European Patent Application EP 4 137 153 A1, published February 22, 2023. Title: HPV vaccine. Applicant: Sirion Biotech GmbH. The sequence listing filed with the application follows.

SEQUENCE LISTING (105 sequences)

SEQ ID NO: 1 - DNA, 1881 bp, Macaca fascicularis
  MfPV3 E1
atggacccttctggaattcacggcgagggcaccagatgcaccggatggttcgatgtggaagccatcgtggaaagacggaccggcgacgtggtgtccgaggacgaagatgagaacctggaagataccggcgtggacctggtggacttcatcgacgatacctgcgagtttgagcaggccggcgacgaagctcctagagcactgctgcatgcccaagagacacaggcccatgtgaacgccgtgcactacctgaagcggaagttcacatgcagccctaccgtgtctcccctgggcaatgtgcagtgttctatcgagggcgagctgagccctagactgcacgccatccaactgaatgaaggcagcggcaaggccaagcggagactgtttctgcctgatagcggctacggcaataccgaggtggaaacccagctgtctcaggtggcaggatccgatggcgaatctcaagcccctggcggcaaagaaaatgtgcagcctgctgaaggcgctggcggagatgttcgacagctgctgagaagcagcaacctgaaggccacactgctgggcaagttcaaggacgtgtacggcatcggcttcaacgaactcgtgcggtgcttcaagagcgacaagaccgtgtgcaccgattgggttgtgggagctgctggcgtgcaccattctgtggccgaaggactgaagcacctgatcgagcctttctgcacatacgcccacatgcagtgcctgacctgcaactggggagtgtttctgctgctgctcatccggttcaagtgcggcaagaacagactgaccgtggccaagtgcatctctaccctgctgaacgtgcaagagccctacctgctgatcgaacctccaaagctgagatccacagccgccgctctgtactggtacagaaccggcatcagcaacgtgtccgaagtgatcggagagcctcctgagtggatcgtgcggcagaccatgtttcagcacagcctcgaggacagcatcttcgacctgtctcagatggtgcagtgggcctacgaccacgatctggtggacgatagcgccattgcctaccagtatgcccagctggccgacgtggactctaatgccgccgctttcctgaagtctaacgctcaggccaaatacgtgaaggactgcgccaccatgtgcagacactacaagagagccgagaagcaggccatgaccatgagccagtggatcagagccagatgcgataagaccgacgacggcggagattggaggcctatcgtgcagttcctgagataccagaacgtcgagttcatcacctttctgagcgcctttaaggccttcctgaagggaatccccaagagaagctgcatcgtgctgtacggccctccaaacaccggcaagagctacttcggaatgagcctgatgcagtttctgcagggcagcatcatcagctacgtgaacagcaacagccacttttggctggcccctctggccgaagctaaagtggccatgctggacgatgccacaccacagtgctggtcctacatcgacacctacatgcggagcgtgctggacggcaaccccatgagcattgaccggaagcacaagaacctgatccagatgaagtgtccgcctctgatcatcaccagcaacaccaacgtgggcgaagatgacagatggcgctacctgcactccagagtggtggtgttcaagttcgagcagacctttccattcgaccagaacggcaatcccgtgtacgagctgtccgacaagaattggaagtccttcttcagccggacctggtccagactcgagctgcaagaggatgaggacaccgagcaggatggctctacagtgcgggcctttaagtgtgtgcccggccagaacaccaatatcctg

SEQ ID NO: 2 - protein, 627 aa, Macaca fascicularis
  MfPV3 E1 translated
MDPSGIHGEGTRCTGWFDVEAIVERRTGDVVSEDEDENLEDTGVDLVDFIDDTCEFEQAGDEAPRALLHAQETQAHVNAVHYLKRKFTCSPTVSPLGNVQCSIEGELSPRLHAIQLNEGSGKAKRRLFLPDSGYGNTEVETQLSQVAGSDGESQAPGGKENVQPAEGAGGDVRQLLRSSNLKATLLGKFKDVYGIGFNELVRCFKSDKTVCTDWVVGAAGVHHSVAEGLKHLIEPFCTYAHMQCLTCNWGVFLLLLIRFKCGKNRLTVAKCISTLLNVQEPYLLIEPPKLRSTAAALYWYRTGISNVSEVIGEPPEWIVRQTMFQHSLEDSIFDLSQMVQWAYDHDLVDDSAIAYQYAQLADVDSNAAAFLKSNAQAKYVKDCATMCRHYKRAEKQAMTMSQWIRARCDKTDDGGDWRPIVQFLRYQNVEFITFLSAFKAFLKGIPKRSCIVLYGPPNTGKSYFGMSLMQFLQGSIISYVNSNSHFWLAPLAEAKVAMLDDATPQCWSYIDTYMRSVLDGNPMSIDRKHKNLIQMKCPPLIITSNTNVGEDDRWRYLHSRVVVFKFEQTFPFDQNGNPVYELSDKNWKSFFSRTWSRLELQEDEDTEQDGSTVRAFKCVPGQNTNIL

SEQ ID NO: 3 - DNA, 1080 bp, Macaca fascicularis
  MfPV3 E2
atggaagccctgagcgagagactgaacgcctaccaggacaagatcctgaccttctacgaagaggactccaaggacctgagggaccagatcgagcattggagatgtgtgcggggagagtgcgccgtgttctacaaggccagagagatgggccacagccacatcaaccaccagcaggttccacctctgcacgtgtccagaggcaaggcccacaatgccattgagctgcagatggccctggaaagcctgaaccagagcgacttcaacaccgaggaatggaccctgcaggacacaagcctggaaatgtggcggaccgagcctcagtgctgcttcaaaaagaaaggcgagacagtgaccgtgctgtatgactgcgacaaggacaacagcatggactacaccctgtggggccacgtgtacgtgtggggagatacaggctgggacaaagtgtgcggaaaggtggactacggcggcctgtactatgtgctgcacggcctgaaagtgtactacgttgagttccagcaagaggccgtgaagtacagcaagaccaacaagtgggaagtgcatatcggcagaacagtgatcccctacagcgagtccgtgtcctctacagccctgtgcgaaagagtgcctatcgccgagatcgccaatggcctccagcagaccagcattccctctcacacacacgccaccaccaaagagaacgcttgggtttcctctcagcctcctaccaagcggtccagaagatctgatccaggcggcgatcctgtcagagccctggatgccaatagcagaaccctgctgtctggaaccgcctgcgagaataccaccggcaactcttacagcgactgcacccctgtggtgcacctgaaaggcgaccccaattgtctgaaggccctgcggttcagattcgtgaaacacaagaatctgttcgtgaacgtgtcctccacctggcggtggaccaacaacaccgaagagaaggccatcgtgactgtgacctttaaggacgagcagcagagacagcagttcctcggcagcgtgaagatccccaactccatctgtgtgtgcaagggcgtgatgacagtt

SEQ ID NO: 4 - protein, 360 aa, Macaca fascicularis
  MfPV3 E2 translated
MEALSERLNAYQDKILTFYEEDSKDLRDQIEHWRCVRGECAVFYKAREMGHSHINHQQVPPLHVSRGKAHNAIELQMALESLNQSDFNTEEWTLQDTSLEMWRTEPQCCFKKKGETVTVLYDCDKDNSMDYTLWGHVYVWGDTGWDKVCGKVDYGGLYYVLHGLKVYYVEFQQEAVKYSKTNKWEVHIGRTVIPYSESVSSTALCERVPIAEIANGLQQTSIPSHTHATTKENAWVSSQPPTKRSRRSDPGGDPVRALDANSRTLLSGTACENTTGNSYSDCTPVVHLKGDPNCLKALRFRFVKHKNLFVNVSSTWRWTNNTEEKAIVTVTFKDEQQRQQFLGSVKIPNSICVCKGVMTV

SEQ ID NO: 5 - DNA, 441 bp, Macaca fascicularis
  MfPV3 E6
atggtggaaggcagccaagagagagcccggacactgcacgaactgtgcgagcagagagaacagacccagcacgacatcgagctggactgcgtgtactgcctgaatcctctgaccagaaccgaggtgtacgacttcgccagatgggagctgagaatcgtgtacagacgggataccgcctacggcgtgtgcaagctgtgcctgaggttccacagcaaagtgcggaagtacaggcggtacaactactccatctacggccccacactggaacggcggacaaagaagcagctcgaagaactcgtgatccggtgctactgctgccagaaacctcagtgccccgtggaaaagcagcgccacgttgaccagggccagagattccacaacattgccgagcagtggaccggcagatgcctgcaatgttggaggccaacagccgctgaaacc

SEQ ID NO: 6 - protein, 147 aa, Macaca fascicularis
  MfPV3 E6 translated
MVEGSQERARTLHELCEQREQTQHDIELDCVYCLNPLTRTEVYDFARWELRIVYRRDTAYGVCKLCLRFHSKVRKYRRYNYSIYGPTLERRTKKQLEELVIRCYCCQKPQCPVEKQRHVDQGQRFHNIAEQWTGRCLQCWRPTAAET

SEQ ID NO: 7 - DNA, 300 bp, Macaca fascicularis
  MfPV3 E7
atgatcggccctggacctacactgcaggatatcgtgcttgagctggaacccgagcctgtggacctgagaggatatgagcagctggactccagcgaggacgaggacgagattgaccaccaccaacagcaggacagacccgatgtgcaagaagatgacggcgagcggtttagaatcctgagcgactgtcacgtgtgccagaataccgtgtcaagagtggtgcacagcacccacgacgacctgcacattctcgaggacctgcttatgggcaccctcgagatcgtggcccctaattgtgccgtg

SEQ ID NO: 8 - protein, 100 aa, Macaca fascicularis
  MfPV3 E7 translated
MIGPGPTLQDIVLELEPEPVDLRGYEQLDSSEDEDEIDHHQQQDRPDVQEDDGERFRILSDCHVCQNTVSRVVHSTHDDLHILEDLLMGTLEIVAPNCAV

SEQ ID NO: 9 - DNA, 1947 bp, Human papillomavirus type 16
  HPV16 E1
atggccgatcctgctggcacaaacggcgaagaaggcacaggctgcaacggctggttttacgtggaagccgtggtggaaaagaaaaccggcgacgccatcagcgacgacgagaacgagaatgacagcgacaccggcgaggacctggtggacttcatcgtgaacgacaacgactacctgacacaggccgagacagagacagcccacgctctgtttacagcccaagaggccaagcagcacagagatgccgttcaggtgctgaagagaaagtacctgggcagccctctgagcgacatcagcggctgtgtggacaacaacatcagccccagactgaaggccatctgcatcgagaagcagagcagagccgccaagcggagactgtttgagagcgaggatagcggctacggcaataccgaggtggaaacccagcaaatgctgcaggtcgagggcagacacgaaaccgagacaccttgcagccagtacagcggaggatctggcggaggctgtagccagtactcttctggaagtggcggagagggcgtgtccgagagacacaccatttgtcagacccctctgaccaacatcctgaacgtgctgaaaaccagcaacgccaaggccgccatgctggccaagttcaaagagctgtacggcgtcagcttcagcgaactcgtgcggcccttcaagagcaacaagtccacctgttgcgactggtgcattgccgcctttggcctgacaccttctatcgccgacagcatcaagaccctgctccagcagtactgtctgtacctgcacattcagagcctggcctgctcttggggaatggtggtgctgctgctcgtgcggtacaagtgcggcaagaacagagagacaattgagaagctgctgagcaaactgctgtgcgtgtcccctatgtgcatgatgatcgagcctccaaagctgcggtctacagccgccgctctgtactggtacaagaccggcatcagcaatatctccgaggtgtacggcgacacccctgagtggattcagagacagaccgtcctgcagcacagcttcaacgactgcaccttcgagctgtcccagatggtgcagtgggcctacgacaatgacatcgtggacgactccgagatcgcctataagtacgcccagctggccgacaccaacagcaatgccagcgccttcctgaagtccaacagccaggccaagatcgtgaaggactgcgccaccatgtgcagacactacaagcgggccgagaagaaacagatgagcatgagccagtggatcaagtacagatgcgacagagtggacgacggcggcgattggaagcagatcgtgatgttcctgagataccagggcgtcgagttcatgagctttctgacagccctgaagcggttcctgcagggcatccccaagaagaactgcatcctgctgtatggcgccgctaacaccggcaagagcctgttcggaatgagcctgatgaagtttctgcagggctccgtgatctgctttgtgaacagcaagagccacttctggctccagccactggccgatgccaagattggcatgctggacgatgccaccgtgccttgctggaactacatcgacgacaacctgagaaacgccctggacggcaacctggtttctatggacgtgaagcacagacccctggtgcagctgaagtgtcctccactgctgatcaccagcaacatcaacgccggcaccgattccagatggccctatctgcacaaccggctggtggtgtttacctttcctaacgagttccccttcgacgaaaacggcaaccccgtgtacgagctgaacgataagaattggaagtccttcttcagccggacctggtccagactgagcctgcacgaggatgaggacaaagagaacgacggcgacagcctgcctaccttcaaatgtgtcagcggccagaacaccaacacactg

SEQ ID NO: 10 - protein, 649 aa, Human papillomavirus type 16
  HPV16 E1 translated
MADPAGTNGEEGTGCNGWFYVEAVVEKKTGDAISDDENENDSDTGEDLVDFIVNDNDYLTQAETETAHALFTAQEAKQHRDAVQVLKRKYLGSPLSDISGCVDNNISPRLKAICIEKQSRAAKRRLFESEDSGYGNTEVETQQMLQVEGRHETETPCSQYSGGSGGGCSQYSSGSGGEGVSERHTICQTPLTNILNVLKTSNAKAAMLAKFKELYGVSFSELVRPFKSNKSTCCDWCIAAFGLTPSIADSIKTLLQQYCLYLHIQSLACSWGMVVLLLVRYKCGKNRETIEKLLSKLLCVSPMCMMIEPPKLRSTAAALYWYKTGISNISEVYGDTPEWIQRQTVLQHSFNDCTFELSQMVQWAYDNDIVDDSEIAYKYAQLADTNSNASAFLKSNSQAKIVKDCATMCRHYKRAEKKQMSMSQWIKYRCDRVDDGGDWKQIVMFLRYQGVEFMSFLTALKRFLQGIPKKNCILLYGAANTGKSLFGMSLMKFLQGSVICFVNSKSHFWLQPLADAKIGMLDDATVPCWNYIDDNLRNALDGNLVSMDVKHRPLVQLKCPPLLITSNINAGTDSRWPYLHNRLVVFTFPNEFPFDENGNPVYELNDKNWKSFFSRTWSRLSLHEDEDKENDGDSLPTFKCVSGQNTNTL

SEQ ID NO: 11 - DNA, 1095 bp, Human papillomavirus type 16
  HPV16 E2
atggaaacactgtgccagcggctgaacgtgtgccaggacaagattctgacccactatgagaacgacagcaccgacctgagggaccacatcgactactggaagcacatgcggctggaatgcgccatctactacaaggctagagagatgggcttcaagcacatcaaccaccaggtggtgcctacactggccgtgtctaagaacaaggctctgcaggccatcgaactgcagctgaccctggaaacaatctacaactcccagtactccaacgagaagtggaccctccaggacgtgtcactggaagtgtacctgaccgctcctaccggctgcatcaagaaacacggctacaccgtggaagtgcagtttgacggcgatatctgcaataccatgcactacaccaactggacccacatctacatctgcgaagaggccagcgtgacagtggtggaaggccaggtcgactactacggcctgtactacgtgcacgagggcatcagaacctacttcgtgcagttcaaggatgacgccgagaagtacagcaagaacaaagtgtgggaagtgcacgctggcggccaagtgatcctgtgtcctacaagcgtgttcagcagcaacgaagtgtctagccccgagatcatcagacagcacctggccaatcatcctgccgccacacacacaaaagctgtggccctgggcaccgaggaaacacagaccacaattcagaggcccagaagcgagcccgataccggcaatccttgtcacaccaccaagctgctgcaccgggattccgtggattctgcccctatcctgaccgccttcaacagctcccacaaaggccggatcaactgcaacagcaacaccacacctatcgtgcacctgaaaggggacgccaacactctgaaggccctgcggtacagattcaagaagcactgtaccctgtataccgccgtgtccagcacatggcactggaccggacacaacgtgaaacacaagagcgccatcgtgaccctgacctacgatagcgagtggcagagggaccagttcctgagccaagtgaagatccctaagaccatcaccgtgtccaccggctttatgagcatt

SEQ ID NO: 12 - protein, 365 aa, Human papillomavirus type 16
  HPV16 E2 translated
METLCQRLNVCQDKILTHYENDSTDLRDHIDYWKHMRLECAIYYKAREMGFKHINHQVVPTLAVSKNKALQAIELQLTLETIYNSQYSNEKWTLQDVSLEVYLTAPTGCIKKHGYTVEVQFDGDICNTMHYTNWTHIYICEEASVTVVEGQVDYYGLYYVHEGIRTYFVQFKDDAEKYSKNKVWEVHAGGQVILCPTSVFSSNEVSSPEIIRQHLANHPAATHTKAVALGTEETQTTIQRPRSEPDTGNPCHTTKLLHRDSVDSAPILTAFNSSHKGRINCNSNTTPIVHLKGDANTLKALRYRFKKHCTLYTAVSSTWHWTGHNVKHKSAIVTLTYDSEWQRDQFLSQVKIPKTITVSTGFMSI

SEQ ID NO: 13 - DNA, 462 bp, Human papillomavirus type 16
  HPV16 E6
atgcaccagaaacggacagccatgttccaggatcctcaagagcggccacggaagctgcctcagctgtgtacagaactgcagaccaccatccacgacatcatcctcgagtgcgtgtactgcaagcagcagctcctgcggagagaagtgtacgacttcgccttccgggatctgtgcatcgtgtacagagatggcaacccctacgccgtgtgcgacaagtgcctgaagttctactccaagatcagcgagtaccggcactactgctactccctgtacggcaccacacttgagcagcagtacaacaagcccctgtgcgatctgctgatccggtgcatcaactgccagaaacctcagtgccccgaggaaaagcagagacacctggacaagaagcagcggttccacaacattagaggcagatggacaggccggtgcatgagctgctgtagaagcagcagaacaagacgg

SEQ ID NO: 14 - protein, 154 aa, Human papillomavirus type 16
  HPV16 E6 translated
MHQKRTAMFQDPQERPRKLPQLCTELQTTIHDIILECVYCKQQLLRREVYDFAFRDLCIVYRDGNPYAVCDKCLKFYSKISEYRHYCYSLYGTTLEQQYNKPLCDLLIRCINCQKPQCPEEKQRHLDKKQRFHNIRGRWTGRCMSCCRSSRTRR

SEQ ID NO: 15 - DNA, 294 bp, Human papillomavirus type 16
  HPV16 E7
atgcacggcgataccccaacactgcacgagtacatgctggatctgcagcccgagacaaccgatctgtacggctatgagcagctgaatgactccagcgaggaagaggacgagatcgacggacctgctggacaggctgaacctgatagagcccactacaatatcgtgaccttctgctgcaagtgcgatagcaccctgagaagatgcgtgcagagcacccacgtggacatcaggaccctcgaggatctgctcatgggcaccctgggaattgtggccccaatctgctctcagaagcct

SEQ ID NO: 16 - protein, 98 aa, Human papillomavirus type 16
  HPV16 E7 translated
MHGDTPTLHEYMLDLQPETTDLYGYEQLNDSSEEEDEIDGPAGQAEPDRAHYNIVTFCCKCDSTLRRCVQSTHVDIRTLEDLLMGTLGIVAPICSQKP

SEQ ID NO: 17 - DNA, 1971 bp, Human papillomavirus type 18
  HPV18 E1
atggccgatcctgagggaacagatggcgaaggcacaggctgcaacggctggttttacgtgcaagccatcgtggacaagaagaccggcgacgtcatcagcgacgacgaggatgagaatgccaccgacaccggcagcgacatggtggactttatcgatacccagggcacgttctgcgagcaggccgaactggaaacagcccaggcactgtttcacgcccaagaggtgcacaacgatgcccaggtgctgcacgtgctgaagagaaagtttgccggcggaagcaccgagaacagcccactgggagaaagactggaagtggacaccgagctgagccccagactgcaagagatcagcctgaacagcggccagaagaaggccaagcggagactgttcaccatctccgacagcggctacggctgtagcgaagtggaagccacacagatccaagtgaccaccaatggcgagcacggcggcaatgtttgttctggcggatctaccgaggccatcgacaatggcggaaccgagggcaacaatagctccgtggatggcaccagcgacaacagcaacatcgagaacgtgaaccctcagtgcacaatcgcccagctgaaggacctgctgaaagtgaacaacaagcagggcgccatgctggccgtgtttaaggatacctacggcctgagcttcaccgacctcgtgcggaacttcaagagcgacaagaccacctgtaccgactgggtcaccgccatctttggcgtgaacccaacaatcgccgagggcttcaagaccctgatccagcctttcatcctgtacgcccacatccagtgtctggactgcaaatggggcgtgctgattctggccctgctgagatacaagtgcggcaagagcagactgaccgtggccaagggactgagcactctgctgcatgtgcccgagacatgcatgctgattcagcctccaaagctgcggtctagcgtggccgctctgtactggtacagaaccggcatcagcaatatcagcgaagtgatgggcgacacccctgagtggattcagcggctgacaatcatccagcacggcatcgacgactccaacttcgacctgagcgagatggtgcagtgggccttcgataacgagctgaccgacgagtccgacatggcctttgaatacgccctgctggcagacagcaactccaatgccgccgctttcctgaagtccaactgccaggccaagtacctgaaggactgcgccaccatgtgcaagcactaccgcagagcacagaaacggcagatgaacatgagccagtggatccggttccggtgcagcaagatcgatgaaggtggcgactggcggcctatcgtgcagttcctgagataccagcagatcgagttcatcacctttctgggcgccctgaagtcattcctgaagggaacccctaaaaagaactgcctggtgttctgcggccctgccaataccggcaagtcctacttcggcatgagctttatccacttcatccagggcgccgtgatcagcttcgtgaacagcaccagccacttttggctggaacccctgaccgataccaaggtggcaatgctggacgacgccaccaccacctgttggacctacttcgacacctacatgcggaacgccctggacggcaaccccatcagcatcgacagaaagcacaagcccctcatccagctgaaatgccctccaatcctgctgaccacaaacattcaccccgccaaggacaatcggtggccctacctggaaagccggatcaccgtgttcgagttccccaacgcctttccattcgacaagaacggcaatcccgtgtacgagatcaacgacaagaattggaagtgcttcttcgagcggacctggtccagactggatctgcacgaggaagaagaggacgccgacacagagggcaatcccttcggcacctttaagtgtgtggccgggcagaatcacagacccctg

SEQ ID NO: 18 - protein, 657 aa, Human papillomavirus type 18
  HPV18 E1 translated
MADPEGTDGEGTGCNGWFYVQAIVDKKTGDVISDDEDENATDTGSDMVDFIDTQGTFCEQAELETAQALFHAQEVHNDAQVLHVLKRKFAGGSTENSPLGERLEVDTELSPRLQEISLNSGQKKAKRRLFTISDSGYGCSEVEATQIQVTTNGEHGGNVCSGGSTEAIDNGGTEGNNSSVDGTSDNSNIENVNPQCTIAQLKDLLKVNNKQGAMLAVFKDTYGLSFTDLVRNFKSDKTTCTDWVTAIFGVNPTIAEGFKTLIQPFILYAHIQCLDCKWGVLILALLRYKCGKSRLTVAKGLSTLLHVPETCMLIQPPKLRSSVAALYWYRTGISNISEVMGDTPEWIQRLTIIQHGIDDSNFDLSEMVQWAFDNELTDESDMAFEYALLADSNSNAAAFLKSNCQAKYLKDCATMCKHYRRAQKRQMNMSQWIRFRCSKIDEGGDWRPIVQFLRYQQIEFITFLGALKSFLKGTPKKNCLVFCGPANTGKSYFGMSFIHFIQGAVISFVNSTSHFWLEPLTDTKVAMLDDATTTCWTYFDTYMRNALDGNPISIDRKHKPLIQLKCPPILLTTNIHPAKDNRWPYLESRITVFEFPNAFPFDKNGNPVYEINDKNWKCFFERTWSRLDLHEEEEDADTEGNPFGTFKCVAGQNHRPL

SEQ ID NO: 19 - DNA, 1095 bp, Human papillomavirus type 18
  HPV18 E2
atgcagaccccaaaagagacactgagcgagcggctgagcgccctccaggacaagatcatcgaccactacgagaacgacagcaaggacatcgacagccagattcagtactggcagctgatcagatgggagaacgccatcttcttcgccgctagagagcacggaattcagaccctgaaccaccaggtggtgcccgcctacaacatcagcaagagcaaggcccacaaggccattgaactccagatggccctgcaaggactggctcagagcgcctacaagaccgaggattggacactccaggatacctgcgaggaactgtggaacacagagcccacacactgcttcaagaaaggcggccagaccgtgcaggtctacttcgatggcaacaaggataactgcatgacctacgtggcctgggacagcgtgtactacatgacagatgccggcacctgggacaagaccgccacctgtgtttctcaccggggcctgtactacgtgaaagagggctacaacaccttctacatcgagtttaagagcgagtgcgagaagtatggcaacaccggcacatgggaagtgcatttcggcaacaacgtgatcgactgcaacgactccatgtgctccacctccgatgacaccgtgtctgccacacagctggtcaagcagctccagcacaccccatctccatacagctctacagtgtctgtgggcaccgccaagacctatggccaaacaagcgctgccacaagacctggccattgtggactggccgagaagcagcactgtggccctgttaatcctctgctgggagccgccacacctacaggcaacaacaagagaagaaagctgtgcagcggcaacaccacacctatcattcacctgaagggcgacagaaacagcctgaagtgcctgcggtacagactgaggaagcacagcgatcactaccgggacatcagctccacctggcactggacaggtgctggcaacgaaaagaccggcatcctgacagtgacctaccacagcgagactcagcggaccaagttcctgaacaccgtggctatccccgacagcgtgcagattctcgtgggctacatgaccatg

SEQ ID NO: 20 - protein, 365 aa, Human papillomavirus type 18
  HPV18 E2 translated
MQTPKETLSERLSALQDKIIDHYENDSKDIDSQIQYWQLIRWENAIFFAAREHGIQTLNHQVVPAYNISKSKAHKAIELQMALQGLAQSAYKTEDWTLQDTCEELWNTEPTHCFKKGGQTVQVYFDGNKDNCMTYVAWDSVYYMTDAGTWDKTATCVSHRGLYYVKEGYNTFYIEFKSECEKYGNTGTWEVHFGNNVIDCNDSMCSTSDDTVSATQLVKQLQHTPSPYSSTVSVGTAKTYGQTSAATRPGHCGLAEKQHCGPVNPLLGAATPTGNNKRRKLCSGNTTPIIHLKGDRNSLKCLRYRLRKHSDHYRDISSTWHWTGAGNEKTGILTVTYHSETQRTKFLNTVAIPDSVQILVGYMTM

SEQ ID NO: 21 - DNA, 462 bp, Human papillomavirus type 18
  HPV18 E6
atggccagattcgaggaccctaccagacggccctacaagctgcctgatctgtgcaccgaactgaacaccagccttcaggatatcgagatcacctgtgtgtactgcaagaccgtgctcgagctgacagaagtgtttgagttcgccttcaaggacctgttcgtggtgtacagagacagcatccctcacgccgcctgtcacaagtgcatcgacttctacagcagaatcagagagctgcggcactacagcgactccgtgtacggcgataccctggaaaaactgaccaacaccggactgtacaacctgctgatccggtgcctgagatgccagaaacctcagaaccccgccgagaaactgagacatctgaacgagaagcggcggttccacaatatcgccggccactacagaggccagtgccacagctgttgcaaccgggccagacaagaaagactccagcggagaaga

SEQ ID NO: 22 - protein, 154 aa, Human papillomavirus type 18
  HPV18 E6 translated
MARFEDPTRRPYKLPDLCTELNTSLQDIEITCVYCKTVLELTEVFEFAFKDLFVVYRDSIPHAACHKCIDFYSRIRELRHYSDSVYGDTLEKLTNTGLYNLLIRCLRCQKPQNPAEKLRHLNEKRRFHNIAGHYRGQCHSCCNRARQERLQRRR

SEQ ID NO: 23 - DNA, 315 bp, Human papillomavirus type 18
  HPV18 E7
atgcacggacctaaagccacacttcaggacatcgtgctgcacctcgagcctcagaatgagatccccgtggatctgctcggccatgagcagctgagcgatagcgaggaagagaacgacgagatcgacggcgtcaaccaccagcatctgcctgccagaagggccgaacctcagagacacaccatgctgtgcatgtgctgcaagtgcgaggcccggatcgagagagtggtggaatctagcgccgacgacctgagagctttccagcagctgttcctgaatactctgagcttcgtggccccttggtgcgctagtcagcag

SEQ ID NO: 24 - protein, 105 aa, Human papillomavirus type 18
  HPV18 E7 translated
MHGPKATLQDIVLHLEPQNEIPVDLLGHEQLSDSEEENDEIDGVNHQHLPARRAEPQRHTMLCMCCKCEARIERVVESSADDLRAFQQLFLNTLSFVAPWCASQQ

SEQ ID NO: 25 - DNA, 4455 bp, Macaca fascicularis
  MfPV3 Ii-E1E2E6E7
atgcacagaaggcggagcagaagctgccgcgaggatcagaaacccgtgatggacgaccagcgggacctgatcagcaacaacgagcagctgcctatgctcggcagaaggcctggcgctcctgagagcaaatgttctagaggcgccctgtacaccggcttcagcatcctggttacactgctgctggccggacaggctaccaccgcctactttctgtatcagcagcagggcagactggacaagctgaccgtgaccagccagaacctgcagctggaaaacctgcggatgaagctgcccaagcctcctaagcctgtgtccaagatgcggatggccacacctctgctgatgcaggctttgcctatgggagcactgcctcagggccctatgcagaacgccaccaaatacggcaacatgaccgaggaccacgtgatgcatctgctgcagaatgccgatcctctgaaggtgtaccctccactgaagggcagctttcccgagaacctgcggcacctgaagaacaccatggaaaccatcgactggaaggtgttcgagagctggatgcaccactggctgctgttcgagatgagccggcacagcctggaacagaagcctacagacgcccctcctaaagagtccctggaactggaagatcccagctctggcctgggcgtgacaaagcaagatctgggccctgtgcctatgatggacccttctggaattcacggcgagggcaccagatgcaccggatggttcgatgtggaagccatcgtggaaagacggaccggcgacgtggtgtccgaggacgaagatgagaacctggaagataccggcgtggacctggtggacttcatcgacgatacctgcgagtttgagcaggccggcgacgaagctcctagagcactgctgcatgcccaagagacacaggcccatgtgaacgccgtgcactacctgaagcggaagttcacatgcagccctaccgtgtctcccctgggcaatgtgcagtgttctatcgagggcgagctgagccctagactgcacgccatccaactgaatgaaggcagcggcaaggccaagcggagactgtttctgcctgatagcggctacggcaataccgaggtggaaacccagctgtctcaggtggcaggatccgatggcgaatctcaagcccctggcggcaaagaaaatgtgcagcctgctgaaggcgctggcggagatgttcgacagctgctgagaagcagcaacctgaaggccacactgctgggcaagttcaaggacgtgtacggcatcggcttcaacgaactcgtgcggtgcttcaagagcgacaagaccgtgtgcaccgattgggttgtgggagctgctggcgtgcaccattctgtggccgaaggactgaagcacctgatcgagcctttctgcacatacgcccacatgcagtgcctgacctgcaactggggagtgtttctgctgctgctcatccggttcaagtgcggcaagaacagactgaccgtggccaagtgcatctctaccctgctgaacgtgcaagagccctacctgctgatcgaacctccaaagctgagatccacagccgccgctctgtactggtacagaaccggcatcagcaacgtgtccgaagtgatcggagagcctcctgagtggatcgtgcggcagaccatgtttcagcacagcctcgaggacagcatcttcgacctgtctcagatggtgcagtgggcctacgaccacgatctggtggacgatagcgccattgcctaccagtatgcccagctggccgacgtggactctaatgccgccgctttcctgaagtctaacgctcaggccaaatacgtgaaggactgcgccaccatgtgcagacactacaagagagccgagaagcaggccatgaccatgagccagtggatcagagccagatgcgataagaccgacgacggcggagattggaggcctatcgtgcagttcctgagataccagaacgtcgagttcatcacctttctgagcgcctttaaggccttcctgaagggaatccccaagagaagctgcatcgtgctgtacggccctccaaacaccggcaagagctacttcggaatgagcctgatgcagtttctgcagggcagcatcatcagctacgtgaacagcaacagccacttttggctggcccctctggccgaagctaaagtggccatgctggacgatgccacaccacagtgctggtcctacatcgacacctacatgcggagcgtgctggacggcaaccccatgagcattgaccggaagcacaagaacctgatccagatgaagtgtccgcctctgatcatcaccagcaacaccaacgtgggcgaagatgacagatggcgctacctgcactccagagtggtggtgttcaagttcgagcagacctttccattcgaccagaacggcaatcccgtgtacgagctgtccgacaagaattggaagtccttcttcagccggacctggtccagactcgagctgcaagaggatgaggacaccgagcaggatggctctacagtgcgggcctttaagtgtgtgcccggccagaacaccaatatcctgggctctatggaagccctgagcgagagactgaacgcctaccaggacaagatcctgaccttctacgaagaggactccaaggacctgagggaccagatcgagcattggagatgtgtgcggggagagtgcgccgtgttctacaaggccagagagatgggccacagccacatcaaccaccagcaggttccacctctgcacgtgtccagaggcaaggcccacaatgccattgagctgcagatggccctggaaagcctgaaccagagcgacttcaacaccgaggaatggaccctgcaggacacaagcctggaaatgtggcggaccgagcctcagtgctgcttcaaaaagaaaggcgagacagtgaccgtgctgtatgactgcgacaaggacaacagcatggactacaccctgtggggccacgtgtacgtgtggggagatacaggctgggacaaagtgtgcggaaaggtggactacggcggcctgtactatgtgctgcacggcctgaaagtgtactacgttgagttccagcaagaggccgtgaagtacagcaagaccaacaagtgggaagtgcatatcggcagaacagtgatcccctacagcgagtccgtgtcctctacagccctgtgcgaaagagtgcctatcgccgagatcgccaatggcctccagcagaccagcattccctctcacacacacgccaccaccaaagagaacgcttgggtttcctctcagcctcctaccaagcggtccagaagatctgatccaggcggcgatcctgtcagagccctggatgccaatagcagaaccctgctgtctggaaccgcctgcgagaataccaccggcaactcttacagcgactgcacccctgtggtgcacctgaaaggcgaccccaattgtctgaaggccctgcggttcagattcgtgaaacacaagaatctgttcgtgaacgtgtcctccacctggcggtggaccaacaacaccgaagagaaggccatcgtgactgtgacctttaaggacgagcagcagagacagcagttcctcggcagcgtgaagatccccaactccatctgtgtgtgcaagggcgtgatgacagttggcagcatggtggaaggcagccaagagagagcccggacactgcacgaactgtgcgagcagagagaacagacccagcacgacatcgagctggactgcgtgtactgcctgaatcctctgaccagaaccgaggtgtacgacttcgccagatgggagctgagaatcgtgtacagacgggataccgcctacggcgtgtgcaagctgtgcctgaggttccacagcaaagtgcggaagtacaggcggtacaactactccatctacggccccacactggaacggcggacaaagaagcagctcgaagaactcgtgatccggtgctactgctgccagaaacctcagtgccccgtggaaaagcagcgccacgttgaccagggccagagattccacaacattgccgagcagtggaccggcagatgcctgcaatgttggaggccaacagccgctgaaaccggctctatgatcggccctggacctacactgcaggatatcgtgcttgagctggaacccgagcctgtggacctgagaggatatgagcagctggactccagcgaggacgaggacgagattgaccaccaccaacagcaggacagacccgatgtgcaagaagatgacggcgagcggtttagaatcctgagcgactgtcacgtgtgccagaataccgtgtcaagagtggtgcacagcacccacgacgacctgcacattctcgaggacctgcttatgggcaccctcgagatcgtggcccctaattgtgccgtgggcagcgaacagaaactgatctccgaggaagatctctga

SEQ ID NO: 26 - protein, 1484 aa, Macaca fascicularis
  MfPV3 Ii-E1E2E6E7 translated
MHRRRSRSCREDQKPVMDDQRDLISNNEQLPMLGRRPGAPESKCSRGALYTGFSILVTLLLAGQATTAYFLYQQQGRLDKLTVTSQNLQLENLRMKLPKPPKPVSKMRMATPLLMQALPMGALPQGPMQNATKYGNMTEDHVMHLLQNADPLKVYPPLKGSFPENLRHLKNTMETIDWKVFESWMHHWLLFEMSRHSLEQKPTDAPPKESLELEDPSSGLGVTKQDLGPVPMMDPSGIHGEGTRCTGWFDVEAIVERRTGDVVSEDEDENLEDTGVDLVDFIDDTCEFEQAGDEAPRALLHAQETQAHVNAVHYLKRKFTCSPTVSPLGNVQCSIEGELSPRLHAIQLNEGSGKAKRRLFLPDSGYGNTEVETQLSQVAGSDGESQAPGGKENVQPAEGAGGDVRQLLRSSNLKATLLGKFKDVYGIGFNELVRCFKSDKTVCTDWVVGAAGVHHSVAEGLKHLIEPFCTYAHMQCLTCNWGVFLLLLIRFKCGKNRLTVAKCISTLLNVQEPYLLIEPPKLRSTAAALYWYRTGISNVSEVIGEPPEWIVRQTMFQHSLEDSIFDLSQMVQWAYDHDLVDDSAIAYQYAQLADVDSNAAAFLKSNAQAKYVKDCATMCRHYKRAEKQAMTMSQWIRARCDKTDDGGDWRPIVQFLRYQNVEFITFLSAFKAFLKGIPKRSCIVLYGPPNTGKSYFGMSLMQFLQGSIISYVNSNSHFWLAPLAEAKVAMLDDATPQCWSYIDTYMRSVLDGNPMSIDRKHKNLIQMKCPPLIITSNTNVGEDDRWRYLHSRVVVFKFEQTFPFDQNGNPVYELSDKNWKSFFSRTWSRLELQEDEDTEQDGSTVRAFKCVPGQNTNILGSMEALSERLNAYQDKILTFYEEDSKDLRDQIEHWRCVRGECAVFYKAREMGHSHINHQQVPPLHVSRGKAHNAIELQMALESLNQSDFNTEEWTLQDTSLEMWRTEPQCCFKKKGETVTVLYDCDKDNSMDYTLWGHVYVWGDTGWDKVCGKVDYGGLYYVLHGLKVYYVEFQQEAVKYSKTNKWEVHIGRTVIPYSESVSSTALCERVPIAEIANGLQQTSIPSHTHATTKENAWVSSQPPTKRSRRSDPGGDPVRALDANSRTLLSGTACENTTGNSYSDCTPVVHLKGDPNCLKALRFRFVKHKNLFVNVSSTWRWTNNTEEKAIVTVTFKDEQQRQQFLGSVKIPNSICVCKGVMTVGSMVEGSQERARTLHELCEQREQTQHDIELDCVYCLNPLTRTEVYDFARWELRIVYRRDTAYGVCKLCLRFHSKVRKYRRYNYSIYGPTLERRTKKQLEELVIRCYCCQKPQCPVEKQRHVDQGQRFHNIAEQWTGRCLQCWRPTAAETGSMIGPGPTLQDIVLELEPEPVDLRGYEQLDSSEDEDEIDHHQQQDRPDVQEDDGERFRILSDCHVCQNTVSRVVHSTHDDLHILEDLLMGTLEIVAPNCAVGSEQKLISEEDL

SEQ ID NO: 27 - DNA, 5211 bp, Macaca fascicularis
  MfPV3 Ii-E1E2-p2a-Ii-E6E7
atgcacagaaggcggagcagaagctgccgcgaggatcagaaacccgtgatggacgaccagcgggacctgatcagcaacaacgagcagctgcctatgctcggcagaaggcctggcgctcctgagagcaaatgttctagaggcgccctgtacaccggcttcagcatcctggttacactgctgctggccggacaggctaccaccgcctactttctgtatcagcagcagggcagactggacaagctgaccgtgaccagccagaacctgcagctggaaaacctgcggatgaagctgcccaagcctcctaagcctgtgtccaagatgcggatggccacacctctgctgatgcaggctttgcctatgggagcactgcctcagggccctatgcagaacgccaccaaatacggcaacatgaccgaggaccacgtgatgcatctgctgcagaatgccgatcctctgaaggtgtaccctccactgaagggcagctttcccgagaacctgcggcacctgaagaacaccatggaaaccatcgactggaaggtgttcgagagctggatgcaccactggctgctgttcgagatgagccggcacagcctggaacagaagcctacagacgcccctcctaaagagtccctggaactggaagatcccagctctggcctgggcgtgacaaagcaagatctgggccctgtgcctatgatggacccttctggaattcacggcgagggcaccagatgcaccggatggttcgatgtggaagccatcgtggaaagacggaccggcgacgtggtgtccgaggacgaagatgagaacctggaagataccggcgtggacctggtggacttcatcgacgatacctgcgagtttgagcaggccggcgacgaagctcctagagcactgctgcatgcccaagagacacaggcccatgtgaacgccgtgcactacctgaagcggaagttcacatgcagccctaccgtgtctcccctgggcaatgtgcagtgttctatcgagggcgagctgagccctagactgcacgccatccaactgaatgaaggcagcggcaaggccaagcggagactgtttctgcctgatagcggctacggcaataccgaggtggaaacccagctgtctcaggtggcaggatccgatggcgaatctcaagcccctggcggcaaagaaaatgtgcagcctgctgaaggcgctggcggagatgttcgacagctgctgagaagcagcaacctgaaggccacactgctgggcaagttcaaggacgtgtacggcatcggcttcaacgaactcgtgcggtgcttcaagagcgacaagaccgtgtgcaccgattgggttgtgggagctgctggcgtgcaccattctgtggccgaaggactgaagcacctgatcgagcctttctgcacatacgcccacatgcagtgcctgacctgcaactggggagtgtttctgctgctgctcatccggttcaagtgcggcaagaacagactgaccgtggccaagtgcatctctaccctgctgaacgtgcaagagccctacctgctgatcgaacctccaaagctgagatccacagccgccgctctgtactggtacagaaccggcatcagcaacgtgtccgaagtgatcggagagcctcctgagtggatcgtgcggcagaccatgtttcagcacagcctcgaggacagcatcttcgacctgtctcagatggtgcagtgggcctacgaccacgatctggtggacgatagcgccattgcctaccagtatgcccagctggccgacgtggactctaatgccgccgctttcctgaagtctaacgctcaggccaaatacgtgaaggactgcgccaccatgtgcagacactacaagagagccgagaagcaggccatgaccatgagccagtggatcagagccagatgcgataagaccgacgacggcggagattggaggcctatcgtgcagttcctgagataccagaacgtcgagttcatcacctttctgagcgcctttaaggccttcctgaagggaatccccaagagaagctgcatcgtgctgtacggccctccaaacaccggcaagagctacttcggaatgagcctgatgcagtttctgcagggcagcatcatcagctacgtgaacagcaacagccacttttggctggcccctctggccgaagctaaagtggccatgctggacgatgccacaccacagtgctggtcctacatcgacacctacatgcggagcgtgctggacggcaaccccatgagcattgaccggaagcacaagaacctgatccagatgaagtgtccgcctctgatcatcaccagcaacaccaacgtgggcgaagatgacagatggcgctacctgcactccagagtggtggtgttcaagttcgagcagacctttccattcgaccagaacggcaatcccgtgtacgagctgtccgacaagaattggaagtccttcttcagccggacctggtccagactcgagctgcaagaggatgaggacaccgagcaggatggctctacagtgcgggcctttaagtgtgtgcccggccagaacaccaatatcctgggctctatggaagccctgagcgagagactgaacgcctaccaggacaagatcctgaccttctacgaagaggactccaaggacctgagggaccagatcgagcattggagatgtgtgcggggagagtgcgccgtgttctacaaggccagagagatgggccacagccacatcaaccaccagcaggttccacctctgcacgtgtccagaggcaaggcccacaatgccattgagctgcagatggccctggaaagcctgaaccagagcgacttcaacaccgaggaatggaccctgcaggacacaagcctggaaatgtggcggaccgagcctcagtgctgcttcaaaaagaaaggcgagacagtgaccgtgctgtatgactgcgacaaggacaacagcatggactacaccctgtggggccacgtgtacgtgtggggagatacaggctgggacaaagtgtgcggaaaggtggactacggcggcctgtactatgtgctgcacggcctgaaagtgtactacgttgagttccagcaagaggccgtgaagtacagcaagaccaacaagtgggaagtgcatatcggcagaacagtgatcccctacagcgagtccgtgtcctctacagccctgtgcgaaagagtgcctatcgccgagatcgccaatggcctccagcagaccagcattccctctcacacacacgccaccaccaaagagaacgcttgggtttcctctcagcctcctaccaagcggtccagaagatctgatccaggcggcgatcctgtcagagccctggatgccaatagcagaaccctgctgtctggaaccgcctgcgagaataccaccggcaactcttacagcgactgcacccctgtggtgcacctgaaaggcgaccccaattgtctgaaggccctgcggttcagattcgtgaaacacaagaatctgttcgtgaacgtgtcctccacctggcggtggaccaacaacaccgaagagaaggccatcgtgactgtgacctttaaggacgagcagcagagacagcagttcctcggcagcgtgaagatccccaactccatctgtgtgtgcaagggcgtgatgacagttggcagcggcgccaccaatttcagtctgcttaaacaggccggggacgtcgaagagaaccccggacctatgcatcggcgcagatctcggtcttgtagagaagaccaaaagcctgtcatggatgatcaaagagatttaatttctaataatgaacaattacccatgttgggacggcgccccggagcccccgaatctaagtgcagccggggagctttatatacaggattttctattttagtgaccttattattagctggccaagccacaacagcttatttcttataccaacaacaaggacggttagataaattaacagtcacatctcaaaatttacaattagagaatttaagaatgaaattacctaaaccacccaaacccgtcagtaaaatgagaatggctacccccttattaatgcaagccctccccatgggcgccttaccccaaggacccatgcaaaatgctacaaagtatggaaatatgacagaagatcatgtcatgcacttattacaaaacgctgaccccttaaaagtctatccccctttaaaaggatctttccctgaaaatttaagacatttaaaaaatacaatggagacaattgattggaaagtctttgaatcttggatgcatcattggttattatttgaaatgtctaggcattctttagagcaaaaacccaccgatgctccacccaaggaaagtttagagttagaggacccttctagcggattaggagtcaccaaacaggacttaggacccgtccccatgatggtggaaggcagccaagagagagcccggacactgcacgaactgtgcgagcagagagaacagacccagcacgacatcgagctggactgcgtgtactgcctgaatcctctgaccagaaccgaggtgtacgacttcgccagatgggagctgagaatcgtgtacagacgggataccgcctacggcgtgtgcaagctgtgcctgaggttccacagcaaagtgcggaagtacaggcggtacaactactccatctacggccccacactggaacggcggacaaagaagcagctcgaagaactcgtgatccggtgctactgctgccagaaacctcagtgccccgtggaaaagcagcgccacgttgaccagggccagagattccacaacattgccgagcagtggaccggcagatgcctgcaatgttggaggccaacagccgctgaaaccggctctatgatcggccctggacctacactgcaggatatcgtgcttgagctggaacccgagcctgtggacctgagaggatatgagcagctggactccagcgaggacgaggacgagattgaccaccaccaacagcaggacagacccgatgtgcaagaagatgacggcgagcggtttagaatcctgagcgactgtcacgtgtgccagaataccgtgtcaagagtggtgcacagcacccacgacgacctgcacattctcgaggacctgcttatgggcaccctcgagatcgtggcccctaattgtgccgtgggcagcgaacagaaactgatctccgaggaagatctctga

SEQ ID NO: 28 - protein, 1736 aa, Macaca fascicularis
  MfPV3 Ii-E1E2-p2a-Ii-E6E7 translated
MHRRRSRSCREDQKPVMDDQRDLISNNEQLPMLGRRPGAPESKCSRGALYTGFSILVTLLLAGQATTAYFLYQQQGRLDKLTVTSQNLQLENLRMKLPKPPKPVSKMRMATPLLMQALPMGALPQGPMQNATKYGNMTEDHVMHLLQNADPLKVYPPLKGSFPENLRHLKNTMETIDWKVFESWMHHWLLFEMSRHSLEQKPTDAPPKESLELEDPSSGLGVTKQDLGPVPMMDPSGIHGEGTRCTGWFDVEAIVERRTGDVVSEDEDENLEDTGVDLVDFIDDTCEFEQAGDEAPRALLHAQETQAHVNAVHYLKRKFTCSPTVSPLGNVQCSIEGELSPRLHAIQLNEGSGKAKRRLFLPDSGYGNTEVETQLSQVAGSDGESQAPGGKENVQPAEGAGGDVRQLLRSSNLKATLLGKFKDVYGIGFNELVRCFKSDKTVCTDWVVGAAGVHHSVAEGLKHLIEPFCTYAHMQCLTCNWGVFLLLLIRFKCGKNRLTVAKCISTLLNVQEPYLLIEPPKLRSTAAALYWYRTGISNVSEVIGEPPEWIVRQTMFQHSLEDSIFDLSQMVQWAYDHDLVDDSAIAYQYAQLADVDSNAAAFLKSNAQAKYVKDCATMCRHYKRAEKQAMTMSQWIRARCDKTDDGGDWRPIVQFLRYQNVEFITFLSAFKAFLKGIPKRSCIVLYGPPNTGKSYFGMSLMQFLQGSIISYVNSNSHFWLAPLAEAKVAMLDDATPQCWSYIDTYMRSVLDGNPMSIDRKHKNLIQMKCPPLIITSNTNVGEDDRWRYLHSRVVVFKFEQTFPFDQNGNPVYELSDKNWKSFFSRTWSRLELQEDEDTEQDGSTVRAFKCVPGQNTNILGSMEALSERLNAYQDKILTFYEEDSKDLRDQIEHWRCVRGECAVFYKAREMGHSHINHQQVPPLHVSRGKAHNAIELQMALESLNQSDFNTEEWTLQDTSLEMWRTEPQCCFKKKGETVTVLYDCDKDNSMDYTLWGHVYVWGDTGWDKVCGKVDYGGLYYVLHGLKVYYVEFQQEAVKYSKTNKWEVHIGRTVIPYSESVSSTALCERVPIAEIANGLQQTSIPSHTHATTKENAWVSSQPPTKRSRRSDPGGDPVRALDANSRTLLSGTACENTTGNSYSDCTPVVHLKGDPNCLKALRFRFVKHKNLFVNVSSTWRWTNNTEEKAIVTVTFKDEQQRQQFLGSVKIPNSICVCKGVMTVGSGATNFSLLKQAGDVEENPGPMHRRRSRSCREDQKPVMDDQRDLISNNEQLPMLGRRPGAPESKCSRGALYTGFSILVTLLLAGQATTAYFLYQQQGRLDKLTVTSQNLQLENLRMKLPKPPKPVSKMRMATPLLMQALPMGALPQGPMQNATKYGNMTEDHVMHLLQNADPLKVYPPLKGSFPENLRHLKNTMETIDWKVFESWMHHWLLFEMSRHSLEQKPTDAPPKESLELEDPSSGLGVTKQDLGPVPMMVEGSQERARTLHELCEQREQTQHDIELDCVYCLNPLTRTEVYDFARWELRIVYRRDTAYGVCKLCLRFHSKVRKYRRYNYSIYGPTLERRTKKQLEELVIRCYCCQKPQCPVEKQRHVDQGQRFHNIAEQWTGRCLQCWRPTAAETGSMIGPGPTLQDIVLELEPEPVDLRGYEQLDSSEDEDEIDHHQQQDRPDVQEDDGERFRILSDCHVCQNTVSRVVHSTHDDLHILEDLLMGTLEIVAPNCAVGSEQKLISEEDL

SEQ ID NO: 29 - DNA, 3759 bp, Macaca fascicularis
  MfPV3 E1E2E6E7
atggacccttctggaattcacggcgagggcaccagatgcaccggatggttcgatgtggaagccatcgtggaaagacggaccggcgacgtggtgtccgaggacgaagatgagaacctggaagataccggcgtggacctggtggacttcatcgacgatacctgcgagtttgagcaggccggcgacgaagctcctagagcactgctgcatgcccaagagacacaggcccatgtgaacgccgtgcactacctgaagcggaagttcacatgcagccctaccgtgtctcccctgggcaatgtgcagtgttctatcgagggcgagctgagccctagactgcacgccatccaactgaatgaaggcagcggcaaggccaagcggagactgtttctgcctgatagcggctacggcaataccgaggtggaaacccagctgtctcaggtggcaggatccgatggcgaatctcaagcccctggcggcaaagaaaatgtgcagcctgctgaaggcgctggcggagatgttcgacagctgctgagaagcagcaacctgaaggccacactgctgggcaagttcaaggacgtgtacggcatcggcttcaacgaactcgtgcggtgcttcaagagcgacaagaccgtgtgcaccgattgggttgtgggagctgctggcgtgcaccattctgtggccgaaggactgaagcacctgatcgagcctttctgcacatacgcccacatgcagtgcctgacctgcaactggggagtgtttctgctgctgctcatccggttcaagtgcggcaagaacagactgaccgtggccaagtgcatctctaccctgctgaacgtgcaagagccctacctgctgatcgaacctccaaagctgagatccacagccgccgctctgtactggtacagaaccggcatcagcaacgtgtccgaagtgatcggagagcctcctgagtggatcgtgcggcagaccatgtttcagcacagcctcgaggacagcatcttcgacctgtctcagatggtgcagtgggcctacgaccacgatctggtggacgatagcgccattgcctaccagtatgcccagctggccgacgtggactctaatgccgccgctttcctgaagtctaacgctcaggccaaatacgtgaaggactgcgccaccatgtgcagacactacaagagagccgagaagcaggccatgaccatgagccagtggatcagagccagatgcgataagaccgacgacggcggagattggaggcctatcgtgcagttcctgagataccagaacgtcgagttcatcacctttctgagcgcctttaaggccttcctgaagggaatccccaagagaagctgcatcgtgctgtacggccctccaaacaccggcaagagctacttcggaatgagcctgatgcagtttctgcagggcagcatcatcagctacgtgaacagcaacagccacttttggctggcccctctggccgaagctaaagtggccatgctggacgatgccacaccacagtgctggtcctacatcgacacctacatgcggagcgtgctggacggcaaccccatgagcattgaccggaagcacaagaacctgatccagatgaagtgtccgcctctgatcatcaccagcaacaccaacgtgggcgaagatgacagatggcgctacctgcactccagagtggtggtgttcaagttcgagcagacctttccattcgaccagaacggcaatcccgtgtacgagctgtccgacaagaattggaagtccttcttcagccggacctggtccagactcgagctgcaagaggatgaggacaccgagcaggatggctctacagtgcgggcctttaagtgtgtgcccggccagaacaccaatatcctgggctctatggaagccctgagcgagagactgaacgcctaccaggacaagatcctgaccttctacgaagaggactccaaggacctgagggaccagatcgagcattggagatgtgtgcggggagagtgcgccgtgttctacaaggccagagagatgggccacagccacatcaaccaccagcaggttccacctctgcacgtgtccagaggcaaggcccacaatgccattgagctgcagatggccctggaaagcctgaaccagagcgacttcaacaccgaggaatggaccctgcaggacacaagcctggaaatgtggcggaccgagcctcagtgctgcttcaaaaagaaaggcgagacagtgaccgtgctgtatgactgcgacaaggacaacagcatggactacaccctgtggggccacgtgtacgtgtggggagatacaggctgggacaaagtgtgcggaaaggtggactacggcggcctgtactatgtgctgcacggcctgaaagtgtactacgttgagttccagcaagaggccgtgaagtacagcaagaccaacaagtgggaagtgcatatcggcagaacagtgatcccctacagcgagtccgtgtcctctacagccctgtgcgaaagagtgcctatcgccgagatcgccaatggcctccagcagaccagcattccctctcacacacacgccaccaccaaagagaacgcttgggtttcctctcagcctcctaccaagcggtccagaagatctgatccaggcggcgatcctgtcagagccctggatgccaatagcagaaccctgctgtctggaaccgcctgcgagaataccaccggcaactcttacagcgactgcacccctgtggtgcacctgaaaggcgaccccaattgtctgaaggccctgcggttcagattcgtgaaacacaagaatctgttcgtgaacgtgtcctccacctggcggtggaccaacaacaccgaagagaaggccatcgtgactgtgacctttaaggacgagcagcagagacagcagttcctcggcagcgtgaagatccccaactccatctgtgtgtgcaagggcgtgatgacagttggcagcatggtggaaggcagccaagagagagcccggacactgcacgaactgtgcgagcagagagaacagacccagcacgacatcgagctggactgcgtgtactgcctgaatcctctgaccagaaccgaggtgtacgacttcgccagatgggagctgagaatcgtgtacagacgggataccgcctacggcgtgtgcaagctgtgcctgaggttccacagcaaagtgcggaagtacaggcggtacaactactccatctacggccccacactggaacggcggacaaagaagcagctcgaagaactcgtgatccggtgctactgctgccagaaacctcagtgccccgtggaaaagcagcgccacgttgaccagggccagagattccacaacattgccgagcagtggaccggcagatgcctgcaatgttggaggccaacagccgctgaaaccggctctatgatcggccctggacctacactgcaggatatcgtgcttgagctggaacccgagcctgtggacctgagaggatatgagcagctggactccagcgaggacgaggacgagattgaccaccaccaacagcaggacagacccgatgtgcaagaagatgacggcgagcggtttagaatcctgagcgactgtcacgtgtgccagaataccgtgtcaagagtggtgcacagcacccacgacgacctgcacattctcgaggacctgcttatgggcaccctcgagatcgtggcccctaattgtgccgtgggcagcgaacagaaactgatctccgaggaagatctctga

SEQ ID NO: 30 - protein, 1252 aa, Macaca fascicularis
  MfPV3 E1E2E6E7 translated
MDPSGIHGEGTRCTGWFDVEAIVERRTGDVVSEDEDENLEDTGVDLVDFIDDTCEFEQAGDEAPRALLHAQETQAHVNAVHYLKRKFTCSPTVSPLGNVQCSIEGELSPRLHAIQLNEGSGKAKRRLFLPDSGYGNTEVETQLSQVAGSDGESQAPGGKENVQPAEGAGGDVRQLLRSSNLKATLLGKFKDVYGIGFNELVRCFKSDKTVCTDWVVGAAGVHHSVAEGLKHLIEPFCTYAHMQCLTCNWGVFLLLLIRFKCGKNRLTVAKCISTLLNVQEPYLLIEPPKLRSTAAALYWYRTGISNVSEVIGEPPEWIVRQTMFQHSLEDSIFDLSQMVQWAYDHDLVDDSAIAYQYAQLADVDSNAAAFLKSNAQAKYVKDCATMCRHYKRAEKQAMTMSQWIRARCDKTDDGGDWRPIVQFLRYQNVEFITFLSAFKAFLKGIPKRSCIVLYGPPNTGKSYFGMSLMQFLQGSIISYVNSNSHFWLAPLAEAKVAMLDDATPQCWSYIDTYMRSVLDGNPMSIDRKHKNLIQMKCPPLIITSNTNVGEDDRWRYLHSRVVVFKFEQTFPFDQNGNPVYELSDKNWKSFFSRTWSRLELQEDEDTEQDGSTVRAFKCVPGQNTNILGSMEALSERLNAYQDKILTFYEEDSKDLRDQIEHWRCVRGECAVFYKAREMGHSHINHQQVPPLHVSRGKAHNAIELQMALESLNQSDFNTEEWTLQDTSLEMWRTEPQCCFKKKGETVTVLYDCDKDNSMDYTLWGHVYVWGDTGWDKVCGKVDYGGLYYVLHGLKVYYVEFQQEAVKYSKTNKWEVHIGRTVIPYSESVSSTALCERVPIAEIANGLQQTSIPSHTHATTKENAWVSSQPPTKRSRRSDPGGDPVRALDANSRTLLSGTACENTTGNSYSDCTPVVHLKGDPNCLKALRFRFVKHKNLFVNVSSTWRWTNNTEEKAIVTVTFKDEQQRQQFLGSVKIPNSICVCKGVMTVGSMVEGSQERARTLHELCEQREQTQHDIELDCVYCLNPLTRTEVYDFARWELRIVYRRDTAYGVCKLCLRFHSKVRKYRRYNYSIYGPTLERRTKKQLEELVIRCYCCQKPQCPVEKQRHVDQGQRFHNIAEQWTGRCLQCWRPTAAETGSMIGPGPTLQDIVLELEPEPVDLRGYEQLDSSEDEDEIDHHQQQDRPDVQEDDGERFRILSDCHVCQNTVSRVVHSTHDDLHILEDLLMGTLEIVAPNCAVGSEQKLISEEDL

SEQ ID NO: 31 - DNA, 5211 bp, Macaca fascicularis
  MfPV3 Ii-E1E6E7-p2a-Ii-E2
atgcacagaaggcggagcagaagctgccgcgaggatcagaaacccgtgatggacgaccagcgggacctgatcagcaacaacgagcagctgcctatgctcggcagaaggcctggcgctcctgagagcaaatgttctagaggcgccctgtacaccggcttcagcatcctggttacactgctgctggccggacaggctaccaccgcctactttctgtatcagcagcagggcagactggacaagctgaccgtgaccagccagaacctgcagctggaaaacctgcggatgaagctgcccaagcctcctaagcctgtgtccaagatgcggatggccacacctctgctgatgcaggctttgcctatgggagcactgcctcagggccctatgcagaacgccaccaaatacggcaacatgaccgaggaccacgtgatgcatctgctgcagaatgccgatcctctgaaggtgtaccctccactgaagggcagctttcccgagaacctgcggcacctgaagaacaccatggaaaccatcgactggaaggtgttcgagagctggatgcaccactggctgctgttcgagatgagccggcacagcctggaacagaagcctacagacgcccctcctaaagagtccctggaactggaagatcccagctctggcctgggcgtgacaaagcaagatctgggccctgtgcctatgatggacccttctggaattcacggcgagggcaccagatgcaccggatggttcgatgtggaagccatcgtggaaagacggaccggcgacgtggtgtccgaggacgaagatgagaacctggaagataccggcgtggacctggtggacttcatcgacgatacctgcgagtttgagcaggccggcgacgaagctcctagagcactgctgcatgcccaagagacacaggcccatgtgaacgccgtgcactacctgaagcggaagttcacatgcagccctaccgtgtctcccctgggcaatgtgcagtgttctatcgagggcgagctgagccctagactgcacgccatccaactgaatgaaggcagcggcaaggccaagcggagactgtttctgcctgatagcggctacggcaataccgaggtggaaacccagctgtctcaggtggcaggatccgatggcgaatctcaagcccctggcggcaaagaaaatgtgcagcctgctgaaggcgctggcggagatgttcgacagctgctgagaagcagcaacctgaaggccacactgctgggcaagttcaaggacgtgtacggcatcggcttcaacgaactcgtgcggtgcttcaagagcgacaagaccgtgtgcaccgattgggttgtgggagctgctggcgtgcaccattctgtggccgaaggactgaagcacctgatcgagcctttctgcacatacgcccacatgcagtgcctgacctgcaactggggagtgtttctgctgctgctcatccggttcaagtgcggcaagaacagactgaccgtggccaagtgcatctctaccctgctgaacgtgcaagagccctacctgctgatcgaacctccaaagctgagatccacagccgccgctctgtactggtacagaaccggcatcagcaacgtgtccgaagtgatcggagagcctcctgagtggatcgtgcggcagaccatgtttcagcacagcctcgaggacagcatcttcgacctgtctcagatggtgcagtgggcctacgaccacgatctggtggacgatagcgccattgcctaccagtatgcccagctggccgacgtggactctaatgccgccgctttcctgaagtctaacgctcaggccaaatacgtgaaggactgcgccaccatgtgcagacactacaagagagccgagaagcaggccatgaccatgagccagtggatcagagccagatgcgataagaccgacgacggcggagattggaggcctatcgtgcagttcctgagataccagaacgtcgagttcatcacctttctgagcgcctttaaggccttcctgaagggaatccccaagagaagctgcatcgtgctgtacggccctccaaacaccggcaagagctacttcggaatgagcctgatgcagtttctgcagggcagcatcatcagctacgtgaacagcaacagccacttttggctggcccctctggccgaagctaaagtggccatgctggacgatgccacaccacagtgctggtcctacatcgacacctacatgcggagcgtgctggacggcaaccccatgagcattgaccggaagcacaagaacctgatccagatgaagtgtccgcctctgatcatcaccagcaacaccaacgtgggcgaagatgacagatggcgctacctgcactccagagtggtggtgttcaagttcgagcagacctttccattcgaccagaacggcaatcccgtgtacgagctgtccgacaagaattggaagtccttcttcagccggacctggtccagactcgagctgcaagaggatgaggacaccgagcaggatggctctacagtgcgggcctttaagtgtgtgcccggccagaacaccaatatcctgggctctatggtggaaggcagccaagagagagcccggacactgcacgaactgtgcgagcagagagaacagacccagcacgacatcgagctggactgcgtgtactgcctgaatcctctgaccagaaccgaggtgtacgacttcgccagatgggagctgagaatcgtgtacagacgggataccgcctacggcgtgtgcaagctgtgcctgaggttccacagcaaagtgcggaagtacaggcggtacaactactccatctacggccccacactggaacggcggacaaagaagcagctcgaagaactcgtgatccggtgctactgctgccagaaacctcagtgccccgtggaaaagcagcgccacgttgaccagggccagagattccacaacattgccgagcagtggaccggcagatgcctgcaatgttggaggccaacagccgctgaaaccggctctatgatcggccctggacctacactgcaggatatcgtgcttgagctggaacccgagcctgtggacctgagaggatatgagcagctggactccagcgaggacgaggacgagattgaccaccaccaacagcaggacagacccgatgtgcaagaagatgacggcgagcggtttagaatcctgagcgactgtcacgtgtgccagaataccgtgtcaagagtggtgcacagcacccacgacgacctgcacattctcgaggacctgcttatgggcaccctcgagatcgtggcccctaattgtgccgtgggcagcggcgccaccaatttcagtctgcttaaacaggccggggacgtcgaagagaaccccggacctatgcatcggcgcagatctcggtcttgtagagaagaccaaaagcctgtcatggatgatcaaagagatttaatttctaataatgaacaattacccatgttgggacggcgccccggagcccccgaatctaagtgcagccggggagctttatatacaggattttctattttagtgaccttattattagctggccaagccacaacagcttatttcttataccaacaacaaggacggttagataaattaacagtcacatctcaaaatttacaattagagaatttaagaatgaaattacctaaaccacccaaacccgtcagtaaaatgagaatggctacccccttattaatgcaagccctccccatgggcgccttaccccaaggacccatgcaaaatgctacaaagtatggaaatatgacagaagatcatgtcatgcacttattacaaaacgctgaccccttaaaagtctatccccctttaaaaggatctttccctgaaaatttaagacatttaaaaaatacaatggagacaattgattggaaagtctttgaatcttggatgcatcattggttattatttgaaatgtctaggcattctttagagcaaaaacccaccgatgctccacccaaggaaagtttagagttagaggacccttctagcggattaggagtcaccaaacaggacttaggacccgtccccatgatggaagccctgagcgagagactgaacgcctaccaggacaagatcctgaccttctacgaagaggactccaaggacctgagggaccagatcgagcattggagatgtgtgcggggagagtgcgccgtgttctacaaggccagagagatgggccacagccacatcaaccaccagcaggttccacctctgcacgtgtccagaggcaaggcccacaatgccattgagctgcagatggccctggaaagcctgaaccagagcgacttcaacaccgaggaatggaccctgcaggacacaagcctggaaatgtggcggaccgagcctcagtgctgcttcaaaaagaaaggcgagacagtgaccgtgctgtatgactgcgacaaggacaacagcatggactacaccctgtggggccacgtgtacgtgtggggagatacaggctgggacaaagtgtgcggaaaggtggactacggcggcctgtactatgtgctgcacggcctgaaagtgtactacgttgagttccagcaagaggccgtgaagtacagcaagaccaacaagtgggaagtgcatatcggcagaacagtgatcccctacagcgagtccgtgtcctctacagccctgtgcgaaagagtgcctatcgccgagatcgccaatggcctccagcagaccagcattccctctcacacacacgccaccaccaaagagaacgcttgggtttcctctcagcctcctaccaagcggtccagaagatctgatccaggcggcgatcctgtcagagccctggatgccaatagcagaaccctgctgtctggaaccgcctgcgagaataccaccggcaactcttacagcgactgcacccctgtggtgcacctgaaaggcgaccccaattgtctgaaggccctgcggttcagattcgtgaaacacaagaatctgttcgtgaacgtgtcctccacctggcggtggaccaacaacaccgaagagaaggccatcgtgactgtgacctttaaggacgagcagcagagacagcagttcctcggcagcgtgaagatccccaactccatctgtgtgtgcaagggcgtgatgacagttggcagcgaacagaaactgatctccgaggaagatctctga

SEQ ID NO: 32 - protein, 1736 aa, Macaca fascicularis
  MfPV3 Ii-E1E6E7-p2a-Ii-2 translated
MHRRRSRSCREDQKPVMDDQRDLISNNEQLPMLGRRPGAPESKCSRGALYTGFSILVTLLLAGQATTAYFLYQQQGRLDKLTVTSQNLQLENLRMKLPKPPKPVSKMRMATPLLMQALPMGALPQGPMQNATKYGNMTEDHVMHLLQNADPLKVYPPLKGSFPENLRHLKNTMETIDWKVFESWMHHWLLFEMSRHSLEQKPTDAPPKESLELEDPSSGLGVTKQDLGPVPMMDPSGIHGEGTRCTGWFDVEAIVERRTGDVVSEDEDENLEDTGVDLVDFIDDTCEFEQAGDEAPRALLHAQETQAHVNAVHYLKRKFTCSPTVSPLGNVQCSIEGELSPRLHAIQLNEGSGKAKRRLFLPDSGYGNTEVETQLSQVAGSDGESQAPGGKENVQPAEGAGGDVRQLLRSSNLKATLLGKFKDVYGIGFNELVRCFKSDKTVCTDWVVGAAGVHHSVAEGLKHLIEPFCTYAHMQCLTCNWGVFLLLLIRFKCGKNRLTVAKCISTLLNVQEPYLLIEPPKLRSTAAALYWYRTGISNVSEVIGEPPEWIVRQTMFQHSLEDSIFDLSQMVQWAYDHDLVDDSAIAYQYAQLADVDSNAAAFLKSNAQAKYVKDCATMCRHYKRAEKQAMTMSQWIRARCDKTDDGGDWRPIVQFLRYQNVEFITFLSAFKAFLKGIPKRSCIVLYGPPNTGKSYFGMSLMQFLQGSIISYVNSNSHFWLAPLAEAKVAMLDDATPQCWSYIDTYMRSVLDGNPMSIDRKHKNLIQMKCPPLIITSNTNVGEDDRWRYLHSRVVVFKFEQTFPFDQNGNPVYELSDKNWKSFFSRTWSRLELQEDEDTEQDGSTVRAFKCVPGQNTNILGSMVEGSQERARTLHELCEQREQTQHDIELDCVYCLNPLTRTEVYDFARWELRIVYRRDTAYGVCKLCLRFHSKVRKYRRYNYSIYGPTLERRTKKQLEELVIRCYCCQKPQCPVEKQRHVDQGQRFHNIAEQWTGRCLQCWRPTAAETGSMIGPGPTLQDIVLELEPEPVDLRGYEQLDSSEDEDEIDHHQQQDRPDVQEDDGERFRILSDCHVCQNTVSRVVHSTHDDLHILEDLLMGTLEIVAPNCAVGSGATNFSLLKQAGDVEENPGPMHRRRSRSCREDQKPVMDDQRDLISNNEQLPMLGRRPGAPESKCSRGALYTGFSILVTLLLAGQATTAYFLYQQQGRLDKLTVTSQNLQLENLRMKLPKPPKPVSKMRMATPLLMQALPMGALPQGPMQNATKYGNMTEDHVMHLLQNADPLKVYPPLKGSFPENLRHLKNTMETIDWKVFESWMHHWLLFEMSRHSLEQKPTDAPPKESLELEDPSSGLGVTKQDLGPVPMMEALSERLNAYQDKILTFYEEDSKDLRDQIEHWRCVRGECAVFYKAREMGHSHINHQQVPPLHVSRGKAHNAIELQMALESLNQSDFNTEEWTLQDTSLEMWRTEPQCCFKKKGETVTVLYDCDKDNSMDYTLWGHVYVWGDTGWDKVCGKVDYGGLYYVLHGLKVYYVEFQQEAVKYSKTNKWEVHIGRTVIPYSESVSSTALCERVPIAEIANGLQQTSIPSHTHATTKENAWVSSQPPTKRSRRSDPGGDPVRALDANSRTLLSGTACENTTGNSYSDCTPVVHLKGDPNCLKALRFRFVKHKNLFVNVSSTWRWTNNTEEKAIVTVTFKDEQQRQQFLGSVKIPNSICVCKGVMTVGSEQKLISEEDL

SEQ ID NO: 33 - DNA, 3369 bp, Macaca fascicularis
  MfPV3 Ii-E1E6E7
atgcacagaaggcggagcagaagctgccgcgaggatcagaaacccgtgatggacgaccagcgggacctgatcagcaacaacgagcagctgcctatgctcggcagaaggcctggcgctcctgagagcaaatgttctagaggcgccctgtacaccggcttcagcatcctggttacactgctgctggccggacaggctaccaccgcctactttctgtatcagcagcagggcagactggacaagctgaccgtgaccagccagaacctgcagctggaaaacctgcggatgaagctgcccaagcctcctaagcctgtgtccaagatgcggatggccacacctctgctgatgcaggctttgcctatgggagcactgcctcagggccctatgcagaacgccaccaaatacggcaacatgaccgaggaccacgtgatgcatctgctgcagaatgccgatcctctgaaggtgtaccctccactgaagggcagctttcccgagaacctgcggcacctgaagaacaccatggaaaccatcgactggaaggtgttcgagagctggatgcaccactggctgctgttcgagatgagccggcacagcctggaacagaagcctacagacgcccctcctaaagagtccctggaactggaagatcccagctctggcctgggcgtgacaaagcaagatctgggccctgtgcctatgatggacccttctggaattcacggcgagggcaccagatgcaccggatggttcgatgtggaagccatcgtggaaagacggaccggcgacgtggtgtccgaggacgaagatgagaacctggaagataccggcgtggacctggtggacttcatcgacgatacctgcgagtttgagcaggccggcgacgaagctcctagagcactgctgcatgcccaagagacacaggcccatgtgaacgccgtgcactacctgaagcggaagttcacatgcagccctaccgtgtctcccctgggcaatgtgcagtgttctatcgagggcgagctgagccctagactgcacgccatccaactgaatgaaggcagcggcaaggccaagcggagactgtttctgcctgatagcggctacggcaataccgaggtggaaacccagctgtctcaggtggcaggatccgatggcgaatctcaagcccctggcggcaaagaaaatgtgcagcctgctgaaggcgctggcggagatgttcgacagctgctgagaagcagcaacctgaaggccacactgctgggcaagttcaaggacgtgtacggcatcggcttcaacgaactcgtgcggtgcttcaagagcgacaagaccgtgtgcaccgattgggttgtgggagctgctggcgtgcaccattctgtggccgaaggactgaagcacctgatcgagcctttctgcacatacgcccacatgcagtgcctgacctgcaactggggagtgtttctgctgctgctcatccggttcaagtgcggcaagaacagactgaccgtggccaagtgcatctctaccctgctgaacgtgcaagagccctacctgctgatcgaacctccaaagctgagatccacagccgccgctctgtactggtacagaaccggcatcagcaacgtgtccgaagtgatcggagagcctcctgagtggatcgtgcggcagaccatgtttcagcacagcctcgaggacagcatcttcgacctgtctcagatggtgcagtgggcctacgaccacgatctggtggacgatagcgccattgcctaccagtatgcccagctggccgacgtggactctaatgccgccgctttcctgaagtctaacgctcaggccaaatacgtgaaggactgcgccaccatgtgcagacactacaagagagccgagaagcaggccatgaccatgagccagtggatcagagccagatgcgataagaccgacgacggcggagattggaggcctatcgtgcagttcctgagataccagaacgtcgagttcatcacctttctgagcgcctttaaggccttcctgaagggaatccccaagagaagctgcatcgtgctgtacggccctccaaacaccggcaagagctacttcggaatgagcctgatgcagtttctgcagggcagcatcatcagctacgtgaacagcaacagccacttttggctggcccctctggccgaagctaaagtggccatgctggacgatgccacaccacagtgctggtcctacatcgacacctacatgcggagcgtgctggacggcaaccccatgagcattgaccggaagcacaagaacctgatccagatgaagtgtccgcctctgatcatcaccagcaacaccaacgtgggcgaagatgacagatggcgctacctgcactccagagtggtggtgttcaagttcgagcagacctttccattcgaccagaacggcaatcccgtgtacgagctgtccgacaagaattggaagtccttcttcagccggacctggtccagactcgagctgcaagaggatgaggacaccgagcaggatggctctacagtgcgggcctttaagtgtgtgcccggccagaacaccaatatcctgggctctatggtggaaggcagccaagagagagcccggacactgcacgaactgtgcgagcagagagaacagacccagcacgacatcgagctggactgcgtgtactgcctgaatcctctgaccagaaccgaggtgtacgacttcgccagatgggagctgagaatcgtgtacagacgggataccgcctacggcgtgtgcaagctgtgcctgaggttccacagcaaagtgcggaagtacaggcggtacaactactccatctacggccccacactggaacggcggacaaagaagcagctcgaagaactcgtgatccggtgctactgctgccagaaacctcagtgccccgtggaaaagcagcgccacgttgaccagggccagagattccacaacattgccgagcagtggaccggcagatgcctgcaatgttggaggccaacagccgctgaaaccggctctatgatcggccctggacctacactgcaggatatcgtgcttgagctggaacccgagcctgtggacctgagaggatatgagcagctggactccagcgaggacgaggacgagattgaccaccaccaacagcaggacagacccgatgtgcaagaagatgacggcgagcggtttagaatcctgagcgactgtcacgtgtgccagaataccgtgtcaagagtggtgcacagcacccacgacgacctgcacattctcgaggacctgcttatgggcaccctcgagatcgtggcccctaattgtgccgtgggcagcgaacagaaactgatctccgaggaagatctctga

SEQ ID NO: 34 - protein, 1122 aa, Macaca fascicularis
  MfPV3 Ii-E1E6E7 translated
MHRRRSRSCREDQKPVMDDQRDLISNNEQLPMLGRRPGAPESKCSRGALYTGFSILVTLLLAGQATTAYFLYQQQGRLDKLTVTSQNLQLENLRMKLPKPPKPVSKMRMATPLLMQALPMGALPQGPMQNATKYGNMTEDHVMHLLQNADPLKVYPPLKGSFPENLRHLKNTMETIDWKVFESWMHHWLLFEMSRHSLEQKPTDAPPKESLELEDPSSGLGVTKQDLGPVPMMDPSGIHGEGTRCTGWFDVEAIVERRTGDVVSEDEDENLEDTGVDLVDFIDDTCEFEQAGDEAPRALLHAQETQAHVNAVHYLKRKFTCSPTVSPLGNVQCSIEGELSPRLHAIQLNEGSGKAKRRLFLPDSGYGNTEVETQLSQVAGSDGESQAPGGKENVQPAEGAGGDVRQLLRSSNLKATLLGKFKDVYGIGFNELVRCFKSDKTVCTDWVVGAAGVHHSVAEGLKHLIEPFCTYAHMQCLTCNWGVFLLLLIRFKCGKNRLTVAKCISTLLNVQEPYLLIEPPKLRSTAAALYWYRTGISNVSEVIGEPPEWIVRQTMFQHSLEDSIFDLSQMVQWAYDHDLVDDSAIAYQYAQLADVDSNAAAFLKSNAQAKYVKDCATMCRHYKRAEKQAMTMSQWIRARCDKTDDGGDWRPIVQFLRYQNVEFITFLSAFKAFLKGIPKRSCIVLYGPPNTGKSYFGMSLMQFLQGSIISYVNSNSHFWLAPLAEAKVAMLDDATPQCWSYIDTYMRSVLDGNPMSIDRKHKNLIQMKCPPLIITSNTNVGEDDRWRYLHSRVVVFKFEQTFPFDQNGNPVYELSDKNWKSFFSRTWSRLELQEDEDTEQDGSTVRAFKCVPGQNTNILGSMVEGSQERARTLHELCEQREQTQHDIELDCVYCLNPLTRTEVYDFARWELRIVYRRDTAYGVCKLCLRFHSKVRKYRRYNYSIYGPTLERRTKKQLEELVIRCYCCQKPQCPVEKQRHVDQGQRFHNIAEQWTGRCLQCWRPTAAETGSMIGPGPTLQDIVLELEPEPVDLRGYEQLDSSEDEDEIDHHQQQDRPDVQEDDGERFRILSDCHVCQNTVSRVVHSTHDDLHILEDLLMGTLEIVAPNCAVGSEQKLISEEDL

SEQ ID NO: 35 - DNA, 4515 bp, Human papillomavirus type 16
  HPV16 Ii-E1E2E6E7
atgcacagaaggcggagcagaagctgccgcgaggatcagaaacccgtgatggacgaccagcgggacctgatcagcaacaacgagcagctgcctatgctcggcagaaggcctggcgctcctgagagcaaatgttctagaggcgccctgtacaccggcttcagcatcctggttacactgctgctggccggacaggctaccaccgcctactttctgtatcagcagcagggcagactggacaagctgaccgtgaccagccagaacctgcagctggaaaacctgcggatgaagctgcccaagcctcctaagcctgtgtccaagatgcggatggccacacctctgctgatgcaggctttgcctatgggagcactgcctcagggccctatgcagaacgccaccaaatacggcaacatgaccgaggaccacgtgatgcatctgctgcagaatgccgatcctctgaaggtgtaccctccactgaagggcagctttcccgagaacctgcggcacctgaagaacaccatggaaaccatcgactggaaggtgttcgagagctggatgcaccactggctgctgttcgagatgagccggcacagcctggaacagaagcctacagacgcccctcctaaagagtccctggaactggaagatcccagctctggcctgggcgtgacaaagcaagatctgggccctgtgcctatgatggccgatcctgctggcacaaacggcgaagaaggcacaggctgcaacggctggttttacgtggaagccgtggtggaaaagaaaaccggcgacgccatcagcgacgacgagaacgagaatgacagcgacaccggcgaggacctggtggacttcatcgtgaacgacaacgactacctgacacaggccgagacagagacagcccacgctctgtttacagcccaagaggccaagcagcacagagatgccgttcaggtgctgaagagaaagtacctgggcagccctctgagcgacatcagcggctgtgtggacaacaacatcagccccagactgaaggccatctgcatcgagaagcagagcagagccgccaagcggagactgtttgagagcgaggatagcggctacggcaataccgaggtggaaacccagcaaatgctgcaggtcgagggcagacacgaaaccgagacaccttgcagccagtacagcggaggatctggcggaggctgtagccagtactcttctggaagtggcggagagggcgtgtccgagagacacaccatttgtcagacccctctgaccaacatcctgaacgtgctgaaaaccagcaacgccaaggccgccatgctggccaagttcaaagagctgtacggcgtcagcttcagcgaactcgtgcggcccttcaagagcaacaagtccacctgttgcgactggtgcattgccgcctttggcctgacaccttctatcgccgacagcatcaagaccctgctccagcagtactgtctgtacctgcacattcagagcctggcctgctcttggggaatggtggtgctgctgctcgtgcggtacaagtgcggcaagaacagagagacaattgagaagctgctgagcaaactgctgtgcgtgtcccctatgtgcatgatgatcgagcctccaaagctgcggtctacagccgccgctctgtactggtacaagaccggcatcagcaatatctccgaggtgtacggcgacacccctgagtggattcagagacagaccgtcctgcagcacagcttcaacgactgcaccttcgagctgtcccagatggtgcagtgggcctacgacaatgacatcgtggacgactccgagatcgcctataagtacgcccagctggccgacaccaacagcaatgccagcgccttcctgaagtccaacagccaggccaagatcgtgaaggactgcgccaccatgtgcagacactacaagcgggccgagaagaaacagatgagcatgagccagtggatcaagtacagatgcgacagagtggacgacggcggcgattggaagcagatcgtgatgttcctgagataccagggcgtcgagttcatgagctttctgacagccctgaagcggttcctgcagggcatccccaagaagaactgcatcctgctgtatggcgccgctaacaccggcaagagcctgttcggaatgagcctgatgaagtttctgcagggctccgtgatctgctttgtgaacagcaagagccacttctggctccagccactggccgatgccaagattggcatgctggacgatgccaccgtgccttgctggaactacatcgacgacaacctgagaaacgccctggacggcaacctggtttctatggacgtgaagcacagacccctggtgcagctgaagtgtcctccactgctgatcaccagcaacatcaacgccggcaccgattccagatggccctatctgcacaaccggctggtggtgtttacctttcctaacgagttccccttcgacgaaaacggcaaccccgtgtacgagctgaacgataagaattggaagtccttcttcagccggacctggtccagactgagcctgcacgaggatgaggacaaagagaacgacggcgacagcctgcctaccttcaaatgtgtcagcggccagaacaccaacacactgggcagcatggaaacactgtgccagcggctgaacgtgtgccaggacaagattctgacccactatgagaacgacagcaccgacctgagggaccacatcgactactggaagcacatgcggctggaatgcgccatctactacaaggctagagagatgggcttcaagcacatcaaccaccaggtggtgcctacactggccgtgtctaagaacaaggctctgcaggccatcgaactgcagctgaccctggaaacaatctacaactcccagtactccaacgagaagtggaccctccaggacgtgtcactggaagtgtacctgaccgctcctaccggctgcatcaagaaacacggctacaccgtggaagtgcagtttgacggcgatatctgcaataccatgcactacaccaactggacccacatctacatctgcgaagaggccagcgtgacagtggtggaaggccaggtcgactactacggcctgtactacgtgcacgagggcatcagaacctacttcgtgcagttcaaggatgacgccgagaagtacagcaagaacaaagtgtgggaagtgcacgctggcggccaagtgatcctgtgtcctacaagcgtgttcagcagcaacgaagtgtctagccccgagatcatcagacagcacctggccaatcatcctgccgccacacacacaaaagctgtggccctgggcaccgaggaaacacagaccacaattcagaggcccagaagcgagcccgataccggcaatccttgtcacaccaccaagctgctgcaccgggattccgtggattctgcccctatcctgaccgccttcaacagctcccacaaaggccggatcaactgcaacagcaacaccacacctatcgtgcacctgaaaggggacgccaacactctgaaggccctgcggtacagattcaagaagcactgtaccctgtataccgccgtgtccagcacatggcactggaccggacacaacgtgaaacacaagagcgccatcgtgaccctgacctacgatagcgagtggcagagggaccagttcctgagccaagtgaagatccctaagaccatcaccgtgtccaccggctttatgagcattggcagcatgcaccagaaacggacagccatgttccaggatcctcaagagcggccacggaagctgcctcagctgtgtacagaactgcagaccaccatccacgacatcatcctcgagtgcgtgtactgcaagcagcagctcctgcggagagaagtgtacgacttcgccttccgggatctgtgcatcgtgtacagagatggcaacccctacgccgtgtgcgacaagtgcctgaagttctactccaagatcagcgagtaccggcactactgctactccctgtacggcaccacacttgagcagcagtacaacaagcccctgtgcgatctgctgatccggtgcatcaactgccagaaacctcagtgccccgaggaaaagcagagacacctggacaagaagcagcggttccacaacattagaggcagatggacaggccggtgcatgagctgctgtagaagcagcagaacaagacggggctccatgcacggcgataccccaacactgcacgagtacatgctggatctgcagcccgagacaaccgatctgtacggctatgagcagctgaatgactccagcgaggaagaggacgagatcgacggacctgctggacaggctgaacctgatagagcccactacaatatcgtgaccttctgctgcaagtgcgatagcaccctgagaagatgcgtgcagagcacccacgtggacatcaggaccctcgaggatctgctcatgggcaccctgggaattgtggccccaatctgctctcagaagccttga

SEQ ID NO: 36 - protein, 1504 aa, Human papillomavirus type 16
  HPV16 Ii-E1E2E6E7 translated
MHRRRSRSCREDQKPVMDDQRDLISNNEQLPMLGRRPGAPESKCSRGALYTGFSILVTLLLAGQATTAYFLYQQQGRLDKLTVTSQNLQLENLRMKLPKPPKPVSKMRMATPLLMQALPMGALPQGPMQNATKYGNMTEDHVMHLLQNADPLKVYPPLKGSFPENLRHLKNTMETIDWKVFESWMHHWLLFEMSRHSLEQKPTDAPPKESLELEDPSSGLGVTKQDLGPVPMMADPAGTNGEEGTGCNGWFYVEAVVEKKTGDAISDDENENDSDTGEDLVDFIVNDNDYLTQAETETAHALFTAQEAKQHRDAVQVLKRKYLGSPLSDISGCVDNNISPRLKAICIEKQSRAAKRRLFESEDSGYGNTEVETQQMLQVEGRHETETPCSQYSGGSGGGCSQYSSGSGGEGVSERHTICQTPLTNILNVLKTSNAKAAMLAKFKELYGVSFSELVRPFKSNKSTCCDWCIAAFGLTPSIADSIKTLLQQYCLYLHIQSLACSWGMVVLLLVRYKCGKNRETIEKLLSKLLCVSPMCMMIEPPKLRSTAAALYWYKTGISNISEVYGDTPEWIQRQTVLQHSFNDCTFELSQMVQWAYDNDIVDDSEIAYKYAQLADTNSNASAFLKSNSQAKIVKDCATMCRHYKRAEKKQMSMSQWIKYRCDRVDDGGDWKQIVMFLRYQGVEFMSFLTALKRFLQGIPKKNCILLYGAANTGKSLFGMSLMKFLQGSVICFVNSKSHFWLQPLADAKIGMLDDATVPCWNYIDDNLRNALDGNLVSMDVKHRPLVQLKCPPLLITSNINAGTDSRWPYLHNRLVVFTFPNEFPFDENGNPVYELNDKNWKSFFSRTWSRLSLHEDEDKENDGDSLPTFKCVSGQNTNTLGSMETLCQRLNVCQDKILTHYENDSTDLRDHIDYWKHMRLECAIYYKAREMGFKHINHQVVPTLAVSKNKALQAIELQLTLETIYNSQYSNEKWTLQDVSLEVYLTAPTGCIKKHGYTVEVQFDGDICNTMHYTNWTHIYICEEASVTVVEGQVDYYGLYYVHEGIRTYFVQFKDDAEKYSKNKVWEVHAGGQVILCPTSVFSSNEVSSPEIIRQHLANHPAATHTKAVALGTEETQTTIQRPRSEPDTGNPCHTTKLLHRDSVDSAPILTAFNSSHKGRINCNSNTTPIVHLKGDANTLKALRYRFKKHCTLYTAVSSTWHWTGHNVKHKSAIVTLTYDSEWQRDQFLSQVKIPKTITVSTGFMSIGSMHQKRTAMFQDPQERPRKLPQLCTELQTTIHDIILECVYCKQQLLRREVYDFAFRDLCIVYRDGNPYAVCDKCLKFYSKISEYRHYCYSLYGTTLEQQYNKPLCDLLIRCINCQKPQCPEEKQRHLDKKQRFHNIRGRWTGRCMSCCRSSRTRRGSMHGDTPTLHEYMLDLQPETTDLYGYEQLNDSSEEEDEIDGPAGQAEPDRAHYNIVTFCCKCDSTLRRCVQSTHVDIRTLEDLLMGTLGIVAPICSQKP

SEQ ID NO: 37 - DNA, 5277 bp, Human papillomavirus type 16
  HPV16 Ii-E1E2-p2a-Ii-E6E7
atgcacagaaggcggagcagaagctgccgcgaggatcagaaacccgtgatggacgaccagcgggacctgatcagcaacaacgagcagctgcctatgctcggcagaaggcctggcgctcctgagagcaaatgttctagaggcgccctgtacaccggcttcagcatcctggttacactgctgctggccggacaggctaccaccgcctactttctgtatcagcagcagggcagactggacaagctgaccgtgaccagccagaacctgcagctggaaaacctgcggatgaagctgcccaagcctcctaagcctgtgtccaagatgcggatggccacacctctgctgatgcaggctttgcctatgggagcactgcctcagggccctatgcagaacgccaccaaatacggcaacatgaccgaggaccacgtgatgcatctgctgcagaatgccgatcctctgaaggtgtaccctccactgaagggcagctttcccgagaacctgcggcacctgaagaacaccatggaaaccatcgactggaaggtgttcgagagctggatgcaccactggctgctgttcgagatgagccggcacagcctggaacagaagcctacagacgcccctcctaaagagtccctggaactggaagatcccagctctggcctgggcgtgacaaagcaagatctgggccctgtgcctatgatggccgatcctgctggcacaaacggcgaagaaggcacaggctgcaacggctggttttacgtggaagccgtggtggaaaagaaaaccggcgacgccatcagcgacgacgagaacgagaatgacagcgacaccggcgaggacctggtggacttcatcgtgaacgacaacgactacctgacacaggccgagacagagacagcccacgctctgtttacagcccaagaggccaagcagcacagagatgccgttcaggtgctgaagagaaagtacctgggcagccctctgagcgacatcagcggctgtgtggacaacaacatcagccccagactgaaggccatctgcatcgagaagcagagcagagccgccaagcggagactgtttgagagcgaggatagcggctacggcaataccgaggtggaaacccagcaaatgctgcaggtcgagggcagacacgaaaccgagacaccttgcagccagtacagcggaggatctggcggaggctgtagccagtactcttctggaagtggcggagagggcgtgtccgagagacacaccatttgtcagacccctctgaccaacatcctgaacgtgctgaaaaccagcaacgccaaggccgccatgctggccaagttcaaagagctgtacggcgtcagcttcagcgaactcgtgcggcccttcaagagcaacaagtccacctgttgcgactggtgcattgccgcctttggcctgacaccttctatcgccgacagcatcaagaccctgctccagcagtactgtctgtacctgcacattcagagcctggcctgctcttggggaatggtggtgctgctgctcgtgcggtacaagtgcggcaagaacagagagacaattgagaagctgctgagcaaactgctgtgcgtgtcccctatgtgcatgatgatcgagcctccaaagctgcggtctacagccgccgctctgtactggtacaagaccggcatcagcaatatctccgaggtgtacggcgacacccctgagtggattcagagacagaccgtcctgcagcacagcttcaacgactgcaccttcgagctgtcccagatggtgcagtgggcctacgacaatgacatcgtggacgactccgagatcgcctataagtacgcccagctggccgacaccaacagcaatgccagcgccttcctgaagtccaacagccaggccaagatcgtgaaggactgcgccaccatgtgcagacactacaagcgggccgagaagaaacagatgagcatgagccagtggatcaagtacagatgcgacagagtggacgacggcggcgattggaagcagatcgtgatgttcctgagataccagggcgtcgagttcatgagctttctgacagccctgaagcggttcctgcagggcatccccaagaagaactgcatcctgctgtatggcgccgctaacaccggcaagagcctgttcggaatgagcctgatgaagtttctgcagggctccgtgatctgctttgtgaacagcaagagccacttctggctccagccactggccgatgccaagattggcatgctggacgatgccaccgtgccttgctggaactacatcgacgacaacctgagaaacgccctggacggcaacctggtttctatggacgtgaagcacagacccctggtgcagctgaagtgtcctccactgctgatcaccagcaacatcaacgccggcaccgattccagatggccctatctgcacaaccggctggtggtgtttacctttcctaacgagttccccttcgacgaaaacggcaaccccgtgtacgagctgaacgataagaattggaagtccttcttcagccggacctggtccagactgagcctgcacgaggatgaggacaaagagaacgacggcgacagcctgcctaccttcaaatgtgtcagcggccagaacaccaacacactgggcagcatggaaacactgtgccagcggctgaacgtgtgccaggacaagattctgacccactatgagaacgacagcaccgacctgagggaccacatcgactactggaagcacatgcggctggaatgcgccatctactacaaggctagagagatgggcttcaagcacatcaaccaccaggtggtgcctacactggccgtgtctaagaacaaggctctgcaggccatcgaactgcagctgaccctggaaacaatctacaactcccagtactccaacgagaagtggaccctccaggacgtgtcactggaagtgtacctgaccgctcctaccggctgcatcaagaaacacggctacaccgtggaagtgcagtttgacggcgatatctgcaataccatgcactacaccaactggacccacatctacatctgcgaagaggccagcgtgacagtggtggaaggccaggtcgactactacggcctgtactacgtgcacgagggcatcagaacctacttcgtgcagttcaaggatgacgccgagaagtacagcaagaacaaagtgtgggaagtgcacgctggcggccaagtgatcctgtgtcctacaagcgtgttcagcagcaacgaagtgtctagccccgagatcatcagacagcacctggccaatcatcctgccgccacacacacaaaagctgtggccctgggcaccgaggaaacacagaccacaattcagaggcccagaagcgagcccgataccggcaatccttgtcacaccaccaagctgctgcaccgggattccgtggattctgcccctatcctgaccgccttcaacagctcccacaaaggccggatcaactgcaacagcaacaccacacctatcgtgcacctgaaaggggacgccaacactctgaaggccctgcggtacagattcaagaagcactgtaccctgtataccgccgtgtccagcacatggcactggaccggacacaacgtgaaacacaagagcgccatcgtgaccctgacctacgatagcgagtggcagagggaccagttcctgagccaagtgaagatccctaagaccatcaccgtgtccaccggctttatgagcattggcagcggcagcggcgccaccaatttcagtctgcttaaacaggccggggacgtcgaagagaaccccggacctatgcatcggcgcagatctcggtcttgtagagaagaccaaaagcctgtcatggatgatcaaagagatttaatttctaataatgaacaattacccatgttgggacggcgccccggagcccccgaatctaagtgcagccggggagctttatatacaggattttctattttagtgaccttattattagctggccaagccacaacagcttatttcttataccaacaacaaggacggttagataaattaacagtcacatctcaaaatttacaattagagaatttaagaatgaaattacctaaaccacccaaacccgtcagtaaaatgagaatggctacccccttattaatgcaagccctccccatgggcgccttaccccaaggacccatgcaaaatgctacaaagtatggaaatatgacagaagatcatgtcatgcacttattacaaaacgctgaccccttaaaagtctatccccctttaaaaggatctttccctgaaaatttaagacatttaaaaaatacaatggagacaattgattggaaagtctttgaatcttggatgcatcattggttattatttgaaatgtctaggcattctttagagcaaaaacccaccgatgctccacccaaggaaagtttagagttagaggacccttctagcggattaggagtcaccaaacaggacttaggacccgtccccatgatgcaccagaaacggacagccatgttccaggatcctcaagagcggccacggaagctgcctcagctgtgtacagaactgcagaccaccatccacgacatcatcctcgagtgcgtgtactgcaagcagcagctcctgcggagagaagtgtacgacttcgccttccgggatctgtgcatcgtgtacagagatggcaacccctacgccgtgtgcgacaagtgcctgaagttctactccaagatcagcgagtaccggcactactgctactccctgtacggcaccacacttgagcagcagtacaacaagcccctgtgcgatctgctgatccggtgcatcaactgccagaaacctcagtgccccgaggaaaagcagagacacctggacaagaagcagcggttccacaacattagaggcagatggacaggccggtgcatgagctgctgtagaagcagcagaacaagacggggctccatgcacggcgataccccaacactgcacgagtacatgctggatctgcagcccgagacaaccgatctgtacggctatgagcagctgaatgactccagcgaggaagaggacgagatcgacggacctgctggacaggctgaacctgatagagcccactacaatatcgtgaccttctgctgcaagtgcgatagcaccctgagaagatgcgtgcagagcacccacgtggacatcaggaccctcgaggatctgctcatgggcaccctgggaattgtggccccaatctgctctcagaagccttga

SEQ ID NO: 38 - protein, 1758 aa, Human papillomavirus type 16
  HPV16 Ii-E1E2-p2a-Ii-E6E7 translated
MHRRRSRSCREDQKPVMDDQRDLISNNEQLPMLGRRPGAPESKCSRGALYTGFSILVTLLLAGQATTAYFLYQQQGRLDKLTVTSQNLQLENLRMKLPKPPKPVSKMRMATPLLMQALPMGALPQGPMQNATKYGNMTEDHVMHLLQNADPLKVYPPLKGSFPENLRHLKNTMETIDWKVFESWMHHWLLFEMSRHSLEQKPTDAPPKESLELEDPSSGLGVTKQDLGPVPMMADPAGTNGEEGTGCNGWFYVEAVVEKKTGDAISDDENENDSDTGEDLVDFIVNDNDYLTQAETETAHALFTAQEAKQHRDAVQVLKRKYLGSPLSDISGCVDNNISPRLKAICIEKQSRAAKRRLFESEDSGYGNTEVETQQMLQVEGRHETETPCSQYSGGSGGGCSQYSSGSGGEGVSERHTICQTPLTNILNVLKTSNAKAAMLAKFKELYGVSFSELVRPFKSNKSTCCDWCIAAFGLTPSIADSIKTLLQQYCLYLHIQSLACSWGMVVLLLVRYKCGKNRETIEKLLSKLLCVSPMCMMIEPPKLRSTAAALYWYKTGISNISEVYGDTPEWIQRQTVLQHSFNDCTFELSQMVQWAYDNDIVDDSEIAYKYAQLADTNSNASAFLKSNSQAKIVKDCATMCRHYKRAEKKQMSMSQWIKYRCDRVDDGGDWKQIVMFLRYQGVEFMSFLTALKRFLQGIPKKNCILLYGAANTGKSLFGMSLMKFLQGSVICFVNSKSHFWLQPLADAKIGMLDDATVPCWNYIDDNLRNALDGNLVSMDVKHRPLVQLKCPPLLITSNINAGTDSRWPYLHNRLVVFTFPNEFPFDENGNPVYELNDKNWKSFFSRTWSRLSLHEDEDKENDGDSLPTFKCVSGQNTNTLGSMETLCQRLNVCQDKILTHYENDSTDLRDHIDYWKHMRLECAIYYKAREMGFKHINHQVVPTLAVSKNKALQAIELQLTLETIYNSQYSNEKWTLQDVSLEVYLTAPTGCIKKHGYTVEVQFDGDICNTMHYTNWTHIYICEEASVTVVEGQVDYYGLYYVHEGIRTYFVQFKDDAEKYSKNKVWEVHAGGQVILCPTSVFSSNEVSSPEIIRQHLANHPAATHTKAVALGTEETQTTIQRPRSEPDTGNPCHTTKLLHRDSVDSAPILTAFNSSHKGRINCNSNTTPIVHLKGDANTLKALRYRFKKHCTLYTAVSSTWHWTGHNVKHKSAIVTLTYDSEWQRDQFLSQVKIPKTITVSTGFMSIGSGSGATNFSLLKQAGDVEENPGPMHRRRSRSCREDQKPVMDDQRDLISNNEQLPMLGRRPGAPESKCSRGALYTGFSILVTLLLAGQATTAYFLYQQQGRLDKLTVTSQNLQLENLRMKLPKPPKPVSKMRMATPLLMQALPMGALPQGPMQNATKYGNMTEDHVMHLLQNADPLKVYPPLKGSFPENLRHLKNTMETIDWKVFESWMHHWLLFEMSRHSLEQKPTDAPPKESLELEDPSSGLGVTKQDLGPVPMMHQKRTAMFQDPQERPRKLPQLCTELQTTIHDIILECVYCKQQLLRREVYDFAFRDLCIVYRDGNPYAVCDKCLKFYSKISEYRHYCYSLYGTTLEQQYNKPLCDLLIRCINCQKPQCPEEKQRHLDKKQRFHNIRGRWTGRCMSCCRSSRTRRGSMHGDTPTLHEYMLDLQPETTDLYGYEQLNDSSEEEDEIDGPAGQAEPDRAHYNIVTFCCKCDSTLRRCVQSTHVDIRTLEDLLMGTLGIVAPICSQKP

SEQ ID NO: 39 - DNA, 3819 bp, Human papillomavirus type 16
  HPV16 E1E2E6E7
atggccgatcctgctggcacaaacggcgaagaaggcacaggctgcaacggctggttttacgtggaagccgtggtggaaaagaaaaccggcgacgccatcagcgacgacgagaacgagaatgacagcgacaccggcgaggacctggtggacttcatcgtgaacgacaacgactacctgacacaggccgagacagagacagcccacgctctgtttacagcccaagaggccaagcagcacagagatgccgttcaggtgctgaagagaaagtacctgggcagccctctgagcgacatcagcggctgtgtggacaacaacatcagccccagactgaaggccatctgcatcgagaagcagagcagagccgccaagcggagactgtttgagagcgaggatagcggctacggcaataccgaggtggaaacccagcaaatgctgcaggtcgagggcagacacgaaaccgagacaccttgcagccagtacagcggaggatctggcggaggctgtagccagtactcttctggaagtggcggagagggcgtgtccgagagacacaccatttgtcagacccctctgaccaacatcctgaacgtgctgaaaaccagcaacgccaaggccgccatgctggccaagttcaaagagctgtacggcgtcagcttcagcgaactcgtgcggcccttcaagagcaacaagtccacctgttgcgactggtgcattgccgcctttggcctgacaccttctatcgccgacagcatcaagaccctgctccagcagtactgtctgtacctgcacattcagagcctggcctgctcttggggaatggtggtgctgctgctcgtgcggtacaagtgcggcaagaacagagagacaattgagaagctgctgagcaaactgctgtgcgtgtcccctatgtgcatgatgatcgagcctccaaagctgcggtctacagccgccgctctgtactggtacaagaccggcatcagcaatatctccgaggtgtacggcgacacccctgagtggattcagagacagaccgtcctgcagcacagcttcaacgactgcaccttcgagctgtcccagatggtgcagtgggcctacgacaatgacatcgtggacgactccgagatcgcctataagtacgcccagctggccgacaccaacagcaatgccagcgccttcctgaagtccaacagccaggccaagatcgtgaaggactgcgccaccatgtgcagacactacaagcgggccgagaagaaacagatgagcatgagccagtggatcaagtacagatgcgacagagtggacgacggcggcgattggaagcagatcgtgatgttcctgagataccagggcgtcgagttcatgagctttctgacagccctgaagcggttcctgcagggcatccccaagaagaactgcatcctgctgtatggcgccgctaacaccggcaagagcctgttcggaatgagcctgatgaagtttctgcagggctccgtgatctgctttgtgaacagcaagagccacttctggctccagccactggccgatgccaagattggcatgctggacgatgccaccgtgccttgctggaactacatcgacgacaacctgagaaacgccctggacggcaacctggtttctatggacgtgaagcacagacccctggtgcagctgaagtgtcctccactgctgatcaccagcaacatcaacgccggcaccgattccagatggccctatctgcacaaccggctggtggtgtttacctttcctaacgagttccccttcgacgaaaacggcaaccccgtgtacgagctgaacgataagaattggaagtccttcttcagccggacctggtccagactgagcctgcacgaggatgaggacaaagagaacgacggcgacagcctgcctaccttcaaatgtgtcagcggccagaacaccaacacactgggcagcatggaaacactgtgccagcggctgaacgtgtgccaggacaagattctgacccactatgagaacgacagcaccgacctgagggaccacatcgactactggaagcacatgcggctggaatgcgccatctactacaaggctagagagatgggcttcaagcacatcaaccaccaggtggtgcctacactggccgtgtctaagaacaaggctctgcaggccatcgaactgcagctgaccctggaaacaatctacaactcccagtactccaacgagaagtggaccctccaggacgtgtcactggaagtgtacctgaccgctcctaccggctgcatcaagaaacacggctacaccgtggaagtgcagtttgacggcgatatctgcaataccatgcactacaccaactggacccacatctacatctgcgaagaggccagcgtgacagtggtggaaggccaggtcgactactacggcctgtactacgtgcacgagggcatcagaacctacttcgtgcagttcaaggatgacgccgagaagtacagcaagaacaaagtgtgggaagtgcacgctggcggccaagtgatcctgtgtcctacaagcgtgttcagcagcaacgaagtgtctagccccgagatcatcagacagcacctggccaatcatcctgccgccacacacacaaaagctgtggccctgggcaccgaggaaacacagaccacaattcagaggcccagaagcgagcccgataccggcaatccttgtcacaccaccaagctgctgcaccgggattccgtggattctgcccctatcctgaccgccttcaacagctcccacaaaggccggatcaactgcaacagcaacaccacacctatcgtgcacctgaaaggggacgccaacactctgaaggccctgcggtacagattcaagaagcactgtaccctgtataccgccgtgtccagcacatggcactggaccggacacaacgtgaaacacaagagcgccatcgtgaccctgacctacgatagcgagtggcagagggaccagttcctgagccaagtgaagatccctaagaccatcaccgtgtccaccggctttatgagcattggcagcatgcaccagaaacggacagccatgttccaggatcctcaagagcggccacggaagctgcctcagctgtgtacagaactgcagaccaccatccacgacatcatcctcgagtgcgtgtactgcaagcagcagctcctgcggagagaagtgtacgacttcgccttccgggatctgtgcatcgtgtacagagatggcaacccctacgccgtgtgcgacaagtgcctgaagttctactccaagatcagcgagtaccggcactactgctactccctgtacggcaccacacttgagcagcagtacaacaagcccctgtgcgatctgctgatccggtgcatcaactgccagaaacctcagtgccccgaggaaaagcagagacacctggacaagaagcagcggttccacaacattagaggcagatggacaggccggtgcatgagctgctgtagaagcagcagaacaagacggggctccatgcacggcgataccccaacactgcacgagtacatgctggatctgcagcccgagacaaccgatctgtacggctatgagcagctgaatgactccagcgaggaagaggacgagatcgacggacctgctggacaggctgaacctgatagagcccactacaatatcgtgaccttctgctgcaagtgcgatagcaccctgagaagatgcgtgcagagcacccacgtggacatcaggaccctcgaggatctgctcatgggcaccctgggaattgtggccccaatctgctctcagaagccttga

SEQ ID NO: 40 - protein, 1272 aa, Human papillomavirus type 16
  HPV16 E1E2E6E7 translated
MADPAGTNGEEGTGCNGWFYVEAVVEKKTGDAISDDENENDSDTGEDLVDFIVNDNDYLTQAETETAHALFTAQEAKQHRDAVQVLKRKYLGSPLSDISGCVDNNISPRLKAICIEKQSRAAKRRLFESEDSGYGNTEVETQQMLQVEGRHETETPCSQYSGGSGGGCSQYSSGSGGEGVSERHTICQTPLTNILNVLKTSNAKAAMLAKFKELYGVSFSELVRPFKSNKSTCCDWCIAAFGLTPSIADSIKTLLQQYCLYLHIQSLACSWGMVVLLLVRYKCGKNRETIEKLLSKLLCVSPMCMMIEPPKLRSTAAALYWYKTGISNISEVYGDTPEWIQRQTVLQHSFNDCTFELSQMVQWAYDNDIVDDSEIAYKYAQLADTNSNASAFLKSNSQAKIVKDCATMCRHYKRAEKKQMSMSQWIKYRCDRVDDGGDWKQIVMFLRYQGVEFMSFLTALKRFLQGIPKKNCILLYGAANTGKSLFGMSLMKFLQGSVICFVNSKSHFWLQPLADAKIGMLDDATVPCWNYIDDNLRNALDGNLVSMDVKHRPLVQLKCPPLLITSNINAGTDSRWPYLHNRLVVFTFPNEFPFDENGNPVYELNDKNWKSFFSRTWSRLSLHEDEDKENDGDSLPTFKCVSGQNTNTLGSMETLCQRLNVCQDKILTHYENDSTDLRDHIDYWKHMRLECAIYYKAREMGFKHINHQVVPTLAVSKNKALQAIELQLTLETIYNSQYSNEKWTLQDVSLEVYLTAPTGCIKKHGYTVEVQFDGDICNTMHYTNWTHIYICEEASVTVVEGQVDYYGLYYVHEGIRTYFVQFKDDAEKYSKNKVWEVHAGGQVILCPTSVFSSNEVSSPEIIRQHLANHPAATHTKAVALGTEETQTTIQRPRSEPDTGNPCHTTKLLHRDSVDSAPILTAFNSSHKGRINCNSNTTPIVHLKGDANTLKALRYRFKKHCTLYTAVSSTWHWTGHNVKHKSAIVTLTYDSEWQRDQFLSQVKIPKTITVSTGFMSIGSMHQKRTAMFQDPQERPRKLPQLCTELQTTIHDIILECVYCKQQLLRREVYDFAFRDLCIVYRDGNPYAVCDKCLKFYSKISEYRHYCYSLYGTTLEQQYNKPLCDLLIRCINCQKPQCPEEKQRHLDKKQRFHNIRGRWTGRCMSCCRSSRTRRGSMHGDTPTLHEYMLDLQPETTDLYGYEQLNDSSEEEDEIDGPAGQAEPDRAHYNIVTFCCKCDSTLRRCVQSTHVDIRTLEDLLMGTLGIVAPICSQKP

SEQ ID NO: 41 - DNA, 5271 bp, Human papillomavirus type 16
  HPV16 Ii-E1E6E7-p2a-Ii-E2
atgcacagaaggcggagcagaagctgccgcgaggatcagaaacccgtgatggacgaccagcgggacctgatcagcaacaacgagcagctgcctatgctcggcagaaggcctggcgctcctgagagcaaatgttctagaggcgccctgtacaccggcttcagcatcctggttacactgctgctggccggacaggctaccaccgcctactttctgtatcagcagcagggcagactggacaagctgaccgtgaccagccagaacctgcagctggaaaacctgcggatgaagctgcccaagcctcctaagcctgtgtccaagatgcggatggccacacctctgctgatgcaggctttgcctatgggagcactgcctcagggccctatgcagaacgccaccaaatacggcaacatgaccgaggaccacgtgatgcatctgctgcagaatgccgatcctctgaaggtgtaccctccactgaagggcagctttcccgagaacctgcggcacctgaagaacaccatggaaaccatcgactggaaggtgttcgagagctggatgcaccactggctgctgttcgagatgagccggcacagcctggaacagaagcctacagacgcccctcctaaagagtccctggaactggaagatcccagctctggcctgggcgtgacaaagcaagatctgggccctgtgcctatgatggccgatcctgctggcacaaacggcgaagaaggcacaggctgcaacggctggttttacgtggaagccgtggtggaaaagaaaaccggcgacgccatcagcgacgacgagaacgagaatgacagcgacaccggcgaggacctggtggacttcatcgtgaacgacaacgactacctgacacaggccgagacagagacagcccacgctctgtttacagcccaagaggccaagcagcacagagatgccgttcaggtgctgaagagaaagtacctgggcagccctctgagcgacatcagcggctgtgtggacaacaacatcagccccagactgaaggccatctgcatcgagaagcagagcagagccgccaagcggagactgtttgagagcgaggatagcggctacggcaataccgaggtggaaacccagcaaatgctgcaggtcgagggcagacacgaaaccgagacaccttgcagccagtacagcggaggatctggcggaggctgtagccagtactcttctggaagtggcggagagggcgtgtccgagagacacaccatttgtcagacccctctgaccaacatcctgaacgtgctgaaaaccagcaacgccaaggccgccatgctggccaagttcaaagagctgtacggcgtcagcttcagcgaactcgtgcggcccttcaagagcaacaagtccacctgttgcgactggtgcattgccgcctttggcctgacaccttctatcgccgacagcatcaagaccctgctccagcagtactgtctgtacctgcacattcagagcctggcctgctcttggggaatggtggtgctgctgctcgtgcggtacaagtgcggcaagaacagagagacaattgagaagctgctgagcaaactgctgtgcgtgtcccctatgtgcatgatgatcgagcctccaaagctgcggtctacagccgccgctctgtactggtacaagaccggcatcagcaatatctccgaggtgtacggcgacacccctgagtggattcagagacagaccgtcctgcagcacagcttcaacgactgcaccttcgagctgtcccagatggtgcagtgggcctacgacaatgacatcgtggacgactccgagatcgcctataagtacgcccagctggccgacaccaacagcaatgccagcgccttcctgaagtccaacagccaggccaagatcgtgaaggactgcgccaccatgtgcagacactacaagcgggccgagaagaaacagatgagcatgagccagtggatcaagtacagatgcgacagagtggacgacggcggcgattggaagcagatcgtgatgttcctgagataccagggcgtcgagttcatgagctttctgacagccctgaagcggttcctgcagggcatccccaagaagaactgcatcctgctgtatggcgccgctaacaccggcaagagcctgttcggaatgagcctgatgaagtttctgcagggctccgtgatctgctttgtgaacagcaagagccacttctggctccagccactggccgatgccaagattggcatgctggacgatgccaccgtgccttgctggaactacatcgacgacaacctgagaaacgccctggacggcaacctggtttctatggacgtgaagcacagacccctggtgcagctgaagtgtcctccactgctgatcaccagcaacatcaacgccggcaccgattccagatggccctatctgcacaaccggctggtggtgtttacctttcctaacgagttccccttcgacgaaaacggcaaccccgtgtacgagctgaacgataagaattggaagtccttcttcagccggacctggtccagactgagcctgcacgaggatgaggacaaagagaacgacggcgacagcctgcctaccttcaaatgtgtcagcggccagaacaccaacacactgggcagcatgcaccagaaacggacagccatgttccaggatcctcaagagcggccacggaagctgcctcagctgtgtacagaactgcagaccaccatccacgacatcatcctcgagtgcgtgtactgcaagcagcagctcctgcggagagaagtgtacgacttcgccttccgggatctgtgcatcgtgtacagagatggcaacccctacgccgtgtgcgacaagtgcctgaagttctactccaagatcagcgagtaccggcactactgctactccctgtacggcaccacacttgagcagcagtacaacaagcccctgtgcgatctgctgatccggtgcatcaactgccagaaacctcagtgccccgaggaaaagcagagacacctggacaagaagcagcggttccacaacattagaggcagatggacaggccggtgcatgagctgctgtagaagcagcagaacaagacggggctccatgcacggcgataccccaacactgcacgagtacatgctggatctgcagcccgagacaaccgatctgtacggctatgagcagctgaatgactccagcgaggaagaggacgagatcgacggacctgctggacaggctgaacctgatagagcccactacaatatcgtgaccttctgctgcaagtgcgatagcaccctgagaagatgcgtgcagagcacccacgtggacatcaggaccctcgaggatctgctcatgggcaccctgggaattgtggccccaatctgctctcagaagcctggcagcggcgccaccaatttcagtctgcttaaacaggccggggacgtcgaagagaaccccggacctatgcatcggcgcagatctcggtcttgtagagaagaccaaaagcctgtcatggatgatcaaagagatttaatttctaataatgaacaattacccatgttgggacggcgccccggagcccccgaatctaagtgcagccggggagctttatatacaggattttctattttagtgaccttattattagctggccaagccacaacagcttatttcttataccaacaacaaggacggttagataaattaacagtcacatctcaaaatttacaattagagaatttaagaatgaaattacctaaaccacccaaacccgtcagtaaaatgagaatggctacccccttattaatgcaagccctccccatgggcgccttaccccaaggacccatgcaaaatgctacaaagtatggaaatatgacagaagatcatgtcatgcacttattacaaaacgctgaccccttaaaagtctatccccctttaaaaggatctttccctgaaaatttaagacatttaaaaaatacaatggagacaattgattggaaagtctttgaatcttggatgcatcattggttattatttgaaatgtctaggcattctttagagcaaaaacccaccgatgctccacccaaggaaagtttagagttagaggacccttctagcggattaggagtcaccaaacaggacttaggacccgtccccatgatggaaacactgtgccagcggctgaacgtgtgccaggacaagattctgacccactatgagaacgacagcaccgacctgagggaccacatcgactactggaagcacatgcggctggaatgcgccatctactacaaggctagagagatgggcttcaagcacatcaaccaccaggtggtgcctacactggccgtgtctaagaacaaggctctgcaggccatcgaactgcagctgaccctggaaacaatctacaactcccagtactccaacgagaagtggaccctccaggacgtgtcactggaagtgtacctgaccgctcctaccggctgcatcaagaaacacggctacaccgtggaagtgcagtttgacggcgatatctgcaataccatgcactacaccaactggacccacatctacatctgcgaagaggccagcgtgacagtggtggaaggccaggtcgactactacggcctgtactacgtgcacgagggcatcagaacctacttcgtgcagttcaaggatgacgccgagaagtacagcaagaacaaagtgtgggaagtgcacgctggcggccaagtgatcctgtgtcctacaagcgtgttcagcagcaacgaagtgtctagccccgagatcatcagacagcacctggccaatcatcctgccgccacacacacaaaagctgtggccctgggcaccgaggaaacacagaccacaattcagaggcccagaagcgagcccgataccggcaatccttgtcacaccaccaagctgctgcaccgggattccgtggattctgcccctatcctgaccgccttcaacagctcccacaaaggccggatcaactgcaacagcaacaccacacctatcgtgcacctgaaaggggacgccaacactctgaaggccctgcggtacagattcaagaagcactgtaccctgtataccgccgtgtccagcacatggcactggaccggacacaacgtgaaacacaagagcgccatcgtgaccctgacctacgatagcgagtggcagagggaccagttcctgagccaagtgaagatccctaagaccatcaccgtgtccaccggctttatgagcatttga

SEQ ID NO: 42 - protein, 1756 aa, Human papillomavirus type 16
  HPV16 Ii-E1E6E7-p2a-Ii-E2 translated
MHRRRSRSCREDQKPVMDDQRDLISNNEQLPMLGRRPGAPESKCSRGALYTGFSILVTLLLAGQATTAYFLYQQQGRLDKLTVTSQNLQLENLRMKLPKPPKPVSKMRMATPLLMQALPMGALPQGPMQNATKYGNMTEDHVMHLLQNADPLKVYPPLKGSFPENLRHLKNTMETIDWKVFESWMHHWLLFEMSRHSLEQKPTDAPPKESLELEDPSSGLGVTKQDLGPVPMMADPAGTNGEEGTGCNGWFYVEAVVEKKTGDAISDDENENDSDTGEDLVDFIVNDNDYLTQAETETAHALFTAQEAKQHRDAVQVLKRKYLGSPLSDISGCVDNNISPRLKAICIEKQSRAAKRRLFESEDSGYGNTEVETQQMLQVEGRHETETPCSQYSGGSGGGCSQYSSGSGGEGVSERHTICQTPLTNILNVLKTSNAKAAMLAKFKELYGVSFSELVRPFKSNKSTCCDWCIAAFGLTPSIADSIKTLLQQYCLYLHIQSLACSWGMVVLLLVRYKCGKNRETIEKLLSKLLCVSPMCMMIEPPKLRSTAAALYWYKTGISNISEVYGDTPEWIQRQTVLQHSFNDCTFELSQMVQWAYDNDIVDDSEIAYKYAQLADTNSNASAFLKSNSQAKIVKDCATMCRHYKRAEKKQMSMSQWIKYRCDRVDDGGDWKQIVMFLRYQGVEFMSFLTALKRFLQGIPKKNCILLYGAANTGKSLFGMSLMKFLQGSVICFVNSKSHFWLQPLADAKIGMLDDATVPCWNYIDDNLRNALDGNLVSMDVKHRPLVQLKCPPLLITSNINAGTDSRWPYLHNRLVVFTFPNEFPFDENGNPVYELNDKNWKSFFSRTWSRLSLHEDEDKENDGDSLPTFKCVSGQNTNTLGSMHQKRTAMFQDPQERPRKLPQLCTELQTTIHDIILECVYCKQQLLRREVYDFAFRDLCIVYRDGNPYAVCDKCLKFYSKISEYRHYCYSLYGTTLEQQYNKPLCDLLIRCINCQKPQCPEEKQRHLDKKQRFHNIRGRWTGRCMSCCRSSRTRRGSMHGDTPTLHEYMLDLQPETTDLYGYEQLNDSSEEEDEIDGPAGQAEPDRAHYNIVTFCCKCDSTLRRCVQSTHVDIRTLEDLLMGTLGIVAPICSQKPGSGATNFSLLKQAGDVEENPGPMHRRRSRSCREDQKPVMDDQRDLISNNEQLPMLGRRPGAPESKCSRGALYTGFSILVTLLLAGQATTAYFLYQQQGRLDKLTVTSQNLQLENLRMKLPKPPKPVSKMRMATPLLMQALPMGALPQGPMQNATKYGNMTEDHVMHLLQNADPLKVYPPLKGSFPENLRHLKNTMETIDWKVFESWMHHWLLFEMSRHSLEQKPTDAPPKESLELEDPSSGLGVTKQDLGPVPMMETLCQRLNVCQDKILTHYENDSTDLRDHIDYWKHMRLECAIYYKAREMGFKHINHQVVPTLAVSKNKALQAIELQLTLETIYNSQYSNEKWTLQDVSLEVYLTAPTGCIKKHGYTVEVQFDGDICNTMHYTNWTHIYICEEASVTVVEGQVDYYGLYYVHEGIRTYFVQFKDDAEKYSKNKVWEVHAGGQVILCPTSVFSSNEVSSPEIIRQHLANHPAATHTKAVALGTEETQTTIQRPRSEPDTGNPCHTTKLLHRDSVDSAPILTAFNSSHKGRINCNSNTTPIVHLKGDANTLKALRYRFKKHCTLYTAVSSTWHWTGHNVKHKSAIVTLTYDSEWQRDQFLSQVKIPKTITVSTGFMSI

SEQ ID NO: 43 - DNA, 3414 bp, Human papillomavirus type 16
  HPV16 Ii-E1E6E7
atgcacagaaggcggagcagaagctgccgcgaggatcagaaacccgtgatggacgaccagcgggacctgatcagcaacaacgagcagctgcctatgctcggcagaaggcctggcgctcctgagagcaaatgttctagaggcgccctgtacaccggcttcagcatcctggttacactgctgctggccggacaggctaccaccgcctactttctgtatcagcagcagggcagactggacaagctgaccgtgaccagccagaacctgcagctggaaaacctgcggatgaagctgcccaagcctcctaagcctgtgtccaagatgcggatggccacacctctgctgatgcaggctttgcctatgggagcactgcctcagggccctatgcagaacgccaccaaatacggcaacatgaccgaggaccacgtgatgcatctgctgcagaatgccgatcctctgaaggtgtaccctccactgaagggcagctttcccgagaacctgcggcacctgaagaacaccatggaaaccatcgactggaaggtgttcgagagctggatgcaccactggctgctgttcgagatgagccggcacagcctggaacagaagcctacagacgcccctcctaaagagtccctggaactggaagatcccagctctggcctgggcgtgacaaagcaagatctgggccctgtgcctatgatggccgatcctgctggcacaaacggcgaagaaggcacaggctgcaacggctggttttacgtggaagccgtggtggaaaagaaaaccggcgacgccatcagcgacgacgagaacgagaatgacagcgacaccggcgaggacctggtggacttcatcgtgaacgacaacgactacctgacacaggccgagacagagacagcccacgctctgtttacagcccaagaggccaagcagcacagagatgccgttcaggtgctgaagagaaagtacctgggcagccctctgagcgacatcagcggctgtgtggacaacaacatcagccccagactgaaggccatctgcatcgagaagcagagcagagccgccaagcggagactgtttgagagcgaggatagcggctacggcaataccgaggtggaaacccagcaaatgctgcaggtcgagggcagacacgaaaccgagacaccttgcagccagtacagcggaggatctggcggaggctgtagccagtactcttctggaagtggcggagagggcgtgtccgagagacacaccatttgtcagacccctctgaccaacatcctgaacgtgctgaaaaccagcaacgccaaggccgccatgctggccaagttcaaagagctgtacggcgtcagcttcagcgaactcgtgcggcccttcaagagcaacaagtccacctgttgcgactggtgcattgccgcctttggcctgacaccttctatcgccgacagcatcaagaccctgctccagcagtactgtctgtacctgcacattcagagcctggcctgctcttggggaatggtggtgctgctgctcgtgcggtacaagtgcggcaagaacagagagacaattgagaagctgctgagcaaactgctgtgcgtgtcccctatgtgcatgatgatcgagcctccaaagctgcggtctacagccgccgctctgtactggtacaagaccggcatcagcaatatctccgaggtgtacggcgacacccctgagtggattcagagacagaccgtcctgcagcacagcttcaacgactgcaccttcgagctgtcccagatggtgcagtgggcctacgacaatgacatcgtggacgactccgagatcgcctataagtacgcccagctggccgacaccaacagcaatgccagcgccttcctgaagtccaacagccaggccaagatcgtgaaggactgcgccaccatgtgcagacactacaagcgggccgagaagaaacagatgagcatgagccagtggatcaagtacagatgcgacagagtggacgacggcggcgattggaagcagatcgtgatgttcctgagataccagggcgtcgagttcatgagctttctgacagccctgaagcggttcctgcagggcatccccaagaagaactgcatcctgctgtatggcgccgctaacaccggcaagagcctgttcggaatgagcctgatgaagtttctgcagggctccgtgatctgctttgtgaacagcaagagccacttctggctccagccactggccgatgccaagattggcatgctggacgatgccaccgtgccttgctggaactacatcgacgacaacctgagaaacgccctggacggcaacctggtttctatggacgtgaagcacagacccctggtgcagctgaagtgtcctccactgctgatcaccagcaacatcaacgccggcaccgattccagatggccctatctgcacaaccggctggtggtgtttacctttcctaacgagttccccttcgacgaaaacggcaaccccgtgtacgagctgaacgataagaattggaagtccttcttcagccggacctggtccagactgagcctgcacgaggatgaggacaaagagaacgacggcgacagcctgcctaccttcaaatgtgtcagcggccagaacaccaacacactgggcagcatgcaccagaaacggacagccatgttccaggatcctcaagagcggccacggaagctgcctcagctgtgtacagaactgcagaccaccatccacgacatcatcctcgagtgcgtgtactgcaagcagcagctcctgcggagagaagtgtacgacttcgccttccgggatctgtgcatcgtgtacagagatggcaacccctacgccgtgtgcgacaagtgcctgaagttctactccaagatcagcgagtaccggcactactgctactccctgtacggcaccacacttgagcagcagtacaacaagcccctgtgcgatctgctgatccggtgcatcaactgccagaaacctcagtgccccgaggaaaagcagagacacctggacaagaagcagcggttccacaacattagaggcagatggacaggccggtgcatgagctgctgtagaagcagcagaacaagacggggctccatgcacggcgataccccaacactgcacgagtacatgctggatctgcagcccgagacaaccgatctgtacggctatgagcagctgaatgactccagcgaggaagaggacgagatcgacggacctgctggacaggctgaacctgatagagcccactacaatatcgtgaccttctgctgcaagtgcgatagcaccctgagaagatgcgtgcagagcacccacgtggacatcaggaccctcgaggatctgctcatgggcaccctgggaattgtggccccaatctgctctcagaagccttga

SEQ ID NO: 44 - protein, 1137 aa, Human papillomavirus type 16
  HPV16 Ii-E1E6E7 translated
MHRRRSRSCREDQKPVMDDQRDLISNNEQLPMLGRRPGAPESKCSRGALYTGFSILVTLLLAGQATTAYFLYQQQGRLDKLTVTSQNLQLENLRMKLPKPPKPVSKMRMATPLLMQALPMGALPQGPMQNATKYGNMTEDHVMHLLQNADPLKVYPPLKGSFPENLRHLKNTMETIDWKVFESWMHHWLLFEMSRHSLEQKPTDAPPKESLELEDPSSGLGVTKQDLGPVPMMADPAGTNGEEGTGCNGWFYVEAVVEKKTGDAISDDENENDSDTGEDLVDFIVNDNDYLTQAETETAHALFTAQEAKQHRDAVQVLKRKYLGSPLSDISGCVDNNISPRLKAICIEKQSRAAKRRLFESEDSGYGNTEVETQQMLQVEGRHETETPCSQYSGGSGGGCSQYSSGSGGEGVSERHTICQTPLTNILNVLKTSNAKAAMLAKFKELYGVSFSELVRPFKSNKSTCCDWCIAAFGLTPSIADSIKTLLQQYCLYLHIQSLACSWGMVVLLLVRYKCGKNRETIEKLLSKLLCVSPMCMMIEPPKLRSTAAALYWYKTGISNISEVYGDTPEWIQRQTVLQHSFNDCTFELSQMVQWAYDNDIVDDSEIAYKYAQLADTNSNASAFLKSNSQAKIVKDCATMCRHYKRAEKKQMSMSQWIKYRCDRVDDGGDWKQIVMFLRYQGVEFMSFLTALKRFLQGIPKKNCILLYGAANTGKSLFGMSLMKFLQGSVICFVNSKSHFWLQPLADAKIGMLDDATVPCWNYIDDNLRNALDGNLVSMDVKHRPLVQLKCPPLLITSNINAGTDSRWPYLHNRLVVFTFPNEFPFDENGNPVYELNDKNWKSFFSRTWSRLSLHEDEDKENDGDSLPTFKCVSGQNTNTLGSMHQKRTAMFQDPQERPRKLPQLCTELQTTIHDIILECVYCKQQLLRREVYDFAFRDLCIVYRDGNPYAVCDKCLKFYSKISEYRHYCYSLYGTTLEQQYNKPLCDLLIRCINCQKPQCPEEKQRHLDKKQRFHNIRGRWTGRCMSCCRSSRTRRGSMHGDTPTLHEYMLDLQPETTDLYGYEQLNDSSEEEDEIDGPAGQAEPDRAHYNIVTFCCKCDSTLRRCVQSTHVDIRTLEDLLMGTLGIVAPICSQKP

SEQ ID NO: 45 - DNA, 4560 bp, Human papillomavirus type 18
  HPV18 Ii-E1E2E6E7
atgcacagaaggcggagcagaagctgccgcgaggatcagaaacccgtgatggacgaccagcgggacctgatcagcaacaacgagcagctgcctatgctcggcagaaggcctggcgctcctgagagcaaatgttctagaggcgccctgtacaccggcttcagcatcctggttacactgctgctggccggacaggctaccaccgcctactttctgtatcagcagcagggcagactggacaagctgaccgtgaccagccagaacctgcagctggaaaacctgcggatgaagctgcccaagcctcctaagcctgtgtccaagatgcggatggccacacctctgctgatgcaggctttgcctatgggagcactgcctcagggccctatgcagaacgccaccaaatacggcaacatgaccgaggaccacgtgatgcatctgctgcagaatgccgatcctctgaaggtgtaccctccactgaagggcagctttcccgagaacctgcggcacctgaagaacaccatggaaaccatcgactggaaggtgttcgagagctggatgcaccactggctgctgttcgagatgagccggcacagcctggaacagaagcctacagacgcccctcctaaagagtccctggaactggaagatcccagctctggcctgggcgtgacaaagcaagatctgggccctgtgcctatgatggccgatcctgagggaacagatggcgaaggcacaggctgcaacggctggttttacgtgcaagccatcgtggacaagaagaccggcgacgtcatcagcgacgacgaggatgagaatgccaccgacaccggcagcgacatggtggactttatcgatacccagggcacgttctgcgagcaggccgaactggaaacagcccaggcactgtttcacgcccaagaggtgcacaacgatgcccaggtgctgcacgtgctgaagagaaagtttgccggcggaagcaccgagaacagcccactgggagaaagactggaagtggacaccgagctgagccccagactgcaagagatcagcctgaacagcggccagaagaaggccaagcggagactgttcaccatctccgacagcggctacggctgtagcgaagtggaagccacacagatccaagtgaccaccaatggcgagcacggcggcaatgtttgttctggcggatctaccgaggccatcgacaatggcggaaccgagggcaacaatagctccgtggatggcaccagcgacaacagcaacatcgagaacgtgaaccctcagtgcacaatcgcccagctgaaggacctgctgaaagtgaacaacaagcagggcgccatgctggccgtgtttaaggatacctacggcctgagcttcaccgacctcgtgcggaacttcaagagcgacaagaccacctgtaccgactgggtcaccgccatctttggcgtgaacccaacaatcgccgagggcttcaagaccctgatccagcctttcatcctgtacgcccacatccagtgtctggactgcaaatggggcgtgctgattctggccctgctgagatacaagtgcggcaagagcagactgaccgtggccaagggactgagcactctgctgcatgtgcccgagacatgcatgctgattcagcctccaaagctgcggtctagcgtggccgctctgtactggtacagaaccggcatcagcaatatcagcgaagtgatgggcgacacccctgagtggattcagcggctgacaatcatccagcacggcatcgacgactccaacttcgacctgagcgagatggtgcagtgggccttcgataacgagctgaccgacgagtccgacatggcctttgaatacgccctgctggcagacagcaactccaatgccgccgctttcctgaagtccaactgccaggccaagtacctgaaggactgcgccaccatgtgcaagcactaccgcagagcacagaaacggcagatgaacatgagccagtggatccggttccggtgcagcaagatcgatgaaggtggcgactggcggcctatcgtgcagttcctgagataccagcagatcgagttcatcacctttctgggcgccctgaagtcattcctgaagggaacccctaaaaagaactgcctggtgttctgcggccctgccaataccggcaagtcctacttcggcatgagctttatccacttcatccagggcgccgtgatcagcttcgtgaacagcaccagccacttttggctggaacccctgaccgataccaaggtggcaatgctggacgacgccaccaccacctgttggacctacttcgacacctacatgcggaacgccctggacggcaaccccatcagcatcgacagaaagcacaagcccctcatccagctgaaatgccctccaatcctgctgaccacaaacattcaccccgccaaggacaatcggtggccctacctggaaagccggatcaccgtgttcgagttccccaacgcctttccattcgacaagaacggcaatcccgtgtacgagatcaacgacaagaattggaagtgcttcttcgagcggacctggtccagactggatctgcacgaggaagaagaggacgccgacacagagggcaatcccttcggcacctttaagtgtgtggccgggcagaatcacagacccctgggatctatgcagaccccaaaagagacactgagcgagcggctgagcgccctccaggacaagatcatcgaccactacgagaacgacagcaaggacatcgacagccagattcagtactggcagctgatcagatgggagaacgccatcttcttcgccgctagagagcacggaattcagaccctgaaccaccaggtggtgcccgcctacaacatcagcaagagcaaggcccacaaggccattgaactccagatggccctgcaaggactggctcagagcgcctacaagaccgaggattggacactccaggatacctgcgaggaactgtggaacacagagcccacacactgcttcaagaaaggcggccagaccgtgcaggtctacttcgatggcaacaaggataactgcatgacctacgtggcctgggacagcgtgtactacatgacagatgccggcacctgggacaagaccgccacctgtgtttctcaccggggcctgtactacgtgaaagagggctacaacaccttctacatcgagtttaagagcgagtgcgagaagtatggcaacaccggcacatgggaagtgcatttcggcaacaacgtgatcgactgcaacgactccatgtgctccacctccgatgacaccgtgtctgccacacagctggtcaagcagctccagcacaccccatctccatacagctctacagtgtctgtgggcaccgccaagacctatggccaaacaagcgctgccacaagacctggccattgtggactggccgagaagcagcactgtggccctgttaatcctctgctgggagccgccacacctacaggcaacaacaagagaagaaagctgtgcagcggcaacaccacacctatcattcacctgaagggcgacagaaacagcctgaagtgcctgcggtacagactgaggaagcacagcgatcactaccgggacatcagctccacctggcactggacaggtgctggcaacgaaaagaccggcatcctgacagtgacctaccacagcgagactcagcggaccaagttcctgaacaccgtggctatccccgacagcgtgcagattctcgtgggctacatgaccatgggcagcatggccagattcgaggaccctaccagacggccctacaagctgcctgatctgtgcaccgaactgaacaccagccttcaggatatcgagatcacctgtgtgtactgcaagaccgtgctcgagctgacagaagtgtttgagttcgccttcaaggacctgttcgtggtgtacagagacagcatccctcacgccgcctgtcacaagtgcatcgacttctacagcagaatcagagagctgcggcactacagcgactccgtgtacggcgataccctggaaaaactgaccaacaccggactgtacaacctgctgatccggtgcctgagatgccagaaacctcagaaccccgccgagaaactgagacatctgaacgagaagcggcggttccacaatatcgccggccactacagaggccagtgccacagctgttgcaaccgggccagacaagaaagactccagcggagaagaggcagcatgcacggacctaaagccacacttcaggacatcgtgctgcacctcgagcctcagaatgagatccccgtggatctgctcggccatgagcagctgagcgatagcgaggaagagaacgacgagatcgacggcgtcaaccaccagcatctgcctgccagaagggccgaacctcagagacacaccatgctgtgcatgtgctgcaagtgcgaggcccggatcgagagagtggtggaatctagcgccgacgacctgagagctttccagcagctgttcctgaatactctgagcttcgtggccccttggtgcgctagtcagcagtga

SEQ ID NO: 46 - protein, 1519 aa, Human papillomavirus type 18
  HPV18 Ii-E1E2E6E7 translated
MHRRRSRSCREDQKPVMDDQRDLISNNEQLPMLGRRPGAPESKCSRGALYTGFSILVTLLLAGQATTAYFLYQQQGRLDKLTVTSQNLQLENLRMKLPKPPKPVSKMRMATPLLMQALPMGALPQGPMQNATKYGNMTEDHVMHLLQNADPLKVYPPLKGSFPENLRHLKNTMETIDWKVFESWMHHWLLFEMSRHSLEQKPTDAPPKESLELEDPSSGLGVTKQDLGPVPMMADPEGTDGEGTGCNGWFYVQAIVDKKTGDVISDDEDENATDTGSDMVDFIDTQGTFCEQAELETAQALFHAQEVHNDAQVLHVLKRKFAGGSTENSPLGERLEVDTELSPRLQEISLNSGQKKAKRRLFTISDSGYGCSEVEATQIQVTTNGEHGGNVCSGGSTEAIDNGGTEGNNSSVDGTSDNSNIENVNPQCTIAQLKDLLKVNNKQGAMLAVFKDTYGLSFTDLVRNFKSDKTTCTDWVTAIFGVNPTIAEGFKTLIQPFILYAHIQCLDCKWGVLILALLRYKCGKSRLTVAKGLSTLLHVPETCMLIQPPKLRSSVAALYWYRTGISNISEVMGDTPEWIQRLTIIQHGIDDSNFDLSEMVQWAFDNELTDESDMAFEYALLADSNSNAAAFLKSNCQAKYLKDCATMCKHYRRAQKRQMNMSQWIRFRCSKIDEGGDWRPIVQFLRYQQIEFITFLGALKSFLKGTPKKNCLVFCGPANTGKSYFGMSFIHFIQGAVISFVNSTSHFWLEPLTDTKVAMLDDATTTCWTYFDTYMRNALDGNPISIDRKHKPLIQLKCPPILLTTNIHPAKDNRWPYLESRITVFEFPNAFPFDKNGNPVYEINDKNWKCFFERTWSRLDLHEEEEDADTEGNPFGTFKCVAGQNHRPLGSMQTPKETLSERLSALQDKIIDHYENDSKDIDSQIQYWQLIRWENAIFFAAREHGIQTLNHQVVPAYNISKSKAHKAIELQMALQGLAQSAYKTEDWTLQDTCEELWNTEPTHCFKKGGQTVQVYFDGNKDNCMTYVAWDSVYYMTDAGTWDKTATCVSHRGLYYVKEGYNTFYIEFKSECEKYGNTGTWEVHFGNNVIDCNDSMCSTSDDTVSATQLVKQLQHTPSPYSSTVSVGTAKTYGQTSAATRPGHCGLAEKQHCGPVNPLLGAATPTGNNKRRKLCSGNTTPIIHLKGDRNSLKCLRYRLRKHSDHYRDISSTWHWTGAGNEKTGILTVTYHSETQRTKFLNTVAIPDSVQILVGYMTMGSMARFEDPTRRPYKLPDLCTELNTSLQDIEITCVYCKTVLELTEVFEFAFKDLFVVYRDSIPHAACHKCIDFYSRIRELRHYSDSVYGDTLEKLTNTGLYNLLIRCLRCQKPQNPAEKLRHLNEKRRFHNIAGHYRGQCHSCCNRARQERLQRRRGSMHGPKATLQDIVLHLEPQNEIPVDLLGHEQLSDSEEENDEIDGVNHQHLPARRAEPQRHTMLCMCCKCEARIERVVESSADDLRAFQQLFLNTLSFVAPWCASQQ

SEQ ID NO: 47 - DNA, 5316 bp, Human papillomavirus type 18
  HPV18 Ii-E1E2-p2a-Ii-E6E7
atgcacagaaggcggagcagaagctgccgcgaggatcagaaacccgtgatggacgaccagcgggacctgatcagcaacaacgagcagctgcctatgctcggcagaaggcctggcgctcctgagagcaaatgttctagaggcgccctgtacaccggcttcagcatcctggttacactgctgctggccggacaggctaccaccgcctactttctgtatcagcagcagggcagactggacaagctgaccgtgaccagccagaacctgcagctggaaaacctgcggatgaagctgcccaagcctcctaagcctgtgtccaagatgcggatggccacacctctgctgatgcaggctttgcctatgggagcactgcctcagggccctatgcagaacgccaccaaatacggcaacatgaccgaggaccacgtgatgcatctgctgcagaatgccgatcctctgaaggtgtaccctccactgaagggcagctttcccgagaacctgcggcacctgaagaacaccatggaaaccatcgactggaaggtgttcgagagctggatgcaccactggctgctgttcgagatgagccggcacagcctggaacagaagcctacagacgcccctcctaaagagtccctggaactggaagatcccagctctggcctgggcgtgacaaagcaagatctgggccctgtgcctatgatggccgatcctgagggaacagatggcgaaggcacaggctgcaacggctggttttacgtgcaagccatcgtggacaagaagaccggcgacgtcatcagcgacgacgaggatgagaatgccaccgacaccggcagcgacatggtggactttatcgatacccagggcacgttctgcgagcaggccgaactggaaacagcccaggcactgtttcacgcccaagaggtgcacaacgatgcccaggtgctgcacgtgctgaagagaaagtttgccggcggaagcaccgagaacagcccactgggagaaagactggaagtggacaccgagctgagccccagactgcaagagatcagcctgaacagcggccagaagaaggccaagcggagactgttcaccatctccgacagcggctacggctgtagcgaagtggaagccacacagatccaagtgaccaccaatggcgagcacggcggcaatgtttgttctggcggatctaccgaggccatcgacaatggcggaaccgagggcaacaatagctccgtggatggcaccagcgacaacagcaacatcgagaacgtgaaccctcagtgcacaatcgcccagctgaaggacctgctgaaagtgaacaacaagcagggcgccatgctggccgtgtttaaggatacctacggcctgagcttcaccgacctcgtgcggaacttcaagagcgacaagaccacctgtaccgactgggtcaccgccatctttggcgtgaacccaacaatcgccgagggcttcaagaccctgatccagcctttcatcctgtacgcccacatccagtgtctggactgcaaatggggcgtgctgattctggccctgctgagatacaagtgcggcaagagcagactgaccgtggccaagggactgagcactctgctgcatgtgcccgagacatgcatgctgattcagcctccaaagctgcggtctagcgtggccgctctgtactggtacagaaccggcatcagcaatatcagcgaagtgatgggcgacacccctgagtggattcagcggctgacaatcatccagcacggcatcgacgactccaacttcgacctgagcgagatggtgcagtgggccttcgataacgagctgaccgacgagtccgacatggcctttgaatacgccctgctggcagacagcaactccaatgccgccgctttcctgaagtccaactgccaggccaagtacctgaaggactgcgccaccatgtgcaagcactaccgcagagcacagaaacggcagatgaacatgagccagtggatccggttccggtgcagcaagatcgatgaaggtggcgactggcggcctatcgtgcagttcctgagataccagcagatcgagttcatcacctttctgggcgccctgaagtcattcctgaagggaacccctaaaaagaactgcctggtgttctgcggccctgccaataccggcaagtcctacttcggcatgagctttatccacttcatccagggcgccgtgatcagcttcgtgaacagcaccagccacttttggctggaacccctgaccgataccaaggtggcaatgctggacgacgccaccaccacctgttggacctacttcgacacctacatgcggaacgccctggacggcaaccccatcagcatcgacagaaagcacaagcccctcatccagctgaaatgccctccaatcctgctgaccacaaacattcaccccgccaaggacaatcggtggccctacctggaaagccggatcaccgtgttcgagttccccaacgcctttccattcgacaagaacggcaatcccgtgtacgagatcaacgacaagaattggaagtgcttcttcgagcggacctggtccagactggatctgcacgaggaagaagaggacgccgacacagagggcaatcccttcggcacctttaagtgtgtggccgggcagaatcacagacccctgggatctatgcagaccccaaaagagacactgagcgagcggctgagcgccctccaggacaagatcatcgaccactacgagaacgacagcaaggacatcgacagccagattcagtactggcagctgatcagatgggagaacgccatcttcttcgccgctagagagcacggaattcagaccctgaaccaccaggtggtgcccgcctacaacatcagcaagagcaaggcccacaaggccattgaactccagatggccctgcaaggactggctcagagcgcctacaagaccgaggattggacactccaggatacctgcgaggaactgtggaacacagagcccacacactgcttcaagaaaggcggccagaccgtgcaggtctacttcgatggcaacaaggataactgcatgacctacgtggcctgggacagcgtgtactacatgacagatgccggcacctgggacaagaccgccacctgtgtttctcaccggggcctgtactacgtgaaagagggctacaacaccttctacatcgagtttaagagcgagtgcgagaagtatggcaacaccggcacatgggaagtgcatttcggcaacaacgtgatcgactgcaacgactccatgtgctccacctccgatgacaccgtgtctgccacacagctggtcaagcagctccagcacaccccatctccatacagctctacagtgtctgtgggcaccgccaagacctatggccaaacaagcgctgccacaagacctggccattgtggactggccgagaagcagcactgtggccctgttaatcctctgctgggagccgccacacctacaggcaacaacaagagaagaaagctgtgcagcggcaacaccacacctatcattcacctgaagggcgacagaaacagcctgaagtgcctgcggtacagactgaggaagcacagcgatcactaccgggacatcagctccacctggcactggacaggtgctggcaacgaaaagaccggcatcctgacagtgacctaccacagcgagactcagcggaccaagttcctgaacaccgtggctatccccgacagcgtgcagattctcgtgggctacatgaccatgggcagcggcgccaccaatttcagtctgcttaaacaggccggggacgtcgaagagaaccccggacctatgcatcggcgcagatctcggtcttgtagagaagaccaaaagcctgtcatggatgatcaaagagatttaatttctaataatgaacaattacccatgttgggacggcgccccggagcccccgaatctaagtgcagccggggagctttatatacaggattttctattttagtgaccttattattagctggccaagccacaacagcttatttcttataccaacaacaaggacggttagataaattaacagtcacatctcaaaatttacaattagagaatttaagaatgaaattacctaaaccacccaaacccgtcagtaaaatgagaatggctacccccttattaatgcaagccctccccatgggcgccttaccccaaggacccatgcaaaatgctacaaagtatggaaatatgacagaagatcatgtcatgcacttattacaaaacgctgaccccttaaaagtctatccccctttaaaaggatctttccctgaaaatttaagacatttaaaaaatacaatggagacaattgattggaaagtctttgaatcttggatgcatcattggttattatttgaaatgtctaggcattctttagagcaaaaacccaccgatgctccacccaaggaaagtttagagttagaggacccttctagcggattaggagtcaccaaacaggacttaggacccgtccccatgatggccagattcgaggaccctaccagacggccctacaagctgcctgatctgtgcaccgaactgaacaccagccttcaggatatcgagatcacctgtgtgtactgcaagaccgtgctcgagctgacagaagtgtttgagttcgccttcaaggacctgttcgtggtgtacagagacagcatccctcacgccgcctgtcacaagtgcatcgacttctacagcagaatcagagagctgcggcactacagcgactccgtgtacggcgataccctggaaaaactgaccaacaccggactgtacaacctgctgatccggtgcctgagatgccagaaacctcagaaccccgccgagaaactgagacatctgaacgagaagcggcggttccacaatatcgccggccactacagaggccagtgccacagctgttgcaaccgggccagacaagaaagactccagcggagaagaggcagcatgcacggacctaaagccacacttcaggacatcgtgctgcacctcgagcctcagaatgagatccccgtggatctgctcggccatgagcagctgagcgatagcgaggaagagaacgacgagatcgacggcgtcaaccaccagcatctgcctgccagaagggccgaacctcagagacacaccatgctgtgcatgtgctgcaagtgcgaggcccggatcgagagagtggtggaatctagcgccgacgacctgagagctttccagcagctgttcctgaatactctgagcttcgtggccccttggtgcgctagtcagcagtga

SEQ ID NO: 48 - protein, 1771 aa, Human papillomavirus type 18
  HPV18 Ii-E1E2-p2a-Ii-E6E7 translated
MHRRRSRSCREDQKPVMDDQRDLISNNEQLPMLGRRPGAPESKCSRGALYTGFSILVTLLLAGQATTAYFLYQQQGRLDKLTVTSQNLQLENLRMKLPKPPKPVSKMRMATPLLMQALPMGALPQGPMQNATKYGNMTEDHVMHLLQNADPLKVYPPLKGSFPENLRHLKNTMETIDWKVFESWMHHWLLFEMSRHSLEQKPTDAPPKESLELEDPSSGLGVTKQDLGPVPMMADPEGTDGEGTGCNGWFYVQAIVDKKTGDVISDDEDENATDTGSDMVDFIDTQGTFCEQAELETAQALFHAQEVHNDAQVLHVLKRKFAGGSTENSPLGERLEVDTELSPRLQEISLNSGQKKAKRRLFTISDSGYGCSEVEATQIQVTTNGEHGGNVCSGGSTEAIDNGGTEGNNSSVDGTSDNSNIENVNPQCTIAQLKDLLKVNNKQGAMLAVFKDTYGLSFTDLVRNFKSDKTTCTDWVTAIFGVNPTIAEGFKTLIQPFILYAHIQCLDCKWGVLILALLRYKCGKSRLTVAKGLSTLLHVPETCMLIQPPKLRSSVAALYWYRTGISNISEVMGDTPEWIQRLTIIQHGIDDSNFDLSEMVQWAFDNELTDESDMAFEYALLADSNSNAAAFLKSNCQAKYLKDCATMCKHYRRAQKRQMNMSQWIRFRCSKIDEGGDWRPIVQFLRYQQIEFITFLGALKSFLKGTPKKNCLVFCGPANTGKSYFGMSFIHFIQGAVISFVNSTSHFWLEPLTDTKVAMLDDATTTCWTYFDTYMRNALDGNPISIDRKHKPLIQLKCPPILLTTNIHPAKDNRWPYLESRITVFEFPNAFPFDKNGNPVYEINDKNWKCFFERTWSRLDLHEEEEDADTEGNPFGTFKCVAGQNHRPLGSMQTPKETLSERLSALQDKIIDHYENDSKDIDSQIQYWQLIRWENAIFFAAREHGIQTLNHQVVPAYNISKSKAHKAIELQMALQGLAQSAYKTEDWTLQDTCEELWNTEPTHCFKKGGQTVQVYFDGNKDNCMTYVAWDSVYYMTDAGTWDKTATCVSHRGLYYVKEGYNTFYIEFKSECEKYGNTGTWEVHFGNNVIDCNDSMCSTSDDTVSATQLVKQLQHTPSPYSSTVSVGTAKTYGQTSAATRPGHCGLAEKQHCGPVNPLLGAATPTGNNKRRKLCSGNTTPIIHLKGDRNSLKCLRYRLRKHSDHYRDISSTWHWTGAGNEKTGILTVTYHSETQRTKFLNTVAIPDSVQILVGYMTMGSGATNFSLLKQAGDVEENPGPMHRRRSRSCREDQKPVMDDQRDLISNNEQLPMLGRRPGAPESKCSRGALYTGFSILVTLLLAGQATTAYFLYQQQGRLDKLTVTSQNLQLENLRMKLPKPPKPVSKMRMATPLLMQALPMGALPQGPMQNATKYGNMTEDHVMHLLQNADPLKVYPPLKGSFPENLRHLKNTMETIDWKVFESWMHHWLLFEMSRHSLEQKPTDAPPKESLELEDPSSGLGVTKQDLGPVPMMARFEDPTRRPYKLPDLCTELNTSLQDIEITCVYCKTVLELTEVFEFAFKDLFVVYRDSIPHAACHKCIDFYSRIRELRHYSDSVYGDTLEKLTNTGLYNLLIRCLRCQKPQNPAEKLRHLNEKRRFHNIAGHYRGQCHSCCNRARQERLQRRRGSMHGPKATLQDIVLHLEPQNEIPVDLLGHEQLSDSEEENDEIDGVNHQHLPARRAEPQRHTMLCMCCKCEARIERVVESSADDLRAFQQLFLNTLSFVAPWCASQQ

SEQ ID NO: 49 - DNA, 3864 bp, Human papillomavirus type 18
  HPV18 #4 E1E2E6E7
atggccgatcctgagggaacagatggcgaaggcacaggctgcaacggctggttttacgtgcaagccatcgtggacaagaagaccggcgacgtcatcagcgacgacgaggatgagaatgccaccgacaccggcagcgacatggtggactttatcgatacccagggcacgttctgcgagcaggccgaactggaaacagcccaggcactgtttcacgcccaagaggtgcacaacgatgcccaggtgctgcacgtgctgaagagaaagtttgccggcggaagcaccgagaacagcccactgggagaaagactggaagtggacaccgagctgagccccagactgcaagagatcagcctgaacagcggccagaagaaggccaagcggagactgttcaccatctccgacagcggctacggctgtagcgaagtggaagccacacagatccaagtgaccaccaatggcgagcacggcggcaatgtttgttctggcggatctaccgaggccatcgacaatggcggaaccgagggcaacaatagctccgtggatggcaccagcgacaacagcaacatcgagaacgtgaaccctcagtgcacaatcgcccagctgaaggacctgctgaaagtgaacaacaagcagggcgccatgctggccgtgtttaaggatacctacggcctgagcttcaccgacctcgtgcggaacttcaagagcgacaagaccacctgtaccgactgggtcaccgccatctttggcgtgaacccaacaatcgccgagggcttcaagaccctgatccagcctttcatcctgtacgcccacatccagtgtctggactgcaaatggggcgtgctgattctggccctgctgagatacaagtgcggcaagagcagactgaccgtggccaagggactgagcactctgctgcatgtgcccgagacatgcatgctgattcagcctccaaagctgcggtctagcgtggccgctctgtactggtacagaaccggcatcagcaatatcagcgaagtgatgggcgacacccctgagtggattcagcggctgacaatcatccagcacggcatcgacgactccaacttcgacctgagcgagatggtgcagtgggccttcgataacgagctgaccgacgagtccgacatggcctttgaatacgccctgctggcagacagcaactccaatgccgccgctttcctgaagtccaactgccaggccaagtacctgaaggactgcgccaccatgtgcaagcactaccgcagagcacagaaacggcagatgaacatgagccagtggatccggttccggtgcagcaagatcgatgaaggtggcgactggcggcctatcgtgcagttcctgagataccagcagatcgagttcatcacctttctgggcgccctgaagtcattcctgaagggaacccctaaaaagaactgcctggtgttctgcggccctgccaataccggcaagtcctacttcggcatgagctttatccacttcatccagggcgccgtgatcagcttcgtgaacagcaccagccacttttggctggaacccctgaccgataccaaggtggcaatgctggacgacgccaccaccacctgttggacctacttcgacacctacatgcggaacgccctggacggcaaccccatcagcatcgacagaaagcacaagcccctcatccagctgaaatgccctccaatcctgctgaccacaaacattcaccccgccaaggacaatcggtggccctacctggaaagccggatcaccgtgttcgagttccccaacgcctttccattcgacaagaacggcaatcccgtgtacgagatcaacgacaagaattggaagtgcttcttcgagcggacctggtccagactggatctgcacgaggaagaagaggacgccgacacagagggcaatcccttcggcacctttaagtgtgtggccgggcagaatcacagacccctgggatctatgcagaccccaaaagagacactgagcgagcggctgagcgccctccaggacaagatcatcgaccactacgagaacgacagcaaggacatcgacagccagattcagtactggcagctgatcagatgggagaacgccatcttcttcgccgctagagagcacggaattcagaccctgaaccaccaggtggtgcccgcctacaacatcagcaagagcaaggcccacaaggccattgaactccagatggccctgcaaggactggctcagagcgcctacaagaccgaggattggacactccaggatacctgcgaggaactgtggaacacagagcccacacactgcttcaagaaaggcggccagaccgtgcaggtctacttcgatggcaacaaggataactgcatgacctacgtggcctgggacagcgtgtactacatgacagatgccggcacctgggacaagaccgccacctgtgtttctcaccggggcctgtactacgtgaaagagggctacaacaccttctacatcgagtttaagagcgagtgcgagaagtatggcaacaccggcacatgggaagtgcatttcggcaacaacgtgatcgactgcaacgactccatgtgctccacctccgatgacaccgtgtctgccacacagctggtcaagcagctccagcacaccccatctccatacagctctacagtgtctgtgggcaccgccaagacctatggccaaacaagcgctgccacaagacctggccattgtggactggccgagaagcagcactgtggccctgttaatcctctgctgggagccgccacacctacaggcaacaacaagagaagaaagctgtgcagcggcaacaccacacctatcattcacctgaagggcgacagaaacagcctgaagtgcctgcggtacagactgaggaagcacagcgatcactaccgggacatcagctccacctggcactggacaggtgctggcaacgaaaagaccggcatcctgacagtgacctaccacagcgagactcagcggaccaagttcctgaacaccgtggctatccccgacagcgtgcagattctcgtgggctacatgaccatgggcagcatggccagattcgaggaccctaccagacggccctacaagctgcctgatctgtgcaccgaactgaacaccagccttcaggatatcgagatcacctgtgtgtactgcaagaccgtgctcgagctgacagaagtgtttgagttcgccttcaaggacctgttcgtggtgtacagagacagcatccctcacgccgcctgtcacaagtgcatcgacttctacagcagaatcagagagctgcggcactacagcgactccgtgtacggcgataccctggaaaaactgaccaacaccggactgtacaacctgctgatccggtgcctgagatgccagaaacctcagaaccccgccgagaaactgagacatctgaacgagaagcggcggttccacaatatcgccggccactacagaggccagtgccacagctgttgcaaccgggccagacaagaaagactccagcggagaagaggcagcatgcacggacctaaagccacacttcaggacatcgtgctgcacctcgagcctcagaatgagatccccgtggatctgctcggccatgagcagctgagcgatagcgaggaagagaacgacgagatcgacggcgtcaaccaccagcatctgcctgccagaagggccgaacctcagagacacaccatgctgtgcatgtgctgcaagtgcgaggcccggatcgagagagtggtggaatctagcgccgacgacctgagagctttccagcagctgttcctgaatactctgagcttcgtggccccttggtgcgctagtcagcagtga

SEQ ID NO: 50 - protein, 1287 aa, Human papillomavirus type 18
  HPV18 #4 E1E2E6E7 translated
MADPEGTDGEGTGCNGWFYVQAIVDKKTGDVISDDEDENATDTGSDMVDFIDTQGTFCEQAELETAQALFHAQEVHNDAQVLHVLKRKFAGGSTENSPLGERLEVDTELSPRLQEISLNSGQKKAKRRLFTISDSGYGCSEVEATQIQVTTNGEHGGNVCSGGSTEAIDNGGTEGNNSSVDGTSDNSNIENVNPQCTIAQLKDLLKVNNKQGAMLAVFKDTYGLSFTDLVRNFKSDKTTCTDWVTAIFGVNPTIAEGFKTLIQPFILYAHIQCLDCKWGVLILALLRYKCGKSRLTVAKGLSTLLHVPETCMLIQPPKLRSSVAALYWYRTGISNISEVMGDTPEWIQRLTIIQHGIDDSNFDLSEMVQWAFDNELTDESDMAFEYALLADSNSNAAAFLKSNCQAKYLKDCATMCKHYRRAQKRQMNMSQWIRFRCSKIDEGGDWRPIVQFLRYQQIEFITFLGALKSFLKGTPKKNCLVFCGPANTGKSYFGMSFIHFIQGAVISFVNSTSHFWLEPLTDTKVAMLDDATTTCWTYFDTYMRNALDGNPISIDRKHKPLIQLKCPPILLTTNIHPAKDNRWPYLESRITVFEFPNAFPFDKNGNPVYEINDKNWKCFFERTWSRLDLHEEEEDADTEGNPFGTFKCVAGQNHRPLGSMQTPKETLSERLSALQDKIIDHYENDSKDIDSQIQYWQLIRWENAIFFAAREHGIQTLNHQVVPAYNISKSKAHKAIELQMALQGLAQSAYKTEDWTLQDTCEELWNTEPTHCFKKGGQTVQVYFDGNKDNCMTYVAWDSVYYMTDAGTWDKTATCVSHRGLYYVKEGYNTFYIEFKSECEKYGNTGTWEVHFGNNVIDCNDSMCSTSDDTVSATQLVKQLQHTPSPYSSTVSVGTAKTYGQTSAATRPGHCGLAEKQHCGPVNPLLGAATPTGNNKRRKLCSGNTTPIIHLKGDRNSLKCLRYRLRKHSDHYRDISSTWHWTGAGNEKTGILTVTYHSETQRTKFLNTVAIPDSVQILVGYMTMGSMARFEDPTRRPYKLPDLCTELNTSLQDIEITCVYCKTVLELTEVFEFAFKDLFVVYRDSIPHAACHKCIDFYSRIRELRHYSDSVYGDTLEKLTNTGLYNLLIRCLRCQKPQNPAEKLRHLNEKRRFHNIAGHYRGQCHSCCNRARQERLQRRRGSMHGPKATLQDIVLHLEPQNEIPVDLLGHEQLSDSEEENDEIDGVNHQHLPARRAEPQRHTMLCMCCKCEARIERVVESSADDLRAFQQLFLNTLSFVAPWCASQQ

SEQ ID NO: 51 - DNA, 5316 bp, Human papillomavirus type 18
  HPV18 Ii-E1E6E7-p2a-Ii-E2
atgcacagaaggcggagcagaagctgccgcgaggatcagaaacccgtgatggacgaccagcgggacctgatcagcaacaacgagcagctgcctatgctcggcagaaggcctggcgctcctgagagcaaatgttctagaggcgccctgtacaccggcttcagcatcctggttacactgctgctggccggacaggctaccaccgcctactttctgtatcagcagcagggcagactggacaagctgaccgtgaccagccagaacctgcagctggaaaacctgcggatgaagctgcccaagcctcctaagcctgtgtccaagatgcggatggccacacctctgctgatgcaggctttgcctatgggagcactgcctcagggccctatgcagaacgccaccaaatacggcaacatgaccgaggaccacgtgatgcatctgctgcagaatgccgatcctctgaaggtgtaccctccactgaagggcagctttcccgagaacctgcggcacctgaagaacaccatggaaaccatcgactggaaggtgttcgagagctggatgcaccactggctgctgttcgagatgagccggcacagcctggaacagaagcctacagacgcccctcctaaagagtccctggaactggaagatcccagctctggcctgggcgtgacaaagcaagatctgggccctgtgcctatgatggccgatcctgagggaacagatggcgaaggcacaggctgcaacggctggttttacgtgcaagccatcgtggacaagaagaccggcgacgtcatcagcgacgacgaggatgagaatgccaccgacaccggcagcgacatggtggactttatcgatacccagggcacgttctgcgagcaggccgaactggaaacagcccaggcactgtttcacgcccaagaggtgcacaacgatgcccaggtgctgcacgtgctgaagagaaagtttgccggcggaagcaccgagaacagcccactgggagaaagactggaagtggacaccgagctgagccccagactgcaagagatcagcctgaacagcggccagaagaaggccaagcggagactgttcaccatctccgacagcggctacggctgtagcgaagtggaagccacacagatccaagtgaccaccaatggcgagcacggcggcaatgtttgttctggcggatctaccgaggccatcgacaatggcggaaccgagggcaacaatagctccgtggatggcaccagcgacaacagcaacatcgagaacgtgaaccctcagtgcacaatcgcccagctgaaggacctgctgaaagtgaacaacaagcagggcgccatgctggccgtgtttaaggatacctacggcctgagcttcaccgacctcgtgcggaacttcaagagcgacaagaccacctgtaccgactgggtcaccgccatctttggcgtgaacccaacaatcgccgagggcttcaagaccctgatccagcctttcatcctgtacgcccacatccagtgtctggactgcaaatggggcgtgctgattctggccctgctgagatacaagtgcggcaagagcagactgaccgtggccaagggactgagcactctgctgcatgtgcccgagacatgcatgctgattcagcctccaaagctgcggtctagcgtggccgctctgtactggtacagaaccggcatcagcaatatcagcgaagtgatgggcgacacccctgagtggattcagcggctgacaatcatccagcacggcatcgacgactccaacttcgacctgagcgagatggtgcagtgggccttcgataacgagctgaccgacgagtccgacatggcctttgaatacgccctgctggcagacagcaactccaatgccgccgctttcctgaagtccaactgccaggccaagtacctgaaggactgcgccaccatgtgcaagcactaccgcagagcacagaaacggcagatgaacatgagccagtggatccggttccggtgcagcaagatcgatgaaggtggcgactggcggcctatcgtgcagttcctgagataccagcagatcgagttcatcacctttctgggcgccctgaagtcattcctgaagggaacccctaaaaagaactgcctggtgttctgcggccctgccaataccggcaagtcctacttcggcatgagctttatccacttcatccagggcgccgtgatcagcttcgtgaacagcaccagccacttttggctggaacccctgaccgataccaaggtggcaatgctggacgacgccaccaccacctgttggacctacttcgacacctacatgcggaacgccctggacggcaaccccatcagcatcgacagaaagcacaagcccctcatccagctgaaatgccctccaatcctgctgaccacaaacattcaccccgccaaggacaatcggtggccctacctggaaagccggatcaccgtgttcgagttccccaacgcctttccattcgacaagaacggcaatcccgtgtacgagatcaacgacaagaattggaagtgcttcttcgagcggacctggtccagactggatctgcacgaggaagaagaggacgccgacacagagggcaatcccttcggcacctttaagtgtgtggccgggcagaatcacagacccctgggcagcatggccagattcgaggaccctaccagacggccctacaagctgcctgatctgtgcaccgaactgaacaccagccttcaggatatcgagatcacctgtgtgtactgcaagaccgtgctcgagctgacagaagtgtttgagttcgccttcaaggacctgttcgtggtgtacagagacagcatccctcacgccgcctgtcacaagtgcatcgacttctacagcagaatcagagagctgcggcactacagcgactccgtgtacggcgataccctggaaaaactgaccaacaccggactgtacaacctgctgatccggtgcctgagatgccagaaacctcagaaccccgccgagaaactgagacatctgaacgagaagcggcggttccacaatatcgccggccactacagaggccagtgccacagctgttgcaaccgggccagacaagaaagactccagcggagaagaggcagcatgcacggacctaaagccacacttcaggacatcgtgctgcacctcgagcctcagaatgagatccccgtggatctgctcggccatgagcagctgagcgatagcgaggaagagaacgacgagatcgacggcgtcaaccaccagcatctgcctgccagaagggccgaacctcagagacacaccatgctgtgcatgtgctgcaagtgcgaggcccggatcgagagagtggtggaatctagcgccgacgacctgagagctttccagcagctgttcctgaatactctgagcttcgtggccccttggtgcgctagtcagcagggcagcggcgccaccaatttcagtctgcttaaacaggccggggacgtcgaagagaaccccggacctatgcatcggcgcagatctcggtcttgtagagaagaccaaaagcctgtcatggatgatcaaagagatttaatttctaataatgaacaattacccatgttgggacggcgccccggagcccccgaatctaagtgcagccggggagctttatatacaggattttctattttagtgaccttattattagctggccaagccacaacagcttatttcttataccaacaacaaggacggttagataaattaacagtcacatctcaaaatttacaattagagaatttaagaatgaaattacctaaaccacccaaacccgtcagtaaaatgagaatggctacccccttattaatgcaagccctccccatgggcgccttaccccaaggacccatgcaaaatgctacaaagtatggaaatatgacagaagatcatgtcatgcacttattacaaaacgctgaccccttaaaagtctatccccctttaaaaggatctttccctgaaaatttaagacatttaaaaaatacaatggagacaattgattggaaagtctttgaatcttggatgcatcattggttattatttgaaatgtctaggcattctttagagcaaaaacccaccgatgctccacccaaggaaagtttagagttagaggacccttctagcggattaggagtcaccaaacaggacttaggacccgtccccatgatgcagaccccaaaagagacactgagcgagcggctgagcgccctccaggacaagatcatcgaccactacgagaacgacagcaaggacatcgacagccagattcagtactggcagctgatcagatgggagaacgccatcttcttcgccgctagagagcacggaattcagaccctgaaccaccaggtggtgcccgcctacaacatcagcaagagcaaggcccacaaggccattgaactccagatggccctgcaaggactggctcagagcgcctacaagaccgaggattggacactccaggatacctgcgaggaactgtggaacacagagcccacacactgcttcaagaaaggcggccagaccgtgcaggtctacttcgatggcaacaaggataactgcatgacctacgtggcctgggacagcgtgtactacatgacagatgccggcacctgggacaagaccgccacctgtgtttctcaccggggcctgtactacgtgaaagagggctacaacaccttctacatcgagtttaagagcgagtgcgagaagtatggcaacaccggcacatgggaagtgcatttcggcaacaacgtgatcgactgcaacgactccatgtgctccacctccgatgacaccgtgtctgccacacagctggtcaagcagctccagcacaccccatctccatacagctctacagtgtctgtgggcaccgccaagacctatggccaaacaagcgctgccacaagacctggccattgtggactggccgagaagcagcactgtggccctgttaatcctctgctgggagccgccacacctacaggcaacaacaagagaagaaagctgtgcagcggcaacaccacacctatcattcacctgaagggcgacagaaacagcctgaagtgcctgcggtacagactgaggaagcacagcgatcactaccgggacatcagctccacctggcactggacaggtgctggcaacgaaaagaccggcatcctgacagtgacctaccacagcgagactcagcggaccaagttcctgaacaccgtggctatccccgacagcgtgcagattctcgtgggctacatgaccatgtga

SEQ ID NO: 52 - protein, 1771 aa, Human papillomavirus type 18
  HPV18 Ii-E1E6E7-p2a-Ii-E2 translated
MHRRRSRSCREDQKPVMDDQRDLISNNEQLPMLGRRPGAPESKCSRGALYTGFSILVTLLLAGQATTAYFLYQQQGRLDKLTVTSQNLQLENLRMKLPKPPKPVSKMRMATPLLMQALPMGALPQGPMQNATKYGNMTEDHVMHLLQNADPLKVYPPLKGSFPENLRHLKNTMETIDWKVFESWMHHWLLFEMSRHSLEQKPTDAPPKESLELEDPSSGLGVTKQDLGPVPMMADPEGTDGEGTGCNGWFYVQAIVDKKTGDVISDDEDENATDTGSDMVDFIDTQGTFCEQAELETAQALFHAQEVHNDAQVLHVLKRKFAGGSTENSPLGERLEVDTELSPRLQEISLNSGQKKAKRRLFTISDSGYGCSEVEATQIQVTTNGEHGGNVCSGGSTEAIDNGGTEGNNSSVDGTSDNSNIENVNPQCTIAQLKDLLKVNNKQGAMLAVFKDTYGLSFTDLVRNFKSDKTTCTDWVTAIFGVNPTIAEGFKTLIQPFILYAHIQCLDCKWGVLILALLRYKCGKSRLTVAKGLSTLLHVPETCMLIQPPKLRSSVAALYWYRTGISNISEVMGDTPEWIQRLTIIQHGIDDSNFDLSEMVQWAFDNELTDESDMAFEYALLADSNSNAAAFLKSNCQAKYLKDCATMCKHYRRAQKRQMNMSQWIRFRCSKIDEGGDWRPIVQFLRYQQIEFITFLGALKSFLKGTPKKNCLVFCGPANTGKSYFGMSFIHFIQGAVISFVNSTSHFWLEPLTDTKVAMLDDATTTCWTYFDTYMRNALDGNPISIDRKHKPLIQLKCPPILLTTNIHPAKDNRWPYLESRITVFEFPNAFPFDKNGNPVYEINDKNWKCFFERTWSRLDLHEEEEDADTEGNPFGTFKCVAGQNHRPLGSMARFEDPTRRPYKLPDLCTELNTSLQDIEITCVYCKTVLELTEVFEFAFKDLFVVYRDSIPHAACHKCIDFYSRIRELRHYSDSVYGDTLEKLTNTGLYNLLIRCLRCQKPQNPAEKLRHLNEKRRFHNIAGHYRGQCHSCCNRARQERLQRRRGSMHGPKATLQDIVLHLEPQNEIPVDLLGHEQLSDSEEENDEIDGVNHQHLPARRAEPQRHTMLCMCCKCEARIERVVESSADDLRAFQQLFLNTLSFVAPWCASQQGSGATNFSLLKQAGDVEENPGPMHRRRSRSCREDQKPVMDDQRDLISNNEQLPMLGRRPGAPESKCSRGALYTGFSILVTLLLAGQATTAYFLYQQQGRLDKLTVTSQNLQLENLRMKLPKPPKPVSKMRMATPLLMQALPMGALPQGPMQNATKYGNMTEDHVMHLLQNADPLKVYPPLKGSFPENLRHLKNTMETIDWKVFESWMHHWLLFEMSRHSLEQKPTDAPPKESLELEDPSSGLGVTKQDLGPVPMMQTPKETLSERLSALQDKIIDHYENDSKDIDSQIQYWQLIRWENAIFFAAREHGIQTLNHQVVPAYNISKSKAHKAIELQMALQGLAQSAYKTEDWTLQDTCEELWNTEPTHCFKKGGQTVQVYFDGNKDNCMTYVAWDSVYYMTDAGTWDKTATCVSHRGLYYVKEGYNTFYIEFKSECEKYGNTGTWEVHFGNNVIDCNDSMCSTSDDTVSATQLVKQLQHTPSPYSSTVSVGTAKTYGQTSAATRPGHCGLAEKQHCGPVNPLLGAATPTGNNKRRKLCSGNTTPIIHLKGDRNSLKCLRYRLRKHSDHYRDISSTWHWTGAGNEKTGILTVTYHSETQRTKFLNTVAIPDSVQILVGYMTM

SEQ ID NO: 53 - DNA, 3459 bp, Human papillomavirus type 18
  HPV18 Ii-E1E6E7
atgcacagaaggcggagcagaagctgccgcgaggatcagaaacccgtgatggacgaccagcgggacctgatcagcaacaacgagcagctgcctatgctcggcagaaggcctggcgctcctgagagcaaatgttctagaggcgccctgtacaccggcttcagcatcctggttacactgctgctggccggacaggctaccaccgcctactttctgtatcagcagcagggcagactggacaagctgaccgtgaccagccagaacctgcagctggaaaacctgcggatgaagctgcccaagcctcctaagcctgtgtccaagatgcggatggccacacctctgctgatgcaggctttgcctatgggagcactgcctcagggccctatgcagaacgccaccaaatacggcaacatgaccgaggaccacgtgatgcatctgctgcagaatgccgatcctctgaaggtgtaccctccactgaagggcagctttcccgagaacctgcggcacctgaagaacaccatggaaaccatcgactggaaggtgttcgagagctggatgcaccactggctgctgttcgagatgagccggcacagcctggaacagaagcctacagacgcccctcctaaagagtccctggaactggaagatcccagctctggcctgggcgtgacaaagcaagatctgggccctgtgcctatgatggccgatcctgagggaacagatggcgaaggcacaggctgcaacggctggttttacgtgcaagccatcgtggacaagaagaccggcgacgtcatcagcgacgacgaggatgagaatgccaccgacaccggcagcgacatggtggactttatcgatacccagggcacgttctgcgagcaggccgaactggaaacagcccaggcactgtttcacgcccaagaggtgcacaacgatgcccaggtgctgcacgtgctgaagagaaagtttgccggcggaagcaccgagaacagcccactgggagaaagactggaagtggacaccgagctgagccccagactgcaagagatcagcctgaacagcggccagaagaaggccaagcggagactgttcaccatctccgacagcggctacggctgtagcgaagtggaagccacacagatccaagtgaccaccaatggcgagcacggcggcaatgtttgttctggcggatctaccgaggccatcgacaatggcggaaccgagggcaacaatagctccgtggatggcaccagcgacaacagcaacatcgagaacgtgaaccctcagtgcacaatcgcccagctgaaggacctgctgaaagtgaacaacaagcagggcgccatgctggccgtgtttaaggatacctacggcctgagcttcaccgacctcgtgcggaacttcaagagcgacaagaccacctgtaccgactgggtcaccgccatctttggcgtgaacccaacaatcgccgagggcttcaagaccctgatccagcctttcatcctgtacgcccacatccagtgtctggactgcaaatggggcgtgctgattctggccctgctgagatacaagtgcggcaagagcagactgaccgtggccaagggactgagcactctgctgcatgtgcccgagacatgcatgctgattcagcctccaaagctgcggtctagcgtggccgctctgtactggtacagaaccggcatcagcaatatcagcgaagtgatgggcgacacccctgagtggattcagcggctgacaatcatccagcacggcatcgacgactccaacttcgacctgagcgagatggtgcagtgggccttcgataacgagctgaccgacgagtccgacatggcctttgaatacgccctgctggcagacagcaactccaatgccgccgctttcctgaagtccaactgccaggccaagtacctgaaggactgcgccaccatgtgcaagcactaccgcagagcacagaaacggcagatgaacatgagccagtggatccggttccggtgcagcaagatcgatgaaggtggcgactggcggcctatcgtgcagttcctgagataccagcagatcgagttcatcacctttctgggcgccctgaagtcattcctgaagggaacccctaaaaagaactgcctggtgttctgcggccctgccaataccggcaagtcctacttcggcatgagctttatccacttcatccagggcgccgtgatcagcttcgtgaacagcaccagccacttttggctggaacccctgaccgataccaaggtggcaatgctggacgacgccaccaccacctgttggacctacttcgacacctacatgcggaacgccctggacggcaaccccatcagcatcgacagaaagcacaagcccctcatccagctgaaatgccctccaatcctgctgaccacaaacattcaccccgccaaggacaatcggtggccctacctggaaagccggatcaccgtgttcgagttccccaacgcctttccattcgacaagaacggcaatcccgtgtacgagatcaacgacaagaattggaagtgcttcttcgagcggacctggtccagactggatctgcacgaggaagaagaggacgccgacacagagggcaatcccttcggcacctttaagtgtgtggccgggcagaatcacagacccctgggcagcatggccagattcgaggaccctaccagacggccctacaagctgcctgatctgtgcaccgaactgaacaccagccttcaggatatcgagatcacctgtgtgtactgcaagaccgtgctcgagctgacagaagtgtttgagttcgccttcaaggacctgttcgtggtgtacagagacagcatccctcacgccgcctgtcacaagtgcatcgacttctacagcagaatcagagagctgcggcactacagcgactccgtgtacggcgataccctggaaaaactgaccaacaccggactgtacaacctgctgatccggtgcctgagatgccagaaacctcagaaccccgccgagaaactgagacatctgaacgagaagcggcggttccacaatatcgccggccactacagaggccagtgccacagctgttgcaaccgggccagacaagaaagactccagcggagaagaggcagcatgcacggacctaaagccacacttcaggacatcgtgctgcacctcgagcctcagaatgagatccccgtggatctgctcggccatgagcagctgagcgatagcgaggaagagaacgacgagatcgacggcgtcaaccaccagcatctgcctgccagaagggccgaacctcagagacacaccatgctgtgcatgtgctgcaagtgcgaggcccggatcgagagagtggtggaatctagcgccgacgacctgagagctttccagcagctgttcctgaatactctgagcttcgtggccccttggtgcgctagtcagcagtga

SEQ ID NO: 54 - protein, 1152 aa, Human papillomavirus type 18
  HPV18 Ii-E1E6E7 translated
MHRRRSRSCREDQKPVMDDQRDLISNNEQLPMLGRRPGAPESKCSRGALYTGFSILVTLLLAGQATTAYFLYQQQGRLDKLTVTSQNLQLENLRMKLPKPPKPVSKMRMATPLLMQALPMGALPQGPMQNATKYGNMTEDHVMHLLQNADPLKVYPPLKGSFPENLRHLKNTMETIDWKVFESWMHHWLLFEMSRHSLEQKPTDAPPKESLELEDPSSGLGVTKQDLGPVPMMADPEGTDGEGTGCNGWFYVQAIVDKKTGDVISDDEDENATDTGSDMVDFIDTQGTFCEQAELETAQALFHAQEVHNDAQVLHVLKRKFAGGSTENSPLGERLEVDTELSPRLQEISLNSGQKKAKRRLFTISDSGYGCSEVEATQIQVTTNGEHGGNVCSGGSTEAIDNGGTEGNNSSVDGTSDNSNIENVNPQCTIAQLKDLLKVNNKQGAMLAVFKDTYGLSFTDLVRNFKSDKTTCTDWVTAIFGVNPTIAEGFKTLIQPFILYAHIQCLDCKWGVLILALLRYKCGKSRLTVAKGLSTLLHVPETCMLIQPPKLRSSVAALYWYRTGISNISEVMGDTPEWIQRLTIIQHGIDDSNFDLSEMVQWAFDNELTDESDMAFEYALLADSNSNAAAFLKSNCQAKYLKDCATMCKHYRRAQKRQMNMSQWIRFRCSKIDEGGDWRPIVQFLRYQQIEFITFLGALKSFLKGTPKKNCLVFCGPANTGKSYFGMSFIHFIQGAVISFVNSTSHFWLEPLTDTKVAMLDDATTTCWTYFDTYMRNALDGNPISIDRKHKPLIQLKCPPILLTTNIHPAKDNRWPYLESRITVFEFPNAFPFDKNGNPVYEINDKNWKCFFERTWSRLDLHEEEEDADTEGNPFGTFKCVAGQNHRPLGSMARFEDPTRRPYKLPDLCTELNTSLQDIEITCVYCKTVLELTEVFEFAFKDLFVVYRDSIPHAACHKCIDFYSRIRELRHYSDSVYGDTLEKLTNTGLYNLLIRCLRCQKPQNPAEKLRHLNEKRRFHNIAGHYRGQCHSCCNRARQERLQRRRGSMHGPKATLQDIVLHLEPQNEIPVDLLGHEQLSDSEEENDEIDGVNHQHLPARRAEPQRHTMLCMCCKCEARIERVVESSADDLRAFQQLFLNTLSFVAPWCASQQ

SEQ ID NO: 55 - DNA, 5033 bp, Artificial Sequence
  MfPV3 Ii-E1E2E6E7 as carried by Adenoviral vector
gtgatgcggttttggcagtacatcaatgggcgtggatagcggtttgactcacggggatttccaagtctccaccccattgacgtcaatgggagtttgttttggaaccaaaatcaacgggactttccaaaatgtcgtaacaactccgccccattgacgcaaatgggcggtaggcgtgtacggtgggaggtctatataagcagagctctccctatcagtgatagagatctccctatcagtgatagagatcgtcgacgagctcgtttagtgaaccgtcagatcgcctggagacgccatccacgctgttttgacctctagcaccggtgccaccatgcacagaaggcggagcagaagctgccgcgaggatcagaaacccgtgatggacgaccagcgggacctgatcagcaacaacgagcagctgcctatgctcggcagaaggcctggcgctcctgagagcaaatgttctagaggcgccctgtacaccggcttcagcatcctggttacactgctgctggccggacaggctaccaccgcctactttctgtatcagcagcagggcagactggacaagctgaccgtgaccagccagaacctgcagctggaaaacctgcggatgaagctgcccaagcctcctaagcctgtgtccaagatgcggatggccacacctctgctgatgcaggctttgcctatgggagcactgcctcagggccctatgcagaacgccaccaaatacggcaacatgaccgaggaccacgtgatgcatctgctgcagaatgccgatcctctgaaggtgtaccctccactgaagggcagctttcccgagaacctgcggcacctgaagaacaccatggaaaccatcgactggaaggtgttcgagagctggatgcaccactggctgctgttcgagatgagccggcacagcctggaacagaagcctacagacgcccctcctaaagagtccctggaactggaagatcccagctctggcctgggcgtgacaaagcaagatctgggccctgtgcctatgatggacccttctggaattcacggcgagggcaccagatgcaccggatggttcgatgtggaagccatcgtggaaagacggaccggcgacgtggtgtccgaggacgaagatgagaacctggaagataccggcgtggacctggtggacttcatcgacgatacctgcgagtttgagcaggccggcgacgaagctcctagagcactgctgcatgcccaagagacacaggcccatgtgaacgccgtgcactacctgaagcggaagttcacatgcagccctaccgtgtctcccctgggcaatgtgcagtgttctatcgagggcgagctgagccctagactgcacgccatccaactgaatgaaggcagcggcaaggccaagcggagactgtttctgcctgatagcggctacggcaataccgaggtggaaacccagctgtctcaggtggcaggatccgatggcgaatctcaagcccctggcggcaaagaaaatgtgcagcctgctgaaggcgctggcggagatgttcgacagctgctgagaagcagcaacctgaaggccacactgctgggcaagttcaaggacgtgtacggcatcggcttcaacgaactcgtgcggtgcttcaagagcgacaagaccgtgtgcaccgattgggttgtgggagctgctggcgtgcaccattctgtggccgaaggactgaagcacctgatcgagcctttctgcacatacgcccacatgcagtgcctgacctgcaactggggagtgtttctgctgctgctcatccggttcaagtgcggcaagaacagactgaccgtggccaagtgcatctctaccctgctgaacgtgcaagagccctacctgctgatcgaacctccaaagctgagatccacagccgccgctctgtactggtacagaaccggcatcagcaacgtgtccgaagtgatcggagagcctcctgagtggatcgtgcggcagaccatgtttcagcacagcctcgaggacagcatcttcgacctgtctcagatggtgcagtgggcctacgaccacgatctggtggacgatagcgccattgcctaccagtatgcccagctggccgacgtggactctaatgccgccgctttcctgaagtctaacgctcaggccaaatacgtgaaggactgcgccaccatgtgcagacactacaagagagccgagaagcaggccatgaccatgagccagtggatcagagccagatgcgataagaccgacgacggcggagattggaggcctatcgtgcagttcctgagataccagaacgtcgagttcatcacctttctgagcgcctttaaggccttcctgaagggaatccccaagagaagctgcatcgtgctgtacggccctccaaacaccggcaagagctacttcggaatgagcctgatgcagtttctgcagggcagcatcatcagctacgtgaacagcaacagccacttttggctggcccctctggccgaagctaaagtggccatgctggacgatgccacaccacagtgctggtcctacatcgacacctacatgcggagcgtgctggacggcaaccccatgagcattgaccggaagcacaagaacctgatccagatgaagtgtccgcctctgatcatcaccagcaacaccaacgtgggcgaagatgacagatggcgctacctgcactccagagtggtggtgttcaagttcgagcagacctttccattcgaccagaacggcaatcccgtgtacgagctgtccgacaagaattggaagtccttcttcagccggacctggtccagactcgagctgcaagaggatgaggacaccgagcaggatggctctacagtgcgggcctttaagtgtgtgcccggccagaacaccaatatcctgggctctatggaagccctgagcgagagactgaacgcctaccaggacaagatcctgaccttctacgaagaggactccaaggacctgagggaccagatcgagcattggagatgtgtgcggggagagtgcgccgtgttctacaaggccagagagatgggccacagccacatcaaccaccagcaggttccacctctgcacgtgtccagaggcaaggcccacaatgccattgagctgcagatggccctggaaagcctgaaccagagcgacttcaacaccgaggaatggaccctgcaggacacaagcctggaaatgtggcggaccgagcctcagtgctgcttcaaaaagaaaggcgagacagtgaccgtgctgtatgactgcgacaaggacaacagcatggactacaccctgtggggccacgtgtacgtgtggggagatacaggctgggacaaagtgtgcggaaaggtggactacggcggcctgtactatgtgctgcacggcctgaaagtgtactacgttgagttccagcaagaggccgtgaagtacagcaagaccaacaagtgggaagtgcatatcggcagaacagtgatcccctacagcgagtccgtgtcctctacagccctgtgcgaaagagtgcctatcgccgagatcgccaatggcctccagcagaccagcattccctctcacacacacgccaccaccaaagagaacgcttgggtttcctctcagcctcctaccaagcggtccagaagatctgatccaggcggcgatcctgtcagagccctggatgccaatagcagaaccctgctgtctggaaccgcctgcgagaataccaccggcaactcttacagcgactgcacccctgtggtgcacctgaaaggcgaccccaattgtctgaaggccctgcggttcagattcgtgaaacacaagaatctgttcgtgaacgtgtcctccacctggcggtggaccaacaacaccgaagagaaggccatcgtgactgtgacctttaaggacgagcagcagagacagcagttcctcggcagcgtgaagatccccaactccatctgtgtgtgcaagggcgtgatgacagttggcagcatggtggaaggcagccaagagagagcccggacactgcacgaactgtgcgagcagagagaacagacccagcacgacatcgagctggactgcgtgtactgcctgaatcctctgaccagaaccgaggtgtacgacttcgccagatgggagctgagaatcgtgtacagacgggataccgcctacggcgtgtgcaagctgtgcctgaggttccacagcaaagtgcggaagtacaggcggtacaactactccatctacggccccacactggaacggcggacaaagaagcagctcgaagaactcgtgatccggtgctactgctgccagaaacctcagtgccccgtggaaaagcagcgccacgttgaccagggccagagattccacaacattgccgagcagtggaccggcagatgcctgcaatgttggaggccaacagccgctgaaaccggctctatgatcggccctggacctacactgcaggatatcgtgcttgagctggaacccgagcctgtggacctgagaggatatgagcagctggactccagcgaggacgaggacgagattgaccaccaccaacagcaggacagacccgatgtgcaagaagatgacggcgagcggtttagaatcctgagcgactgtcacgtgtgccagaataccgtgtcaagagtggtgcacagcacccacgacgacctgcacattctcgaggacctgcttatgggcaccctcgagatcgtggcccctaattgtgccgtgggcagcgaacagaaactgatctccgaggaagatctctgaggaagaatgtgcacagtgctaaccagaaaattcaggacaagactagtgcggccgcgactctagatcataatcagccataccacatttgtagaggttttacttgctttaaaaaacctcccacacctccccctgaacctgaaacataaaatgaatgcaattgttgttgttaacttgtttattgcagcttataatggttacaaataaagcaatagcatcacaaatttcacaaataaagcatttttttcactgc

SEQ ID NO: 56 - DNA, 5789 bp, Artificial Sequence
  MfPV3 Ii-E1E2-p2a-Ii-E6E7 as carried by Adenoviral vector
gtgatgcggttttggcagtacatcaatgggcgtggatagcggtttgactcacggggatttccaagtctccaccccattgacgtcaatgggagtttgttttggaaccaaaatcaacgggactttccaaaatgtcgtaacaactccgccccattgacgcaaatgggcggtaggcgtgtacggtgggaggtctatataagcagagctctccctatcagtgatagagatctccctatcagtgatagagatcgtcgacgagctcgtttagtgaaccgtcagatcgcctggagacgccatccacgctgttttgacctctagcaccggtgccaccatgcacagaaggcggagcagaagctgccgcgaggatcagaaacccgtgatggacgaccagcgggacctgatcagcaacaacgagcagctgcctatgctcggcagaaggcctggcgctcctgagagcaaatgttctagaggcgccctgtacaccggcttcagcatcctggttacactgctgctggccggacaggctaccaccgcctactttctgtatcagcagcagggcagactggacaagctgaccgtgaccagccagaacctgcagctggaaaacctgcggatgaagctgcccaagcctcctaagcctgtgtccaagatgcggatggccacacctctgctgatgcaggctttgcctatgggagcactgcctcagggccctatgcagaacgccaccaaatacggcaacatgaccgaggaccacgtgatgcatctgctgcagaatgccgatcctctgaaggtgtaccctccactgaagggcagctttcccgagaacctgcggcacctgaagaacaccatggaaaccatcgactggaaggtgttcgagagctggatgcaccactggctgctgttcgagatgagccggcacagcctggaacagaagcctacagacgcccctcctaaagagtccctggaactggaagatcccagctctggcctgggcgtgacaaagcaagatctgggccctgtgcctatgatggacccttctggaattcacggcgagggcaccagatgcaccggatggttcgatgtggaagccatcgtggaaagacggaccggcgacgtggtgtccgaggacgaagatgagaacctggaagataccggcgtggacctggtggacttcatcgacgatacctgcgagtttgagcaggccggcgacgaagctcctagagcactgctgcatgcccaagagacacaggcccatgtgaacgccgtgcactacctgaagcggaagttcacatgcagccctaccgtgtctcccctgggcaatgtgcagtgttctatcgagggcgagctgagccctagactgcacgccatccaactgaatgaaggcagcggcaaggccaagcggagactgtttctgcctgatagcggctacggcaataccgaggtggaaacccagctgtctcaggtggcaggatccgatggcgaatctcaagcccctggcggcaaagaaaatgtgcagcctgctgaaggcgctggcggagatgttcgacagctgctgagaagcagcaacctgaaggccacactgctgggcaagttcaaggacgtgtacggcatcggcttcaacgaactcgtgcggtgcttcaagagcgacaagaccgtgtgcaccgattgggttgtgggagctgctggcgtgcaccattctgtggccgaaggactgaagcacctgatcgagcctttctgcacatacgcccacatgcagtgcctgacctgcaactggggagtgtttctgctgctgctcatccggttcaagtgcggcaagaacagactgaccgtggccaagtgcatctctaccctgctgaacgtgcaagagccctacctgctgatcgaacctccaaagctgagatccacagccgccgctctgtactggtacagaaccggcatcagcaacgtgtccgaagtgatcggagagcctcctgagtggatcgtgcggcagaccatgtttcagcacagcctcgaggacagcatcttcgacctgtctcagatggtgcagtgggcctacgaccacgatctggtggacgatagcgccattgcctaccagtatgcccagctggccgacgtggactctaatgccgccgctttcctgaagtctaacgctcaggccaaatacgtgaaggactgcgccaccatgtgcagacactacaagagagccgagaagcaggccatgaccatgagccagtggatcagagccagatgcgataagaccgacgacggcggagattggaggcctatcgtgcagttcctgagataccagaacgtcgagttcatcacctttctgagcgcctttaaggccttcctgaagggaatccccaagagaagctgcatcgtgctgtacggccctccaaacaccggcaagagctacttcggaatgagcctgatgcagtttctgcagggcagcatcatcagctacgtgaacagcaacagccacttttggctggcccctctggccgaagctaaagtggccatgctggacgatgccacaccacagtgctggtcctacatcgacacctacatgcggagcgtgctggacggcaaccccatgagcattgaccggaagcacaagaacctgatccagatgaagtgtccgcctctgatcatcaccagcaacaccaacgtgggcgaagatgacagatggcgctacctgcactccagagtggtggtgttcaagttcgagcagacctttccattcgaccagaacggcaatcccgtgtacgagctgtccgacaagaattggaagtccttcttcagccggacctggtccagactcgagctgcaagaggatgaggacaccgagcaggatggctctacagtgcgggcctttaagtgtgtgcccggccagaacaccaatatcctgggctctatggaagccctgagcgagagactgaacgcctaccaggacaagatcctgaccttctacgaagaggactccaaggacctgagggaccagatcgagcattggagatgtgtgcggggagagtgcgccgtgttctacaaggccagagagatgggccacagccacatcaaccaccagcaggttccacctctgcacgtgtccagaggcaaggcccacaatgccattgagctgcagatggccctggaaagcctgaaccagagcgacttcaacaccgaggaatggaccctgcaggacacaagcctggaaatgtggcggaccgagcctcagtgctgcttcaaaaagaaaggcgagacagtgaccgtgctgtatgactgcgacaaggacaacagcatggactacaccctgtggggccacgtgtacgtgtggggagatacaggctgggacaaagtgtgcggaaaggtggactacggcggcctgtactatgtgctgcacggcctgaaagtgtactacgttgagttccagcaagaggccgtgaagtacagcaagaccaacaagtgggaagtgcatatcggcagaacagtgatcccctacagcgagtccgtgtcctctacagccctgtgcgaaagagtgcctatcgccgagatcgccaatggcctccagcagaccagcattccctctcacacacacgccaccaccaaagagaacgcttgggtttcctctcagcctcctaccaagcggtccagaagatctgatccaggcggcgatcctgtcagagccctggatgccaatagcagaaccctgctgtctggaaccgcctgcgagaataccaccggcaactcttacagcgactgcacccctgtggtgcacctgaaaggcgaccccaattgtctgaaggccctgcggttcagattcgtgaaacacaagaatctgttcgtgaacgtgtcctccacctggcggtggaccaacaacaccgaagagaaggccatcgtgactgtgacctttaaggacgagcagcagagacagcagttcctcggcagcgtgaagatccccaactccatctgtgtgtgcaagggcgtgatgacagttggcagcggcgccaccaatttcagtctgcttaaacaggccggggacgtcgaagagaaccccggacctatgcatcggcgcagatctcggtcttgtagagaagaccaaaagcctgtcatggatgatcaaagagatttaatttctaataatgaacaattacccatgttgggacggcgccccggagcccccgaatctaagtgcagccggggagctttatatacaggattttctattttagtgaccttattattagctggccaagccacaacagcttatttcttataccaacaacaaggacggttagataaattaacagtcacatctcaaaatttacaattagagaatttaagaatgaaattacctaaaccacccaaacccgtcagtaaaatgagaatggctacccccttattaatgcaagccctccccatgggcgccttaccccaaggacccatgcaaaatgctacaaagtatggaaatatgacagaagatcatgtcatgcacttattacaaaacgctgaccccttaaaagtctatccccctttaaaaggatctttccctgaaaatttaagacatttaaaaaatacaatggagacaattgattggaaagtctttgaatcttggatgcatcattggttattatttgaaatgtctaggcattctttagagcaaaaacccaccgatgctccacccaaggaaagtttagagttagaggacccttctagcggattaggagtcaccaaacaggacttaggacccgtccccatgatggtggaaggcagccaagagagagcccggacactgcacgaactgtgcgagcagagagaacagacccagcacgacatcgagctggactgcgtgtactgcctgaatcctctgaccagaaccgaggtgtacgacttcgccagatgggagctgagaatcgtgtacagacgggataccgcctacggcgtgtgcaagctgtgcctgaggttccacagcaaagtgcggaagtacaggcggtacaactactccatctacggccccacactggaacggcggacaaagaagcagctcgaagaactcgtgatccggtgctactgctgccagaaacctcagtgccccgtggaaaagcagcgccacgttgaccagggccagagattccacaacattgccgagcagtggaccggcagatgcctgcaatgttggaggccaacagccgctgaaaccggctctatgatcggccctggacctacactgcaggatatcgtgcttgagctggaacccgagcctgtggacctgagaggatatgagcagctggactccagcgaggacgaggacgagattgaccaccaccaacagcaggacagacccgatgtgcaagaagatgacggcgagcggtttagaatcctgagcgactgtcacgtgtgccagaataccgtgtcaagagtggtgcacagcacccacgacgacctgcacattctcgaggacctgcttatgggcaccctcgagatcgtggcccctaattgtgccgtgggcagcgaacagaaactgatctccgaggaagatctctgaggaagaatgtgcacagtgctaaccagaaaattcaggacaagactagtgcggccgcgactctagatcataatcagccataccacatttgtagaggttttacttgctttaaaaaacctcccacacctccccctgaacctgaaacataaaatgaatgcaattgttgttgttaacttgtttattgcagcttataatggttacaaataaagcaatagcatcacaaatttcacaaataaagcatttttttcactgc

SEQ ID NO: 57 - DNA, 4337 bp, Artificial Sequence
  MfPV3 E1E2E6E7 as carried by Adenoviral vector
gtgatgcggttttggcagtacatcaatgggcgtggatagcggtttgactcacggggatttccaagtctccaccccattgacgtcaatgggagtttgttttggaaccaaaatcaacgggactttccaaaatgtcgtaacaactccgccccattgacgcaaatgggcggtaggcgtgtacggtgggaggtctatataagcagagctctccctatcagtgatagagatctccctatcagtgatagagatcgtcgacgagctcgtttagtgaaccgtcagatcgcctggagacgccatccacgctgttttgacctctagcaccggtgccaccatggacccttctggaattcacggcgagggcaccagatgcaccggatggttcgatgtggaagccatcgtggaaagacggaccggcgacgtggtgtccgaggacgaagatgagaacctggaagataccggcgtggacctggtggacttcatcgacgatacctgcgagtttgagcaggccggcgacgaagctcctagagcactgctgcatgcccaagagacacaggcccatgtgaacgccgtgcactacctgaagcggaagttcacatgcagccctaccgtgtctcccctgggcaatgtgcagtgttctatcgagggcgagctgagccctagactgcacgccatccaactgaatgaaggcagcggcaaggccaagcggagactgtttctgcctgatagcggctacggcaataccgaggtggaaacccagctgtctcaggtggcaggatccgatggcgaatctcaagcccctggcggcaaagaaaatgtgcagcctgctgaaggcgctggcggagatgttcgacagctgctgagaagcagcaacctgaaggccacactgctgggcaagttcaaggacgtgtacggcatcggcttcaacgaactcgtgcggtgcttcaagagcgacaagaccgtgtgcaccgattgggttgtgggagctgctggcgtgcaccattctgtggccgaaggactgaagcacctgatcgagcctttctgcacatacgcccacatgcagtgcctgacctgcaactggggagtgtttctgctgctgctcatccggttcaagtgcggcaagaacagactgaccgtggccaagtgcatctctaccctgctgaacgtgcaagagccctacctgctgatcgaacctccaaagctgagatccacagccgccgctctgtactggtacagaaccggcatcagcaacgtgtccgaagtgatcggagagcctcctgagtggatcgtgcggcagaccatgtttcagcacagcctcgaggacagcatcttcgacctgtctcagatggtgcagtgggcctacgaccacgatctggtggacgatagcgccattgcctaccagtatgcccagctggccgacgtggactctaatgccgccgctttcctgaagtctaacgctcaggccaaatacgtgaaggactgcgccaccatgtgcagacactacaagagagccgagaagcaggccatgaccatgagccagtggatcagagccagatgcgataagaccgacgacggcggagattggaggcctatcgtgcagttcctgagataccagaacgtcgagttcatcacctttctgagcgcctttaaggccttcctgaagggaatccccaagagaagctgcatcgtgctgtacggccctccaaacaccggcaagagctacttcggaatgagcctgatgcagtttctgcagggcagcatcatcagctacgtgaacagcaacagccacttttggctggcccctctggccgaagctaaagtggccatgctggacgatgccacaccacagtgctggtcctacatcgacacctacatgcggagcgtgctggacggcaaccccatgagcattgaccggaagcacaagaacctgatccagatgaagtgtccgcctctgatcatcaccagcaacaccaacgtgggcgaagatgacagatggcgctacctgcactccagagtggtggtgttcaagttcgagcagacctttccattcgaccagaacggcaatcccgtgtacgagctgtccgacaagaattggaagtccttcttcagccggacctggtccagactcgagctgcaagaggatgaggacaccgagcaggatggctctacagtgcgggcctttaagtgtgtgcccggccagaacaccaatatcctgggctctatggaagccctgagcgagagactgaacgcctaccaggacaagatcctgaccttctacgaagaggactccaaggacctgagggaccagatcgagcattggagatgtgtgcggggagagtgcgccgtgttctacaaggccagagagatgggccacagccacatcaaccaccagcaggttccacctctgcacgtgtccagaggcaaggcccacaatgccattgagctgcagatggccctggaaagcctgaaccagagcgacttcaacaccgaggaatggaccctgcaggacacaagcctggaaatgtggcggaccgagcctcagtgctgcttcaaaaagaaaggcgagacagtgaccgtgctgtatgactgcgacaaggacaacagcatggactacaccctgtggggccacgtgtacgtgtggggagatacaggctgggacaaagtgtgcggaaaggtggactacggcggcctgtactatgtgctgcacggcctgaaagtgtactacgttgagttccagcaagaggccgtgaagtacagcaagaccaacaagtgggaagtgcatatcggcagaacagtgatcccctacagcgagtccgtgtcctctacagccctgtgcgaaagagtgcctatcgccgagatcgccaatggcctccagcagaccagcattccctctcacacacacgccaccaccaaagagaacgcttgggtttcctctcagcctcctaccaagcggtccagaagatctgatccaggcggcgatcctgtcagagccctggatgccaatagcagaaccctgctgtctggaaccgcctgcgagaataccaccggcaactcttacagcgactgcacccctgtggtgcacctgaaaggcgaccccaattgtctgaaggccctgcggttcagattcgtgaaacacaagaatctgttcgtgaacgtgtcctccacctggcggtggaccaacaacaccgaagagaaggccatcgtgactgtgacctttaaggacgagcagcagagacagcagttcctcggcagcgtgaagatccccaactccatctgtgtgtgcaagggcgtgatgacagttggcagcatggtggaaggcagccaagagagagcccggacactgcacgaactgtgcgagcagagagaacagacccagcacgacatcgagctggactgcgtgtactgcctgaatcctctgaccagaaccgaggtgtacgacttcgccagatgggagctgagaatcgtgtacagacgggataccgcctacggcgtgtgcaagctgtgcctgaggttccacagcaaagtgcggaagtacaggcggtacaactactccatctacggccccacactggaacggcggacaaagaagcagctcgaagaactcgtgatccggtgctactgctgccagaaacctcagtgccccgtggaaaagcagcgccacgttgaccagggccagagattccacaacattgccgagcagtggaccggcagatgcctgcaatgttggaggccaacagccgctgaaaccggctctatgatcggccctggacctacactgcaggatatcgtgcttgagctggaacccgagcctgtggacctgagaggatatgagcagctggactccagcgaggacgaggacgagattgaccaccaccaacagcaggacagacccgatgtgcaagaagatgacggcgagcggtttagaatcctgagcgactgtcacgtgtgccagaataccgtgtcaagagtggtgcacagcacccacgacgacctgcacattctcgaggacctgcttatgggcaccctcgagatcgtggcccctaattgtgccgtgggcagcgaacagaaactgatctccgaggaagatctctgaggaagaatgtgcacagtgctaaccagaaaattcaggacaagactagtgcggccgcgactctagatcataatcagccataccacatttgtagaggttttacttgctttaaaaaacctcccacacctccccctgaacctgaaacataaaatgaatgcaattgttgttgttaacttgtttattgcagcttataatggttacaaataaagcaatagcatcacaaatttcacaaataaagcatttttttcactgc

SEQ ID NO: 58 - DNA, 5789 bp, Artificial Sequence
  MfPV3 Ii-E1E6E7-p2a-Ii-E2 as carried by Adenoviral vector
gtgatgcggttttggcagtacatcaatgggcgtggatagcggtttgactcacggggatttccaagtctccaccccattgacgtcaatgggagtttgttttggaaccaaaatcaacgggactttccaaaatgtcgtaacaactccgccccattgacgcaaatgggcggtaggcgtgtacggtgggaggtctatataagcagagctctccctatcagtgatagagatctccctatcagtgatagagatcgtcgacgagctcgtttagtgaaccgtcagatcgcctggagacgccatccacgctgttttgacctctagcaccggtgccaccatgcacagaaggcggagcagaagctgccgcgaggatcagaaacccgtgatggacgaccagcgggacctgatcagcaacaacgagcagctgcctatgctcggcagaaggcctggcgctcctgagagcaaatgttctagaggcgccctgtacaccggcttcagcatcctggttacactgctgctggccggacaggctaccaccgcctactttctgtatcagcagcagggcagactggacaagctgaccgtgaccagccagaacctgcagctggaaaacctgcggatgaagctgcccaagcctcctaagcctgtgtccaagatgcggatggccacacctctgctgatgcaggctttgcctatgggagcactgcctcagggccctatgcagaacgccaccaaatacggcaacatgaccgaggaccacgtgatgcatctgctgcagaatgccgatcctctgaaggtgtaccctccactgaagggcagctttcccgagaacctgcggcacctgaagaacaccatggaaaccatcgactggaaggtgttcgagagctggatgcaccactggctgctgttcgagatgagccggcacagcctggaacagaagcctacagacgcccctcctaaagagtccctggaactggaagatcccagctctggcctgggcgtgacaaagcaagatctgggccctgtgcctatgatggacccttctggaattcacggcgagggcaccagatgcaccggatggttcgatgtggaagccatcgtggaaagacggaccggcgacgtggtgtccgaggacgaagatgagaacctggaagataccggcgtggacctggtggacttcatcgacgatacctgcgagtttgagcaggccggcgacgaagctcctagagcactgctgcatgcccaagagacacaggcccatgtgaacgccgtgcactacctgaagcggaagttcacatgcagccctaccgtgtctcccctgggcaatgtgcagtgttctatcgagggcgagctgagccctagactgcacgccatccaactgaatgaaggcagcggcaaggccaagcggagactgtttctgcctgatagcggctacggcaataccgaggtggaaacccagctgtctcaggtggcaggatccgatggcgaatctcaagcccctggcggcaaagaaaatgtgcagcctgctgaaggcgctggcggagatgttcgacagctgctgagaagcagcaacctgaaggccacactgctgggcaagttcaaggacgtgtacggcatcggcttcaacgaactcgtgcggtgcttcaagagcgacaagaccgtgtgcaccgattgggttgtgggagctgctggcgtgcaccattctgtggccgaaggactgaagcacctgatcgagcctttctgcacatacgcccacatgcagtgcctgacctgcaactggggagtgtttctgctgctgctcatccggttcaagtgcggcaagaacagactgaccgtggccaagtgcatctctaccctgctgaacgtgcaagagccctacctgctgatcgaacctccaaagctgagatccacagccgccgctctgtactggtacagaaccggcatcagcaacgtgtccgaagtgatcggagagcctcctgagtggatcgtgcggcagaccatgtttcagcacagcctcgaggacagcatcttcgacctgtctcagatggtgcagtgggcctacgaccacgatctggtggacgatagcgccattgcctaccagtatgcccagctggccgacgtggactctaatgccgccgctttcctgaagtctaacgctcaggccaaatacgtgaaggactgcgccaccatgtgcagacactacaagagagccgagaagcaggccatgaccatgagccagtggatcagagccagatgcgataagaccgacgacggcggagattggaggcctatcgtgcagttcctgagataccagaacgtcgagttcatcacctttctgagcgcctttaaggccttcctgaagggaatccccaagagaagctgcatcgtgctgtacggccctccaaacaccggcaagagctacttcggaatgagcctgatgcagtttctgcagggcagcatcatcagctacgtgaacagcaacagccacttttggctggcccctctggccgaagctaaagtggccatgctggacgatgccacaccacagtgctggtcctacatcgacacctacatgcggagcgtgctggacggcaaccccatgagcattgaccggaagcacaagaacctgatccagatgaagtgtccgcctctgatcatcaccagcaacaccaacgtgggcgaagatgacagatggcgctacctgcactccagagtggtggtgttcaagttcgagcagacctttccattcgaccagaacggcaatcccgtgtacgagctgtccgacaagaattggaagtccttcttcagccggacctggtccagactcgagctgcaagaggatgaggacaccgagcaggatggctctacagtgcgggcctttaagtgtgtgcccggccagaacaccaatatcctgggctctatggtggaaggcagccaagagagagcccggacactgcacgaactgtgcgagcagagagaacagacccagcacgacatcgagctggactgcgtgtactgcctgaatcctctgaccagaaccgaggtgtacgacttcgccagatgggagctgagaatcgtgtacagacgggataccgcctacggcgtgtgcaagctgtgcctgaggttccacagcaaagtgcggaagtacaggcggtacaactactccatctacggccccacactggaacggcggacaaagaagcagctcgaagaactcgtgatccggtgctactgctgccagaaacctcagtgccccgtggaaaagcagcgccacgttgaccagggccagagattccacaacattgccgagcagtggaccggcagatgcctgcaatgttggaggccaacagccgctgaaaccggctctatgatcggccctggacctacactgcaggatatcgtgcttgagctggaacccgagcctgtggacctgagaggatatgagcagctggactccagcgaggacgaggacgagattgaccaccaccaacagcaggacagacccgatgtgcaagaagatgacggcgagcggtttagaatcctgagcgactgtcacgtgtgccagaataccgtgtcaagagtggtgcacagcacccacgacgacctgcacattctcgaggacctgcttatgggcaccctcgagatcgtggcccctaattgtgccgtgggcagcggcgccaccaatttcagtctgcttaaacaggccggggacgtcgaagagaaccccggacctatgcatcggcgcagatctcggtcttgtagagaagaccaaaagcctgtcatggatgatcaaagagatttaatttctaataatgaacaattacccatgttgggacggcgccccggagcccccgaatctaagtgcagccggggagctttatatacaggattttctattttagtgaccttattattagctggccaagccacaacagcttatttcttataccaacaacaaggacggttagataaattaacagtcacatctcaaaatttacaattagagaatttaagaatgaaattacctaaaccacccaaacccgtcagtaaaatgagaatggctacccccttattaatgcaagccctccccatgggcgccttaccccaaggacccatgcaaaatgctacaaagtatggaaatatgacagaagatcatgtcatgcacttattacaaaacgctgaccccttaaaagtctatccccctttaaaaggatctttccctgaaaatttaagacatttaaaaaatacaatggagacaattgattggaaagtctttgaatcttggatgcatcattggttattatttgaaatgtctaggcattctttagagcaaaaacccaccgatgctccacccaaggaaagtttagagttagaggacccttctagcggattaggagtcaccaaacaggacttaggacccgtccccatgatggaagccctgagcgagagactgaacgcctaccaggacaagatcctgaccttctacgaagaggactccaaggacctgagggaccagatcgagcattggagatgtgtgcggggagagtgcgccgtgttctacaaggccagagagatgggccacagccacatcaaccaccagcaggttccacctctgcacgtgtccagaggcaaggcccacaatgccattgagctgcagatggccctggaaagcctgaaccagagcgacttcaacaccgaggaatggaccctgcaggacacaagcctggaaatgtggcggaccgagcctcagtgctgcttcaaaaagaaaggcgagacagtgaccgtgctgtatgactgcgacaaggacaacagcatggactacaccctgtggggccacgtgtacgtgtggggagatacaggctgggacaaagtgtgcggaaaggtggactacggcggcctgtactatgtgctgcacggcctgaaagtgtactacgttgagttccagcaagaggccgtgaagtacagcaagaccaacaagtgggaagtgcatatcggcagaacagtgatcccctacagcgagtccgtgtcctctacagccctgtgcgaaagagtgcctatcgccgagatcgccaatggcctccagcagaccagcattccctctcacacacacgccaccaccaaagagaacgcttgggtttcctctcagcctcctaccaagcggtccagaagatctgatccaggcggcgatcctgtcagagccctggatgccaatagcagaaccctgctgtctggaaccgcctgcgagaataccaccggcaactcttacagcgactgcacccctgtggtgcacctgaaaggcgaccccaattgtctgaaggccctgcggttcagattcgtgaaacacaagaatctgttcgtgaacgtgtcctccacctggcggtggaccaacaacaccgaagagaaggccatcgtgactgtgacctttaaggacgagcagcagagacagcagttcctcggcagcgtgaagatccccaactccatctgtgtgtgcaagggcgtgatgacagttggcagcgaacagaaactgatctccgaggaagatctctgaggaagaatgtgcacagtgctaaccagaaaattcaggacaagactagtgcggccgcgactctagatcataatcagccataccacatttgtagaggttttacttgctttaaaaaacctcccacacctccccctgaacctgaaacataaaatgaatgcaattgttgttgttaacttgtttattgcagcttataatggttacaaataaagcaatagcatcacaaatttcacaaataaagcatttttttcactgc

SEQ ID NO: 59 - DNA, 3947 bp, Artificial Sequence
  MfPV3 Ii-E1E6E7 as carried by Adenoviral vector
gtgatgcggttttggcagtacatcaatgggcgtggatagcggtttgactcacggggatttccaagtctccaccccattgacgtcaatgggagtttgttttggaaccaaaatcaacgggactttccaaaatgtcgtaacaactccgccccattgacgcaaatgggcggtaggcgtgtacggtgggaggtctatataagcagagctctccctatcagtgatagagatctccctatcagtgatagagatcgtcgacgagctcgtttagtgaaccgtcagatcgcctggagacgccatccacgctgttttgacctctagcaccggtgccaccatgcacagaaggcggagcagaagctgccgcgaggatcagaaacccgtgatggacgaccagcgggacctgatcagcaacaacgagcagctgcctatgctcggcagaaggcctggcgctcctgagagcaaatgttctagaggcgccctgtacaccggcttcagcatcctggttacactgctgctggccggacaggctaccaccgcctactttctgtatcagcagcagggcagactggacaagctgaccgtgaccagccagaacctgcagctggaaaacctgcggatgaagctgcccaagcctcctaagcctgtgtccaagatgcggatggccacacctctgctgatgcaggctttgcctatgggagcactgcctcagggccctatgcagaacgccaccaaatacggcaacatgaccgaggaccacgtgatgcatctgctgcagaatgccgatcctctgaaggtgtaccctccactgaagggcagctttcccgagaacctgcggcacctgaagaacaccatggaaaccatcgactggaaggtgttcgagagctggatgcaccactggctgctgttcgagatgagccggcacagcctggaacagaagcctacagacgcccctcctaaagagtccctggaactggaagatcccagctctggcctgggcgtgacaaagcaagatctgggccctgtgcctatgatggacccttctggaattcacggcgagggcaccagatgcaccggatggttcgatgtggaagccatcgtggaaagacggaccggcgacgtggtgtccgaggacgaagatgagaacctggaagataccggcgtggacctggtggacttcatcgacgatacctgcgagtttgagcaggccggcgacgaagctcctagagcactgctgcatgcccaagagacacaggcccatgtgaacgccgtgcactacctgaagcggaagttcacatgcagccctaccgtgtctcccctgggcaatgtgcagtgttctatcgagggcgagctgagccctagactgcacgccatccaactgaatgaaggcagcggcaaggccaagcggagactgtttctgcctgatagcggctacggcaataccgaggtggaaacccagctgtctcaggtggcaggatccgatggcgaatctcaagcccctggcggcaaagaaaatgtgcagcctgctgaaggcgctggcggagatgttcgacagctgctgagaagcagcaacctgaaggccacactgctgggcaagttcaaggacgtgtacggcatcggcttcaacgaactcgtgcggtgcttcaagagcgacaagaccgtgtgcaccgattgggttgtgggagctgctggcgtgcaccattctgtggccgaaggactgaagcacctgatcgagcctttctgcacatacgcccacatgcagtgcctgacctgcaactggggagtgtttctgctgctgctcatccggttcaagtgcggcaagaacagactgaccgtggccaagtgcatctctaccctgctgaacgtgcaagagccctacctgctgatcgaacctccaaagctgagatccacagccgccgctctgtactggtacagaaccggcatcagcaacgtgtccgaagtgatcggagagcctcctgagtggatcgtgcggcagaccatgtttcagcacagcctcgaggacagcatcttcgacctgtctcagatggtgcagtgggcctacgaccacgatctggtggacgatagcgccattgcctaccagtatgcccagctggccgacgtggactctaatgccgccgctttcctgaagtctaacgctcaggccaaatacgtgaaggactgcgccaccatgtgcagacactacaagagagccgagaagcaggccatgaccatgagccagtggatcagagccagatgcgataagaccgacgacggcggagattggaggcctatcgtgcagttcctgagataccagaacgtcgagttcatcacctttctgagcgcctttaaggccttcctgaagggaatccccaagagaagctgcatcgtgctgtacggccctccaaacaccggcaagagctacttcggaatgagcctgatgcagtttctgcagggcagcatcatcagctacgtgaacagcaacagccacttttggctggcccctctggccgaagctaaagtggccatgctggacgatgccacaccacagtgctggtcctacatcgacacctacatgcggagcgtgctggacggcaaccccatgagcattgaccggaagcacaagaacctgatccagatgaagtgtccgcctctgatcatcaccagcaacaccaacgtgggcgaagatgacagatggcgctacctgcactccagagtggtggtgttcaagttcgagcagacctttccattcgaccagaacggcaatcccgtgtacgagctgtccgacaagaattggaagtccttcttcagccggacctggtccagactcgagctgcaagaggatgaggacaccgagcaggatggctctacagtgcgggcctttaagtgtgtgcccggccagaacaccaatatcctgggctctatggtggaaggcagccaagagagagcccggacactgcacgaactgtgcgagcagagagaacagacccagcacgacatcgagctggactgcgtgtactgcctgaatcctctgaccagaaccgaggtgtacgacttcgccagatgggagctgagaatcgtgtacagacgggataccgcctacggcgtgtgcaagctgtgcctgaggttccacagcaaagtgcggaagtacaggcggtacaactactccatctacggccccacactggaacggcggacaaagaagcagctcgaagaactcgtgatccggtgctactgctgccagaaacctcagtgccccgtggaaaagcagcgccacgttgaccagggccagagattccacaacattgccgagcagtggaccggcagatgcctgcaatgttggaggccaacagccgctgaaaccggctctatgatcggccctggacctacactgcaggatatcgtgcttgagctggaacccgagcctgtggacctgagaggatatgagcagctggactccagcgaggacgaggacgagattgaccaccaccaacagcaggacagacccgatgtgcaagaagatgacggcgagcggtttagaatcctgagcgactgtcacgtgtgccagaataccgtgtcaagagtggtgcacagcacccacgacgacctgcacattctcgaggacctgcttatgggcaccctcgagatcgtggcccctaattgtgccgtgggcagcgaacagaaactgatctccgaggaagatctctgaggaagaatgtgcacagtgctaaccagaaaattcaggacaagactagtgcggccgcgactctagatcataatcagccataccacatttgtagaggttttacttgctttaaaaaacctcccacacctccccctgaacctgaaacataaaatgaatgcaattgttgttgttaacttgtttattgcagcttataatggttacaaataaagcaatagcatcacaaatttcacaaataaagcatttttttcactgc

SEQ ID NO: 60 - DNA, 5095 bp, Artificial Sequence
  HPV16 Ii-E1E2E6E7 as carried by Adenoviral vector
gtgatgcggttttggcagtacatcaatgggcgtggatagcggtttgactcacggggatttccaagtctccaccccattgacgtcaatgggagtttgttttggaaccaaaatcaacgggactttccaaaatgtcgtaacaactccgccccattgacgcaaatgggcggtaggcgtgtacggtgggaggtctatataagcagagctctccctatcagtgatagagatctccctatcagtgatagagatcgtcgacgagctcgtttagtgaaccgtcagatcgcctggagacgccatccacgctgttttgacctctagcaccggtgccaccatgcacagaaggcggagcagaagctgccgcgaggatcagaaacccgtgatggacgaccagcgggacctgatcagcaacaacgagcagctgcctatgctcggcagaaggcctggcgctcctgagagcaaatgttctagaggcgccctgtacaccggcttcagcatcctggttacactgctgctggccggacaggctaccaccgcctactttctgtatcagcagcagggcagactggacaagctgaccgtgaccagccagaacctgcagctggaaaacctgcggatgaagctgcccaagcctcctaagcctgtgtccaagatgcggatggccacacctctgctgatgcaggctttgcctatgggagcactgcctcagggccctatgcagaacgccaccaaatacggcaacatgaccgaggaccacgtgatgcatctgctgcagaatgccgatcctctgaaggtgtaccctccactgaagggcagctttcccgagaacctgcggcacctgaagaacaccatggaaaccatcgactggaaggtgttcgagagctggatgcaccactggctgctgttcgagatgagccggcacagcctggaacagaagcctacagacgcccctcctaaagagtccctggaactggaagatcccagctctggcctgggcgtgacaaagcaagatctgggccctgtgcctatgatggccgatcctgctggcacaaacggcgaagaaggcacaggctgcaacggctggttttacgtggaagccgtggtggaaaagaaaaccggcgacgccatcagcgacgacgagaacgagaatgacagcgacaccggcgaggacctggtggacttcatcgtgaacgacaacgactacctgacacaggccgagacagagacagcccacgctctgtttacagcccaagaggccaagcagcacagagatgccgttcaggtgctgaagagaaagtacctgggcagccctctgagcgacatcagcggctgtgtggacaacaacatcagccccagactgaaggccatctgcatcgagaagcagagcagagccgccaagcggagactgtttgagagcgaggatagcggctacggcaataccgaggtggaaacccagcaaatgctgcaggtcgagggcagacacgaaaccgagacaccttgcagccagtacagcggaggatctggcggaggctgtagccagtactcttctggaagtggcggagagggcgtgtccgagagacacaccatttgtcagacccctctgaccaacatcctgaacgtgctgaaaaccagcaacgccaaggccgccatgctggccaagttcaaagagctgtacggcgtcagcttcagcgaactcgtgcggcccttcaagagcaacaagtccacctgttgcgactggtgcattgccgcctttggcctgacaccttctatcgccgacagcatcaagaccctgctccagcagtactgtctgtacctgcacattcagagcctggcctgctcttggggaatggtggtgctgctgctcgtgcggtacaagtgcggcaagaacagagagacaattgagaagctgctgagcaaactgctgtgcgtgtcccctatgtgcatgatgatcgagcctccaaagctgcggtctacagccgccgctctgtactggtacaagaccggcatcagcaatatctccgaggtgtacggcgacacccctgagtggattcagagacagaccgtcctgcagcacagcttcaacgactgcaccttcgagctgtcccagatggtgcagtgggcctacgacaatgacatcgtggacgactccgagatcgcctataagtacgcccagctggccgacaccaacagcaatgccagcgccttcctgaagtccaacagccaggccaagatcgtgaaggactgcgccaccatgtgcagacactacaagcgggccgagaagaaacagatgagcatgagccagtggatcaagtacagatgcgacagagtggacgacggcggcgattggaagcagatcgtgatgttcctgagataccagggcgtcgagttcatgagctttctgacagccctgaagcggttcctgcagggcatccccaagaagaactgcatcctgctgtatggcgccgctaacaccggcaagagcctgttcggaatgagcctgatgaagtttctgcagggctccgtgatctgctttgtgaacagcaagagccacttctggctccagccactggccgatgccaagattggcatgctggacgatgccaccgtgccttgctggaactacatcgacgacaacctgagaaacgccctggacggcaacctggtttctatggacgtgaagcacagacccctggtgcagctgaagtgtcctccactgctgatcaccagcaacatcaacgccggcaccgattccagatggccctatctgcacaaccggctggtggtgtttacctttcctaacgagttccccttcgacgaaaacggcaaccccgtgtacgagctgaacgataagaattggaagtccttcttcagccggacctggtccagactgagcctgcacgaggatgaggacaaagagaacgacggcgacagcctgcctaccttcaaatgtgtcagcggccagaacaccaacacactgggcagcatggaaacactgtgccagcggctgaacgtgtgccaggacaagattctgacccactatgagaacgacagcaccgacctgagggaccacatcgactactggaagcacatgcggctggaatgcgccatctactacaaggctagagagatgggcttcaagcacatcaaccaccaggtggtgcctacactggccgtgtctaagaacaaggctctgcaggccatcgaactgcagctgaccctggaaacaatctacaactcccagtactccaacgagaagtggaccctccaggacgtgtcactggaagtgtacctgaccgctcctaccggctgcatcaagaaacacggctacaccgtggaagtgcagtttgacggcgatatctgcaataccatgcactacaccaactggacccacatctacatctgcgaagaggccagcgtgacagtggtggaaggccaggtcgactactacggcctgtactacgtgcacgagggcatcagaacctacttcgtgcagttcaaggatgacgccgagaagtacagcaagaacaaagtgtgggaagtgcacgctggcggccaagtgatcctgtgtcctacaagcgtgttcagcagcaacgaagtgtctagccccgagatcatcagacagcacctggccaatcatcctgccgccacacacacaaaagctgtggccctgggcaccgaggaaacacagaccacaattcagaggcccagaagcgagcccgataccggcaatccttgtcacaccaccaagctgctgcaccgggattccgtggattctgcccctatcctgaccgccttcaacagctcccacaaaggccggatcaactgcaacagcaacaccacacctatcgtgcacctgaaaggggacgccaacactctgaaggccctgcggtacagattcaagaagcactgtaccctgtataccgccgtgtccagcacatggcactggaccggacacaacgtgaaacacaagagcgccatcgtgaccctgacctacgatagcgagtggcagagggaccagttcctgagccaagtgaagatccctaagaccatcaccgtgtccaccggctttatgagcattggcagcatgcaccagaaacggacagccatgttccaggatcctcaagagcggccacggaagctgcctcagctgtgtacagaactgcagaccaccatccacgacatcatcctcgagtgcgtgtactgcaagcagcagctcctgcggagagaagtgtacgacttcgccttccgggatctgtgcatcgtgtacagagatggcaacccctacgccgtgtgcgacaagtgcctgaagttctactccaagatcagcgagtaccggcactactgctactccctgtacggcaccacacttgagcagcagtacaacaagcccctgtgcgatctgctgatccggtgcatcaactgccagaaacctcagtgccccgaggaaaagcagagacacctggacaagaagcagcggttccacaacattagaggcagatggacaggccggtgcatgagctgctgtagaagcagcagaacaagacggggctccatgcacggcgataccccaacactgcacgagtacatgctggatctgcagcccgagacaaccgatctgtacggctatgagcagctgaatgactccagcgaggaagaggacgagatcgacggacctgctggacaggctgaacctgatagagcccactacaatatcgtgaccttctgctgcaagtgcgatagcaccctgagaagatgcgtgcagagcacccacgtggacatcaggaccctcgaggatctgctcatgggcaccctgggaattgtggccccaatctgctctcagaagccttgagcgcggccgcggaagaatgtgcacagtgctaaccagaaaattcaggacaagactagtgactctagatcataatcagccataccacatttgtagaggttttacttgctttaaaaaacctcccacacctccccctgaacctgaaacataaaatgaatgcaattgttgttgttaacttgtttattgcagcttataatggttacaaataaagcaatagcatcacaaatttcacaaataaagcatttttttcactgc

SEQ ID NO: 61 - DNA, 5855 bp, Artificial Sequence
  HPV16 Ii-E1E2-p2a-Ii-E6E7 as carried by Adenoviral vector
gtgatgcggttttggcagtacatcaatgggcgtggatagcggtttgactcacggggatttccaagtctccaccccattgacgtcaatgggagtttgttttggaaccaaaatcaacgggactttccaaaatgtcgtaacaactccgccccattgacgcaaatgggcggtaggcgtgtacggtgggaggtctatataagcagagctctccctatcagtgatagagatctccctatcagtgatagagatcgtcgacgagctcgtttagtgaaccgtcagatcgcctggagacgccatccacgctgttttgacctctagcaccggtgccaccatgcacagaaggcggagcagaagctgccgcgaggatcagaaacccgtgatggacgaccagcgggacctgatcagcaacaacgagcagctgcctatgctcggcagaaggcctggcgctcctgagagcaaatgttctagaggcgccctgtacaccggcttcagcatcctggttacactgctgctggccggacaggctaccaccgcctactttctgtatcagcagcagggcagactggacaagctgaccgtgaccagccagaacctgcagctggaaaacctgcggatgaagctgcccaagcctcctaagcctgtgtccaagatgcggatggccacacctctgctgatgcaggctttgcctatgggagcactgcctcagggccctatgcagaacgccaccaaatacggcaacatgaccgaggaccacgtgatgcatctgctgcagaatgccgatcctctgaaggtgtaccctccactgaagggcagctttcccgagaacctgcggcacctgaagaacaccatggaaaccatcgactggaaggtgttcgagagctggatgcaccactggctgctgttcgagatgagccggcacagcctggaacagaagcctacagacgcccctcctaaagagtccctggaactggaagatcccagctctggcctgggcgtgacaaagcaagatctgggccctgtgcctatgatggccgatcctgctggcacaaacggcgaagaaggcacaggctgcaacggctggttttacgtggaagccgtggtggaaaagaaaaccggcgacgccatcagcgacgacgagaacgagaatgacagcgacaccggcgaggacctggtggacttcatcgtgaacgacaacgactacctgacacaggccgagacagagacagcccacgctctgtttacagcccaagaggccaagcagcacagagatgccgttcaggtgctgaagagaaagtacctgggcagccctctgagcgacatcagcggctgtgtggacaacaacatcagccccagactgaaggccatctgcatcgagaagcagagcagagccgccaagcggagactgtttgagagcgaggatagcggctacggcaataccgaggtggaaacccagcaaatgctgcaggtcgagggcagacacgaaaccgagacaccttgcagccagtacagcggaggatctggcggaggctgtagccagtactcttctggaagtggcggagagggcgtgtccgagagacacaccatttgtcagacccctctgaccaacatcctgaacgtgctgaaaaccagcaacgccaaggccgccatgctggccaagttcaaagagctgtacggcgtcagcttcagcgaactcgtgcggcccttcaagagcaacaagtccacctgttgcgactggtgcattgccgcctttggcctgacaccttctatcgccgacagcatcaagaccctgctccagcagtactgtctgtacctgcacattcagagcctggcctgctcttggggaatggtggtgctgctgctcgtgcggtacaagtgcggcaagaacagagagacaattgagaagctgctgagcaaactgctgtgcgtgtcccctatgtgcatgatgatcgagcctccaaagctgcggtctacagccgccgctctgtactggtacaagaccggcatcagcaatatctccgaggtgtacggcgacacccctgagtggattcagagacagaccgtcctgcagcacagcttcaacgactgcaccttcgagctgtcccagatggtgcagtgggcctacgacaatgacatcgtggacgactccgagatcgcctataagtacgcccagctggccgacaccaacagcaatgccagcgccttcctgaagtccaacagccaggccaagatcgtgaaggactgcgccaccatgtgcagacactacaagcgggccgagaagaaacagatgagcatgagccagtggatcaagtacagatgcgacagagtggacgacggcggcgattggaagcagatcgtgatgttcctgagataccagggcgtcgagttcatgagctttctgacagccctgaagcggttcctgcagggcatccccaagaagaactgcatcctgctgtatggcgccgctaacaccggcaagagcctgttcggaatgagcctgatgaagtttctgcagggctccgtgatctgctttgtgaacagcaagagccacttctggctccagccactggccgatgccaagattggcatgctggacgatgccaccgtgccttgctggaactacatcgacgacaacctgagaaacgccctggacggcaacctggtttctatggacgtgaagcacagacccctggtgcagctgaagtgtcctccactgctgatcaccagcaacatcaacgccggcaccgattccagatggccctatctgcacaaccggctggtggtgtttacctttcctaacgagttccccttcgacgaaaacggcaaccccgtgtacgagctgaacgataagaattggaagtccttcttcagccggacctggtccagactgagcctgcacgaggatgaggacaaagagaacgacggcgacagcctgcctaccttcaaatgtgtcagcggccagaacaccaacacactgggcagcatggaaacactgtgccagcggctgaacgtgtgccaggacaagattctgacccactatgagaacgacagcaccgacctgagggaccacatcgactactggaagcacatgcggctggaatgcgccatctactacaaggctagagagatgggcttcaagcacatcaaccaccaggtggtgcctacactggccgtgtctaagaacaaggctctgcaggccatcgaactgcagctgaccctggaaacaatctacaactcccagtactccaacgagaagtggaccctccaggacgtgtcactggaagtgtacctgaccgctcctaccggctgcatcaagaaacacggctacaccgtggaagtgcagtttgacggcgatatctgcaataccatgcactacaccaactggacccacatctacatctgcgaagaggccagcgtgacagtggtggaaggccaggtcgactactacggcctgtactacgtgcacgagggcatcagaacctacttcgtgcagttcaaggatgacgccgagaagtacagcaagaacaaagtgtgggaagtgcacgctggcggccaagtgatcctgtgtcctacaagcgtgttcagcagcaacgaagtgtctagccccgagatcatcagacagcacctggccaatcatcctgccgccacacacacaaaagctgtggccctgggcaccgaggaaacacagaccacaattcagaggcccagaagcgagcccgataccggcaatccttgtcacaccaccaagctgctgcaccgggattccgtggattctgcccctatcctgaccgccttcaacagctcccacaaaggccggatcaactgcaacagcaacaccacacctatcgtgcacctgaaaggggacgccaacactctgaaggccctgcggtacagattcaagaagcactgtaccctgtataccgccgtgtccagcacatggcactggaccggacacaacgtgaaacacaagagcgccatcgtgaccctgacctacgatagcgagtggcagagggaccagttcctgagccaagtgaagatccctaagaccatcaccgtgtccaccggctttatgagcattggcagcggcagcggcgccaccaatttcagtctgcttaaacaggccggggacgtcgaagagaaccccggacctatgcatcggcgcagatctcggtcttgtagagaagaccaaaagcctgtcatggatgatcaaagagatttaatttctaataatgaacaattacccatgttgggacggcgccccggagcccccgaatctaagtgcagccggggagctttatatacaggattttctattttagtgaccttattattagctggccaagccacaacagcttatttcttataccaacaacaaggacggttagataaattaacagtcacatctcaaaatttacaattagagaatttaagaatgaaattacctaaaccacccaaacccgtcagtaaaatgagaatggctacccccttattaatgcaagccctccccatgggcgccttaccccaaggacccatgcaaaatgctacaaagtatggaaatatgacagaagatcatgtcatgcacttattacaaaacgctgaccccttaaaagtctatccccctttaaaaggatctttccctgaaaatttaagacatttaaaaaatacaatggagacaattgattggaaagtctttgaatcttggatgcatcattggttattatttgaaatgtctaggcattctttagagcaaaaacccaccgatgctccacccaaggaaagtttagagttagaggacccttctagcggattaggagtcaccaaacaggacttaggacccgtccccatgatgcaccagaaacggacagccatgttccaggatcctcaagagcggccacggaagctgcctcagctgtgtacagaactgcagaccaccatccacgacatcatcctcgagtgcgtgtactgcaagcagcagctcctgcggagagaagtgtacgacttcgccttccgggatctgtgcatcgtgtacagagatggcaacccctacgccgtgtgcgacaagtgcctgaagttctactccaagatcagcgagtaccggcactactgctactccctgtacggcaccacacttgagcagcagtacaacaagcccctgtgcgatctgctgatccggtgcatcaactgccagaaacctcagtgccccgaggaaaagcagagacacctggacaagaagcagcggttccacaacattagaggcagatggacaggccggtgcatgagctgctgtagaagcagcagaacaagacggggctccatgcacggcgataccccaacactgcacgagtacatgctggatctgcagcccgagacaaccgatctgtacggctatgagcagctgaatgactccagcgaggaagaggacgagatcgacggacctgctggacaggctgaacctgatagagcccactacaatatcgtgaccttctgctgcaagtgcgatagcaccctgagaagatgcgtgcagagcacccacgtggacatcaggaccctcgaggatctgctcatgggcaccctgggaattgtggccccaatctgctctcagaagccttgagcggccgcggaagaatgtgcacagtgctaaccagaaaattcaggacaagactagtgactctagatcataatcagccataccacatttgtagaggttttacttgctttaaaaaacctcccacacctccccctgaacctgaaacataaaatgaatgcaattgttgttgttaacttgtttattgcagcttataatggttacaaataaagcaatagcatcacaaatttcacaaataaagcatttttttcactgc

SEQ ID NO: 62 - DNA, 4397 bp, Artificial Sequence
  HPV16 E1E2E6E7 as carried by Adenoviral vector
gtgatgcggttttggcagtacatcaatgggcgtggatagcggtttgactcacggggatttccaagtctccaccccattgacgtcaatgggagtttgttttggaaccaaaatcaacgggactttccaaaatgtcgtaacaactccgccccattgacgcaaatgggcggtaggcgtgtacggtgggaggtctatataagcagagctctccctatcagtgatagagatctccctatcagtgatagagatcgtcgacgagctcgtttagtgaaccgtcagatcgcctggagacgccatccacgctgttttgacctctagcaccggtgccaccatggccgatcctgctggcacaaacggcgaagaaggcacaggctgcaacggctggttttacgtggaagccgtggtggaaaagaaaaccggcgacgccatcagcgacgacgagaacgagaatgacagcgacaccggcgaggacctggtggacttcatcgtgaacgacaacgactacctgacacaggccgagacagagacagcccacgctctgtttacagcccaagaggccaagcagcacagagatgccgttcaggtgctgaagagaaagtacctgggcagccctctgagcgacatcagcggctgtgtggacaacaacatcagccccagactgaaggccatctgcatcgagaagcagagcagagccgccaagcggagactgtttgagagcgaggatagcggctacggcaataccgaggtggaaacccagcaaatgctgcaggtcgagggcagacacgaaaccgagacaccttgcagccagtacagcggaggatctggcggaggctgtagccagtactcttctggaagtggcggagagggcgtgtccgagagacacaccatttgtcagacccctctgaccaacatcctgaacgtgctgaaaaccagcaacgccaaggccgccatgctggccaagttcaaagagctgtacggcgtcagcttcagcgaactcgtgcggcccttcaagagcaacaagtccacctgttgcgactggtgcattgccgcctttggcctgacaccttctatcgccgacagcatcaagaccctgctccagcagtactgtctgtacctgcacattcagagcctggcctgctcttggggaatggtggtgctgctgctcgtgcggtacaagtgcggcaagaacagagagacaattgagaagctgctgagcaaactgctgtgcgtgtcccctatgtgcatgatgatcgagcctccaaagctgcggtctacagccgccgctctgtactggtacaagaccggcatcagcaatatctccgaggtgtacggcgacacccctgagtggattcagagacagaccgtcctgcagcacagcttcaacgactgcaccttcgagctgtcccagatggtgcagtgggcctacgacaatgacatcgtggacgactccgagatcgcctataagtacgcccagctggccgacaccaacagcaatgccagcgccttcctgaagtccaacagccaggccaagatcgtgaaggactgcgccaccatgtgcagacactacaagcgggccgagaagaaacagatgagcatgagccagtggatcaagtacagatgcgacagagtggacgacggcggcgattggaagcagatcgtgatgttcctgagataccagggcgtcgagttcatgagctttctgacagccctgaagcggttcctgcagggcatccccaagaagaactgcatcctgctgtatggcgccgctaacaccggcaagagcctgttcggaatgagcctgatgaagtttctgcagggctccgtgatctgctttgtgaacagcaagagccacttctggctccagccactggccgatgccaagattggcatgctggacgatgccaccgtgccttgctggaactacatcgacgacaacctgagaaacgccctggacggcaacctggtttctatggacgtgaagcacagacccctggtgcagctgaagtgtcctccactgctgatcaccagcaacatcaacgccggcaccgattccagatggccctatctgcacaaccggctggtggtgtttacctttcctaacgagttccccttcgacgaaaacggcaaccccgtgtacgagctgaacgataagaattggaagtccttcttcagccggacctggtccagactgagcctgcacgaggatgaggacaaagagaacgacggcgacagcctgcctaccttcaaatgtgtcagcggccagaacaccaacacactgggcagcatggaaacactgtgccagcggctgaacgtgtgccaggacaagattctgacccactatgagaacgacagcaccgacctgagggaccacatcgactactggaagcacatgcggctggaatgcgccatctactacaaggctagagagatgggcttcaagcacatcaaccaccaggtggtgcctacactggccgtgtctaagaacaaggctctgcaggccatcgaactgcagctgaccctggaaacaatctacaactcccagtactccaacgagaagtggaccctccaggacgtgtcactggaagtgtacctgaccgctcctaccggctgcatcaagaaacacggctacaccgtggaagtgcagtttgacggcgatatctgcaataccatgcactacaccaactggacccacatctacatctgcgaagaggccagcgtgacagtggtggaaggccaggtcgactactacggcctgtactacgtgcacgagggcatcagaacctacttcgtgcagttcaaggatgacgccgagaagtacagcaagaacaaagtgtgggaagtgcacgctggcggccaagtgatcctgtgtcctacaagcgtgttcagcagcaacgaagtgtctagccccgagatcatcagacagcacctggccaatcatcctgccgccacacacacaaaagctgtggccctgggcaccgaggaaacacagaccacaattcagaggcccagaagcgagcccgataccggcaatccttgtcacaccaccaagctgctgcaccgggattccgtggattctgcccctatcctgaccgccttcaacagctcccacaaaggccggatcaactgcaacagcaacaccacacctatcgtgcacctgaaaggggacgccaacactctgaaggccctgcggtacagattcaagaagcactgtaccctgtataccgccgtgtccagcacatggcactggaccggacacaacgtgaaacacaagagcgccatcgtgaccctgacctacgatagcgagtggcagagggaccagttcctgagccaagtgaagatccctaagaccatcaccgtgtccaccggctttatgagcattggcagcatgcaccagaaacggacagccatgttccaggatcctcaagagcggccacggaagctgcctcagctgtgtacagaactgcagaccaccatccacgacatcatcctcgagtgcgtgtactgcaagcagcagctcctgcggagagaagtgtacgacttcgccttccgggatctgtgcatcgtgtacagagatggcaacccctacgccgtgtgcgacaagtgcctgaagttctactccaagatcagcgagtaccggcactactgctactccctgtacggcaccacacttgagcagcagtacaacaagcccctgtgcgatctgctgatccggtgcatcaactgccagaaacctcagtgccccgaggaaaagcagagacacctggacaagaagcagcggttccacaacattagaggcagatggacaggccggtgcatgagctgctgtagaagcagcagaacaagacggggctccatgcacggcgataccccaacactgcacgagtacatgctggatctgcagcccgagacaaccgatctgtacggctatgagcagctgaatgactccagcgaggaagaggacgagatcgacggacctgctggacaggctgaacctgatagagcccactacaatatcgtgaccttctgctgcaagtgcgatagcaccctgagaagatgcgtgcagagcacccacgtggacatcaggaccctcgaggatctgctcatgggcaccctgggaattgtggccccaatctgctctcagaagccttgagcggccgcggaagaatgtgcacagtgctaaccagaaaattcaggacaagactagtgactctagatcataatcagccataccacatttgtagaggttttacttgctttaaaaaacctcccacacctccccctgaacctgaaacataaaatgaatgcaattgttgttgttaacttgtttattgcagcttataatggttacaaataaagcaatagcatcacaaatttcacaaataaagcatttttttcactgc

SEQ ID NO: 63 - DNA, 5849 bp, Artificial Sequence
  HPV16 Ii-E1E6E7-p2a-Ii-E2 as carried by Adenoviral vector
gtgatgcggttttggcagtacatcaatgggcgtggatagcggtttgactcacggggatttccaagtctccaccccattgacgtcaatgggagtttgttttggaaccaaaatcaacgggactttccaaaatgtcgtaacaactccgccccattgacgcaaatgggcggtaggcgtgtacggtgggaggtctatataagcagagctctccctatcagtgatagagatctccctatcagtgatagagatcgtcgacgagctcgtttagtgaaccgtcagatcgcctggagacgccatccacgctgttttgacctctagcaccggtgccaccatgcacagaaggcggagcagaagctgccgcgaggatcagaaacccgtgatggacgaccagcgggacctgatcagcaacaacgagcagctgcctatgctcggcagaaggcctggcgctcctgagagcaaatgttctagaggcgccctgtacaccggcttcagcatcctggttacactgctgctggccggacaggctaccaccgcctactttctgtatcagcagcagggcagactggacaagctgaccgtgaccagccagaacctgcagctggaaaacctgcggatgaagctgcccaagcctcctaagcctgtgtccaagatgcggatggccacacctctgctgatgcaggctttgcctatgggagcactgcctcagggccctatgcagaacgccaccaaatacggcaacatgaccgaggaccacgtgatgcatctgctgcagaatgccgatcctctgaaggtgtaccctccactgaagggcagctttcccgagaacctgcggcacctgaagaacaccatggaaaccatcgactggaaggtgttcgagagctggatgcaccactggctgctgttcgagatgagccggcacagcctggaacagaagcctacagacgcccctcctaaagagtccctggaactggaagatcccagctctggcctgggcgtgacaaagcaagatctgggccctgtgcctatgatggccgatcctgctggcacaaacggcgaagaaggcacaggctgcaacggctggttttacgtggaagccgtggtggaaaagaaaaccggcgacgccatcagcgacgacgagaacgagaatgacagcgacaccggcgaggacctggtggacttcatcgtgaacgacaacgactacctgacacaggccgagacagagacagcccacgctctgtttacagcccaagaggccaagcagcacagagatgccgttcaggtgctgaagagaaagtacctgggcagccctctgagcgacatcagcggctgtgtggacaacaacatcagccccagactgaaggccatctgcatcgagaagcagagcagagccgccaagcggagactgtttgagagcgaggatagcggctacggcaataccgaggtggaaacccagcaaatgctgcaggtcgagggcagacacgaaaccgagacaccttgcagccagtacagcggaggatctggcggaggctgtagccagtactcttctggaagtggcggagagggcgtgtccgagagacacaccatttgtcagacccctctgaccaacatcctgaacgtgctgaaaaccagcaacgccaaggccgccatgctggccaagttcaaagagctgtacggcgtcagcttcagcgaactcgtgcggcccttcaagagcaacaagtccacctgttgcgactggtgcattgccgcctttggcctgacaccttctatcgccgacagcatcaagaccctgctccagcagtactgtctgtacctgcacattcagagcctggcctgctcttggggaatggtggtgctgctgctcgtgcggtacaagtgcggcaagaacagagagacaattgagaagctgctgagcaaactgctgtgcgtgtcccctatgtgcatgatgatcgagcctccaaagctgcggtctacagccgccgctctgtactggtacaagaccggcatcagcaatatctccgaggtgtacggcgacacccctgagtggattcagagacagaccgtcctgcagcacagcttcaacgactgcaccttcgagctgtcccagatggtgcagtgggcctacgacaatgacatcgtggacgactccgagatcgcctataagtacgcccagctggccgacaccaacagcaatgccagcgccttcctgaagtccaacagccaggccaagatcgtgaaggactgcgccaccatgtgcagacactacaagcgggccgagaagaaacagatgagcatgagccagtggatcaagtacagatgcgacagagtggacgacggcggcgattggaagcagatcgtgatgttcctgagataccagggcgtcgagttcatgagctttctgacagccctgaagcggttcctgcagggcatccccaagaagaactgcatcctgctgtatggcgccgctaacaccggcaagagcctgttcggaatgagcctgatgaagtttctgcagggctccgtgatctgctttgtgaacagcaagagccacttctggctccagccactggccgatgccaagattggcatgctggacgatgccaccgtgccttgctggaactacatcgacgacaacctgagaaacgccctggacggcaacctggtttctatggacgtgaagcacagacccctggtgcagctgaagtgtcctccactgctgatcaccagcaacatcaacgccggcaccgattccagatggccctatctgcacaaccggctggtggtgtttacctttcctaacgagttccccttcgacgaaaacggcaaccccgtgtacgagctgaacgataagaattggaagtccttcttcagccggacctggtccagactgagcctgcacgaggatgaggacaaagagaacgacggcgacagcctgcctaccttcaaatgtgtcagcggccagaacaccaacacactgggcagcatgcaccagaaacggacagccatgttccaggatcctcaagagcggccacggaagctgcctcagctgtgtacagaactgcagaccaccatccacgacatcatcctcgagtgcgtgtactgcaagcagcagctcctgcggagagaagtgtacgacttcgccttccgggatctgtgcatcgtgtacagagatggcaacccctacgccgtgtgcgacaagtgcctgaagttctactccaagatcagcgagtaccggcactactgctactccctgtacggcaccacacttgagcagcagtacaacaagcccctgtgcgatctgctgatccggtgcatcaactgccagaaacctcagtgccccgaggaaaagcagagacacctggacaagaagcagcggttccacaacattagaggcagatggacaggccggtgcatgagctgctgtagaagcagcagaacaagacggggctccatgcacggcgataccccaacactgcacgagtacatgctggatctgcagcccgagacaaccgatctgtacggctatgagcagctgaatgactccagcgaggaagaggacgagatcgacggacctgctggacaggctgaacctgatagagcccactacaatatcgtgaccttctgctgcaagtgcgatagcaccctgagaagatgcgtgcagagcacccacgtggacatcaggaccctcgaggatctgctcatgggcaccctgggaattgtggccccaatctgctctcagaagcctggcagcggcgccaccaatttcagtctgcttaaacaggccggggacgtcgaagagaaccccggacctatgcatcggcgcagatctcggtcttgtagagaagaccaaaagcctgtcatggatgatcaaagagatttaatttctaataatgaacaattacccatgttgggacggcgccccggagcccccgaatctaagtgcagccggggagctttatatacaggattttctattttagtgaccttattattagctggccaagccacaacagcttatttcttataccaacaacaaggacggttagataaattaacagtcacatctcaaaatttacaattagagaatttaagaatgaaattacctaaaccacccaaacccgtcagtaaaatgagaatggctacccccttattaatgcaagccctccccatgggcgccttaccccaaggacccatgcaaaatgctacaaagtatggaaatatgacagaagatcatgtcatgcacttattacaaaacgctgaccccttaaaagtctatccccctttaaaaggatctttccctgaaaatttaagacatttaaaaaatacaatggagacaattgattggaaagtctttgaatcttggatgcatcattggttattatttgaaatgtctaggcattctttagagcaaaaacccaccgatgctccacccaaggaaagtttagagttagaggacccttctagcggattaggagtcaccaaacaggacttaggacccgtccccatgatggaaacactgtgccagcggctgaacgtgtgccaggacaagattctgacccactatgagaacgacagcaccgacctgagggaccacatcgactactggaagcacatgcggctggaatgcgccatctactacaaggctagagagatgggcttcaagcacatcaaccaccaggtggtgcctacactggccgtgtctaagaacaaggctctgcaggccatcgaactgcagctgaccctggaaacaatctacaactcccagtactccaacgagaagtggaccctccaggacgtgtcactggaagtgtacctgaccgctcctaccggctgcatcaagaaacacggctacaccgtggaagtgcagtttgacggcgatatctgcaataccatgcactacaccaactggacccacatctacatctgcgaagaggccagcgtgacagtggtggaaggccaggtcgactactacggcctgtactacgtgcacgagggcatcagaacctacttcgtgcagttcaaggatgacgccgagaagtacagcaagaacaaagtgtgggaagtgcacgctggcggccaagtgatcctgtgtcctacaagcgtgttcagcagcaacgaagtgtctagccccgagatcatcagacagcacctggccaatcatcctgccgccacacacacaaaagctgtggccctgggcaccgaggaaacacagaccacaattcagaggcccagaagcgagcccgataccggcaatccttgtcacaccaccaagctgctgcaccgggattccgtggattctgcccctatcctgaccgccttcaacagctcccacaaaggccggatcaactgcaacagcaacaccacacctatcgtgcacctgaaaggggacgccaacactctgaaggccctgcggtacagattcaagaagcactgtaccctgtataccgccgtgtccagcacatggcactggaccggacacaacgtgaaacacaagagcgccatcgtgaccctgacctacgatagcgagtggcagagggaccagttcctgagccaagtgaagatccctaagaccatcaccgtgtccaccggctttatgagcatttgagcggccgcggaagaatgtgcacagtgctaaccagaaaattcaggacaagactagtgactctagatcataatcagccataccacatttgtagaggttttacttgctttaaaaaacctcccacacctccccctgaacctgaaacataaaatgaatgcaattgttgttgttaacttgtttattgcagcttataatggttacaaataaagcaatagcatcacaaatttcacaaataaagcatttttttcactgc

SEQ ID NO: 64 - DNA, 3992 bp, Artificial Sequence
  HPV16 Ii-E1E6E7 as carried by Adenoviral vector
gtgatgcggttttggcagtacatcaatgggcgtggatagcggtttgactcacggggatttccaagtctccaccccattgacgtcaatgggagtttgttttggaaccaaaatcaacgggactttccaaaatgtcgtaacaactccgccccattgacgcaaatgggcggtaggcgtgtacggtgggaggtctatataagcagagctctccctatcagtgatagagatctccctatcagtgatagagatcgtcgacgagctcgtttagtgaaccgtcagatcgcctggagacgccatccacgctgttttgacctctagcaccggtgccaccatgcacagaaggcggagcagaagctgccgcgaggatcagaaacccgtgatggacgaccagcgggacctgatcagcaacaacgagcagctgcctatgctcggcagaaggcctggcgctcctgagagcaaatgttctagaggcgccctgtacaccggcttcagcatcctggttacactgctgctggccggacaggctaccaccgcctactttctgtatcagcagcagggcagactggacaagctgaccgtgaccagccagaacctgcagctggaaaacctgcggatgaagctgcccaagcctcctaagcctgtgtccaagatgcggatggccacacctctgctgatgcaggctttgcctatgggagcactgcctcagggccctatgcagaacgccaccaaatacggcaacatgaccgaggaccacgtgatgcatctgctgcagaatgccgatcctctgaaggtgtaccctccactgaagggcagctttcccgagaacctgcggcacctgaagaacaccatggaaaccatcgactggaaggtgttcgagagctggatgcaccactggctgctgttcgagatgagccggcacagcctggaacagaagcctacagacgcccctcctaaagagtccctggaactggaagatcccagctctggcctgggcgtgacaaagcaagatctgggccctgtgcctatgatggccgatcctgctggcacaaacggcgaagaaggcacaggctgcaacggctggttttacgtggaagccgtggtggaaaagaaaaccggcgacgccatcagcgacgacgagaacgagaatgacagcgacaccggcgaggacctggtggacttcatcgtgaacgacaacgactacctgacacaggccgagacagagacagcccacgctctgtttacagcccaagaggccaagcagcacagagatgccgttcaggtgctgaagagaaagtacctgggcagccctctgagcgacatcagcggctgtgtggacaacaacatcagccccagactgaaggccatctgcatcgagaagcagagcagagccgccaagcggagactgtttgagagcgaggatagcggctacggcaataccgaggtggaaacccagcaaatgctgcaggtcgagggcagacacgaaaccgagacaccttgcagccagtacagcggaggatctggcggaggctgtagccagtactcttctggaagtggcggagagggcgtgtccgagagacacaccatttgtcagacccctctgaccaacatcctgaacgtgctgaaaaccagcaacgccaaggccgccatgctggccaagttcaaagagctgtacggcgtcagcttcagcgaactcgtgcggcccttcaagagcaacaagtccacctgttgcgactggtgcattgccgcctttggcctgacaccttctatcgccgacagcatcaagaccctgctccagcagtactgtctgtacctgcacattcagagcctggcctgctcttggggaatggtggtgctgctgctcgtgcggtacaagtgcggcaagaacagagagacaattgagaagctgctgagcaaactgctgtgcgtgtcccctatgtgcatgatgatcgagcctccaaagctgcggtctacagccgccgctctgtactggtacaagaccggcatcagcaatatctccgaggtgtacggcgacacccctgagtggattcagagacagaccgtcctgcagcacagcttcaacgactgcaccttcgagctgtcccagatggtgcagtgggcctacgacaatgacatcgtggacgactccgagatcgcctataagtacgcccagctggccgacaccaacagcaatgccagcgccttcctgaagtccaacagccaggccaagatcgtgaaggactgcgccaccatgtgcagacactacaagcgggccgagaagaaacagatgagcatgagccagtggatcaagtacagatgcgacagagtggacgacggcggcgattggaagcagatcgtgatgttcctgagataccagggcgtcgagttcatgagctttctgacagccctgaagcggttcctgcagggcatccccaagaagaactgcatcctgctgtatggcgccgctaacaccggcaagagcctgttcggaatgagcctgatgaagtttctgcagggctccgtgatctgctttgtgaacagcaagagccacttctggctccagccactggccgatgccaagattggcatgctggacgatgccaccgtgccttgctggaactacatcgacgacaacctgagaaacgccctggacggcaacctggtttctatggacgtgaagcacagacccctggtgcagctgaagtgtcctccactgctgatcaccagcaacatcaacgccggcaccgattccagatggccctatctgcacaaccggctggtggtgtttacctttcctaacgagttccccttcgacgaaaacggcaaccccgtgtacgagctgaacgataagaattggaagtccttcttcagccggacctggtccagactgagcctgcacgaggatgaggacaaagagaacgacggcgacagcctgcctaccttcaaatgtgtcagcggccagaacaccaacacactgggcagcatgcaccagaaacggacagccatgttccaggatcctcaagagcggccacggaagctgcctcagctgtgtacagaactgcagaccaccatccacgacatcatcctcgagtgcgtgtactgcaagcagcagctcctgcggagagaagtgtacgacttcgccttccgggatctgtgcatcgtgtacagagatggcaacccctacgccgtgtgcgacaagtgcctgaagttctactccaagatcagcgagtaccggcactactgctactccctgtacggcaccacacttgagcagcagtacaacaagcccctgtgcgatctgctgatccggtgcatcaactgccagaaacctcagtgccccgaggaaaagcagagacacctggacaagaagcagcggttccacaacattagaggcagatggacaggccggtgcatgagctgctgtagaagcagcagaacaagacggggctccatgcacggcgataccccaacactgcacgagtacatgctggatctgcagcccgagacaaccgatctgtacggctatgagcagctgaatgactccagcgaggaagaggacgagatcgacggacctgctggacaggctgaacctgatagagcccactacaatatcgtgaccttctgctgcaagtgcgatagcaccctgagaagatgcgtgcagagcacccacgtggacatcaggaccctcgaggatctgctcatgggcaccctgggaattgtggccccaatctgctctcagaagccttgagcggccgcggaagaatgtgcacagtgctaaccagaaaattcaggacaagactagtgactctagatcataatcagccataccacatttgtagaggttttacttgctttaaaaaacctcccacacctccccctgaacctgaaacataaaatgaatgcaattgttgttgttaacttgtttattgcagcttataatggttacaaataaagcaatagcatcacaaatttcacaaataaagcatttttttcactgc

SEQ ID NO: 65 - DNA, 5138 bp, Artificial Sequence
  HPV18 Ii-E1E2E6E7 as carried by Adenoviral vector
gtgatgcggttttggcagtacatcaatgggcgtggatagcggtttgactcacggggatttccaagtctccaccccattgacgtcaatgggagtttgttttggaaccaaaatcaacgggactttccaaaatgtcgtaacaactccgccccattgacgcaaatgggcggtaggcgtgtacggtgggaggtctatataagcagagctctccctatcagtgatagagatctccctatcagtgatagagatcgtcgacgagctcgtttagtgaaccgtcagatcgcctggagacgccatccacgctgttttgacctctagcaccggtgccaccatgcacagaaggcggagcagaagctgccgcgaggatcagaaacccgtgatggacgaccagcgggacctgatcagcaacaacgagcagctgcctatgctcggcagaaggcctggcgctcctgagagcaaatgttctagaggcgccctgtacaccggcttcagcatcctggttacactgctgctggccggacaggctaccaccgcctactttctgtatcagcagcagggcagactggacaagctgaccgtgaccagccagaacctgcagctggaaaacctgcggatgaagctgcccaagcctcctaagcctgtgtccaagatgcggatggccacacctctgctgatgcaggctttgcctatgggagcactgcctcagggccctatgcagaacgccaccaaatacggcaacatgaccgaggaccacgtgatgcatctgctgcagaatgccgatcctctgaaggtgtaccctccactgaagggcagctttcccgagaacctgcggcacctgaagaacaccatggaaaccatcgactggaaggtgttcgagagctggatgcaccactggctgctgttcgagatgagccggcacagcctggaacagaagcctacagacgcccctcctaaagagtccctggaactggaagatcccagctctggcctgggcgtgacaaagcaagatctgggccctgtgcctatgatggccgatcctgagggaacagatggcgaaggcacaggctgcaacggctggttttacgtgcaagccatcgtggacaagaagaccggcgacgtcatcagcgacgacgaggatgagaatgccaccgacaccggcagcgacatggtggactttatcgatacccagggcacgttctgcgagcaggccgaactggaaacagcccaggcactgtttcacgcccaagaggtgcacaacgatgcccaggtgctgcacgtgctgaagagaaagtttgccggcggaagcaccgagaacagcccactgggagaaagactggaagtggacaccgagctgagccccagactgcaagagatcagcctgaacagcggccagaagaaggccaagcggagactgttcaccatctccgacagcggctacggctgtagcgaagtggaagccacacagatccaagtgaccaccaatggcgagcacggcggcaatgtttgttctggcggatctaccgaggccatcgacaatggcggaaccgagggcaacaatagctccgtggatggcaccagcgacaacagcaacatcgagaacgtgaaccctcagtgcacaatcgcccagctgaaggacctgctgaaagtgaacaacaagcagggcgccatgctggccgtgtttaaggatacctacggcctgagcttcaccgacctcgtgcggaacttcaagagcgacaagaccacctgtaccgactgggtcaccgccatctttggcgtgaacccaacaatcgccgagggcttcaagaccctgatccagcctttcatcctgtacgcccacatccagtgtctggactgcaaatggggcgtgctgattctggccctgctgagatacaagtgcggcaagagcagactgaccgtggccaagggactgagcactctgctgcatgtgcccgagacatgcatgctgattcagcctccaaagctgcggtctagcgtggccgctctgtactggtacagaaccggcatcagcaatatcagcgaagtgatgggcgacacccctgagtggattcagcggctgacaatcatccagcacggcatcgacgactccaacttcgacctgagcgagatggtgcagtgggccttcgataacgagctgaccgacgagtccgacatggcctttgaatacgccctgctggcagacagcaactccaatgccgccgctttcctgaagtccaactgccaggccaagtacctgaaggactgcgccaccatgtgcaagcactaccgcagagcacagaaacggcagatgaacatgagccagtggatccggttccggtgcagcaagatcgatgaaggtggcgactggcggcctatcgtgcagttcctgagataccagcagatcgagttcatcacctttctgggcgccctgaagtcattcctgaagggaacccctaaaaagaactgcctggtgttctgcggccctgccaataccggcaagtcctacttcggcatgagctttatccacttcatccagggcgccgtgatcagcttcgtgaacagcaccagccacttttggctggaacccctgaccgataccaaggtggcaatgctggacgacgccaccaccacctgttggacctacttcgacacctacatgcggaacgccctggacggcaaccccatcagcatcgacagaaagcacaagcccctcatccagctgaaatgccctccaatcctgctgaccacaaacattcaccccgccaaggacaatcggtggccctacctggaaagccggatcaccgtgttcgagttccccaacgcctttccattcgacaagaacggcaatcccgtgtacgagatcaacgacaagaattggaagtgcttcttcgagcggacctggtccagactggatctgcacgaggaagaagaggacgccgacacagagggcaatcccttcggcacctttaagtgtgtggccgggcagaatcacagacccctgggatctatgcagaccccaaaagagacactgagcgagcggctgagcgccctccaggacaagatcatcgaccactacgagaacgacagcaaggacatcgacagccagattcagtactggcagctgatcagatgggagaacgccatcttcttcgccgctagagagcacggaattcagaccctgaaccaccaggtggtgcccgcctacaacatcagcaagagcaaggcccacaaggccattgaactccagatggccctgcaaggactggctcagagcgcctacaagaccgaggattggacactccaggatacctgcgaggaactgtggaacacagagcccacacactgcttcaagaaaggcggccagaccgtgcaggtctacttcgatggcaacaaggataactgcatgacctacgtggcctgggacagcgtgtactacatgacagatgccggcacctgggacaagaccgccacctgtgtttctcaccggggcctgtactacgtgaaagagggctacaacaccttctacatcgagtttaagagcgagtgcgagaagtatggcaacaccggcacatgggaagtgcatttcggcaacaacgtgatcgactgcaacgactccatgtgctccacctccgatgacaccgtgtctgccacacagctggtcaagcagctccagcacaccccatctccatacagctctacagtgtctgtgggcaccgccaagacctatggccaaacaagcgctgccacaagacctggccattgtggactggccgagaagcagcactgtggccctgttaatcctctgctgggagccgccacacctacaggcaacaacaagagaagaaagctgtgcagcggcaacaccacacctatcattcacctgaagggcgacagaaacagcctgaagtgcctgcggtacagactgaggaagcacagcgatcactaccgggacatcagctccacctggcactggacaggtgctggcaacgaaaagaccggcatcctgacagtgacctaccacagcgagactcagcggaccaagttcctgaacaccgtggctatccccgacagcgtgcagattctcgtgggctacatgaccatgggcagcatggccagattcgaggaccctaccagacggccctacaagctgcctgatctgtgcaccgaactgaacaccagccttcaggatatcgagatcacctgtgtgtactgcaagaccgtgctcgagctgacagaagtgtttgagttcgccttcaaggacctgttcgtggtgtacagagacagcatccctcacgccgcctgtcacaagtgcatcgacttctacagcagaatcagagagctgcggcactacagcgactccgtgtacggcgataccctggaaaaactgaccaacaccggactgtacaacctgctgatccggtgcctgagatgccagaaacctcagaaccccgccgagaaactgagacatctgaacgagaagcggcggttccacaatatcgccggccactacagaggccagtgccacagctgttgcaaccgggccagacaagaaagactccagcggagaagaggcagcatgcacggacctaaagccacacttcaggacatcgtgctgcacctcgagcctcagaatgagatccccgtggatctgctcggccatgagcagctgagcgatagcgaggaagagaacgacgagatcgacggcgtcaaccaccagcatctgcctgccagaagggccgaacctcagagacacaccatgctgtgcatgtgctgcaagtgcgaggcccggatcgagagagtggtggaatctagcgccgacgacctgagagctttccagcagctgttcctgaatactctgagcttcgtggccccttggtgcgctagtcagcagtgagcggccgcggaagaatgtgcacagtgctaaccagaaaattcaggacaagactagtgactctagatcataatcagccataccacatttgtagaggttttacttgctttaaaaaacctcccacacctccccctgaacctgaaacataaaatgaatgcaattgttgttgttaacttgtttattgcagcttataatggttacaaataaagcaatagcatcacaaatttcacaaataaagcatttttttcactgc

SEQ ID NO: 66 - DNA, 5894 bp, Artificial Sequence
  HPV18 Ii-E1E2-p2a-Ii-E6E7 as carried by Adenoviral vector
gtgatgcggttttggcagtacatcaatgggcgtggatagcggtttgactcacggggatttccaagtctccaccccattgacgtcaatgggagtttgttttggaaccaaaatcaacgggactttccaaaatgtcgtaacaactccgccccattgacgcaaatgggcggtaggcgtgtacggtgggaggtctatataagcagagctctccctatcagtgatagagatctccctatcagtgatagagatcgtcgacgagctcgtttagtgaaccgtcagatcgcctggagacgccatccacgctgttttgacctctagcaccggtgccaccatgcacagaaggcggagcagaagctgccgcgaggatcagaaacccgtgatggacgaccagcgggacctgatcagcaacaacgagcagctgcctatgctcggcagaaggcctggcgctcctgagagcaaatgttctagaggcgccctgtacaccggcttcagcatcctggttacactgctgctggccggacaggctaccaccgcctactttctgtatcagcagcagggcagactggacaagctgaccgtgaccagccagaacctgcagctggaaaacctgcggatgaagctgcccaagcctcctaagcctgtgtccaagatgcggatggccacacctctgctgatgcaggctttgcctatgggagcactgcctcagggccctatgcagaacgccaccaaatacggcaacatgaccgaggaccacgtgatgcatctgctgcagaatgccgatcctctgaaggtgtaccctccactgaagggcagctttcccgagaacctgcggcacctgaagaacaccatggaaaccatcgactggaaggtgttcgagagctggatgcaccactggctgctgttcgagatgagccggcacagcctggaacagaagcctacagacgcccctcctaaagagtccctggaactggaagatcccagctctggcctgggcgtgacaaagcaagatctgggccctgtgcctatgatggccgatcctgagggaacagatggcgaaggcacaggctgcaacggctggttttacgtgcaagccatcgtggacaagaagaccggcgacgtcatcagcgacgacgaggatgagaatgccaccgacaccggcagcgacatggtggactttatcgatacccagggcacgttctgcgagcaggccgaactggaaacagcccaggcactgtttcacgcccaagaggtgcacaacgatgcccaggtgctgcacgtgctgaagagaaagtttgccggcggaagcaccgagaacagcccactgggagaaagactggaagtggacaccgagctgagccccagactgcaagagatcagcctgaacagcggccagaagaaggccaagcggagactgttcaccatctccgacagcggctacggctgtagcgaagtggaagccacacagatccaagtgaccaccaatggcgagcacggcggcaatgtttgttctggcggatctaccgaggccatcgacaatggcggaaccgagggcaacaatagctccgtggatggcaccagcgacaacagcaacatcgagaacgtgaaccctcagtgcacaatcgcccagctgaaggacctgctgaaagtgaacaacaagcagggcgccatgctggccgtgtttaaggatacctacggcctgagcttcaccgacctcgtgcggaacttcaagagcgacaagaccacctgtaccgactgggtcaccgccatctttggcgtgaacccaacaatcgccgagggcttcaagaccctgatccagcctttcatcctgtacgcccacatccagtgtctggactgcaaatggggcgtgctgattctggccctgctgagatacaagtgcggcaagagcagactgaccgtggccaagggactgagcactctgctgcatgtgcccgagacatgcatgctgattcagcctccaaagctgcggtctagcgtggccgctctgtactggtacagaaccggcatcagcaatatcagcgaagtgatgggcgacacccctgagtggattcagcggctgacaatcatccagcacggcatcgacgactccaacttcgacctgagcgagatggtgcagtgggccttcgataacgagctgaccgacgagtccgacatggcctttgaatacgccctgctggcagacagcaactccaatgccgccgctttcctgaagtccaactgccaggccaagtacctgaaggactgcgccaccatgtgcaagcactaccgcagagcacagaaacggcagatgaacatgagccagtggatccggttccggtgcagcaagatcgatgaaggtggcgactggcggcctatcgtgcagttcctgagataccagcagatcgagttcatcacctttctgggcgccctgaagtcattcctgaagggaacccctaaaaagaactgcctggtgttctgcggccctgccaataccggcaagtcctacttcggcatgagctttatccacttcatccagggcgccgtgatcagcttcgtgaacagcaccagccacttttggctggaacccctgaccgataccaaggtggcaatgctggacgacgccaccaccacctgttggacctacttcgacacctacatgcggaacgccctggacggcaaccccatcagcatcgacagaaagcacaagcccctcatccagctgaaatgccctccaatcctgctgaccacaaacattcaccccgccaaggacaatcggtggccctacctggaaagccggatcaccgtgttcgagttccccaacgcctttccattcgacaagaacggcaatcccgtgtacgagatcaacgacaagaattggaagtgcttcttcgagcggacctggtccagactggatctgcacgaggaagaagaggacgccgacacagagggcaatcccttcggcacctttaagtgtgtggccgggcagaatcacagacccctgggatctatgcagaccccaaaagagacactgagcgagcggctgagcgccctccaggacaagatcatcgaccactacgagaacgacagcaaggacatcgacagccagattcagtactggcagctgatcagatgggagaacgccatcttcttcgccgctagagagcacggaattcagaccctgaaccaccaggtggtgcccgcctacaacatcagcaagagcaaggcccacaaggccattgaactccagatggccctgcaaggactggctcagagcgcctacaagaccgaggattggacactccaggatacctgcgaggaactgtggaacacagagcccacacactgcttcaagaaaggcggccagaccgtgcaggtctacttcgatggcaacaaggataactgcatgacctacgtggcctgggacagcgtgtactacatgacagatgccggcacctgggacaagaccgccacctgtgtttctcaccggggcctgtactacgtgaaagagggctacaacaccttctacatcgagtttaagagcgagtgcgagaagtatggcaacaccggcacatgggaagtgcatttcggcaacaacgtgatcgactgcaacgactccatgtgctccacctccgatgacaccgtgtctgccacacagctggtcaagcagctccagcacaccccatctccatacagctctacagtgtctgtgggcaccgccaagacctatggccaaacaagcgctgccacaagacctggccattgtggactggccgagaagcagcactgtggccctgttaatcctctgctgggagccgccacacctacaggcaacaacaagagaagaaagctgtgcagcggcaacaccacacctatcattcacctgaagggcgacagaaacagcctgaagtgcctgcggtacagactgaggaagcacagcgatcactaccgggacatcagctccacctggcactggacaggtgctggcaacgaaaagaccggcatcctgacagtgacctaccacagcgagactcagcggaccaagttcctgaacaccgtggctatccccgacagcgtgcagattctcgtgggctacatgaccatgggcagcggcgccaccaatttcagtctgcttaaacaggccggggacgtcgaagagaaccccggacctatgcatcggcgcagatctcggtcttgtagagaagaccaaaagcctgtcatggatgatcaaagagatttaatttctaataatgaacaattacccatgttgggacggcgccccggagcccccgaatctaagtgcagccggggagctttatatacaggattttctattttagtgaccttattattagctggccaagccacaacagcttatttcttataccaacaacaaggacggttagataaattaacagtcacatctcaaaatttacaattagagaatttaagaatgaaattacctaaaccacccaaacccgtcagtaaaatgagaatggctacccccttattaatgcaagccctccccatgggcgccttaccccaaggacccatgcaaaatgctacaaagtatggaaatatgacagaagatcatgtcatgcacttattacaaaacgctgaccccttaaaagtctatccccctttaaaaggatctttccctgaaaatttaagacatttaaaaaatacaatggagacaattgattggaaagtctttgaatcttggatgcatcattggttattatttgaaatgtctaggcattctttagagcaaaaacccaccgatgctccacccaaggaaagtttagagttagaggacccttctagcggattaggagtcaccaaacaggacttaggacccgtccccatgatggccagattcgaggaccctaccagacggccctacaagctgcctgatctgtgcaccgaactgaacaccagccttcaggatatcgagatcacctgtgtgtactgcaagaccgtgctcgagctgacagaagtgtttgagttcgccttcaaggacctgttcgtggtgtacagagacagcatccctcacgccgcctgtcacaagtgcatcgacttctacagcagaatcagagagctgcggcactacagcgactccgtgtacggcgataccctggaaaaactgaccaacaccggactgtacaacctgctgatccggtgcctgagatgccagaaacctcagaaccccgccgagaaactgagacatctgaacgagaagcggcggttccacaatatcgccggccactacagaggccagtgccacagctgttgcaaccgggccagacaagaaagactccagcggagaagaggcagcatgcacggacctaaagccacacttcaggacatcgtgctgcacctcgagcctcagaatgagatccccgtggatctgctcggccatgagcagctgagcgatagcgaggaagagaacgacgagatcgacggcgtcaaccaccagcatctgcctgccagaagggccgaacctcagagacacaccatgctgtgcatgtgctgcaagtgcgaggcccggatcgagagagtggtggaatctagcgccgacgacctgagagctttccagcagctgttcctgaatactctgagcttcgtggccccttggtgcgctagtcagcagtgagcggccgcggaagaatgtgcacagtgctaaccagaaaattcaggacaagactagtgactctagatcataatcagccataccacatttgtagaggttttacttgctttaaaaaacctcccacacctccccctgaacctgaaacataaaatgaatgcaattgttgttgttaacttgtttattgcagcttataatggttacaaataaagcaatagcatcacaaatttcacaaataaagcatttttttcactgc

SEQ ID NO: 67 - DNA, 4442 bp, Artificial Sequence
  HPV18 E1E2E6E7 as carried by Adenoviral vector
gtgatgcggttttggcagtacatcaatgggcgtggatagcggtttgactcacggggatttccaagtctccaccccattgacgtcaatgggagtttgttttggaaccaaaatcaacgggactttccaaaatgtcgtaacaactccgccccattgacgcaaatgggcggtaggcgtgtacggtgggaggtctatataagcagagctctccctatcagtgatagagatctccctatcagtgatagagatcgtcgacgagctcgtttagtgaaccgtcagatcgcctggagacgccatccacgctgttttgacctctagcaccggtgccaccatggccgatcctgagggaacagatggcgaaggcacaggctgcaacggctggttttacgtgcaagccatcgtggacaagaagaccggcgacgtcatcagcgacgacgaggatgagaatgccaccgacaccggcagcgacatggtggactttatcgatacccagggcacgttctgcgagcaggccgaactggaaacagcccaggcactgtttcacgcccaagaggtgcacaacgatgcccaggtgctgcacgtgctgaagagaaagtttgccggcggaagcaccgagaacagcccactgggagaaagactggaagtggacaccgagctgagccccagactgcaagagatcagcctgaacagcggccagaagaaggccaagcggagactgttcaccatctccgacagcggctacggctgtagcgaagtggaagccacacagatccaagtgaccaccaatggcgagcacggcggcaatgtttgttctggcggatctaccgaggccatcgacaatggcggaaccgagggcaacaatagctccgtggatggcaccagcgacaacagcaacatcgagaacgtgaaccctcagtgcacaatcgcccagctgaaggacctgctgaaagtgaacaacaagcagggcgccatgctggccgtgtttaaggatacctacggcctgagcttcaccgacctcgtgcggaacttcaagagcgacaagaccacctgtaccgactgggtcaccgccatctttggcgtgaacccaacaatcgccgagggcttcaagaccctgatccagcctttcatcctgtacgcccacatccagtgtctggactgcaaatggggcgtgctgattctggccctgctgagatacaagtgcggcaagagcagactgaccgtggccaagggactgagcactctgctgcatgtgcccgagacatgcatgctgattcagcctccaaagctgcggtctagcgtggccgctctgtactggtacagaaccggcatcagcaatatcagcgaagtgatgggcgacacccctgagtggattcagcggctgacaatcatccagcacggcatcgacgactccaacttcgacctgagcgagatggtgcagtgggccttcgataacgagctgaccgacgagtccgacatggcctttgaatacgccctgctggcagacagcaactccaatgccgccgctttcctgaagtccaactgccaggccaagtacctgaaggactgcgccaccatgtgcaagcactaccgcagagcacagaaacggcagatgaacatgagccagtggatccggttccggtgcagcaagatcgatgaaggtggcgactggcggcctatcgtgcagttcctgagataccagcagatcgagttcatcacctttctgggcgccctgaagtcattcctgaagggaacccctaaaaagaactgcctggtgttctgcggccctgccaataccggcaagtcctacttcggcatgagctttatccacttcatccagggcgccgtgatcagcttcgtgaacagcaccagccacttttggctggaacccctgaccgataccaaggtggcaatgctggacgacgccaccaccacctgttggacctacttcgacacctacatgcggaacgccctggacggcaaccccatcagcatcgacagaaagcacaagcccctcatccagctgaaatgccctccaatcctgctgaccacaaacattcaccccgccaaggacaatcggtggccctacctggaaagccggatcaccgtgttcgagttccccaacgcctttccattcgacaagaacggcaatcccgtgtacgagatcaacgacaagaattggaagtgcttcttcgagcggacctggtccagactggatctgcacgaggaagaagaggacgccgacacagagggcaatcccttcggcacctttaagtgtgtggccgggcagaatcacagacccctgggatctatgcagaccccaaaagagacactgagcgagcggctgagcgccctccaggacaagatcatcgaccactacgagaacgacagcaaggacatcgacagccagattcagtactggcagctgatcagatgggagaacgccatcttcttcgccgctagagagcacggaattcagaccctgaaccaccaggtggtgcccgcctacaacatcagcaagagcaaggcccacaaggccattgaactccagatggccctgcaaggactggctcagagcgcctacaagaccgaggattggacactccaggatacctgcgaggaactgtggaacacagagcccacacactgcttcaagaaaggcggccagaccgtgcaggtctacttcgatggcaacaaggataactgcatgacctacgtggcctgggacagcgtgtactacatgacagatgccggcacctgggacaagaccgccacctgtgtttctcaccggggcctgtactacgtgaaagagggctacaacaccttctacatcgagtttaagagcgagtgcgagaagtatggcaacaccggcacatgggaagtgcatttcggcaacaacgtgatcgactgcaacgactccatgtgctccacctccgatgacaccgtgtctgccacacagctggtcaagcagctccagcacaccccatctccatacagctctacagtgtctgtgggcaccgccaagacctatggccaaacaagcgctgccacaagacctggccattgtggactggccgagaagcagcactgtggccctgttaatcctctgctgggagccgccacacctacaggcaacaacaagagaagaaagctgtgcagcggcaacaccacacctatcattcacctgaagggcgacagaaacagcctgaagtgcctgcggtacagactgaggaagcacagcgatcactaccgggacatcagctccacctggcactggacaggtgctggcaacgaaaagaccggcatcctgacagtgacctaccacagcgagactcagcggaccaagttcctgaacaccgtggctatccccgacagcgtgcagattctcgtgggctacatgaccatgggcagcatggccagattcgaggaccctaccagacggccctacaagctgcctgatctgtgcaccgaactgaacaccagccttcaggatatcgagatcacctgtgtgtactgcaagaccgtgctcgagctgacagaagtgtttgagttcgccttcaaggacctgttcgtggtgtacagagacagcatccctcacgccgcctgtcacaagtgcatcgacttctacagcagaatcagagagctgcggcactacagcgactccgtgtacggcgataccctggaaaaactgaccaacaccggactgtacaacctgctgatccggtgcctgagatgccagaaacctcagaaccccgccgagaaactgagacatctgaacgagaagcggcggttccacaatatcgccggccactacagaggccagtgccacagctgttgcaaccgggccagacaagaaagactccagcggagaagaggcagcatgcacggacctaaagccacacttcaggacatcgtgctgcacctcgagcctcagaatgagatccccgtggatctgctcggccatgagcagctgagcgatagcgaggaagagaacgacgagatcgacggcgtcaaccaccagcatctgcctgccagaagggccgaacctcagagacacaccatgctgtgcatgtgctgcaagtgcgaggcccggatcgagagagtggtggaatctagcgccgacgacctgagagctttccagcagctgttcctgaatactctgagcttcgtggccccttggtgcgctagtcagcagtgagcggccgcggaagaatgtgcacagtgctaaccagaaaattcaggacaagactagtgactctagatcataatcagccataccacatttgtagaggttttacttgctttaaaaaacctcccacacctccccctgaacctgaaacataaaatgaatgcaattgttgttgttaacttgtttattgcagcttataatggttacaaataaagcaatagcatcacaaatttcacaaataaagcatttttttcactgc

SEQ ID NO: 68 - DNA, 5894 bp, Artificial Sequence
  HPV18 Ii-E1E6E7-p2a-Ii-E2 as carried by Adenoviral vector
gtgatgcggttttggcagtacatcaatgggcgtggatagcggtttgactcacggggatttccaagtctccaccccattgacgtcaatgggagtttgttttggaaccaaaatcaacgggactttccaaaatgtcgtaacaactccgccccattgacgcaaatgggcggtaggcgtgtacggtgggaggtctatataagcagagctctccctatcagtgatagagatctccctatcagtgatagagatcgtcgacgagctcgtttagtgaaccgtcagatcgcctggagacgccatccacgctgttttgacctctagcaccggtgccaccatgcacagaaggcggagcagaagctgccgcgaggatcagaaacccgtgatggacgaccagcgggacctgatcagcaacaacgagcagctgcctatgctcggcagaaggcctggcgctcctgagagcaaatgttctagaggcgccctgtacaccggcttcagcatcctggttacactgctgctggccggacaggctaccaccgcctactttctgtatcagcagcagggcagactggacaagctgaccgtgaccagccagaacctgcagctggaaaacctgcggatgaagctgcccaagcctcctaagcctgtgtccaagatgcggatggccacacctctgctgatgcaggctttgcctatgggagcactgcctcagggccctatgcagaacgccaccaaatacggcaacatgaccgaggaccacgtgatgcatctgctgcagaatgccgatcctctgaaggtgtaccctccactgaagggcagctttcccgagaacctgcggcacctgaagaacaccatggaaaccatcgactggaaggtgttcgagagctggatgcaccactggctgctgttcgagatgagccggcacagcctggaacagaagcctacagacgcccctcctaaagagtccctggaactggaagatcccagctctggcctgggcgtgacaaagcaagatctgggccctgtgcctatgatggccgatcctgagggaacagatggcgaaggcacaggctgcaacggctggttttacgtgcaagccatcgtggacaagaagaccggcgacgtcatcagcgacgacgaggatgagaatgccaccgacaccggcagcgacatggtggactttatcgatacccagggcacgttctgcgagcaggccgaactggaaacagcccaggcactgtttcacgcccaagaggtgcacaacgatgcccaggtgctgcacgtgctgaagagaaagtttgccggcggaagcaccgagaacagcccactgggagaaagactggaagtggacaccgagctgagccccagactgcaagagatcagcctgaacagcggccagaagaaggccaagcggagactgttcaccatctccgacagcggctacggctgtagcgaagtggaagccacacagatccaagtgaccaccaatggcgagcacggcggcaatgtttgttctggcggatctaccgaggccatcgacaatggcggaaccgagggcaacaatagctccgtggatggcaccagcgacaacagcaacatcgagaacgtgaaccctcagtgcacaatcgcccagctgaaggacctgctgaaagtgaacaacaagcagggcgccatgctggccgtgtttaaggatacctacggcctgagcttcaccgacctcgtgcggaacttcaagagcgacaagaccacctgtaccgactgggtcaccgccatctttggcgtgaacccaacaatcgccgagggcttcaagaccctgatccagcctttcatcctgtacgcccacatccagtgtctggactgcaaatggggcgtgctgattctggccctgctgagatacaagtgcggcaagagcagactgaccgtggccaagggactgagcactctgctgcatgtgcccgagacatgcatgctgattcagcctccaaagctgcggtctagcgtggccgctctgtactggtacagaaccggcatcagcaatatcagcgaagtgatgggcgacacccctgagtggattcagcggctgacaatcatccagcacggcatcgacgactccaacttcgacctgagcgagatggtgcagtgggccttcgataacgagctgaccgacgagtccgacatggcctttgaatacgccctgctggcagacagcaactccaatgccgccgctttcctgaagtccaactgccaggccaagtacctgaaggactgcgccaccatgtgcaagcactaccgcagagcacagaaacggcagatgaacatgagccagtggatccggttccggtgcagcaagatcgatgaaggtggcgactggcggcctatcgtgcagttcctgagataccagcagatcgagttcatcacctttctgggcgccctgaagtcattcctgaagggaacccctaaaaagaactgcctggtgttctgcggccctgccaataccggcaagtcctacttcggcatgagctttatccacttcatccagggcgccgtgatcagcttcgtgaacagcaccagccacttttggctggaacccctgaccgataccaaggtggcaatgctggacgacgccaccaccacctgttggacctacttcgacacctacatgcggaacgccctggacggcaaccccatcagcatcgacagaaagcacaagcccctcatccagctgaaatgccctccaatcctgctgaccacaaacattcaccccgccaaggacaatcggtggccctacctggaaagccggatcaccgtgttcgagttccccaacgcctttccattcgacaagaacggcaatcccgtgtacgagatcaacgacaagaattggaagtgcttcttcgagcggacctggtccagactggatctgcacgaggaagaagaggacgccgacacagagggcaatcccttcggcacctttaagtgtgtggccgggcagaatcacagacccctgggcagcatggccagattcgaggaccctaccagacggccctacaagctgcctgatctgtgcaccgaactgaacaccagccttcaggatatcgagatcacctgtgtgtactgcaagaccgtgctcgagctgacagaagtgtttgagttcgccttcaaggacctgttcgtggtgtacagagacagcatccctcacgccgcctgtcacaagtgcatcgacttctacagcagaatcagagagctgcggcactacagcgactccgtgtacggcgataccctggaaaaactgaccaacaccggactgtacaacctgctgatccggtgcctgagatgccagaaacctcagaaccccgccgagaaactgagacatctgaacgagaagcggcggttccacaatatcgccggccactacagaggccagtgccacagctgttgcaaccgggccagacaagaaagactccagcggagaagaggcagcatgcacggacctaaagccacacttcaggacatcgtgctgcacctcgagcctcagaatgagatccccgtggatctgctcggccatgagcagctgagcgatagcgaggaagagaacgacgagatcgacggcgtcaaccaccagcatctgcctgccagaagggccgaacctcagagacacaccatgctgtgcatgtgctgcaagtgcgaggcccggatcgagagagtggtggaatctagcgccgacgacctgagagctttccagcagctgttcctgaatactctgagcttcgtggccccttggtgcgctagtcagcagggcagcggcgccaccaatttcagtctgcttaaacaggccggggacgtcgaagagaaccccggacctatgcatcggcgcagatctcggtcttgtagagaagaccaaaagcctgtcatggatgatcaaagagatttaatttctaataatgaacaattacccatgttgggacggcgccccggagcccccgaatctaagtgcagccggggagctttatatacaggattttctattttagtgaccttattattagctggccaagccacaacagcttatttcttataccaacaacaaggacggttagataaattaacagtcacatctcaaaatttacaattagagaatttaagaatgaaattacctaaaccacccaaacccgtcagtaaaatgagaatggctacccccttattaatgcaagccctccccatgggcgccttaccccaaggacccatgcaaaatgctacaaagtatggaaatatgacagaagatcatgtcatgcacttattacaaaacgctgaccccttaaaagtctatccccctttaaaaggatctttccctgaaaatttaagacatttaaaaaatacaatggagacaattgattggaaagtctttgaatcttggatgcatcattggttattatttgaaatgtctaggcattctttagagcaaaaacccaccgatgctccacccaaggaaagtttagagttagaggacccttctagcggattaggagtcaccaaacaggacttaggacccgtccccatgatgcagaccccaaaagagacactgagcgagcggctgagcgccctccaggacaagatcatcgaccactacgagaacgacagcaaggacatcgacagccagattcagtactggcagctgatcagatgggagaacgccatcttcttcgccgctagagagcacggaattcagaccctgaaccaccaggtggtgcccgcctacaacatcagcaagagcaaggcccacaaggccattgaactccagatggccctgcaaggactggctcagagcgcctacaagaccgaggattggacactccaggatacctgcgaggaactgtggaacacagagcccacacactgcttcaagaaaggcggccagaccgtgcaggtctacttcgatggcaacaaggataactgcatgacctacgtggcctgggacagcgtgtactacatgacagatgccggcacctgggacaagaccgccacctgtgtttctcaccggggcctgtactacgtgaaagagggctacaacaccttctacatcgagtttaagagcgagtgcgagaagtatggcaacaccggcacatgggaagtgcatttcggcaacaacgtgatcgactgcaacgactccatgtgctccacctccgatgacaccgtgtctgccacacagctggtcaagcagctccagcacaccccatctccatacagctctacagtgtctgtgggcaccgccaagacctatggccaaacaagcgctgccacaagacctggccattgtggactggccgagaagcagcactgtggccctgttaatcctctgctgggagccgccacacctacaggcaacaacaagagaagaaagctgtgcagcggcaacaccacacctatcattcacctgaagggcgacagaaacagcctgaagtgcctgcggtacagactgaggaagcacagcgatcactaccgggacatcagctccacctggcactggacaggtgctggcaacgaaaagaccggcatcctgacagtgacctaccacagcgagactcagcggaccaagttcctgaacaccgtggctatccccgacagcgtgcagattctcgtgggctacatgaccatgtgagcggccgcggaagaatgtgcacagtgctaaccagaaaattcaggacaagactagtgactctagatcataatcagccataccacatttgtagaggttttacttgctttaaaaaacctcccacacctccccctgaacctgaaacataaaatgaatgcaattgttgttgttaacttgtttattgcagcttataatggttacaaataaagcaatagcatcacaaatttcacaaataaagcatttttttcactgc

SEQ ID NO: 69 - DNA, 4037 bp, Artificial Sequence
  HPV18 Ii-E1E6E7 as carried by Adenoviral vector
gtgatgcggttttggcagtacatcaatgggcgtggatagcggtttgactcacggggatttccaagtctccaccccattgacgtcaatgggagtttgttttggaaccaaaatcaacgggactttccaaaatgtcgtaacaactccgccccattgacgcaaatgggcggtaggcgtgtacggtgggaggtctatataagcagagctctccctatcagtgatagagatctccctatcagtgatagagatcgtcgacgagctcgtttagtgaaccgtcagatcgcctggagacgccatccacgctgttttgacctctagcaccggtgccaccatgcacagaaggcggagcagaagctgccgcgaggatcagaaacccgtgatggacgaccagcgggacctgatcagcaacaacgagcagctgcctatgctcggcagaaggcctggcgctcctgagagcaaatgttctagaggcgccctgtacaccggcttcagcatcctggttacactgctgctggccggacaggctaccaccgcctactttctgtatcagcagcagggcagactggacaagctgaccgtgaccagccagaacctgcagctggaaaacctgcggatgaagctgcccaagcctcctaagcctgtgtccaagatgcggatggccacacctctgctgatgcaggctttgcctatgggagcactgcctcagggccctatgcagaacgccaccaaatacggcaacatgaccgaggaccacgtgatgcatctgctgcagaatgccgatcctctgaaggtgtaccctccactgaagggcagctttcccgagaacctgcggcacctgaagaacaccatggaaaccatcgactggaaggtgttcgagagctggatgcaccactggctgctgttcgagatgagccggcacagcctggaacagaagcctacagacgcccctcctaaagagtccctggaactggaagatcccagctctggcctgggcgtgacaaagcaagatctgggccctgtgcctatgatggccgatcctgagggaacagatggcgaaggcacaggctgcaacggctggttttacgtgcaagccatcgtggacaagaagaccggcgacgtcatcagcgacgacgaggatgagaatgccaccgacaccggcagcgacatggtggactttatcgatacccagggcacgttctgcgagcaggccgaactggaaacagcccaggcactgtttcacgcccaagaggtgcacaacgatgcccaggtgctgcacgtgctgaagagaaagtttgccggcggaagcaccgagaacagcccactgggagaaagactggaagtggacaccgagctgagccccagactgcaagagatcagcctgaacagcggccagaagaaggccaagcggagactgttcaccatctccgacagcggctacggctgtagcgaagtggaagccacacagatccaagtgaccaccaatggcgagcacggcggcaatgtttgttctggcggatctaccgaggccatcgacaatggcggaaccgagggcaacaatagctccgtggatggcaccagcgacaacagcaacatcgagaacgtgaaccctcagtgcacaatcgcccagctgaaggacctgctgaaagtgaacaacaagcagggcgccatgctggccgtgtttaaggatacctacggcctgagcttcaccgacctcgtgcggaacttcaagagcgacaagaccacctgtaccgactgggtcaccgccatctttggcgtgaacccaacaatcgccgagggcttcaagaccctgatccagcctttcatcctgtacgcccacatccagtgtctggactgcaaatggggcgtgctgattctggccctgctgagatacaagtgcggcaagagcagactgaccgtggccaagggactgagcactctgctgcatgtgcccgagacatgcatgctgattcagcctccaaagctgcggtctagcgtggccgctctgtactggtacagaaccggcatcagcaatatcagcgaagtgatgggcgacacccctgagtggattcagcggctgacaatcatccagcacggcatcgacgactccaacttcgacctgagcgagatggtgcagtgggccttcgataacgagctgaccgacgagtccgacatggcctttgaatacgccctgctggcagacagcaactccaatgccgccgctttcctgaagtccaactgccaggccaagtacctgaaggactgcgccaccatgtgcaagcactaccgcagagcacagaaacggcagatgaacatgagccagtggatccggttccggtgcagcaagatcgatgaaggtggcgactggcggcctatcgtgcagttcctgagataccagcagatcgagttcatcacctttctgggcgccctgaagtcattcctgaagggaacccctaaaaagaactgcctggtgttctgcggccctgccaataccggcaagtcctacttcggcatgagctttatccacttcatccagggcgccgtgatcagcttcgtgaacagcaccagccacttttggctggaacccctgaccgataccaaggtggcaatgctggacgacgccaccaccacctgttggacctacttcgacacctacatgcggaacgccctggacggcaaccccatcagcatcgacagaaagcacaagcccctcatccagctgaaatgccctccaatcctgctgaccacaaacattcaccccgccaaggacaatcggtggccctacctggaaagccggatcaccgtgttcgagttccccaacgcctttccattcgacaagaacggcaatcccgtgtacgagatcaacgacaagaattggaagtgcttcttcgagcggacctggtccagactggatctgcacgaggaagaagaggacgccgacacagagggcaatcccttcggcacctttaagtgtgtggccgggcagaatcacagacccctgggcagcatggccagattcgaggaccctaccagacggccctacaagctgcctgatctgtgcaccgaactgaacaccagccttcaggatatcgagatcacctgtgtgtactgcaagaccgtgctcgagctgacagaagtgtttgagttcgccttcaaggacctgttcgtggtgtacagagacagcatccctcacgccgcctgtcacaagtgcatcgacttctacagcagaatcagagagctgcggcactacagcgactccgtgtacggcgataccctggaaaaactgaccaacaccggactgtacaacctgctgatccggtgcctgagatgccagaaacctcagaaccccgccgagaaactgagacatctgaacgagaagcggcggttccacaatatcgccggccactacagaggccagtgccacagctgttgcaaccgggccagacaagaaagactccagcggagaagaggcagcatgcacggacctaaagccacacttcaggacatcgtgctgcacctcgagcctcagaatgagatccccgtggatctgctcggccatgagcagctgagcgatagcgaggaagagaacgacgagatcgacggcgtcaaccaccagcatctgcctgccagaagggccgaacctcagagacacaccatgctgtgcatgtgctgcaagtgcgaggcccggatcgagagagtggtggaatctagcgccgacgacctgagagctttccagcagctgttcctgaatactctgagcttcgtggccccttggtgcgctagtcagcagtgagcggccgcggaagaatgtgcacagtgctaaccagaaaattcaggacaagactagtgactctagatcataatcagccataccacatttgtagaggttttacttgctttaaaaaacctcccacacctccccctgaacctgaaacataaaatgaatgcaattgttgttgttaacttgtttattgcagcttataatggttacaaataaagcaatagcatcacaaatttcacaaataaagcatttttttcactgc

SEQ ID NO: 70 - DNA, 4748 bp, Artificial Sequence
  MfPV3 Ii-E1E2E6E7 integrated into DelIII locus of the poxviral vector
aaaaattaaaattttattttttttttttggaatataaataagatctatccctatcagtgatagagatctccctatcagtgatagagatcgtcgacgagctcgtttagtgaaccgtcagatcgcctggagacgccatccacgctgttttgacctctagcaccggtgccaccatgcacagaaggcggagcagaagctgccgcgaggatcagaaacccgtgatggacgaccagcgggacctgatcagcaacaacgagcagctgcctatgctcggcagaaggcctggcgctcctgagagcaaatgttctagaggcgccctgtacaccggcttcagcatcctggttacactgctgctggccggacaggctaccaccgcctactttctgtatcagcagcagggcagactggacaagctgaccgtgaccagccagaacctgcagctggaaaacctgcggatgaagctgcccaagcctcctaagcctgtgtccaagatgcggatggccacacctctgctgatgcaggctttgcctatgggagcactgcctcagggccctatgcagaacgccaccaaatacggcaacatgaccgaggaccacgtgatgcatctgctgcagaatgccgatcctctgaaggtgtaccctccactgaagggcagctttcccgagaacctgcggcacctgaagaacaccatggaaaccatcgactggaaggtgttcgagagctggatgcaccactggctgctgttcgagatgagccggcacagcctggaacagaagcctacagacgcccctcctaaagagtccctggaactggaagatcccagctctggcctgggcgtgacaaagcaagatctgggccctgtgcctatgatggacccttctggaattcacggcgagggcaccagatgcaccggatggttcgatgtggaagccatcgtggaaagacggaccggcgacgtggtgtccgaggacgaagatgagaacctggaagataccggcgtggacctggtggacttcatcgacgatacctgcgagtttgagcaggccggcgacgaagctcctagagcactgctgcatgcccaagagacacaggcccatgtgaacgccgtgcactacctgaagcggaagttcacatgcagccctaccgtgtctcccctgggcaatgtgcagtgttctatcgagggcgagctgagccctagactgcacgccatccaactgaatgaaggcagcggcaaggccaagcggagactgtttctgcctgatagcggctacggcaataccgaggtggaaacccagctgtctcaggtggcaggatccgatggcgaatctcaagcccctggcggcaaagaaaatgtgcagcctgctgaaggcgctggcggagatgttcgacagctgctgagaagcagcaacctgaaggccacactgctgggcaagttcaaggacgtgtacggcatcggcttcaacgaactcgtgcggtgcttcaagagcgacaagaccgtgtgcaccgattgggttgtgggagctgctggcgtgcaccattctgtggccgaaggactgaagcacctgatcgagcctttctgcacatacgcccacatgcagtgcctgacctgcaactggggagtgtttctgctgctgctcatccggttcaagtgcggcaagaacagactgaccgtggccaagtgcatctctaccctgctgaacgtgcaagagccctacctgctgatcgaacctccaaagctgagatccacagccgccgctctgtactggtacagaaccggcatcagcaacgtgtccgaagtgatcggagagcctcctgagtggatcgtgcggcagaccatgtttcagcacagcctcgaggacagcatcttcgacctgtctcagatggtgcagtgggcctacgaccacgatctggtggacgatagcgccattgcctaccagtatgcccagctggccgacgtggactctaatgccgccgctttcctgaagtctaacgctcaggccaaatacgtgaaggactgcgccaccatgtgcagacactacaagagagccgagaagcaggccatgaccatgagccagtggatcagagccagatgcgataagaccgacgacggcggagattggaggcctatcgtgcagttcctgagataccagaacgtcgagttcatcacctttctgagcgcctttaaggccttcctgaagggaatccccaagagaagctgcatcgtgctgtacggccctccaaacaccggcaagagctacttcggaatgagcctgatgcagtttctgcagggcagcatcatcagctacgtgaacagcaacagccacttttggctggcccctctggccgaagctaaagtggccatgctggacgatgccacaccacagtgctggtcctacatcgacacctacatgcggagcgtgctggacggcaaccccatgagcattgaccggaagcacaagaacctgatccagatgaagtgtccgcctctgatcatcaccagcaacaccaacgtgggcgaagatgacagatggcgctacctgcactccagagtggtggtgttcaagttcgagcagacctttccattcgaccagaacggcaatcccgtgtacgagctgtccgacaagaattggaagtccttcttcagccggacctggtccagactcgagctgcaagaggatgaggacaccgagcaggatggctctacagtgcgggcctttaagtgtgtgcccggccagaacaccaatatcctgggctctatggaagccctgagcgagagactgaacgcctaccaggacaagatcctgaccttctacgaagaggactccaaggacctgagggaccagatcgagcattggagatgtgtgcggggagagtgcgccgtgttctacaaggccagagagatgggccacagccacatcaaccaccagcaggttccacctctgcacgtgtccagaggcaaggcccacaatgccattgagctgcagatggccctggaaagcctgaaccagagcgacttcaacaccgaggaatggaccctgcaggacacaagcctggaaatgtggcggaccgagcctcagtgctgcttcaaaaagaaaggcgagacagtgaccgtgctgtatgactgcgacaaggacaacagcatggactacaccctgtggggccacgtgtacgtgtggggagatacaggctgggacaaagtgtgcggaaaggtggactacggcggcctgtactatgtgctgcacggcctgaaagtgtactacgttgagttccagcaagaggccgtgaagtacagcaagaccaacaagtgggaagtgcatatcggcagaacagtgatcccctacagcgagtccgtgtcctctacagccctgtgcgaaagagtgcctatcgccgagatcgccaatggcctccagcagaccagcattccctctcacacacacgccaccaccaaagagaacgcttgggtttcctctcagcctcctaccaagcggtccagaagatctgatccaggcggcgatcctgtcagagccctggatgccaatagcagaaccctgctgtctggaaccgcctgcgagaataccaccggcaactcttacagcgactgcacccctgtggtgcacctgaaaggcgaccccaattgtctgaaggccctgcggttcagattcgtgaaacacaagaatctgttcgtgaacgtgtcctccacctggcggtggaccaacaacaccgaagagaaggccatcgtgactgtgacctttaaggacgagcagcagagacagcagttcctcggcagcgtgaagatccccaactccatctgtgtgtgcaagggcgtgatgacagttggcagcatggtggaaggcagccaagagagagcccggacactgcacgaactgtgcgagcagagagaacagacccagcacgacatcgagctggactgcgtgtactgcctgaatcctctgaccagaaccgaggtgtacgacttcgccagatgggagctgagaatcgtgtacagacgggataccgcctacggcgtgtgcaagctgtgcctgaggttccacagcaaagtgcggaagtacaggcggtacaactactccatctacggccccacactggaacggcggacaaagaagcagctcgaagaactcgtgatccggtgctactgctgccagaaacctcagtgccccgtggaaaagcagcgccacgttgaccagggccagagattccacaacattgccgagcagtggaccggcagatgcctgcaatgttggaggccaacagccgctgaaaccggctctatgatcggccctggacctacactgcaggatatcgtgcttgagctggaacccgagcctgtggacctgagaggatatgagcagctggactccagcgaggacgaggacgagattgaccaccaccaacagcaggacagacccgatgtgcaagaagatgacggcgagcggtttagaatcctgagcgactgtcacgtgtgccagaataccgtgtcaagagtggtgcacagcacccacgacgacctgcacattctcgaggacctgcttatgggcaccctcgagatcgtggcccctaattgtgccgtgggcagcgaacagaaactgatctccgaggaagatctctgaggaagaatgtgcacagtgctaaccagaaaattcaggacaagactagtgcggccgctttggaaagttttataggtagttgatagaacaaaatacataattttgtaaaaataaatcactttttat

SEQ ID NO: 71 - DNA, 5504 bp, Artificial Sequence
  MfPV3 Ii-E1E2-p2a-Ii-E6E7 integrated into DelIII locus of the poxviral vector
aaaaattaaaattttattttttttttttggaatataaataagatctatccctatcagtgatagagatctccctatcagtgatagagatcgtcgacgagctcgtttagtgaaccgtcagatcgcctggagacgccatccacgctgttttgacctctagcaccggtgccaccatgcacagaaggcggagcagaagctgccgcgaggatcagaaacccgtgatggacgaccagcgggacctgatcagcaacaacgagcagctgcctatgctcggcagaaggcctggcgctcctgagagcaaatgttctagaggcgccctgtacaccggcttcagcatcctggttacactgctgctggccggacaggctaccaccgcctactttctgtatcagcagcagggcagactggacaagctgaccgtgaccagccagaacctgcagctggaaaacctgcggatgaagctgcccaagcctcctaagcctgtgtccaagatgcggatggccacacctctgctgatgcaggctttgcctatgggagcactgcctcagggccctatgcagaacgccaccaaatacggcaacatgaccgaggaccacgtgatgcatctgctgcagaatgccgatcctctgaaggtgtaccctccactgaagggcagctttcccgagaacctgcggcacctgaagaacaccatggaaaccatcgactggaaggtgttcgagagctggatgcaccactggctgctgttcgagatgagccggcacagcctggaacagaagcctacagacgcccctcctaaagagtccctggaactggaagatcccagctctggcctgggcgtgacaaagcaagatctgggccctgtgcctatgatggacccttctggaattcacggcgagggcaccagatgcaccggatggttcgatgtggaagccatcgtggaaagacggaccggcgacgtggtgtccgaggacgaagatgagaacctggaagataccggcgtggacctggtggacttcatcgacgatacctgcgagtttgagcaggccggcgacgaagctcctagagcactgctgcatgcccaagagacacaggcccatgtgaacgccgtgcactacctgaagcggaagttcacatgcagccctaccgtgtctcccctgggcaatgtgcagtgttctatcgagggcgagctgagccctagactgcacgccatccaactgaatgaaggcagcggcaaggccaagcggagactgtttctgcctgatagcggctacggcaataccgaggtggaaacccagctgtctcaggtggcaggatccgatggcgaatctcaagcccctggcggcaaagaaaatgtgcagcctgctgaaggcgctggcggagatgttcgacagctgctgagaagcagcaacctgaaggccacactgctgggcaagttcaaggacgtgtacggcatcggcttcaacgaactcgtgcggtgcttcaagagcgacaagaccgtgtgcaccgattgggttgtgggagctgctggcgtgcaccattctgtggccgaaggactgaagcacctgatcgagcctttctgcacatacgcccacatgcagtgcctgacctgcaactggggagtgtttctgctgctgctcatccggttcaagtgcggcaagaacagactgaccgtggccaagtgcatctctaccctgctgaacgtgcaagagccctacctgctgatcgaacctccaaagctgagatccacagccgccgctctgtactggtacagaaccggcatcagcaacgtgtccgaagtgatcggagagcctcctgagtggatcgtgcggcagaccatgtttcagcacagcctcgaggacagcatcttcgacctgtctcagatggtgcagtgggcctacgaccacgatctggtggacgatagcgccattgcctaccagtatgcccagctggccgacgtggactctaatgccgccgctttcctgaagtctaacgctcaggccaaatacgtgaaggactgcgccaccatgtgcagacactacaagagagccgagaagcaggccatgaccatgagccagtggatcagagccagatgcgataagaccgacgacggcggagattggaggcctatcgtgcagttcctgagataccagaacgtcgagttcatcacctttctgagcgcctttaaggccttcctgaagggaatccccaagagaagctgcatcgtgctgtacggccctccaaacaccggcaagagctacttcggaatgagcctgatgcagtttctgcagggcagcatcatcagctacgtgaacagcaacagccacttttggctggcccctctggccgaagctaaagtggccatgctggacgatgccacaccacagtgctggtcctacatcgacacctacatgcggagcgtgctggacggcaaccccatgagcattgaccggaagcacaagaacctgatccagatgaagtgtccgcctctgatcatcaccagcaacaccaacgtgggcgaagatgacagatggcgctacctgcactccagagtggtggtgttcaagttcgagcagacctttccattcgaccagaacggcaatcccgtgtacgagctgtccgacaagaattggaagtccttcttcagccggacctggtccagactcgagctgcaagaggatgaggacaccgagcaggatggctctacagtgcgggcctttaagtgtgtgcccggccagaacaccaatatcctgggctctatggaagccctgagcgagagactgaacgcctaccaggacaagatcctgaccttctacgaagaggactccaaggacctgagggaccagatcgagcattggagatgtgtgcggggagagtgcgccgtgttctacaaggccagagagatgggccacagccacatcaaccaccagcaggttccacctctgcacgtgtccagaggcaaggcccacaatgccattgagctgcagatggccctggaaagcctgaaccagagcgacttcaacaccgaggaatggaccctgcaggacacaagcctggaaatgtggcggaccgagcctcagtgctgcttcaaaaagaaaggcgagacagtgaccgtgctgtatgactgcgacaaggacaacagcatggactacaccctgtggggccacgtgtacgtgtggggagatacaggctgggacaaagtgtgcggaaaggtggactacggcggcctgtactatgtgctgcacggcctgaaagtgtactacgttgagttccagcaagaggccgtgaagtacagcaagaccaacaagtgggaagtgcatatcggcagaacagtgatcccctacagcgagtccgtgtcctctacagccctgtgcgaaagagtgcctatcgccgagatcgccaatggcctccagcagaccagcattccctctcacacacacgccaccaccaaagagaacgcttgggtttcctctcagcctcctaccaagcggtccagaagatctgatccaggcggcgatcctgtcagagccctggatgccaatagcagaaccctgctgtctggaaccgcctgcgagaataccaccggcaactcttacagcgactgcacccctgtggtgcacctgaaaggcgaccccaattgtctgaaggccctgcggttcagattcgtgaaacacaagaatctgttcgtgaacgtgtcctccacctggcggtggaccaacaacaccgaagagaaggccatcgtgactgtgacctttaaggacgagcagcagagacagcagttcctcggcagcgtgaagatccccaactccatctgtgtgtgcaagggcgtgatgacagttggcagcggcgccaccaatttcagtctgcttaaacaggccggggacgtcgaagagaaccccggacctatgcatcggcgcagatctcggtcttgtagagaagaccaaaagcctgtcatggatgatcaaagagatttaatttctaataatgaacaattacccatgttgggacggcgccccggagcccccgaatctaagtgcagccggggagctttatatacaggattttctattttagtgaccttattattagctggccaagccacaacagcttatttcttataccaacaacaaggacggttagataaattaacagtcacatctcaaaatttacaattagagaatttaagaatgaaattacctaaaccacccaaacccgtcagtaaaatgagaatggctacccccttattaatgcaagccctccccatgggcgccttaccccaaggacccatgcaaaatgctacaaagtatggaaatatgacagaagatcatgtcatgcacttattacaaaacgctgaccccttaaaagtctatccccctttaaaaggatctttccctgaaaatttaagacatttaaaaaatacaatggagacaattgattggaaagtctttgaatcttggatgcatcattggttattatttgaaatgtctaggcattctttagagcaaaaacccaccgatgctccacccaaggaaagtttagagttagaggacccttctagcggattaggagtcaccaaacaggacttaggacccgtccccatgatggtggaaggcagccaagagagagcccggacactgcacgaactgtgcgagcagagagaacagacccagcacgacatcgagctggactgcgtgtactgcctgaatcctctgaccagaaccgaggtgtacgacttcgccagatgggagctgagaatcgtgtacagacgggataccgcctacggcgtgtgcaagctgtgcctgaggttccacagcaaagtgcggaagtacaggcggtacaactactccatctacggccccacactggaacggcggacaaagaagcagctcgaagaactcgtgatccggtgctactgctgccagaaacctcagtgccccgtggaaaagcagcgccacgttgaccagggccagagattccacaacattgccgagcagtggaccggcagatgcctgcaatgttggaggccaacagccgctgaaaccggctctatgatcggccctggacctacactgcaggatatcgtgcttgagctggaacccgagcctgtggacctgagaggatatgagcagctggactccagcgaggacgaggacgagattgaccaccaccaacagcaggacagacccgatgtgcaagaagatgacggcgagcggtttagaatcctgagcgactgtcacgtgtgccagaataccgtgtcaagagtggtgcacagcacccacgacgacctgcacattctcgaggacctgcttatgggcaccctcgagatcgtggcccctaattgtgccgtgggcagcgaacagaaactgatctccgaggaagatctctgaggaagaatgtgcacagtgctaaccagaaaattcaggacaagactagtgcggccgctttggaaagttttataggtagttgatagaacaaaatacataattttgtaaaaataaatcactttttat

SEQ ID NO: 72 - DNA, 4052 bp, Artificial Sequence
  MfPV3 E1E2E6E7 integrated into DelIII locus of the poxviral vector
aaaaattaaaattttattttttttttttggaatataaataagatctatccctatcagtgatagagatctccctatcagtgatagagatcgtcgacgagctcgtttagtgaaccgtcagatcgcctggagacgccatccacgctgttttgacctctagcaccggtgccaccatggacccttctggaattcacggcgagggcaccagatgcaccggatggttcgatgtggaagccatcgtggaaagacggaccggcgacgtggtgtccgaggacgaagatgagaacctggaagataccggcgtggacctggtggacttcatcgacgatacctgcgagtttgagcaggccggcgacgaagctcctagagcactgctgcatgcccaagagacacaggcccatgtgaacgccgtgcactacctgaagcggaagttcacatgcagccctaccgtgtctcccctgggcaatgtgcagtgttctatcgagggcgagctgagccctagactgcacgccatccaactgaatgaaggcagcggcaaggccaagcggagactgtttctgcctgatagcggctacggcaataccgaggtggaaacccagctgtctcaggtggcaggatccgatggcgaatctcaagcccctggcggcaaagaaaatgtgcagcctgctgaaggcgctggcggagatgttcgacagctgctgagaagcagcaacctgaaggccacactgctgggcaagttcaaggacgtgtacggcatcggcttcaacgaactcgtgcggtgcttcaagagcgacaagaccgtgtgcaccgattgggttgtgggagctgctggcgtgcaccattctgtggccgaaggactgaagcacctgatcgagcctttctgcacatacgcccacatgcagtgcctgacctgcaactggggagtgtttctgctgctgctcatccggttcaagtgcggcaagaacagactgaccgtggccaagtgcatctctaccctgctgaacgtgcaagagccctacctgctgatcgaacctccaaagctgagatccacagccgccgctctgtactggtacagaaccggcatcagcaacgtgtccgaagtgatcggagagcctcctgagtggatcgtgcggcagaccatgtttcagcacagcctcgaggacagcatcttcgacctgtctcagatggtgcagtgggcctacgaccacgatctggtggacgatagcgccattgcctaccagtatgcccagctggccgacgtggactctaatgccgccgctttcctgaagtctaacgctcaggccaaatacgtgaaggactgcgccaccatgtgcagacactacaagagagccgagaagcaggccatgaccatgagccagtggatcagagccagatgcgataagaccgacgacggcggagattggaggcctatcgtgcagttcctgagataccagaacgtcgagttcatcacctttctgagcgcctttaaggccttcctgaagggaatccccaagagaagctgcatcgtgctgtacggccctccaaacaccggcaagagctacttcggaatgagcctgatgcagtttctgcagggcagcatcatcagctacgtgaacagcaacagccacttttggctggcccctctggccgaagctaaagtggccatgctggacgatgccacaccacagtgctggtcctacatcgacacctacatgcggagcgtgctggacggcaaccccatgagcattgaccggaagcacaagaacctgatccagatgaagtgtccgcctctgatcatcaccagcaacaccaacgtgggcgaagatgacagatggcgctacctgcactccagagtggtggtgttcaagttcgagcagacctttccattcgaccagaacggcaatcccgtgtacgagctgtccgacaagaattggaagtccttcttcagccggacctggtccagactcgagctgcaagaggatgaggacaccgagcaggatggctctacagtgcgggcctttaagtgtgtgcccggccagaacaccaatatcctgggctctatggaagccctgagcgagagactgaacgcctaccaggacaagatcctgaccttctacgaagaggactccaaggacctgagggaccagatcgagcattggagatgtgtgcggggagagtgcgccgtgttctacaaggccagagagatgggccacagccacatcaaccaccagcaggttccacctctgcacgtgtccagaggcaaggcccacaatgccattgagctgcagatggccctggaaagcctgaaccagagcgacttcaacaccgaggaatggaccctgcaggacacaagcctggaaatgtggcggaccgagcctcagtgctgcttcaaaaagaaaggcgagacagtgaccgtgctgtatgactgcgacaaggacaacagcatggactacaccctgtggggccacgtgtacgtgtggggagatacaggctgggacaaagtgtgcggaaaggtggactacggcggcctgtactatgtgctgcacggcctgaaagtgtactacgttgagttccagcaagaggccgtgaagtacagcaagaccaacaagtgggaagtgcatatcggcagaacagtgatcccctacagcgagtccgtgtcctctacagccctgtgcgaaagagtgcctatcgccgagatcgccaatggcctccagcagaccagcattccctctcacacacacgccaccaccaaagagaacgcttgggtttcctctcagcctcctaccaagcggtccagaagatctgatccaggcggcgatcctgtcagagccctggatgccaatagcagaaccctgctgtctggaaccgcctgcgagaataccaccggcaactcttacagcgactgcacccctgtggtgcacctgaaaggcgaccccaattgtctgaaggccctgcggttcagattcgtgaaacacaagaatctgttcgtgaacgtgtcctccacctggcggtggaccaacaacaccgaagagaaggccatcgtgactgtgacctttaaggacgagcagcagagacagcagttcctcggcagcgtgaagatccccaactccatctgtgtgtgcaagggcgtgatgacagttggcagcatggtggaaggcagccaagagagagcccggacactgcacgaactgtgcgagcagagagaacagacccagcacgacatcgagctggactgcgtgtactgcctgaatcctctgaccagaaccgaggtgtacgacttcgccagatgggagctgagaatcgtgtacagacgggataccgcctacggcgtgtgcaagctgtgcctgaggttccacagcaaagtgcggaagtacaggcggtacaactactccatctacggccccacactggaacggcggacaaagaagcagctcgaagaactcgtgatccggtgctactgctgccagaaacctcagtgccccgtggaaaagcagcgccacgttgaccagggccagagattccacaacattgccgagcagtggaccggcagatgcctgcaatgttggaggccaacagccgctgaaaccggctctatgatcggccctggacctacactgcaggatatcgtgcttgagctggaacccgagcctgtggacctgagaggatatgagcagctggactccagcgaggacgaggacgagattgaccaccaccaacagcaggacagacccgatgtgcaagaagatgacggcgagcggtttagaatcctgagcgactgtcacgtgtgccagaataccgtgtcaagagtggtgcacagcacccacgacgacctgcacattctcgaggacctgcttatgggcaccctcgagatcgtggcccctaattgtgccgtgggcagcgaacagaaactgatctccgaggaagatctctgaggaagaatgtgcacagtgctaaccagaaaattcaggacaagactagtgcggccgctttggaaagttttataggtagttgatagaacaaaatacataattttgtaaaaataaatcactttttat

SEQ ID NO: 73 - DNA, 5504 bp, Artificial Sequence
  MfPV3 Ii-E1E6E7-p2a-Ii-E2 integrated into DelIII locus of the poxviral vector
aaaaattaaaattttattttttttttttggaatataaataagatctatccctatcagtgatagagatctccctatcagtgatagagatcgtcgacgagctcgtttagtgaaccgtcagatcgcctggagacgccatccacgctgttttgacctctagcaccggtgccaccatgcacagaaggcggagcagaagctgccgcgaggatcagaaacccgtgatggacgaccagcgggacctgatcagcaacaacgagcagctgcctatgctcggcagaaggcctggcgctcctgagagcaaatgttctagaggcgccctgtacaccggcttcagcatcctggttacactgctgctggccggacaggctaccaccgcctactttctgtatcagcagcagggcagactggacaagctgaccgtgaccagccagaacctgcagctggaaaacctgcggatgaagctgcccaagcctcctaagcctgtgtccaagatgcggatggccacacctctgctgatgcaggctttgcctatgggagcactgcctcagggccctatgcagaacgccaccaaatacggcaacatgaccgaggaccacgtgatgcatctgctgcagaatgccgatcctctgaaggtgtaccctccactgaagggcagctttcccgagaacctgcggcacctgaagaacaccatggaaaccatcgactggaaggtgttcgagagctggatgcaccactggctgctgttcgagatgagccggcacagcctggaacagaagcctacagacgcccctcctaaagagtccctggaactggaagatcccagctctggcctgggcgtgacaaagcaagatctgggccctgtgcctatgatggacccttctggaattcacggcgagggcaccagatgcaccggatggttcgatgtggaagccatcgtggaaagacggaccggcgacgtggtgtccgaggacgaagatgagaacctggaagataccggcgtggacctggtggacttcatcgacgatacctgcgagtttgagcaggccggcgacgaagctcctagagcactgctgcatgcccaagagacacaggcccatgtgaacgccgtgcactacctgaagcggaagttcacatgcagccctaccgtgtctcccctgggcaatgtgcagtgttctatcgagggcgagctgagccctagactgcacgccatccaactgaatgaaggcagcggcaaggccaagcggagactgtttctgcctgatagcggctacggcaataccgaggtggaaacccagctgtctcaggtggcaggatccgatggcgaatctcaagcccctggcggcaaagaaaatgtgcagcctgctgaaggcgctggcggagatgttcgacagctgctgagaagcagcaacctgaaggccacactgctgggcaagttcaaggacgtgtacggcatcggcttcaacgaactcgtgcggtgcttcaagagcgacaagaccgtgtgcaccgattgggttgtgggagctgctggcgtgcaccattctgtggccgaaggactgaagcacctgatcgagcctttctgcacatacgcccacatgcagtgcctgacctgcaactggggagtgtttctgctgctgctcatccggttcaagtgcggcaagaacagactgaccgtggccaagtgcatctctaccctgctgaacgtgcaagagccctacctgctgatcgaacctccaaagctgagatccacagccgccgctctgtactggtacagaaccggcatcagcaacgtgtccgaagtgatcggagagcctcctgagtggatcgtgcggcagaccatgtttcagcacagcctcgaggacagcatcttcgacctgtctcagatggtgcagtgggcctacgaccacgatctggtggacgatagcgccattgcctaccagtatgcccagctggccgacgtggactctaatgccgccgctttcctgaagtctaacgctcaggccaaatacgtgaaggactgcgccaccatgtgcagacactacaagagagccgagaagcaggccatgaccatgagccagtggatcagagccagatgcgataagaccgacgacggcggagattggaggcctatcgtgcagttcctgagataccagaacgtcgagttcatcacctttctgagcgcctttaaggccttcctgaagggaatccccaagagaagctgcatcgtgctgtacggccctccaaacaccggcaagagctacttcggaatgagcctgatgcagtttctgcagggcagcatcatcagctacgtgaacagcaacagccacttttggctggcccctctggccgaagctaaagtggccatgctggacgatgccacaccacagtgctggtcctacatcgacacctacatgcggagcgtgctggacggcaaccccatgagcattgaccggaagcacaagaacctgatccagatgaagtgtccgcctctgatcatcaccagcaacaccaacgtgggcgaagatgacagatggcgctacctgcactccagagtggtggtgttcaagttcgagcagacctttccattcgaccagaacggcaatcccgtgtacgagctgtccgacaagaattggaagtccttcttcagccggacctggtccagactcgagctgcaagaggatgaggacaccgagcaggatggctctacagtgcgggcctttaagtgtgtgcccggccagaacaccaatatcctgggctctatggtggaaggcagccaagagagagcccggacactgcacgaactgtgcgagcagagagaacagacccagcacgacatcgagctggactgcgtgtactgcctgaatcctctgaccagaaccgaggtgtacgacttcgccagatgggagctgagaatcgtgtacagacgggataccgcctacggcgtgtgcaagctgtgcctgaggttccacagcaaagtgcggaagtacaggcggtacaactactccatctacggccccacactggaacggcggacaaagaagcagctcgaagaactcgtgatccggtgctactgctgccagaaacctcagtgccccgtggaaaagcagcgccacgttgaccagggccagagattccacaacattgccgagcagtggaccggcagatgcctgcaatgttggaggccaacagccgctgaaaccggctctatgatcggccctggacctacactgcaggatatcgtgcttgagctggaacccgagcctgtggacctgagaggatatgagcagctggactccagcgaggacgaggacgagattgaccaccaccaacagcaggacagacccgatgtgcaagaagatgacggcgagcggtttagaatcctgagcgactgtcacgtgtgccagaataccgtgtcaagagtggtgcacagcacccacgacgacctgcacattctcgaggacctgcttatgggcaccctcgagatcgtggcccctaattgtgccgtgggcagcggcgccaccaatttcagtctgcttaaacaggccggggacgtcgaagagaaccccggacctatgcatcggcgcagatctcggtcttgtagagaagaccaaaagcctgtcatggatgatcaaagagatttaatttctaataatgaacaattacccatgttgggacggcgccccggagcccccgaatctaagtgcagccggggagctttatatacaggattttctattttagtgaccttattattagctggccaagccacaacagcttatttcttataccaacaacaaggacggttagataaattaacagtcacatctcaaaatttacaattagagaatttaagaatgaaattacctaaaccacccaaacccgtcagtaaaatgagaatggctacccccttattaatgcaagccctccccatgggcgccttaccccaaggacccatgcaaaatgctacaaagtatggaaatatgacagaagatcatgtcatgcacttattacaaaacgctgaccccttaaaagtctatccccctttaaaaggatctttccctgaaaatttaagacatttaaaaaatacaatggagacaattgattggaaagtctttgaatcttggatgcatcattggttattatttgaaatgtctaggcattctttagagcaaaaacccaccgatgctccacccaaggaaagtttagagttagaggacccttctagcggattaggagtcaccaaacaggacttaggacccgtccccatgatggaagccctgagcgagagactgaacgcctaccaggacaagatcctgaccttctacgaagaggactccaaggacctgagggaccagatcgagcattggagatgtgtgcggggagagtgcgccgtgttctacaaggccagagagatgggccacagccacatcaaccaccagcaggttccacctctgcacgtgtccagaggcaaggcccacaatgccattgagctgcagatggccctggaaagcctgaaccagagcgacttcaacaccgaggaatggaccctgcaggacacaagcctggaaatgtggcggaccgagcctcagtgctgcttcaaaaagaaaggcgagacagtgaccgtgctgtatgactgcgacaaggacaacagcatggactacaccctgtggggccacgtgtacgtgtggggagatacaggctgggacaaagtgtgcggaaaggtggactacggcggcctgtactatgtgctgcacggcctgaaagtgtactacgttgagttccagcaagaggccgtgaagtacagcaagaccaacaagtgggaagtgcatatcggcagaacagtgatcccctacagcgagtccgtgtcctctacagccctgtgcgaaagagtgcctatcgccgagatcgccaatggcctccagcagaccagcattccctctcacacacacgccaccaccaaagagaacgcttgggtttcctctcagcctcctaccaagcggtccagaagatctgatccaggcggcgatcctgtcagagccctggatgccaatagcagaaccctgctgtctggaaccgcctgcgagaataccaccggcaactcttacagcgactgcacccctgtggtgcacctgaaaggcgaccccaattgtctgaaggccctgcggttcagattcgtgaaacacaagaatctgttcgtgaacgtgtcctccacctggcggtggaccaacaacaccgaagagaaggccatcgtgactgtgacctttaaggacgagcagcagagacagcagttcctcggcagcgtgaagatccccaactccatctgtgtgtgcaagggcgtgatgacagttggcagcgaacagaaactgatctccgaggaagatctctgaggaagaatgtgcacagtgctaaccagaaaattcaggacaagactagtgcggccgctttggaaagttttataggtagttgatagaacaaaatacataattttgtaaaaataaatcactttttat

SEQ ID NO: 74 - DNA, 3662 bp, Artificial Sequence
  MfPV3 Ii-E1E6E7 integrated into DelIII locus of the poxviral vector
aaaaattaaaattttattttttttttttggaatataaataagatctatccctatcagtgatagagatctccctatcagtgatagagatcgtcgacgagctcgtttagtgaaccgtcagatcgcctggagacgccatccacgctgttttgacctctagcaccggtgccaccatgcacagaaggcggagcagaagctgccgcgaggatcagaaacccgtgatggacgaccagcgggacctgatcagcaacaacgagcagctgcctatgctcggcagaaggcctggcgctcctgagagcaaatgttctagaggcgccctgtacaccggcttcagcatcctggttacactgctgctggccggacaggctaccaccgcctactttctgtatcagcagcagggcagactggacaagctgaccgtgaccagccagaacctgcagctggaaaacctgcggatgaagctgcccaagcctcctaagcctgtgtccaagatgcggatggccacacctctgctgatgcaggctttgcctatgggagcactgcctcagggccctatgcagaacgccaccaaatacggcaacatgaccgaggaccacgtgatgcatctgctgcagaatgccgatcctctgaaggtgtaccctccactgaagggcagctttcccgagaacctgcggcacctgaagaacaccatggaaaccatcgactggaaggtgttcgagagctggatgcaccactggctgctgttcgagatgagccggcacagcctggaacagaagcctacagacgcccctcctaaagagtccctggaactggaagatcccagctctggcctgggcgtgacaaagcaagatctgggccctgtgcctatgatggacccttctggaattcacggcgagggcaccagatgcaccggatggttcgatgtggaagccatcgtggaaagacggaccggcgacgtggtgtccgaggacgaagatgagaacctggaagataccggcgtggacctggtggacttcatcgacgatacctgcgagtttgagcaggccggcgacgaagctcctagagcactgctgcatgcccaagagacacaggcccatgtgaacgccgtgcactacctgaagcggaagttcacatgcagccctaccgtgtctcccctgggcaatgtgcagtgttctatcgagggcgagctgagccctagactgcacgccatccaactgaatgaaggcagcggcaaggccaagcggagactgtttctgcctgatagcggctacggcaataccgaggtggaaacccagctgtctcaggtggcaggatccgatggcgaatctcaagcccctggcggcaaagaaaatgtgcagcctgctgaaggcgctggcggagatgttcgacagctgctgagaagcagcaacctgaaggccacactgctgggcaagttcaaggacgtgtacggcatcggcttcaacgaactcgtgcggtgcttcaagagcgacaagaccgtgtgcaccgattgggttgtgggagctgctggcgtgcaccattctgtggccgaaggactgaagcacctgatcgagcctttctgcacatacgcccacatgcagtgcctgacctgcaactggggagtgtttctgctgctgctcatccggttcaagtgcggcaagaacagactgaccgtggccaagtgcatctctaccctgctgaacgtgcaagagccctacctgctgatcgaacctccaaagctgagatccacagccgccgctctgtactggtacagaaccggcatcagcaacgtgtccgaagtgatcggagagcctcctgagtggatcgtgcggcagaccatgtttcagcacagcctcgaggacagcatcttcgacctgtctcagatggtgcagtgggcctacgaccacgatctggtggacgatagcgccattgcctaccagtatgcccagctggccgacgtggactctaatgccgccgctttcctgaagtctaacgctcaggccaaatacgtgaaggactgcgccaccatgtgcagacactacaagagagccgagaagcaggccatgaccatgagccagtggatcagagccagatgcgataagaccgacgacggcggagattggaggcctatcgtgcagttcctgagataccagaacgtcgagttcatcacctttctgagcgcctttaaggccttcctgaagggaatccccaagagaagctgcatcgtgctgtacggccctccaaacaccggcaagagctacttcggaatgagcctgatgcagtttctgcagggcagcatcatcagctacgtgaacagcaacagccacttttggctggcccctctggccgaagctaaagtggccatgctggacgatgccacaccacagtgctggtcctacatcgacacctacatgcggagcgtgctggacggcaaccccatgagcattgaccggaagcacaagaacctgatccagatgaagtgtccgcctctgatcatcaccagcaacaccaacgtgggcgaagatgacagatggcgctacctgcactccagagtggtggtgttcaagttcgagcagacctttccattcgaccagaacggcaatcccgtgtacgagctgtccgacaagaattggaagtccttcttcagccggacctggtccagactcgagctgcaagaggatgaggacaccgagcaggatggctctacagtgcgggcctttaagtgtgtgcccggccagaacaccaatatcctgggctctatggtggaaggcagccaagagagagcccggacactgcacgaactgtgcgagcagagagaacagacccagcacgacatcgagctggactgcgtgtactgcctgaatcctctgaccagaaccgaggtgtacgacttcgccagatgggagctgagaatcgtgtacagacgggataccgcctacggcgtgtgcaagctgtgcctgaggttccacagcaaagtgcggaagtacaggcggtacaactactccatctacggccccacactggaacggcggacaaagaagcagctcgaagaactcgtgatccggtgctactgctgccagaaacctcagtgccccgtggaaaagcagcgccacgttgaccagggccagagattccacaacattgccgagcagtggaccggcagatgcctgcaatgttggaggccaacagccgctgaaaccggctctatgatcggccctggacctacactgcaggatatcgtgcttgagctggaacccgagcctgtggacctgagaggatatgagcagctggactccagcgaggacgaggacgagattgaccaccaccaacagcaggacagacccgatgtgcaagaagatgacggcgagcggtttagaatcctgagcgactgtcacgtgtgccagaataccgtgtcaagagtggtgcacagcacccacgacgacctgcacattctcgaggacctgcttatgggcaccctcgagatcgtggcccctaattgtgccgtgggcagcgaacagaaactgatctccgaggaagatctctgaggaagaatgtgcacagtgctaaccagaaaattcaggacaagactagtgcggccgctttggaaagttttataggtagttgatagaacaaaatacataattttgtaaaaataaatcactttttat

SEQ ID NO: 75 - DNA, 4808 bp, Artificial Sequence
  HPV16 Ii-E1E2E6E7 integrated into DelIII locus of the poxviral vector
aaaaattaaaattttattttttttttttggaatataaataagatctatccctatcagtgatagagatctccctatcagtgatagagatcgtcgacgagctcgtttagtgaaccgtcagatcgcctggagacgccatccacgctgttttgacctctagcaccggtgccaccatgcacagaaggcggagcagaagctgccgcgaggatcagaaacccgtgatggacgaccagcgggacctgatcagcaacaacgagcagctgcctatgctcggcagaaggcctggcgctcctgagagcaaatgttctagaggcgccctgtacaccggcttcagcatcctggttacactgctgctggccggacaggctaccaccgcctactttctgtatcagcagcagggcagactggacaagctgaccgtgaccagccagaacctgcagctggaaaacctgcggatgaagctgcccaagcctcctaagcctgtgtccaagatgcggatggccacacctctgctgatgcaggctttgcctatgggagcactgcctcagggccctatgcagaacgccaccaaatacggcaacatgaccgaggaccacgtgatgcatctgctgcagaatgccgatcctctgaaggtgtaccctccactgaagggcagctttcccgagaacctgcggcacctgaagaacaccatggaaaccatcgactggaaggtgttcgagagctggatgcaccactggctgctgttcgagatgagccggcacagcctggaacagaagcctacagacgcccctcctaaagagtccctggaactggaagatcccagctctggcctgggcgtgacaaagcaagatctgggccctgtgcctatgatggccgatcctgctggcacaaacggcgaagaaggcacaggctgcaacggctggttttacgtggaagccgtggtggaaaagaaaaccggcgacgccatcagcgacgacgagaacgagaatgacagcgacaccggcgaggacctggtggacttcatcgtgaacgacaacgactacctgacacaggccgagacagagacagcccacgctctgtttacagcccaagaggccaagcagcacagagatgccgttcaggtgctgaagagaaagtacctgggcagccctctgagcgacatcagcggctgtgtggacaacaacatcagccccagactgaaggccatctgcatcgagaagcagagcagagccgccaagcggagactgtttgagagcgaggatagcggctacggcaataccgaggtggaaacccagcaaatgctgcaggtcgagggcagacacgaaaccgagacaccttgcagccagtacagcggaggatctggcggaggctgtagccagtactcttctggaagtggcggagagggcgtgtccgagagacacaccatttgtcagacccctctgaccaacatcctgaacgtgctgaaaaccagcaacgccaaggccgccatgctggccaagttcaaagagctgtacggcgtcagcttcagcgaactcgtgcggcccttcaagagcaacaagtccacctgttgcgactggtgcattgccgcctttggcctgacaccttctatcgccgacagcatcaagaccctgctccagcagtactgtctgtacctgcacattcagagcctggcctgctcttggggaatggtggtgctgctgctcgtgcggtacaagtgcggcaagaacagagagacaattgagaagctgctgagcaaactgctgtgcgtgtcccctatgtgcatgatgatcgagcctccaaagctgcggtctacagccgccgctctgtactggtacaagaccggcatcagcaatatctccgaggtgtacggcgacacccctgagtggattcagagacagaccgtcctgcagcacagcttcaacgactgcaccttcgagctgtcccagatggtgcagtgggcctacgacaatgacatcgtggacgactccgagatcgcctataagtacgcccagctggccgacaccaacagcaatgccagcgccttcctgaagtccaacagccaggccaagatcgtgaaggactgcgccaccatgtgcagacactacaagcgggccgagaagaaacagatgagcatgagccagtggatcaagtacagatgcgacagagtggacgacggcggcgattggaagcagatcgtgatgttcctgagataccagggcgtcgagttcatgagctttctgacagccctgaagcggttcctgcagggcatccccaagaagaactgcatcctgctgtatggcgccgctaacaccggcaagagcctgttcggaatgagcctgatgaagtttctgcagggctccgtgatctgctttgtgaacagcaagagccacttctggctccagccactggccgatgccaagattggcatgctggacgatgccaccgtgccttgctggaactacatcgacgacaacctgagaaacgccctggacggcaacctggtttctatggacgtgaagcacagacccctggtgcagctgaagtgtcctccactgctgatcaccagcaacatcaacgccggcaccgattccagatggccctatctgcacaaccggctggtggtgtttacctttcctaacgagttccccttcgacgaaaacggcaaccccgtgtacgagctgaacgataagaattggaagtccttcttcagccggacctggtccagactgagcctgcacgaggatgaggacaaagagaacgacggcgacagcctgcctaccttcaaatgtgtcagcggccagaacaccaacacactgggcagcatggaaacactgtgccagcggctgaacgtgtgccaggacaagattctgacccactatgagaacgacagcaccgacctgagggaccacatcgactactggaagcacatgcggctggaatgcgccatctactacaaggctagagagatgggcttcaagcacatcaaccaccaggtggtgcctacactggccgtgtctaagaacaaggctctgcaggccatcgaactgcagctgaccctggaaacaatctacaactcccagtactccaacgagaagtggaccctccaggacgtgtcactggaagtgtacctgaccgctcctaccggctgcatcaagaaacacggctacaccgtggaagtgcagtttgacggcgatatctgcaataccatgcactacaccaactggacccacatctacatctgcgaagaggccagcgtgacagtggtggaaggccaggtcgactactacggcctgtactacgtgcacgagggcatcagaacctacttcgtgcagttcaaggatgacgccgagaagtacagcaagaacaaagtgtgggaagtgcacgctggcggccaagtgatcctgtgtcctacaagcgtgttcagcagcaacgaagtgtctagccccgagatcatcagacagcacctggccaatcatcctgccgccacacacacaaaagctgtggccctgggcaccgaggaaacacagaccacaattcagaggcccagaagcgagcccgataccggcaatccttgtcacaccaccaagctgctgcaccgggattccgtggattctgcccctatcctgaccgccttcaacagctcccacaaaggccggatcaactgcaacagcaacaccacacctatcgtgcacctgaaaggggacgccaacactctgaaggccctgcggtacagattcaagaagcactgtaccctgtataccgccgtgtccagcacatggcactggaccggacacaacgtgaaacacaagagcgccatcgtgaccctgacctacgatagcgagtggcagagggaccagttcctgagccaagtgaagatccctaagaccatcaccgtgtccaccggctttatgagcattggcagcatgcaccagaaacggacagccatgttccaggatcctcaagagcggccacggaagctgcctcagctgtgtacagaactgcagaccaccatccacgacatcatcctcgagtgcgtgtactgcaagcagcagctcctgcggagagaagtgtacgacttcgccttccgggatctgtgcatcgtgtacagagatggcaacccctacgccgtgtgcgacaagtgcctgaagttctactccaagatcagcgagtaccggcactactgctactccctgtacggcaccacacttgagcagcagtacaacaagcccctgtgcgatctgctgatccggtgcatcaactgccagaaacctcagtgccccgaggaaaagcagagacacctggacaagaagcagcggttccacaacattagaggcagatggacaggccggtgcatgagctgctgtagaagcagcagaacaagacggggctccatgcacggcgataccccaacactgcacgagtacatgctggatctgcagcccgagacaaccgatctgtacggctatgagcagctgaatgactccagcgaggaagaggacgagatcgacggacctgctggacaggctgaacctgatagagcccactacaatatcgtgaccttctgctgcaagtgcgatagcaccctgagaagatgcgtgcagagcacccacgtggacatcaggaccctcgaggatctgctcatgggcaccctgggaattgtggccccaatctgctctcagaagccttgaggaagaatgtgcacagtgctaaccagaaaattcaggacaagactagtgcggccgctttggaaagttttataggtagttgatagaacaaaatacataattttgtaaaaataaatcactttttat

SEQ ID NO: 76 - DNA, 5570 bp, Artificial Sequence
  HPV16 Ii-E1E2-p2a-Ii-E6E7 integrated into DelIII locus of the poxviral vector
aaaaattaaaattttattttttttttttggaatataaataagatctatccctatcagtgatagagatctccctatcagtgatagagatcgtcgacgagctcgtttagtgaaccgtcagatcgcctggagacgccatccacgctgttttgacctctagcaccggtgccaccatgcacagaaggcggagcagaagctgccgcgaggatcagaaacccgtgatggacgaccagcgggacctgatcagcaacaacgagcagctgcctatgctcggcagaaggcctggcgctcctgagagcaaatgttctagaggcgccctgtacaccggcttcagcatcctggttacactgctgctggccggacaggctaccaccgcctactttctgtatcagcagcagggcagactggacaagctgaccgtgaccagccagaacctgcagctggaaaacctgcggatgaagctgcccaagcctcctaagcctgtgtccaagatgcggatggccacacctctgctgatgcaggctttgcctatgggagcactgcctcagggccctatgcagaacgccaccaaatacggcaacatgaccgaggaccacgtgatgcatctgctgcagaatgccgatcctctgaaggtgtaccctccactgaagggcagctttcccgagaacctgcggcacctgaagaacaccatggaaaccatcgactggaaggtgttcgagagctggatgcaccactggctgctgttcgagatgagccggcacagcctggaacagaagcctacagacgcccctcctaaagagtccctggaactggaagatcccagctctggcctgggcgtgacaaagcaagatctgggccctgtgcctatgatggccgatcctgctggcacaaacggcgaagaaggcacaggctgcaacggctggttttacgtggaagccgtggtggaaaagaaaaccggcgacgccatcagcgacgacgagaacgagaatgacagcgacaccggcgaggacctggtggacttcatcgtgaacgacaacgactacctgacacaggccgagacagagacagcccacgctctgtttacagcccaagaggccaagcagcacagagatgccgttcaggtgctgaagagaaagtacctgggcagccctctgagcgacatcagcggctgtgtggacaacaacatcagccccagactgaaggccatctgcatcgagaagcagagcagagccgccaagcggagactgtttgagagcgaggatagcggctacggcaataccgaggtggaaacccagcaaatgctgcaggtcgagggcagacacgaaaccgagacaccttgcagccagtacagcggaggatctggcggaggctgtagccagtactcttctggaagtggcggagagggcgtgtccgagagacacaccatttgtcagacccctctgaccaacatcctgaacgtgctgaaaaccagcaacgccaaggccgccatgctggccaagttcaaagagctgtacggcgtcagcttcagcgaactcgtgcggcccttcaagagcaacaagtccacctgttgcgactggtgcattgccgcctttggcctgacaccttctatcgccgacagcatcaagaccctgctccagcagtactgtctgtacctgcacattcagagcctggcctgctcttggggaatggtggtgctgctgctcgtgcggtacaagtgcggcaagaacagagagacaattgagaagctgctgagcaaactgctgtgcgtgtcccctatgtgcatgatgatcgagcctccaaagctgcggtctacagccgccgctctgtactggtacaagaccggcatcagcaatatctccgaggtgtacggcgacacccctgagtggattcagagacagaccgtcctgcagcacagcttcaacgactgcaccttcgagctgtcccagatggtgcagtgggcctacgacaatgacatcgtggacgactccgagatcgcctataagtacgcccagctggccgacaccaacagcaatgccagcgccttcctgaagtccaacagccaggccaagatcgtgaaggactgcgccaccatgtgcagacactacaagcgggccgagaagaaacagatgagcatgagccagtggatcaagtacagatgcgacagagtggacgacggcggcgattggaagcagatcgtgatgttcctgagataccagggcgtcgagttcatgagctttctgacagccctgaagcggttcctgcagggcatccccaagaagaactgcatcctgctgtatggcgccgctaacaccggcaagagcctgttcggaatgagcctgatgaagtttctgcagggctccgtgatctgctttgtgaacagcaagagccacttctggctccagccactggccgatgccaagattggcatgctggacgatgccaccgtgccttgctggaactacatcgacgacaacctgagaaacgccctggacggcaacctggtttctatggacgtgaagcacagacccctggtgcagctgaagtgtcctccactgctgatcaccagcaacatcaacgccggcaccgattccagatggccctatctgcacaaccggctggtggtgtttacctttcctaacgagttccccttcgacgaaaacggcaaccccgtgtacgagctgaacgataagaattggaagtccttcttcagccggacctggtccagactgagcctgcacgaggatgaggacaaagagaacgacggcgacagcctgcctaccttcaaatgtgtcagcggccagaacaccaacacactgggcagcatggaaacactgtgccagcggctgaacgtgtgccaggacaagattctgacccactatgagaacgacagcaccgacctgagggaccacatcgactactggaagcacatgcggctggaatgcgccatctactacaaggctagagagatgggcttcaagcacatcaaccaccaggtggtgcctacactggccgtgtctaagaacaaggctctgcaggccatcgaactgcagctgaccctggaaacaatctacaactcccagtactccaacgagaagtggaccctccaggacgtgtcactggaagtgtacctgaccgctcctaccggctgcatcaagaaacacggctacaccgtggaagtgcagtttgacggcgatatctgcaataccatgcactacaccaactggacccacatctacatctgcgaagaggccagcgtgacagtggtggaaggccaggtcgactactacggcctgtactacgtgcacgagggcatcagaacctacttcgtgcagttcaaggatgacgccgagaagtacagcaagaacaaagtgtgggaagtgcacgctggcggccaagtgatcctgtgtcctacaagcgtgttcagcagcaacgaagtgtctagccccgagatcatcagacagcacctggccaatcatcctgccgccacacacacaaaagctgtggccctgggcaccgaggaaacacagaccacaattcagaggcccagaagcgagcccgataccggcaatccttgtcacaccaccaagctgctgcaccgggattccgtggattctgcccctatcctgaccgccttcaacagctcccacaaaggccggatcaactgcaacagcaacaccacacctatcgtgcacctgaaaggggacgccaacactctgaaggccctgcggtacagattcaagaagcactgtaccctgtataccgccgtgtccagcacatggcactggaccggacacaacgtgaaacacaagagcgccatcgtgaccctgacctacgatagcgagtggcagagggaccagttcctgagccaagtgaagatccctaagaccatcaccgtgtccaccggctttatgagcattggcagcggcagcggcgccaccaatttcagtctgcttaaacaggccggggacgtcgaagagaaccccggacctatgcatcggcgcagatctcggtcttgtagagaagaccaaaagcctgtcatggatgatcaaagagatttaatttctaataatgaacaattacccatgttgggacggcgccccggagcccccgaatctaagtgcagccggggagctttatatacaggattttctattttagtgaccttattattagctggccaagccacaacagcttatttcttataccaacaacaaggacggttagataaattaacagtcacatctcaaaatttacaattagagaatttaagaatgaaattacctaaaccacccaaacccgtcagtaaaatgagaatggctacccccttattaatgcaagccctccccatgggcgccttaccccaaggacccatgcaaaatgctacaaagtatggaaatatgacagaagatcatgtcatgcacttattacaaaacgctgaccccttaaaagtctatccccctttaaaaggatctttccctgaaaatttaagacatttaaaaaatacaatggagacaattgattggaaagtctttgaatcttggatgcatcattggttattatttgaaatgtctaggcattctttagagcaaaaacccaccgatgctccacccaaggaaagtttagagttagaggacccttctagcggattaggagtcaccaaacaggacttaggacccgtccccatgatgcaccagaaacggacagccatgttccaggatcctcaagagcggccacggaagctgcctcagctgtgtacagaactgcagaccaccatccacgacatcatcctcgagtgcgtgtactgcaagcagcagctcctgcggagagaagtgtacgacttcgccttccgggatctgtgcatcgtgtacagagatggcaacccctacgccgtgtgcgacaagtgcctgaagttctactccaagatcagcgagtaccggcactactgctactccctgtacggcaccacacttgagcagcagtacaacaagcccctgtgcgatctgctgatccggtgcatcaactgccagaaacctcagtgccccgaggaaaagcagagacacctggacaagaagcagcggttccacaacattagaggcagatggacaggccggtgcatgagctgctgtagaagcagcagaacaagacggggctccatgcacggcgataccccaacactgcacgagtacatgctggatctgcagcccgagacaaccgatctgtacggctatgagcagctgaatgactccagcgaggaagaggacgagatcgacggacctgctggacaggctgaacctgatagagcccactacaatatcgtgaccttctgctgcaagtgcgatagcaccctgagaagatgcgtgcagagcacccacgtggacatcaggaccctcgaggatctgctcatgggcaccctgggaattgtggccccaatctgctctcagaagccttgaggaagaatgtgcacagtgctaaccagaaaattcaggacaagactagtgcggccgctttggaaagttttataggtagttgatagaacaaaatacataattttgtaaaaataaatcactttttat

SEQ ID NO: 77 - DNA, 4112 bp, Artificial Sequence
  HPV16 E1E2E6E7 integrated into DelIII locus of the poxviral vector
aaaaattaaaattttattttttttttttggaatataaataagatctatccctatcagtgatagagatctccctatcagtgatagagatcgtcgacgagctcgtttagtgaaccgtcagatcgcctggagacgccatccacgctgttttgacctctagcaccggtgccaccatggccgatcctgctggcacaaacggcgaagaaggcacaggctgcaacggctggttttacgtggaagccgtggtggaaaagaaaaccggcgacgccatcagcgacgacgagaacgagaatgacagcgacaccggcgaggacctggtggacttcatcgtgaacgacaacgactacctgacacaggccgagacagagacagcccacgctctgtttacagcccaagaggccaagcagcacagagatgccgttcaggtgctgaagagaaagtacctgggcagccctctgagcgacatcagcggctgtgtggacaacaacatcagccccagactgaaggccatctgcatcgagaagcagagcagagccgccaagcggagactgtttgagagcgaggatagcggctacggcaataccgaggtggaaacccagcaaatgctgcaggtcgagggcagacacgaaaccgagacaccttgcagccagtacagcggaggatctggcggaggctgtagccagtactcttctggaagtggcggagagggcgtgtccgagagacacaccatttgtcagacccctctgaccaacatcctgaacgtgctgaaaaccagcaacgccaaggccgccatgctggccaagttcaaagagctgtacggcgtcagcttcagcgaactcgtgcggcccttcaagagcaacaagtccacctgttgcgactggtgcattgccgcctttggcctgacaccttctatcgccgacagcatcaagaccctgctccagcagtactgtctgtacctgcacattcagagcctggcctgctcttggggaatggtggtgctgctgctcgtgcggtacaagtgcggcaagaacagagagacaattgagaagctgctgagcaaactgctgtgcgtgtcccctatgtgcatgatgatcgagcctccaaagctgcggtctacagccgccgctctgtactggtacaagaccggcatcagcaatatctccgaggtgtacggcgacacccctgagtggattcagagacagaccgtcctgcagcacagcttcaacgactgcaccttcgagctgtcccagatggtgcagtgggcctacgacaatgacatcgtggacgactccgagatcgcctataagtacgcccagctggccgacaccaacagcaatgccagcgccttcctgaagtccaacagccaggccaagatcgtgaaggactgcgccaccatgtgcagacactacaagcgggccgagaagaaacagatgagcatgagccagtggatcaagtacagatgcgacagagtggacgacggcggcgattggaagcagatcgtgatgttcctgagataccagggcgtcgagttcatgagctttctgacagccctgaagcggttcctgcagggcatccccaagaagaactgcatcctgctgtatggcgccgctaacaccggcaagagcctgttcggaatgagcctgatgaagtttctgcagggctccgtgatctgctttgtgaacagcaagagccacttctggctccagccactggccgatgccaagattggcatgctggacgatgccaccgtgccttgctggaactacatcgacgacaacctgagaaacgccctggacggcaacctggtttctatggacgtgaagcacagacccctggtgcagctgaagtgtcctccactgctgatcaccagcaacatcaacgccggcaccgattccagatggccctatctgcacaaccggctggtggtgtttacctttcctaacgagttccccttcgacgaaaacggcaaccccgtgtacgagctgaacgataagaattggaagtccttcttcagccggacctggtccagactgagcctgcacgaggatgaggacaaagagaacgacggcgacagcctgcctaccttcaaatgtgtcagcggccagaacaccaacacactgggcagcatggaaacactgtgccagcggctgaacgtgtgccaggacaagattctgacccactatgagaacgacagcaccgacctgagggaccacatcgactactggaagcacatgcggctggaatgcgccatctactacaaggctagagagatgggcttcaagcacatcaaccaccaggtggtgcctacactggccgtgtctaagaacaaggctctgcaggccatcgaactgcagctgaccctggaaacaatctacaactcccagtactccaacgagaagtggaccctccaggacgtgtcactggaagtgtacctgaccgctcctaccggctgcatcaagaaacacggctacaccgtggaagtgcagtttgacggcgatatctgcaataccatgcactacaccaactggacccacatctacatctgcgaagaggccagcgtgacagtggtggaaggccaggtcgactactacggcctgtactacgtgcacgagggcatcagaacctacttcgtgcagttcaaggatgacgccgagaagtacagcaagaacaaagtgtgggaagtgcacgctggcggccaagtgatcctgtgtcctacaagcgtgttcagcagcaacgaagtgtctagccccgagatcatcagacagcacctggccaatcatcctgccgccacacacacaaaagctgtggccctgggcaccgaggaaacacagaccacaattcagaggcccagaagcgagcccgataccggcaatccttgtcacaccaccaagctgctgcaccgggattccgtggattctgcccctatcctgaccgccttcaacagctcccacaaaggccggatcaactgcaacagcaacaccacacctatcgtgcacctgaaaggggacgccaacactctgaaggccctgcggtacagattcaagaagcactgtaccctgtataccgccgtgtccagcacatggcactggaccggacacaacgtgaaacacaagagcgccatcgtgaccctgacctacgatagcgagtggcagagggaccagttcctgagccaagtgaagatccctaagaccatcaccgtgtccaccggctttatgagcattggcagcatgcaccagaaacggacagccatgttccaggatcctcaagagcggccacggaagctgcctcagctgtgtacagaactgcagaccaccatccacgacatcatcctcgagtgcgtgtactgcaagcagcagctcctgcggagagaagtgtacgacttcgccttccgggatctgtgcatcgtgtacagagatggcaacccctacgccgtgtgcgacaagtgcctgaagttctactccaagatcagcgagtaccggcactactgctactccctgtacggcaccacacttgagcagcagtacaacaagcccctgtgcgatctgctgatccggtgcatcaactgccagaaacctcagtgccccgaggaaaagcagagacacctggacaagaagcagcggttccacaacattagaggcagatggacaggccggtgcatgagctgctgtagaagcagcagaacaagacggggctccatgcacggcgataccccaacactgcacgagtacatgctggatctgcagcccgagacaaccgatctgtacggctatgagcagctgaatgactccagcgaggaagaggacgagatcgacggacctgctggacaggctgaacctgatagagcccactacaatatcgtgaccttctgctgcaagtgcgatagcaccctgagaagatgcgtgcagagcacccacgtggacatcaggaccctcgaggatctgctcatgggcaccctgggaattgtggccccaatctgctctcagaagccttgaggaagaatgtgcacagtgctaaccagaaaattcaggacaagactagtgcggccgctttggaaagttttataggtagttgatagaacaaaatacataattttgtaaaaataaatcactttttat

SEQ ID NO: 78 - DNA, 5564 bp, Artificial Sequence
  HPV16 Ii-E1E6E7-p2a-Ii-E2 integrated into DelIII locus of the poxviral vector
aaaaattaaaattttattttttttttttggaatataaataagatctatccctatcagtgatagagatctccctatcagtgatagagatcgtcgacgagctcgtttagtgaaccgtcagatcgcctggagacgccatccacgctgttttgacctctagcaccggtgccaccatgcacagaaggcggagcagaagctgccgcgaggatcagaaacccgtgatggacgaccagcgggacctgatcagcaacaacgagcagctgcctatgctcggcagaaggcctggcgctcctgagagcaaatgttctagaggcgccctgtacaccggcttcagcatcctggttacactgctgctggccggacaggctaccaccgcctactttctgtatcagcagcagggcagactggacaagctgaccgtgaccagccagaacctgcagctggaaaacctgcggatgaagctgcccaagcctcctaagcctgtgtccaagatgcggatggccacacctctgctgatgcaggctttgcctatgggagcactgcctcagggccctatgcagaacgccaccaaatacggcaacatgaccgaggaccacgtgatgcatctgctgcagaatgccgatcctctgaaggtgtaccctccactgaagggcagctttcccgagaacctgcggcacctgaagaacaccatggaaaccatcgactggaaggtgttcgagagctggatgcaccactggctgctgttcgagatgagccggcacagcctggaacagaagcctacagacgcccctcctaaagagtccctggaactggaagatcccagctctggcctgggcgtgacaaagcaagatctgggccctgtgcctatgatggccgatcctgctggcacaaacggcgaagaaggcacaggctgcaacggctggttttacgtggaagccgtggtggaaaagaaaaccggcgacgccatcagcgacgacgagaacgagaatgacagcgacaccggcgaggacctggtggacttcatcgtgaacgacaacgactacctgacacaggccgagacagagacagcccacgctctgtttacagcccaagaggccaagcagcacagagatgccgttcaggtgctgaagagaaagtacctgggcagccctctgagcgacatcagcggctgtgtggacaacaacatcagccccagactgaaggccatctgcatcgagaagcagagcagagccgccaagcggagactgtttgagagcgaggatagcggctacggcaataccgaggtggaaacccagcaaatgctgcaggtcgagggcagacacgaaaccgagacaccttgcagccagtacagcggaggatctggcggaggctgtagccagtactcttctggaagtggcggagagggcgtgtccgagagacacaccatttgtcagacccctctgaccaacatcctgaacgtgctgaaaaccagcaacgccaaggccgccatgctggccaagttcaaagagctgtacggcgtcagcttcagcgaactcgtgcggcccttcaagagcaacaagtccacctgttgcgactggtgcattgccgcctttggcctgacaccttctatcgccgacagcatcaagaccctgctccagcagtactgtctgtacctgcacattcagagcctggcctgctcttggggaatggtggtgctgctgctcgtgcggtacaagtgcggcaagaacagagagacaattgagaagctgctgagcaaactgctgtgcgtgtcccctatgtgcatgatgatcgagcctccaaagctgcggtctacagccgccgctctgtactggtacaagaccggcatcagcaatatctccgaggtgtacggcgacacccctgagtggattcagagacagaccgtcctgcagcacagcttcaacgactgcaccttcgagctgtcccagatggtgcagtgggcctacgacaatgacatcgtggacgactccgagatcgcctataagtacgcccagctggccgacaccaacagcaatgccagcgccttcctgaagtccaacagccaggccaagatcgtgaaggactgcgccaccatgtgcagacactacaagcgggccgagaagaaacagatgagcatgagccagtggatcaagtacagatgcgacagagtggacgacggcggcgattggaagcagatcgtgatgttcctgagataccagggcgtcgagttcatgagctttctgacagccctgaagcggttcctgcagggcatccccaagaagaactgcatcctgctgtatggcgccgctaacaccggcaagagcctgttcggaatgagcctgatgaagtttctgcagggctccgtgatctgctttgtgaacagcaagagccacttctggctccagccactggccgatgccaagattggcatgctggacgatgccaccgtgccttgctggaactacatcgacgacaacctgagaaacgccctggacggcaacctggtttctatggacgtgaagcacagacccctggtgcagctgaagtgtcctccactgctgatcaccagcaacatcaacgccggcaccgattccagatggccctatctgcacaaccggctggtggtgtttacctttcctaacgagttccccttcgacgaaaacggcaaccccgtgtacgagctgaacgataagaattggaagtccttcttcagccggacctggtccagactgagcctgcacgaggatgaggacaaagagaacgacggcgacagcctgcctaccttcaaatgtgtcagcggccagaacaccaacacactgggcagcatgcaccagaaacggacagccatgttccaggatcctcaagagcggccacggaagctgcctcagctgtgtacagaactgcagaccaccatccacgacatcatcctcgagtgcgtgtactgcaagcagcagctcctgcggagagaagtgtacgacttcgccttccgggatctgtgcatcgtgtacagagatggcaacccctacgccgtgtgcgacaagtgcctgaagttctactccaagatcagcgagtaccggcactactgctactccctgtacggcaccacacttgagcagcagtacaacaagcccctgtgcgatctgctgatccggtgcatcaactgccagaaacctcagtgccccgaggaaaagcagagacacctggacaagaagcagcggttccacaacattagaggcagatggacaggccggtgcatgagctgctgtagaagcagcagaacaagacggggctccatgcacggcgataccccaacactgcacgagtacatgctggatctgcagcccgagacaaccgatctgtacggctatgagcagctgaatgactccagcgaggaagaggacgagatcgacggacctgctggacaggctgaacctgatagagcccactacaatatcgtgaccttctgctgcaagtgcgatagcaccctgagaagatgcgtgcagagcacccacgtggacatcaggaccctcgaggatctgctcatgggcaccctgggaattgtggccccaatctgctctcagaagcctggcagcggcgccaccaatttcagtctgcttaaacaggccggggacgtcgaagagaaccccggacctatgcatcggcgcagatctcggtcttgtagagaagaccaaaagcctgtcatggatgatcaaagagatttaatttctaataatgaacaattacccatgttgggacggcgccccggagcccccgaatctaagtgcagccggggagctttatatacaggattttctattttagtgaccttattattagctggccaagccacaacagcttatttcttataccaacaacaaggacggttagataaattaacagtcacatctcaaaatttacaattagagaatttaagaatgaaattacctaaaccacccaaacccgtcagtaaaatgagaatggctacccccttattaatgcaagccctccccatgggcgccttaccccaaggacccatgcaaaatgctacaaagtatggaaatatgacagaagatcatgtcatgcacttattacaaaacgctgaccccttaaaagtctatccccctttaaaaggatctttccctgaaaatttaagacatttaaaaaatacaatggagacaattgattggaaagtctttgaatcttggatgcatcattggttattatttgaaatgtctaggcattctttagagcaaaaacccaccgatgctccacccaaggaaagtttagagttagaggacccttctagcggattaggagtcaccaaacaggacttaggacccgtccccatgatggaaacactgtgccagcggctgaacgtgtgccaggacaagattctgacccactatgagaacgacagcaccgacctgagggaccacatcgactactggaagcacatgcggctggaatgcgccatctactacaaggctagagagatgggcttcaagcacatcaaccaccaggtggtgcctacactggccgtgtctaagaacaaggctctgcaggccatcgaactgcagctgaccctggaaacaatctacaactcccagtactccaacgagaagtggaccctccaggacgtgtcactggaagtgtacctgaccgctcctaccggctgcatcaagaaacacggctacaccgtggaagtgcagtttgacggcgatatctgcaataccatgcactacaccaactggacccacatctacatctgcgaagaggccagcgtgacagtggtggaaggccaggtcgactactacggcctgtactacgtgcacgagggcatcagaacctacttcgtgcagttcaaggatgacgccgagaagtacagcaagaacaaagtgtgggaagtgcacgctggcggccaagtgatcctgtgtcctacaagcgtgttcagcagcaacgaagtgtctagccccgagatcatcagacagcacctggccaatcatcctgccgccacacacacaaaagctgtggccctgggcaccgaggaaacacagaccacaattcagaggcccagaagcgagcccgataccggcaatccttgtcacaccaccaagctgctgcaccgggattccgtggattctgcccctatcctgaccgccttcaacagctcccacaaaggccggatcaactgcaacagcaacaccacacctatcgtgcacctgaaaggggacgccaacactctgaaggccctgcggtacagattcaagaagcactgtaccctgtataccgccgtgtccagcacatggcactggaccggacacaacgtgaaacacaagagcgccatcgtgaccctgacctacgatagcgagtggcagagggaccagttcctgagccaagtgaagatccctaagaccatcaccgtgtccaccggctttatgagcatttgaggaagaatgtgcacagtgctaaccagaaaattcaggacaagactagtgcggccgctttggaaagttttataggtagttgatagaacaaaatacataattttgtaaaaataaatcactttttat

SEQ ID NO: 79 - DNA, 3707 bp, Artificial Sequence
  HPV16 Ii-E1E6E7 integrated into DelIII locus of the poxviral vector
aaaaattaaaattttattttttttttttggaatataaataagatctatccctatcagtgatagagatctccctatcagtgatagagatcgtcgacgagctcgtttagtgaaccgtcagatcgcctggagacgccatccacgctgttttgacctctagcaccggtgccaccatgcacagaaggcggagcagaagctgccgcgaggatcagaaacccgtgatggacgaccagcgggacctgatcagcaacaacgagcagctgcctatgctcggcagaaggcctggcgctcctgagagcaaatgttctagaggcgccctgtacaccggcttcagcatcctggttacactgctgctggccggacaggctaccaccgcctactttctgtatcagcagcagggcagactggacaagctgaccgtgaccagccagaacctgcagctggaaaacctgcggatgaagctgcccaagcctcctaagcctgtgtccaagatgcggatggccacacctctgctgatgcaggctttgcctatgggagcactgcctcagggccctatgcagaacgccaccaaatacggcaacatgaccgaggaccacgtgatgcatctgctgcagaatgccgatcctctgaaggtgtaccctccactgaagggcagctttcccgagaacctgcggcacctgaagaacaccatggaaaccatcgactggaaggtgttcgagagctggatgcaccactggctgctgttcgagatgagccggcacagcctggaacagaagcctacagacgcccctcctaaagagtccctggaactggaagatcccagctctggcctgggcgtgacaaagcaagatctgggccctgtgcctatgatggccgatcctgctggcacaaacggcgaagaaggcacaggctgcaacggctggttttacgtggaagccgtggtggaaaagaaaaccggcgacgccatcagcgacgacgagaacgagaatgacagcgacaccggcgaggacctggtggacttcatcgtgaacgacaacgactacctgacacaggccgagacagagacagcccacgctctgtttacagcccaagaggccaagcagcacagagatgccgttcaggtgctgaagagaaagtacctgggcagccctctgagcgacatcagcggctgtgtggacaacaacatcagccccagactgaaggccatctgcatcgagaagcagagcagagccgccaagcggagactgtttgagagcgaggatagcggctacggcaataccgaggtggaaacccagcaaatgctgcaggtcgagggcagacacgaaaccgagacaccttgcagccagtacagcggaggatctggcggaggctgtagccagtactcttctggaagtggcggagagggcgtgtccgagagacacaccatttgtcagacccctctgaccaacatcctgaacgtgctgaaaaccagcaacgccaaggccgccatgctggccaagttcaaagagctgtacggcgtcagcttcagcgaactcgtgcggcccttcaagagcaacaagtccacctgttgcgactggtgcattgccgcctttggcctgacaccttctatcgccgacagcatcaagaccctgctccagcagtactgtctgtacctgcacattcagagcctggcctgctcttggggaatggtggtgctgctgctcgtgcggtacaagtgcggcaagaacagagagacaattgagaagctgctgagcaaactgctgtgcgtgtcccctatgtgcatgatgatcgagcctccaaagctgcggtctacagccgccgctctgtactggtacaagaccggcatcagcaatatctccgaggtgtacggcgacacccctgagtggattcagagacagaccgtcctgcagcacagcttcaacgactgcaccttcgagctgtcccagatggtgcagtgggcctacgacaatgacatcgtggacgactccgagatcgcctataagtacgcccagctggccgacaccaacagcaatgccagcgccttcctgaagtccaacagccaggccaagatcgtgaaggactgcgccaccatgtgcagacactacaagcgggccgagaagaaacagatgagcatgagccagtggatcaagtacagatgcgacagagtggacgacggcggcgattggaagcagatcgtgatgttcctgagataccagggcgtcgagttcatgagctttctgacagccctgaagcggttcctgcagggcatccccaagaagaactgcatcctgctgtatggcgccgctaacaccggcaagagcctgttcggaatgagcctgatgaagtttctgcagggctccgtgatctgctttgtgaacagcaagagccacttctggctccagccactggccgatgccaagattggcatgctggacgatgccaccgtgccttgctggaactacatcgacgacaacctgagaaacgccctggacggcaacctggtttctatggacgtgaagcacagacccctggtgcagctgaagtgtcctccactgctgatcaccagcaacatcaacgccggcaccgattccagatggccctatctgcacaaccggctggtggtgtttacctttcctaacgagttccccttcgacgaaaacggcaaccccgtgtacgagctgaacgataagaattggaagtccttcttcagccggacctggtccagactgagcctgcacgaggatgaggacaaagagaacgacggcgacagcctgcctaccttcaaatgtgtcagcggccagaacaccaacacactgggcagcatgcaccagaaacggacagccatgttccaggatcctcaagagcggccacggaagctgcctcagctgtgtacagaactgcagaccaccatccacgacatcatcctcgagtgcgtgtactgcaagcagcagctcctgcggagagaagtgtacgacttcgccttccgggatctgtgcatcgtgtacagagatggcaacccctacgccgtgtgcgacaagtgcctgaagttctactccaagatcagcgagtaccggcactactgctactccctgtacggcaccacacttgagcagcagtacaacaagcccctgtgcgatctgctgatccggtgcatcaactgccagaaacctcagtgccccgaggaaaagcagagacacctggacaagaagcagcggttccacaacattagaggcagatggacaggccggtgcatgagctgctgtagaagcagcagaacaagacggggctccatgcacggcgataccccaacactgcacgagtacatgctggatctgcagcccgagacaaccgatctgtacggctatgagcagctgaatgactccagcgaggaagaggacgagatcgacggacctgctggacaggctgaacctgatagagcccactacaatatcgtgaccttctgctgcaagtgcgatagcaccctgagaagatgcgtgcagagcacccacgtggacatcaggaccctcgaggatctgctcatgggcaccctgggaattgtggccccaatctgctctcagaagccttgaggaagaatgtgcacagtgctaaccagaaaattcaggacaagactagtgcggccgctttggaaagttttataggtagttgatagaacaaaatacataattttgtaaaaataaatcactttttat

SEQ ID NO: 80 - DNA, 4853 bp, Artificial Sequence
  HPV18 Ii-E1E2E6E7 integrated into DelIII locus of the poxviral vector
aaaaattaaaattttattttttttttttggaatataaataagatctatccctatcagtgatagagatctccctatcagtgatagagatcgtcgacgagctcgtttagtgaaccgtcagatcgcctggagacgccatccacgctgttttgacctctagcaccggtgccaccatgcacagaaggcggagcagaagctgccgcgaggatcagaaacccgtgatggacgaccagcgggacctgatcagcaacaacgagcagctgcctatgctcggcagaaggcctggcgctcctgagagcaaatgttctagaggcgccctgtacaccggcttcagcatcctggttacactgctgctggccggacaggctaccaccgcctactttctgtatcagcagcagggcagactggacaagctgaccgtgaccagccagaacctgcagctggaaaacctgcggatgaagctgcccaagcctcctaagcctgtgtccaagatgcggatggccacacctctgctgatgcaggctttgcctatgggagcactgcctcagggccctatgcagaacgccaccaaatacggcaacatgaccgaggaccacgtgatgcatctgctgcagaatgccgatcctctgaaggtgtaccctccactgaagggcagctttcccgagaacctgcggcacctgaagaacaccatggaaaccatcgactggaaggtgttcgagagctggatgcaccactggctgctgttcgagatgagccggcacagcctggaacagaagcctacagacgcccctcctaaagagtccctggaactggaagatcccagctctggcctgggcgtgacaaagcaagatctgggccctgtgcctatgatggccgatcctgagggaacagatggcgaaggcacaggctgcaacggctggttttacgtgcaagccatcgtggacaagaagaccggcgacgtcatcagcgacgacgaggatgagaatgccaccgacaccggcagcgacatggtggactttatcgatacccagggcacgttctgcgagcaggccgaactggaaacagcccaggcactgtttcacgcccaagaggtgcacaacgatgcccaggtgctgcacgtgctgaagagaaagtttgccggcggaagcaccgagaacagcccactgggagaaagactggaagtggacaccgagctgagccccagactgcaagagatcagcctgaacagcggccagaagaaggccaagcggagactgttcaccatctccgacagcggctacggctgtagcgaagtggaagccacacagatccaagtgaccaccaatggcgagcacggcggcaatgtttgttctggcggatctaccgaggccatcgacaatggcggaaccgagggcaacaatagctccgtggatggcaccagcgacaacagcaacatcgagaacgtgaaccctcagtgcacaatcgcccagctgaaggacctgctgaaagtgaacaacaagcagggcgccatgctggccgtgtttaaggatacctacggcctgagcttcaccgacctcgtgcggaacttcaagagcgacaagaccacctgtaccgactgggtcaccgccatctttggcgtgaacccaacaatcgccgagggcttcaagaccctgatccagcctttcatcctgtacgcccacatccagtgtctggactgcaaatggggcgtgctgattctggccctgctgagatacaagtgcggcaagagcagactgaccgtggccaagggactgagcactctgctgcatgtgcccgagacatgcatgctgattcagcctccaaagctgcggtctagcgtggccgctctgtactggtacagaaccggcatcagcaatatcagcgaagtgatgggcgacacccctgagtggattcagcggctgacaatcatccagcacggcatcgacgactccaacttcgacctgagcgagatggtgcagtgggccttcgataacgagctgaccgacgagtccgacatggcctttgaatacgccctgctggcagacagcaactccaatgccgccgctttcctgaagtccaactgccaggccaagtacctgaaggactgcgccaccatgtgcaagcactaccgcagagcacagaaacggcagatgaacatgagccagtggatccggttccggtgcagcaagatcgatgaaggtggcgactggcggcctatcgtgcagttcctgagataccagcagatcgagttcatcacctttctgggcgccctgaagtcattcctgaagggaacccctaaaaagaactgcctggtgttctgcggccctgccaataccggcaagtcctacttcggcatgagctttatccacttcatccagggcgccgtgatcagcttcgtgaacagcaccagccacttttggctggaacccctgaccgataccaaggtggcaatgctggacgacgccaccaccacctgttggacctacttcgacacctacatgcggaacgccctggacggcaaccccatcagcatcgacagaaagcacaagcccctcatccagctgaaatgccctccaatcctgctgaccacaaacattcaccccgccaaggacaatcggtggccctacctggaaagccggatcaccgtgttcgagttccccaacgcctttccattcgacaagaacggcaatcccgtgtacgagatcaacgacaagaattggaagtgcttcttcgagcggacctggtccagactggatctgcacgaggaagaagaggacgccgacacagagggcaatcccttcggcacctttaagtgtgtggccgggcagaatcacagacccctgggatctatgcagaccccaaaagagacactgagcgagcggctgagcgccctccaggacaagatcatcgaccactacgagaacgacagcaaggacatcgacagccagattcagtactggcagctgatcagatgggagaacgccatcttcttcgccgctagagagcacggaattcagaccctgaaccaccaggtggtgcccgcctacaacatcagcaagagcaaggcccacaaggccattgaactccagatggccctgcaaggactggctcagagcgcctacaagaccgaggattggacactccaggatacctgcgaggaactgtggaacacagagcccacacactgcttcaagaaaggcggccagaccgtgcaggtctacttcgatggcaacaaggataactgcatgacctacgtggcctgggacagcgtgtactacatgacagatgccggcacctgggacaagaccgccacctgtgtttctcaccggggcctgtactacgtgaaagagggctacaacaccttctacatcgagtttaagagcgagtgcgagaagtatggcaacaccggcacatgggaagtgcatttcggcaacaacgtgatcgactgcaacgactccatgtgctccacctccgatgacaccgtgtctgccacacagctggtcaagcagctccagcacaccccatctccatacagctctacagtgtctgtgggcaccgccaagacctatggccaaacaagcgctgccacaagacctggccattgtggactggccgagaagcagcactgtggccctgttaatcctctgctgggagccgccacacctacaggcaacaacaagagaagaaagctgtgcagcggcaacaccacacctatcattcacctgaagggcgacagaaacagcctgaagtgcctgcggtacagactgaggaagcacagcgatcactaccgggacatcagctccacctggcactggacaggtgctggcaacgaaaagaccggcatcctgacagtgacctaccacagcgagactcagcggaccaagttcctgaacaccgtggctatccccgacagcgtgcagattctcgtgggctacatgaccatgggcagcatggccagattcgaggaccctaccagacggccctacaagctgcctgatctgtgcaccgaactgaacaccagccttcaggatatcgagatcacctgtgtgtactgcaagaccgtgctcgagctgacagaagtgtttgagttcgccttcaaggacctgttcgtggtgtacagagacagcatccctcacgccgcctgtcacaagtgcatcgacttctacagcagaatcagagagctgcggcactacagcgactccgtgtacggcgataccctggaaaaactgaccaacaccggactgtacaacctgctgatccggtgcctgagatgccagaaacctcagaaccccgccgagaaactgagacatctgaacgagaagcggcggttccacaatatcgccggccactacagaggccagtgccacagctgttgcaaccgggccagacaagaaagactccagcggagaagaggcagcatgcacggacctaaagccacacttcaggacatcgtgctgcacctcgagcctcagaatgagatccccgtggatctgctcggccatgagcagctgagcgatagcgaggaagagaacgacgagatcgacggcgtcaaccaccagcatctgcctgccagaagggccgaacctcagagacacaccatgctgtgcatgtgctgcaagtgcgaggcccggatcgagagagtggtggaatctagcgccgacgacctgagagctttccagcagctgttcctgaatactctgagcttcgtggccccttggtgcgctagtcagcagtgaggaagaatgtgcacagtgctaaccagaaaattcaggacaagactagtgcggccgctttggaaagttttataggtagttgatagaacaaaatacataattttgtaaaaataaatcactttttat

SEQ ID NO: 81 - DNA, 5609 bp, Artificial Sequence
  HPV18 Ii-E1E2-p2a-Ii-E6E7 integrated into DelIII locus of the poxviral vector
aaaaattaaaattttattttttttttttggaatataaataagatctatccctatcagtgatagagatctccctatcagtgatagagatcgtcgacgagctcgtttagtgaaccgtcagatcgcctggagacgccatccacgctgttttgacctctagcaccggtgccaccatgcacagaaggcggagcagaagctgccgcgaggatcagaaacccgtgatggacgaccagcgggacctgatcagcaacaacgagcagctgcctatgctcggcagaaggcctggcgctcctgagagcaaatgttctagaggcgccctgtacaccggcttcagcatcctggttacactgctgctggccggacaggctaccaccgcctactttctgtatcagcagcagggcagactggacaagctgaccgtgaccagccagaacctgcagctggaaaacctgcggatgaagctgcccaagcctcctaagcctgtgtccaagatgcggatggccacacctctgctgatgcaggctttgcctatgggagcactgcctcagggccctatgcagaacgccaccaaatacggcaacatgaccgaggaccacgtgatgcatctgctgcagaatgccgatcctctgaaggtgtaccctccactgaagggcagctttcccgagaacctgcggcacctgaagaacaccatggaaaccatcgactggaaggtgttcgagagctggatgcaccactggctgctgttcgagatgagccggcacagcctggaacagaagcctacagacgcccctcctaaagagtccctggaactggaagatcccagctctggcctgggcgtgacaaagcaagatctgggccctgtgcctatgatggccgatcctgagggaacagatggcgaaggcacaggctgcaacggctggttttacgtgcaagccatcgtggacaagaagaccggcgacgtcatcagcgacgacgaggatgagaatgccaccgacaccggcagcgacatggtggactttatcgatacccagggcacgttctgcgagcaggccgaactggaaacagcccaggcactgtttcacgcccaagaggtgcacaacgatgcccaggtgctgcacgtgctgaagagaaagtttgccggcggaagcaccgagaacagcccactgggagaaagactggaagtggacaccgagctgagccccagactgcaagagatcagcctgaacagcggccagaagaaggccaagcggagactgttcaccatctccgacagcggctacggctgtagcgaagtggaagccacacagatccaagtgaccaccaatggcgagcacggcggcaatgtttgttctggcggatctaccgaggccatcgacaatggcggaaccgagggcaacaatagctccgtggatggcaccagcgacaacagcaacatcgagaacgtgaaccctcagtgcacaatcgcccagctgaaggacctgctgaaagtgaacaacaagcagggcgccatgctggccgtgtttaaggatacctacggcctgagcttcaccgacctcgtgcggaacttcaagagcgacaagaccacctgtaccgactgggtcaccgccatctttggcgtgaacccaacaatcgccgagggcttcaagaccctgatccagcctttcatcctgtacgcccacatccagtgtctggactgcaaatggggcgtgctgattctggccctgctgagatacaagtgcggcaagagcagactgaccgtggccaagggactgagcactctgctgcatgtgcccgagacatgcatgctgattcagcctccaaagctgcggtctagcgtggccgctctgtactggtacagaaccggcatcagcaatatcagcgaagtgatgggcgacacccctgagtggattcagcggctgacaatcatccagcacggcatcgacgactccaacttcgacctgagcgagatggtgcagtgggccttcgataacgagctgaccgacgagtccgacatggcctttgaatacgccctgctggcagacagcaactccaatgccgccgctttcctgaagtccaactgccaggccaagtacctgaaggactgcgccaccatgtgcaagcactaccgcagagcacagaaacggcagatgaacatgagccagtggatccggttccggtgcagcaagatcgatgaaggtggcgactggcggcctatcgtgcagttcctgagataccagcagatcgagttcatcacctttctgggcgccctgaagtcattcctgaagggaacccctaaaaagaactgcctggtgttctgcggccctgccaataccggcaagtcctacttcggcatgagctttatccacttcatccagggcgccgtgatcagcttcgtgaacagcaccagccacttttggctggaacccctgaccgataccaaggtggcaatgctggacgacgccaccaccacctgttggacctacttcgacacctacatgcggaacgccctggacggcaaccccatcagcatcgacagaaagcacaagcccctcatccagctgaaatgccctccaatcctgctgaccacaaacattcaccccgccaaggacaatcggtggccctacctggaaagccggatcaccgtgttcgagttccccaacgcctttccattcgacaagaacggcaatcccgtgtacgagatcaacgacaagaattggaagtgcttcttcgagcggacctggtccagactggatctgcacgaggaagaagaggacgccgacacagagggcaatcccttcggcacctttaagtgtgtggccgggcagaatcacagacccctgggatctatgcagaccccaaaagagacactgagcgagcggctgagcgccctccaggacaagatcatcgaccactacgagaacgacagcaaggacatcgacagccagattcagtactggcagctgatcagatgggagaacgccatcttcttcgccgctagagagcacggaattcagaccctgaaccaccaggtggtgcccgcctacaacatcagcaagagcaaggcccacaaggccattgaactccagatggccctgcaaggactggctcagagcgcctacaagaccgaggattggacactccaggatacctgcgaggaactgtggaacacagagcccacacactgcttcaagaaaggcggccagaccgtgcaggtctacttcgatggcaacaaggataactgcatgacctacgtggcctgggacagcgtgtactacatgacagatgccggcacctgggacaagaccgccacctgtgtttctcaccggggcctgtactacgtgaaagagggctacaacaccttctacatcgagtttaagagcgagtgcgagaagtatggcaacaccggcacatgggaagtgcatttcggcaacaacgtgatcgactgcaacgactccatgtgctccacctccgatgacaccgtgtctgccacacagctggtcaagcagctccagcacaccccatctccatacagctctacagtgtctgtgggcaccgccaagacctatggccaaacaagcgctgccacaagacctggccattgtggactggccgagaagcagcactgtggccctgttaatcctctgctgggagccgccacacctacaggcaacaacaagagaagaaagctgtgcagcggcaacaccacacctatcattcacctgaagggcgacagaaacagcctgaagtgcctgcggtacagactgaggaagcacagcgatcactaccgggacatcagctccacctggcactggacaggtgctggcaacgaaaagaccggcatcctgacagtgacctaccacagcgagactcagcggaccaagttcctgaacaccgtggctatccccgacagcgtgcagattctcgtgggctacatgaccatgggcagcggcgccaccaatttcagtctgcttaaacaggccggggacgtcgaagagaaccccggacctatgcatcggcgcagatctcggtcttgtagagaagaccaaaagcctgtcatggatgatcaaagagatttaatttctaataatgaacaattacccatgttgggacggcgccccggagcccccgaatctaagtgcagccggggagctttatatacaggattttctattttagtgaccttattattagctggccaagccacaacagcttatttcttataccaacaacaaggacggttagataaattaacagtcacatctcaaaatttacaattagagaatttaagaatgaaattacctaaaccacccaaacccgtcagtaaaatgagaatggctacccccttattaatgcaagccctccccatgggcgccttaccccaaggacccatgcaaaatgctacaaagtatggaaatatgacagaagatcatgtcatgcacttattacaaaacgctgaccccttaaaagtctatccccctttaaaaggatctttccctgaaaatttaagacatttaaaaaatacaatggagacaattgattggaaagtctttgaatcttggatgcatcattggttattatttgaaatgtctaggcattctttagagcaaaaacccaccgatgctccacccaaggaaagtttagagttagaggacccttctagcggattaggagtcaccaaacaggacttaggacccgtccccatgatggccagattcgaggaccctaccagacggccctacaagctgcctgatctgtgcaccgaactgaacaccagccttcaggatatcgagatcacctgtgtgtactgcaagaccgtgctcgagctgacagaagtgtttgagttcgccttcaaggacctgttcgtggtgtacagagacagcatccctcacgccgcctgtcacaagtgcatcgacttctacagcagaatcagagagctgcggcactacagcgactccgtgtacggcgataccctggaaaaactgaccaacaccggactgtacaacctgctgatccggtgcctgagatgccagaaacctcagaaccccgccgagaaactgagacatctgaacgagaagcggcggttccacaatatcgccggccactacagaggccagtgccacagctgttgcaaccgggccagacaagaaagactccagcggagaagaggcagcatgcacggacctaaagccacacttcaggacatcgtgctgcacctcgagcctcagaatgagatccccgtggatctgctcggccatgagcagctgagcgatagcgaggaagagaacgacgagatcgacggcgtcaaccaccagcatctgcctgccagaagggccgaacctcagagacacaccatgctgtgcatgtgctgcaagtgcgaggcccggatcgagagagtggtggaatctagcgccgacgacctgagagctttccagcagctgttcctgaatactctgagcttcgtggccccttggtgcgctagtcagcagtgaggaagaatgtgcacagtgctaaccagaaaattcaggacaagactagtgcggccgctttggaaagttttataggtagttgatagaacaaaatacataattttgtaaaaataaatcactttttat

SEQ ID NO: 82 - DNA, 4157 bp, Artificial Sequence
  HPV18 E1E2E6E7 integrated into DelIII locus of the poxviral vector
aaaaattaaaattttattttttttttttggaatataaataagatctatccctatcagtgatagagatctccctatcagtgatagagatcgtcgacgagctcgtttagtgaaccgtcagatcgcctggagacgccatccacgctgttttgacctctagcaccggtgccaccatggccgatcctgagggaacagatggcgaaggcacaggctgcaacggctggttttacgtgcaagccatcgtggacaagaagaccggcgacgtcatcagcgacgacgaggatgagaatgccaccgacaccggcagcgacatggtggactttatcgatacccagggcacgttctgcgagcaggccgaactggaaacagcccaggcactgtttcacgcccaagaggtgcacaacgatgcccaggtgctgcacgtgctgaagagaaagtttgccggcggaagcaccgagaacagcccactgggagaaagactggaagtggacaccgagctgagccccagactgcaagagatcagcctgaacagcggccagaagaaggccaagcggagactgttcaccatctccgacagcggctacggctgtagcgaagtggaagccacacagatccaagtgaccaccaatggcgagcacggcggcaatgtttgttctggcggatctaccgaggccatcgacaatggcggaaccgagggcaacaatagctccgtggatggcaccagcgacaacagcaacatcgagaacgtgaaccctcagtgcacaatcgcccagctgaaggacctgctgaaagtgaacaacaagcagggcgccatgctggccgtgtttaaggatacctacggcctgagcttcaccgacctcgtgcggaacttcaagagcgacaagaccacctgtaccgactgggtcaccgccatctttggcgtgaacccaacaatcgccgagggcttcaagaccctgatccagcctttcatcctgtacgcccacatccagtgtctggactgcaaatggggcgtgctgattctggccctgctgagatacaagtgcggcaagagcagactgaccgtggccaagggactgagcactctgctgcatgtgcccgagacatgcatgctgattcagcctccaaagctgcggtctagcgtggccgctctgtactggtacagaaccggcatcagcaatatcagcgaagtgatgggcgacacccctgagtggattcagcggctgacaatcatccagcacggcatcgacgactccaacttcgacctgagcgagatggtgcagtgggccttcgataacgagctgaccgacgagtccgacatggcctttgaatacgccctgctggcagacagcaactccaatgccgccgctttcctgaagtccaactgccaggccaagtacctgaaggactgcgccaccatgtgcaagcactaccgcagagcacagaaacggcagatgaacatgagccagtggatccggttccggtgcagcaagatcgatgaaggtggcgactggcggcctatcgtgcagttcctgagataccagcagatcgagttcatcacctttctgggcgccctgaagtcattcctgaagggaacccctaaaaagaactgcctggtgttctgcggccctgccaataccggcaagtcctacttcggcatgagctttatccacttcatccagggcgccgtgatcagcttcgtgaacagcaccagccacttttggctggaacccctgaccgataccaaggtggcaatgctggacgacgccaccaccacctgttggacctacttcgacacctacatgcggaacgccctggacggcaaccccatcagcatcgacagaaagcacaagcccctcatccagctgaaatgccctccaatcctgctgaccacaaacattcaccccgccaaggacaatcggtggccctacctggaaagccggatcaccgtgttcgagttccccaacgcctttccattcgacaagaacggcaatcccgtgtacgagatcaacgacaagaattggaagtgcttcttcgagcggacctggtccagactggatctgcacgaggaagaagaggacgccgacacagagggcaatcccttcggcacctttaagtgtgtggccgggcagaatcacagacccctgggatctatgcagaccccaaaagagacactgagcgagcggctgagcgccctccaggacaagatcatcgaccactacgagaacgacagcaaggacatcgacagccagattcagtactggcagctgatcagatgggagaacgccatcttcttcgccgctagagagcacggaattcagaccctgaaccaccaggtggtgcccgcctacaacatcagcaagagcaaggcccacaaggccattgaactccagatggccctgcaaggactggctcagagcgcctacaagaccgaggattggacactccaggatacctgcgaggaactgtggaacacagagcccacacactgcttcaagaaaggcggccagaccgtgcaggtctacttcgatggcaacaaggataactgcatgacctacgtggcctgggacagcgtgtactacatgacagatgccggcacctgggacaagaccgccacctgtgtttctcaccggggcctgtactacgtgaaagagggctacaacaccttctacatcgagtttaagagcgagtgcgagaagtatggcaacaccggcacatgggaagtgcatttcggcaacaacgtgatcgactgcaacgactccatgtgctccacctccgatgacaccgtgtctgccacacagctggtcaagcagctccagcacaccccatctccatacagctctacagtgtctgtgggcaccgccaagacctatggccaaacaagcgctgccacaagacctggccattgtggactggccgagaagcagcactgtggccctgttaatcctctgctgggagccgccacacctacaggcaacaacaagagaagaaagctgtgcagcggcaacaccacacctatcattcacctgaagggcgacagaaacagcctgaagtgcctgcggtacagactgaggaagcacagcgatcactaccgggacatcagctccacctggcactggacaggtgctggcaacgaaaagaccggcatcctgacagtgacctaccacagcgagactcagcggaccaagttcctgaacaccgtggctatccccgacagcgtgcagattctcgtgggctacatgaccatgggcagcatggccagattcgaggaccctaccagacggccctacaagctgcctgatctgtgcaccgaactgaacaccagccttcaggatatcgagatcacctgtgtgtactgcaagaccgtgctcgagctgacagaagtgtttgagttcgccttcaaggacctgttcgtggtgtacagagacagcatccctcacgccgcctgtcacaagtgcatcgacttctacagcagaatcagagagctgcggcactacagcgactccgtgtacggcgataccctggaaaaactgaccaacaccggactgtacaacctgctgatccggtgcctgagatgccagaaacctcagaaccccgccgagaaactgagacatctgaacgagaagcggcggttccacaatatcgccggccactacagaggccagtgccacagctgttgcaaccgggccagacaagaaagactccagcggagaagaggcagcatgcacggacctaaagccacacttcaggacatcgtgctgcacctcgagcctcagaatgagatccccgtggatctgctcggccatgagcagctgagcgatagcgaggaagagaacgacgagatcgacggcgtcaaccaccagcatctgcctgccagaagggccgaacctcagagacacaccatgctgtgcatgtgctgcaagtgcgaggcccggatcgagagagtggtggaatctagcgccgacgacctgagagctttccagcagctgttcctgaatactctgagcttcgtggccccttggtgcgctagtcagcagtgaggaagaatgtgcacagtgctaaccagaaaattcaggacaagactagtgcggccgctttggaaagttttataggtagttgatagaacaaaatacataattttgtaaaaataaatcactttttat

SEQ ID NO: 83 - DNA, 5609 bp, Artificial Sequence
  HPV18 Ii-E1E6E7-p2a-Ii-E2 integrated into DelIII locus of the poxviral vector
aaaaattaaaattttattttttttttttggaatataaataagatctatccctatcagtgatagagatctccctatcagtgatagagatcgtcgacgagctcgtttagtgaaccgtcagatcgcctggagacgccatccacgctgttttgacctctagcaccggtgccaccatgcacagaaggcggagcagaagctgccgcgaggatcagaaacccgtgatggacgaccagcgggacctgatcagcaacaacgagcagctgcctatgctcggcagaaggcctggcgctcctgagagcaaatgttctagaggcgccctgtacaccggcttcagcatcctggttacactgctgctggccggacaggctaccaccgcctactttctgtatcagcagcagggcagactggacaagctgaccgtgaccagccagaacctgcagctggaaaacctgcggatgaagctgcccaagcctcctaagcctgtgtccaagatgcggatggccacacctctgctgatgcaggctttgcctatgggagcactgcctcagggccctatgcagaacgccaccaaatacggcaacatgaccgaggaccacgtgatgcatctgctgcagaatgccgatcctctgaaggtgtaccctccactgaagggcagctttcccgagaacctgcggcacctgaagaacaccatggaaaccatcgactggaaggtgttcgagagctggatgcaccactggctgctgttcgagatgagccggcacagcctggaacagaagcctacagacgcccctcctaaagagtccctggaactggaagatcccagctctggcctgggcgtgacaaagcaagatctgggccctgtgcctatgatggccgatcctgagggaacagatggcgaaggcacaggctgcaacggctggttttacgtgcaagccatcgtggacaagaagaccggcgacgtcatcagcgacgacgaggatgagaatgccaccgacaccggcagcgacatggtggactttatcgatacccagggcacgttctgcgagcaggccgaactggaaacagcccaggcactgtttcacgcccaagaggtgcacaacgatgcccaggtgctgcacgtgctgaagagaaagtttgccggcggaagcaccgagaacagcccactgggagaaagactggaagtggacaccgagctgagccccagactgcaagagatcagcctgaacagcggccagaagaaggccaagcggagactgttcaccatctccgacagcggctacggctgtagcgaagtggaagccacacagatccaagtgaccaccaatggcgagcacggcggcaatgtttgttctggcggatctaccgaggccatcgacaatggcggaaccgagggcaacaatagctccgtggatggcaccagcgacaacagcaacatcgagaacgtgaaccctcagtgcacaatcgcccagctgaaggacctgctgaaagtgaacaacaagcagggcgccatgctggccgtgtttaaggatacctacggcctgagcttcaccgacctcgtgcggaacttcaagagcgacaagaccacctgtaccgactgggtcaccgccatctttggcgtgaacccaacaatcgccgagggcttcaagaccctgatccagcctttcatcctgtacgcccacatccagtgtctggactgcaaatggggcgtgctgattctggccctgctgagatacaagtgcggcaagagcagactgaccgtggccaagggactgagcactctgctgcatgtgcccgagacatgcatgctgattcagcctccaaagctgcggtctagcgtggccgctctgtactggtacagaaccggcatcagcaatatcagcgaagtgatgggcgacacccctgagtggattcagcggctgacaatcatccagcacggcatcgacgactccaacttcgacctgagcgagatggtgcagtgggccttcgataacgagctgaccgacgagtccgacatggcctttgaatacgccctgctggcagacagcaactccaatgccgccgctttcctgaagtccaactgccaggccaagtacctgaaggactgcgccaccatgtgcaagcactaccgcagagcacagaaacggcagatgaacatgagccagtggatccggttccggtgcagcaagatcgatgaaggtggcgactggcggcctatcgtgcagttcctgagataccagcagatcgagttcatcacctttctgggcgccctgaagtcattcctgaagggaacccctaaaaagaactgcctggtgttctgcggccctgccaataccggcaagtcctacttcggcatgagctttatccacttcatccagggcgccgtgatcagcttcgtgaacagcaccagccacttttggctggaacccctgaccgataccaaggtggcaatgctggacgacgccaccaccacctgttggacctacttcgacacctacatgcggaacgccctggacggcaaccccatcagcatcgacagaaagcacaagcccctcatccagctgaaatgccctccaatcctgctgaccacaaacattcaccccgccaaggacaatcggtggccctacctggaaagccggatcaccgtgttcgagttccccaacgcctttccattcgacaagaacggcaatcccgtgtacgagatcaacgacaagaattggaagtgcttcttcgagcggacctggtccagactggatctgcacgaggaagaagaggacgccgacacagagggcaatcccttcggcacctttaagtgtgtggccgggcagaatcacagacccctgggcagcatggccagattcgaggaccctaccagacggccctacaagctgcctgatctgtgcaccgaactgaacaccagccttcaggatatcgagatcacctgtgtgtactgcaagaccgtgctcgagctgacagaagtgtttgagttcgccttcaaggacctgttcgtggtgtacagagacagcatccctcacgccgcctgtcacaagtgcatcgacttctacagcagaatcagagagctgcggcactacagcgactccgtgtacggcgataccctggaaaaactgaccaacaccggactgtacaacctgctgatccggtgcctgagatgccagaaacctcagaaccccgccgagaaactgagacatctgaacgagaagcggcggttccacaatatcgccggccactacagaggccagtgccacagctgttgcaaccgggccagacaagaaagactccagcggagaagaggcagcatgcacggacctaaagccacacttcaggacatcgtgctgcacctcgagcctcagaatgagatccccgtggatctgctcggccatgagcagctgagcgatagcgaggaagagaacgacgagatcgacggcgtcaaccaccagcatctgcctgccagaagggccgaacctcagagacacaccatgctgtgcatgtgctgcaagtgcgaggcccggatcgagagagtggtggaatctagcgccgacgacctgagagctttccagcagctgttcctgaatactctgagcttcgtggccccttggtgcgctagtcagcagggcagcggcgccaccaatttcagtctgcttaaacaggccggggacgtcgaagagaaccccggacctatgcatcggcgcagatctcggtcttgtagagaagaccaaaagcctgtcatggatgatcaaagagatttaatttctaataatgaacaattacccatgttgggacggcgccccggagcccccgaatctaagtgcagccggggagctttatatacaggattttctattttagtgaccttattattagctggccaagccacaacagcttatttcttataccaacaacaaggacggttagataaattaacagtcacatctcaaaatttacaattagagaatttaagaatgaaattacctaaaccacccaaacccgtcagtaaaatgagaatggctacccccttattaatgcaagccctccccatgggcgccttaccccaaggacccatgcaaaatgctacaaagtatggaaatatgacagaagatcatgtcatgcacttattacaaaacgctgaccccttaaaagtctatccccctttaaaaggatctttccctgaaaatttaagacatttaaaaaatacaatggagacaattgattggaaagtctttgaatcttggatgcatcattggttattatttgaaatgtctaggcattctttagagcaaaaacccaccgatgctccacccaaggaaagtttagagttagaggacccttctagcggattaggagtcaccaaacaggacttaggacccgtccccatgatgcagaccccaaaagagacactgagcgagcggctgagcgccctccaggacaagatcatcgaccactacgagaacgacagcaaggacatcgacagccagattcagtactggcagctgatcagatgggagaacgccatcttcttcgccgctagagagcacggaattcagaccctgaaccaccaggtggtgcccgcctacaacatcagcaagagcaaggcccacaaggccattgaactccagatggccctgcaaggactggctcagagcgcctacaagaccgaggattggacactccaggatacctgcgaggaactgtggaacacagagcccacacactgcttcaagaaaggcggccagaccgtgcaggtctacttcgatggcaacaaggataactgcatgacctacgtggcctgggacagcgtgtactacatgacagatgccggcacctgggacaagaccgccacctgtgtttctcaccggggcctgtactacgtgaaagagggctacaacaccttctacatcgagtttaagagcgagtgcgagaagtatggcaacaccggcacatgggaagtgcatttcggcaacaacgtgatcgactgcaacgactccatgtgctccacctccgatgacaccgtgtctgccacacagctggtcaagcagctccagcacaccccatctccatacagctctacagtgtctgtgggcaccgccaagacctatggccaaacaagcgctgccacaagacctggccattgtggactggccgagaagcagcactgtggccctgttaatcctctgctgggagccgccacacctacaggcaacaacaagagaagaaagctgtgcagcggcaacaccacacctatcattcacctgaagggcgacagaaacagcctgaagtgcctgcggtacagactgaggaagcacagcgatcactaccgggacatcagctccacctggcactggacaggtgctggcaacgaaaagaccggcatcctgacagtgacctaccacagcgagactcagcggaccaagttcctgaacaccgtggctatccccgacagcgtgcagattctcgtgggctacatgaccatgtgaggaagaatgtgcacagtgctaaccagaaaattcaggacaagactagtgcggccgctttggaaagttttataggtagttgatagaacaaaatacataattttgtaaaaataaatcactttttat

SEQ ID NO: 84 - DNA, 3752 bp, Artificial Sequence
  HPV18 Ii-E1E6E7 integrated into DelIII locus of the poxviral vector
aaaaattaaaattttattttttttttttggaatataaataagatctatccctatcagtgatagagatctccctatcagtgatagagatcgtcgacgagctcgtttagtgaaccgtcagatcgcctggagacgccatccacgctgttttgacctctagcaccggtgccaccatgcacagaaggcggagcagaagctgccgcgaggatcagaaacccgtgatggacgaccagcgggacctgatcagcaacaacgagcagctgcctatgctcggcagaaggcctggcgctcctgagagcaaatgttctagaggcgccctgtacaccggcttcagcatcctggttacactgctgctggccggacaggctaccaccgcctactttctgtatcagcagcagggcagactggacaagctgaccgtgaccagccagaacctgcagctggaaaacctgcggatgaagctgcccaagcctcctaagcctgtgtccaagatgcggatggccacacctctgctgatgcaggctttgcctatgggagcactgcctcagggccctatgcagaacgccaccaaatacggcaacatgaccgaggaccacgtgatgcatctgctgcagaatgccgatcctctgaaggtgtaccctccactgaagggcagctttcccgagaacctgcggcacctgaagaacaccatggaaaccatcgactggaaggtgttcgagagctggatgcaccactggctgctgttcgagatgagccggcacagcctggaacagaagcctacagacgcccctcctaaagagtccctggaactggaagatcccagctctggcctgggcgtgacaaagcaagatctgggccctgtgcctatgatggccgatcctgagggaacagatggcgaaggcacaggctgcaacggctggttttacgtgcaagccatcgtggacaagaagaccggcgacgtcatcagcgacgacgaggatgagaatgccaccgacaccggcagcgacatggtggactttatcgatacccagggcacgttctgcgagcaggccgaactggaaacagcccaggcactgtttcacgcccaagaggtgcacaacgatgcccaggtgctgcacgtgctgaagagaaagtttgccggcggaagcaccgagaacagcccactgggagaaagactggaagtggacaccgagctgagccccagactgcaagagatcagcctgaacagcggccagaagaaggccaagcggagactgttcaccatctccgacagcggctacggctgtagcgaagtggaagccacacagatccaagtgaccaccaatggcgagcacggcggcaatgtttgttctggcggatctaccgaggccatcgacaatggcggaaccgagggcaacaatagctccgtggatggcaccagcgacaacagcaacatcgagaacgtgaaccctcagtgcacaatcgcccagctgaaggacctgctgaaagtgaacaacaagcagggcgccatgctggccgtgtttaaggatacctacggcctgagcttcaccgacctcgtgcggaacttcaagagcgacaagaccacctgtaccgactgggtcaccgccatctttggcgtgaacccaacaatcgccgagggcttcaagaccctgatccagcctttcatcctgtacgcccacatccagtgtctggactgcaaatggggcgtgctgattctggccctgctgagatacaagtgcggcaagagcagactgaccgtggccaagggactgagcactctgctgcatgtgcccgagacatgcatgctgattcagcctccaaagctgcggtctagcgtggccgctctgtactggtacagaaccggcatcagcaatatcagcgaagtgatgggcgacacccctgagtggattcagcggctgacaatcatccagcacggcatcgacgactccaacttcgacctgagcgagatggtgcagtgggccttcgataacgagctgaccgacgagtccgacatggcctttgaatacgccctgctggcagacagcaactccaatgccgccgctttcctgaagtccaactgccaggccaagtacctgaaggactgcgccaccatgtgcaagcactaccgcagagcacagaaacggcagatgaacatgagccagtggatccggttccggtgcagcaagatcgatgaaggtggcgactggcggcctatcgtgcagttcctgagataccagcagatcgagttcatcacctttctgggcgccctgaagtcattcctgaagggaacccctaaaaagaactgcctggtgttctgcggccctgccaataccggcaagtcctacttcggcatgagctttatccacttcatccagggcgccgtgatcagcttcgtgaacagcaccagccacttttggctggaacccctgaccgataccaaggtggcaatgctggacgacgccaccaccacctgttggacctacttcgacacctacatgcggaacgccctggacggcaaccccatcagcatcgacagaaagcacaagcccctcatccagctgaaatgccctccaatcctgctgaccacaaacattcaccccgccaaggacaatcggtggccctacctggaaagccggatcaccgtgttcgagttccccaacgcctttccattcgacaagaacggcaatcccgtgtacgagatcaacgacaagaattggaagtgcttcttcgagcggacctggtccagactggatctgcacgaggaagaagaggacgccgacacagagggcaatcccttcggcacctttaagtgtgtggccgggcagaatcacagacccctgggcagcatggccagattcgaggaccctaccagacggccctacaagctgcctgatctgtgcaccgaactgaacaccagccttcaggatatcgagatcacctgtgtgtactgcaagaccgtgctcgagctgacagaagtgtttgagttcgccttcaaggacctgttcgtggtgtacagagacagcatccctcacgccgcctgtcacaagtgcatcgacttctacagcagaatcagagagctgcggcactacagcgactccgtgtacggcgataccctggaaaaactgaccaacaccggactgtacaacctgctgatccggtgcctgagatgccagaaacctcagaaccccgccgagaaactgagacatctgaacgagaagcggcggttccacaatatcgccggccactacagaggccagtgccacagctgttgcaaccgggccagacaagaaagactccagcggagaagaggcagcatgcacggacctaaagccacacttcaggacatcgtgctgcacctcgagcctcagaatgagatccccgtggatctgctcggccatgagcagctgagcgatagcgaggaagagaacgacgagatcgacggcgtcaaccaccagcatctgcctgccagaagggccgaacctcagagacacaccatgctgtgcatgtgctgcaagtgcgaggcccggatcgagagagtggtggaatctagcgccgacgacctgagagctttccagcagctgttcctgaatactctgagcttcgtggccccttggtgcgctagtcagcagtgaggaagaatgtgcacagtgctaaccagaaaattcaggacaagactagtgcggccgctttggaaagttttataggtagttgatagaacaaaatacataattttgtaaaaataaatcactttttat

SEQ ID NO: 85 - DNA, 4684 bp, Artificial Sequence
  MfPV3 Ii-E1E2E6E7 integrated into TK locus of the poxviral vector
ggccaaaaattgaaattttattttttttttttggaatataaataatccctatcagtgatagagatctccctatcagtgatagagatcgtcgacgagctcgtttagtgaaccgtcagatcgcctggagacgccatccacgctgttttgacctctagcaccggtgccaccatgcacagaaggcggagcagaagctgccgcgaggatcagaaacccgtgatggacgaccagcgggacctgatcagcaacaacgagcagctgcctatgctcggcagaaggcctggcgctcctgagagcaaatgttctagaggcgccctgtacaccggcttcagcatcctggttacactgctgctggccggacaggctaccaccgcctactttctgtatcagcagcagggcagactggacaagctgaccgtgaccagccagaacctgcagctggaaaacctgcggatgaagctgcccaagcctcctaagcctgtgtccaagatgcggatggccacacctctgctgatgcaggctttgcctatgggagcactgcctcagggccctatgcagaacgccaccaaatacggcaacatgaccgaggaccacgtgatgcatctgctgcagaatgccgatcctctgaaggtgtaccctccactgaagggcagctttcccgagaacctgcggcacctgaagaacaccatggaaaccatcgactggaaggtgttcgagagctggatgcaccactggctgctgttcgagatgagccggcacagcctggaacagaagcctacagacgcccctcctaaagagtccctggaactggaagatcccagctctggcctgggcgtgacaaagcaagatctgggccctgtgcctatgatggacccttctggaattcacggcgagggcaccagatgcaccggatggttcgatgtggaagccatcgtggaaagacggaccggcgacgtggtgtccgaggacgaagatgagaacctggaagataccggcgtggacctggtggacttcatcgacgatacctgcgagtttgagcaggccggcgacgaagctcctagagcactgctgcatgcccaagagacacaggcccatgtgaacgccgtgcactacctgaagcggaagttcacatgcagccctaccgtgtctcccctgggcaatgtgcagtgttctatcgagggcgagctgagccctagactgcacgccatccaactgaatgaaggcagcggcaaggccaagcggagactgtttctgcctgatagcggctacggcaataccgaggtggaaacccagctgtctcaggtggcaggatccgatggcgaatctcaagcccctggcggcaaagaaaatgtgcagcctgctgaaggcgctggcggagatgttcgacagctgctgagaagcagcaacctgaaggccacactgctgggcaagttcaaggacgtgtacggcatcggcttcaacgaactcgtgcggtgcttcaagagcgacaagaccgtgtgcaccgattgggttgtgggagctgctggcgtgcaccattctgtggccgaaggactgaagcacctgatcgagcctttctgcacatacgcccacatgcagtgcctgacctgcaactggggagtgtttctgctgctgctcatccggttcaagtgcggcaagaacagactgaccgtggccaagtgcatctctaccctgctgaacgtgcaagagccctacctgctgatcgaacctccaaagctgagatccacagccgccgctctgtactggtacagaaccggcatcagcaacgtgtccgaagtgatcggagagcctcctgagtggatcgtgcggcagaccatgtttcagcacagcctcgaggacagcatcttcgacctgtctcagatggtgcagtgggcctacgaccacgatctggtggacgatagcgccattgcctaccagtatgcccagctggccgacgtggactctaatgccgccgctttcctgaagtctaacgctcaggccaaatacgtgaaggactgcgccaccatgtgcagacactacaagagagccgagaagcaggccatgaccatgagccagtggatcagagccagatgcgataagaccgacgacggcggagattggaggcctatcgtgcagttcctgagataccagaacgtcgagttcatcacctttctgagcgcctttaaggccttcctgaagggaatccccaagagaagctgcatcgtgctgtacggccctccaaacaccggcaagagctacttcggaatgagcctgatgcagtttctgcagggcagcatcatcagctacgtgaacagcaacagccacttttggctggcccctctggccgaagctaaagtggccatgctggacgatgccacaccacagtgctggtcctacatcgacacctacatgcggagcgtgctggacggcaaccccatgagcattgaccggaagcacaagaacctgatccagatgaagtgtccgcctctgatcatcaccagcaacaccaacgtgggcgaagatgacagatggcgctacctgcactccagagtggtggtgttcaagttcgagcagacctttccattcgaccagaacggcaatcccgtgtacgagctgtccgacaagaattggaagtccttcttcagccggacctggtccagactcgagctgcaagaggatgaggacaccgagcaggatggctctacagtgcgggcctttaagtgtgtgcccggccagaacaccaatatcctgggctctatggaagccctgagcgagagactgaacgcctaccaggacaagatcctgaccttctacgaagaggactccaaggacctgagggaccagatcgagcattggagatgtgtgcggggagagtgcgccgtgttctacaaggccagagagatgggccacagccacatcaaccaccagcaggttccacctctgcacgtgtccagaggcaaggcccacaatgccattgagctgcagatggccctggaaagcctgaaccagagcgacttcaacaccgaggaatggaccctgcaggacacaagcctggaaatgtggcggaccgagcctcagtgctgcttcaaaaagaaaggcgagacagtgaccgtgctgtatgactgcgacaaggacaacagcatggactacaccctgtggggccacgtgtacgtgtggggagatacaggctgggacaaagtgtgcggaaaggtggactacggcggcctgtactatgtgctgcacggcctgaaagtgtactacgttgagttccagcaagaggccgtgaagtacagcaagaccaacaagtgggaagtgcatatcggcagaacagtgatcccctacagcgagtccgtgtcctctacagccctgtgcgaaagagtgcctatcgccgagatcgccaatggcctccagcagaccagcattccctctcacacacacgccaccaccaaagagaacgcttgggtttcctctcagcctcctaccaagcggtccagaagatctgatccaggcggcgatcctgtcagagccctggatgccaatagcagaaccctgctgtctggaaccgcctgcgagaataccaccggcaactcttacagcgactgcacccctgtggtgcacctgaaaggcgaccccaattgtctgaaggccctgcggttcagattcgtgaaacacaagaatctgttcgtgaacgtgtcctccacctggcggtggaccaacaacaccgaagagaaggccatcgtgactgtgacctttaaggacgagcagcagagacagcagttcctcggcagcgtgaagatccccaactccatctgtgtgtgcaagggcgtgatgacagttggcagcatggtggaaggcagccaagagagagcccggacactgcacgaactgtgcgagcagagagaacagacccagcacgacatcgagctggactgcgtgtactgcctgaatcctctgaccagaaccgaggtgtacgacttcgccagatgggagctgagaatcgtgtacagacgggataccgcctacggcgtgtgcaagctgtgcctgaggttccacagcaaagtgcggaagtacaggcggtacaactactccatctacggccccacactggaacggcggacaaagaagcagctcgaagaactcgtgatccggtgctactgctgccagaaacctcagtgccccgtggaaaagcagcgccacgttgaccagggccagagattccacaacattgccgagcagtggaccggcagatgcctgcaatgttggaggccaacagccgctgaaaccggctctatgatcggccctggacctacactgcaggatatcgtgcttgagctggaacccgagcctgtggacctgagaggatatgagcagctggactccagcgaggacgaggacgagattgaccaccaccaacagcaggacagacccgatgtgcaagaagatgacggcgagcggtttagaatcctgagcgactgtcacgtgtgccagaataccgtgtcaagagtggtgcacagcacccacgacgacctgcacattctcgaggacctgcttatgggcaccctcgagatcgtggcccctaattgtgccgtgggcagcgaacagaaactgatctccgaggaagatctctgaggaagaatgtgcacagtgctaaccagaaaattcaggacaagactagtgcggccgcttttat

SEQ ID NO: 86 - DNA, 5440 bp, Artificial Sequence
  MfPV3 Ii-E1E2-p2a-Ii-E6E7 integrated into TK locus of the poxviral vector
ggccaaaaattgaaattttattttttttttttggaatataaataatccctatcagtgatagagatctccctatcagtgatagagatcgtcgacgagctcgtttagtgaaccgtcagatcgcctggagacgccatccacgctgttttgacctctagcaccggtgccaccatgcacagaaggcggagcagaagctgccgcgaggatcagaaacccgtgatggacgaccagcgggacctgatcagcaacaacgagcagctgcctatgctcggcagaaggcctggcgctcctgagagcaaatgttctagaggcgccctgtacaccggcttcagcatcctggttacactgctgctggccggacaggctaccaccgcctactttctgtatcagcagcagggcagactggacaagctgaccgtgaccagccagaacctgcagctggaaaacctgcggatgaagctgcccaagcctcctaagcctgtgtccaagatgcggatggccacacctctgctgatgcaggctttgcctatgggagcactgcctcagggccctatgcagaacgccaccaaatacggcaacatgaccgaggaccacgtgatgcatctgctgcagaatgccgatcctctgaaggtgtaccctccactgaagggcagctttcccgagaacctgcggcacctgaagaacaccatggaaaccatcgactggaaggtgttcgagagctggatgcaccactggctgctgttcgagatgagccggcacagcctggaacagaagcctacagacgcccctcctaaagagtccctggaactggaagatcccagctctggcctgggcgtgacaaagcaagatctgggccctgtgcctatgatggacccttctggaattcacggcgagggcaccagatgcaccggatggttcgatgtggaagccatcgtggaaagacggaccggcgacgtggtgtccgaggacgaagatgagaacctggaagataccggcgtggacctggtggacttcatcgacgatacctgcgagtttgagcaggccggcgacgaagctcctagagcactgctgcatgcccaagagacacaggcccatgtgaacgccgtgcactacctgaagcggaagttcacatgcagccctaccgtgtctcccctgggcaatgtgcagtgttctatcgagggcgagctgagccctagactgcacgccatccaactgaatgaaggcagcggcaaggccaagcggagactgtttctgcctgatagcggctacggcaataccgaggtggaaacccagctgtctcaggtggcaggatccgatggcgaatctcaagcccctggcggcaaagaaaatgtgcagcctgctgaaggcgctggcggagatgttcgacagctgctgagaagcagcaacctgaaggccacactgctgggcaagttcaaggacgtgtacggcatcggcttcaacgaactcgtgcggtgcttcaagagcgacaagaccgtgtgcaccgattgggttgtgggagctgctggcgtgcaccattctgtggccgaaggactgaagcacctgatcgagcctttctgcacatacgcccacatgcagtgcctgacctgcaactggggagtgtttctgctgctgctcatccggttcaagtgcggcaagaacagactgaccgtggccaagtgcatctctaccctgctgaacgtgcaagagccctacctgctgatcgaacctccaaagctgagatccacagccgccgctctgtactggtacagaaccggcatcagcaacgtgtccgaagtgatcggagagcctcctgagtggatcgtgcggcagaccatgtttcagcacagcctcgaggacagcatcttcgacctgtctcagatggtgcagtgggcctacgaccacgatctggtggacgatagcgccattgcctaccagtatgcccagctggccgacgtggactctaatgccgccgctttcctgaagtctaacgctcaggccaaatacgtgaaggactgcgccaccatgtgcagacactacaagagagccgagaagcaggccatgaccatgagccagtggatcagagccagatgcgataagaccgacgacggcggagattggaggcctatcgtgcagttcctgagataccagaacgtcgagttcatcacctttctgagcgcctttaaggccttcctgaagggaatccccaagagaagctgcatcgtgctgtacggccctccaaacaccggcaagagctacttcggaatgagcctgatgcagtttctgcagggcagcatcatcagctacgtgaacagcaacagccacttttggctggcccctctggccgaagctaaagtggccatgctggacgatgccacaccacagtgctggtcctacatcgacacctacatgcggagcgtgctggacggcaaccccatgagcattgaccggaagcacaagaacctgatccagatgaagtgtccgcctctgatcatcaccagcaacaccaacgtgggcgaagatgacagatggcgctacctgcactccagagtggtggtgttcaagttcgagcagacctttccattcgaccagaacggcaatcccgtgtacgagctgtccgacaagaattggaagtccttcttcagccggacctggtccagactcgagctgcaagaggatgaggacaccgagcaggatggctctacagtgcgggcctttaagtgtgtgcccggccagaacaccaatatcctgggctctatggaagccctgagcgagagactgaacgcctaccaggacaagatcctgaccttctacgaagaggactccaaggacctgagggaccagatcgagcattggagatgtgtgcggggagagtgcgccgtgttctacaaggccagagagatgggccacagccacatcaaccaccagcaggttccacctctgcacgtgtccagaggcaaggcccacaatgccattgagctgcagatggccctggaaagcctgaaccagagcgacttcaacaccgaggaatggaccctgcaggacacaagcctggaaatgtggcggaccgagcctcagtgctgcttcaaaaagaaaggcgagacagtgaccgtgctgtatgactgcgacaaggacaacagcatggactacaccctgtggggccacgtgtacgtgtggggagatacaggctgggacaaagtgtgcggaaaggtggactacggcggcctgtactatgtgctgcacggcctgaaagtgtactacgttgagttccagcaagaggccgtgaagtacagcaagaccaacaagtgggaagtgcatatcggcagaacagtgatcccctacagcgagtccgtgtcctctacagccctgtgcgaaagagtgcctatcgccgagatcgccaatggcctccagcagaccagcattccctctcacacacacgccaccaccaaagagaacgcttgggtttcctctcagcctcctaccaagcggtccagaagatctgatccaggcggcgatcctgtcagagccctggatgccaatagcagaaccctgctgtctggaaccgcctgcgagaataccaccggcaactcttacagcgactgcacccctgtggtgcacctgaaaggcgaccccaattgtctgaaggccctgcggttcagattcgtgaaacacaagaatctgttcgtgaacgtgtcctccacctggcggtggaccaacaacaccgaagagaaggccatcgtgactgtgacctttaaggacgagcagcagagacagcagttcctcggcagcgtgaagatccccaactccatctgtgtgtgcaagggcgtgatgacagttggcagcggcgccaccaatttcagtctgcttaaacaggccggggacgtcgaagagaaccccggacctatgcatcggcgcagatctcggtcttgtagagaagaccaaaagcctgtcatggatgatcaaagagatttaatttctaataatgaacaattacccatgttgggacggcgccccggagcccccgaatctaagtgcagccggggagctttatatacaggattttctattttagtgaccttattattagctggccaagccacaacagcttatttcttataccaacaacaaggacggttagataaattaacagtcacatctcaaaatttacaattagagaatttaagaatgaaattacctaaaccacccaaacccgtcagtaaaatgagaatggctacccccttattaatgcaagccctccccatgggcgccttaccccaaggacccatgcaaaatgctacaaagtatggaaatatgacagaagatcatgtcatgcacttattacaaaacgctgaccccttaaaagtctatccccctttaaaaggatctttccctgaaaatttaagacatttaaaaaatacaatggagacaattgattggaaagtctttgaatcttggatgcatcattggttattatttgaaatgtctaggcattctttagagcaaaaacccaccgatgctccacccaaggaaagtttagagttagaggacccttctagcggattaggagtcaccaaacaggacttaggacccgtccccatgatggtggaaggcagccaagagagagcccggacactgcacgaactgtgcgagcagagagaacagacccagcacgacatcgagctggactgcgtgtactgcctgaatcctctgaccagaaccgaggtgtacgacttcgccagatgggagctgagaatcgtgtacagacgggataccgcctacggcgtgtgcaagctgtgcctgaggttccacagcaaagtgcggaagtacaggcggtacaactactccatctacggccccacactggaacggcggacaaagaagcagctcgaagaactcgtgatccggtgctactgctgccagaaacctcagtgccccgtggaaaagcagcgccacgttgaccagggccagagattccacaacattgccgagcagtggaccggcagatgcctgcaatgttggaggccaacagccgctgaaaccggctctatgatcggccctggacctacactgcaggatatcgtgcttgagctggaacccgagcctgtggacctgagaggatatgagcagctggactccagcgaggacgaggacgagattgaccaccaccaacagcaggacagacccgatgtgcaagaagatgacggcgagcggtttagaatcctgagcgactgtcacgtgtgccagaataccgtgtcaagagtggtgcacagcacccacgacgacctgcacattctcgaggacctgcttatgggcaccctcgagatcgtggcccctaattgtgccgtgggcagcgaacagaaactgatctccgaggaagatctctgaggaagaatgtgcacagtgctaaccagaaaattcaggacaagactagtgcggccgcttttat

SEQ ID NO: 87 - DNA, 3988 bp, Artificial Sequence
  MfPV3 E1E2E6E7 integrated into TK locus of the poxviral vector
ggccaaaaattgaaattttattttttttttttggaatataaataatccctatcagtgatagagatctccctatcagtgatagagatcgtcgacgagctcgtttagtgaaccgtcagatcgcctggagacgccatccacgctgttttgacctctagcaccggtgccaccatggacccttctggaattcacggcgagggcaccagatgcaccggatggttcgatgtggaagccatcgtggaaagacggaccggcgacgtggtgtccgaggacgaagatgagaacctggaagataccggcgtggacctggtggacttcatcgacgatacctgcgagtttgagcaggccggcgacgaagctcctagagcactgctgcatgcccaagagacacaggcccatgtgaacgccgtgcactacctgaagcggaagttcacatgcagccctaccgtgtctcccctgggcaatgtgcagtgttctatcgagggcgagctgagccctagactgcacgccatccaactgaatgaaggcagcggcaaggccaagcggagactgtttctgcctgatagcggctacggcaataccgaggtggaaacccagctgtctcaggtggcaggatccgatggcgaatctcaagcccctggcggcaaagaaaatgtgcagcctgctgaaggcgctggcggagatgttcgacagctgctgagaagcagcaacctgaaggccacactgctgggcaagttcaaggacgtgtacggcatcggcttcaacgaactcgtgcggtgcttcaagagcgacaagaccgtgtgcaccgattgggttgtgggagctgctggcgtgcaccattctgtggccgaaggactgaagcacctgatcgagcctttctgcacatacgcccacatgcagtgcctgacctgcaactggggagtgtttctgctgctgctcatccggttcaagtgcggcaagaacagactgaccgtggccaagtgcatctctaccctgctgaacgtgcaagagccctacctgctgatcgaacctccaaagctgagatccacagccgccgctctgtactggtacagaaccggcatcagcaacgtgtccgaagtgatcggagagcctcctgagtggatcgtgcggcagaccatgtttcagcacagcctcgaggacagcatcttcgacctgtctcagatggtgcagtgggcctacgaccacgatctggtggacgatagcgccattgcctaccagtatgcccagctggccgacgtggactctaatgccgccgctttcctgaagtctaacgctcaggccaaatacgtgaaggactgcgccaccatgtgcagacactacaagagagccgagaagcaggccatgaccatgagccagtggatcagagccagatgcgataagaccgacgacggcggagattggaggcctatcgtgcagttcctgagataccagaacgtcgagttcatcacctttctgagcgcctttaaggccttcctgaagggaatccccaagagaagctgcatcgtgctgtacggccctccaaacaccggcaagagctacttcggaatgagcctgatgcagtttctgcagggcagcatcatcagctacgtgaacagcaacagccacttttggctggcccctctggccgaagctaaagtggccatgctggacgatgccacaccacagtgctggtcctacatcgacacctacatgcggagcgtgctggacggcaaccccatgagcattgaccggaagcacaagaacctgatccagatgaagtgtccgcctctgatcatcaccagcaacaccaacgtgggcgaagatgacagatggcgctacctgcactccagagtggtggtgttcaagttcgagcagacctttccattcgaccagaacggcaatcccgtgtacgagctgtccgacaagaattggaagtccttcttcagccggacctggtccagactcgagctgcaagaggatgaggacaccgagcaggatggctctacagtgcgggcctttaagtgtgtgcccggccagaacaccaatatcctgggctctatggaagccctgagcgagagactgaacgcctaccaggacaagatcctgaccttctacgaagaggactccaaggacctgagggaccagatcgagcattggagatgtgtgcggggagagtgcgccgtgttctacaaggccagagagatgggccacagccacatcaaccaccagcaggttccacctctgcacgtgtccagaggcaaggcccacaatgccattgagctgcagatggccctggaaagcctgaaccagagcgacttcaacaccgaggaatggaccctgcaggacacaagcctggaaatgtggcggaccgagcctcagtgctgcttcaaaaagaaaggcgagacagtgaccgtgctgtatgactgcgacaaggacaacagcatggactacaccctgtggggccacgtgtacgtgtggggagatacaggctgggacaaagtgtgcggaaaggtggactacggcggcctgtactatgtgctgcacggcctgaaagtgtactacgttgagttccagcaagaggccgtgaagtacagcaagaccaacaagtgggaagtgcatatcggcagaacagtgatcccctacagcgagtccgtgtcctctacagccctgtgcgaaagagtgcctatcgccgagatcgccaatggcctccagcagaccagcattccctctcacacacacgccaccaccaaagagaacgcttgggtttcctctcagcctcctaccaagcggtccagaagatctgatccaggcggcgatcctgtcagagccctggatgccaatagcagaaccctgctgtctggaaccgcctgcgagaataccaccggcaactcttacagcgactgcacccctgtggtgcacctgaaaggcgaccccaattgtctgaaggccctgcggttcagattcgtgaaacacaagaatctgttcgtgaacgtgtcctccacctggcggtggaccaacaacaccgaagagaaggccatcgtgactgtgacctttaaggacgagcagcagagacagcagttcctcggcagcgtgaagatccccaactccatctgtgtgtgcaagggcgtgatgacagttggcagcatggtggaaggcagccaagagagagcccggacactgcacgaactgtgcgagcagagagaacagacccagcacgacatcgagctggactgcgtgtactgcctgaatcctctgaccagaaccgaggtgtacgacttcgccagatgggagctgagaatcgtgtacagacgggataccgcctacggcgtgtgcaagctgtgcctgaggttccacagcaaagtgcggaagtacaggcggtacaactactccatctacggccccacactggaacggcggacaaagaagcagctcgaagaactcgtgatccggtgctactgctgccagaaacctcagtgccccgtggaaaagcagcgccacgttgaccagggccagagattccacaacattgccgagcagtggaccggcagatgcctgcaatgttggaggccaacagccgctgaaaccggctctatgatcggccctggacctacactgcaggatatcgtgcttgagctggaacccgagcctgtggacctgagaggatatgagcagctggactccagcgaggacgaggacgagattgaccaccaccaacagcaggacagacccgatgtgcaagaagatgacggcgagcggtttagaatcctgagcgactgtcacgtgtgccagaataccgtgtcaagagtggtgcacagcacccacgacgacctgcacattctcgaggacctgcttatgggcaccctcgagatcgtggcccctaattgtgccgtgggcagcgaacagaaactgatctccgaggaagatctctgaggaagaatgtgcacagtgctaaccagaaaattcaggacaagactagtgcggccgcttttat

SEQ ID NO: 88 - DNA, 5440 bp, Artificial Sequence
  MfPV3 Ii-E1E6E7-p2a-Ii-E2 integrated into TK locus of the poxviral vector
ggccaaaaattgaaattttattttttttttttggaatataaataatccctatcagtgatagagatctccctatcagtgatagagatcgtcgacgagctcgtttagtgaaccgtcagatcgcctggagacgccatccacgctgttttgacctctagcaccggtgccaccatgcacagaaggcggagcagaagctgccgcgaggatcagaaacccgtgatggacgaccagcgggacctgatcagcaacaacgagcagctgcctatgctcggcagaaggcctggcgctcctgagagcaaatgttctagaggcgccctgtacaccggcttcagcatcctggttacactgctgctggccggacaggctaccaccgcctactttctgtatcagcagcagggcagactggacaagctgaccgtgaccagccagaacctgcagctggaaaacctgcggatgaagctgcccaagcctcctaagcctgtgtccaagatgcggatggccacacctctgctgatgcaggctttgcctatgggagcactgcctcagggccctatgcagaacgccaccaaatacggcaacatgaccgaggaccacgtgatgcatctgctgcagaatgccgatcctctgaaggtgtaccctccactgaagggcagctttcccgagaacctgcggcacctgaagaacaccatggaaaccatcgactggaaggtgttcgagagctggatgcaccactggctgctgttcgagatgagccggcacagcctggaacagaagcctacagacgcccctcctaaagagtccctggaactggaagatcccagctctggcctgggcgtgacaaagcaagatctgggccctgtgcctatgatggacccttctggaattcacggcgagggcaccagatgcaccggatggttcgatgtggaagccatcgtggaaagacggaccggcgacgtggtgtccgaggacgaagatgagaacctggaagataccggcgtggacctggtggacttcatcgacgatacctgcgagtttgagcaggccggcgacgaagctcctagagcactgctgcatgcccaagagacacaggcccatgtgaacgccgtgcactacctgaagcggaagttcacatgcagccctaccgtgtctcccctgggcaatgtgcagtgttctatcgagggcgagctgagccctagactgcacgccatccaactgaatgaaggcagcggcaaggccaagcggagactgtttctgcctgatagcggctacggcaataccgaggtggaaacccagctgtctcaggtggcaggatccgatggcgaatctcaagcccctggcggcaaagaaaatgtgcagcctgctgaaggcgctggcggagatgttcgacagctgctgagaagcagcaacctgaaggccacactgctgggcaagttcaaggacgtgtacggcatcggcttcaacgaactcgtgcggtgcttcaagagcgacaagaccgtgtgcaccgattgggttgtgggagctgctggcgtgcaccattctgtggccgaaggactgaagcacctgatcgagcctttctgcacatacgcccacatgcagtgcctgacctgcaactggggagtgtttctgctgctgctcatccggttcaagtgcggcaagaacagactgaccgtggccaagtgcatctctaccctgctgaacgtgcaagagccctacctgctgatcgaacctccaaagctgagatccacagccgccgctctgtactggtacagaaccggcatcagcaacgtgtccgaagtgatcggagagcctcctgagtggatcgtgcggcagaccatgtttcagcacagcctcgaggacagcatcttcgacctgtctcagatggtgcagtgggcctacgaccacgatctggtggacgatagcgccattgcctaccagtatgcccagctggccgacgtggactctaatgccgccgctttcctgaagtctaacgctcaggccaaatacgtgaaggactgcgccaccatgtgcagacactacaagagagccgagaagcaggccatgaccatgagccagtggatcagagccagatgcgataagaccgacgacggcggagattggaggcctatcgtgcagttcctgagataccagaacgtcgagttcatcacctttctgagcgcctttaaggccttcctgaagggaatccccaagagaagctgcatcgtgctgtacggccctccaaacaccggcaagagctacttcggaatgagcctgatgcagtttctgcagggcagcatcatcagctacgtgaacagcaacagccacttttggctggcccctctggccgaagctaaagtggccatgctggacgatgccacaccacagtgctggtcctacatcgacacctacatgcggagcgtgctggacggcaaccccatgagcattgaccggaagcacaagaacctgatccagatgaagtgtccgcctctgatcatcaccagcaacaccaacgtgggcgaagatgacagatggcgctacctgcactccagagtggtggtgttcaagttcgagcagacctttccattcgaccagaacggcaatcccgtgtacgagctgtccgacaagaattggaagtccttcttcagccggacctggtccagactcgagctgcaagaggatgaggacaccgagcaggatggctctacagtgcgggcctttaagtgtgtgcccggccagaacaccaatatcctgggctctatggtggaaggcagccaagagagagcccggacactgcacgaactgtgcgagcagagagaacagacccagcacgacatcgagctggactgcgtgtactgcctgaatcctctgaccagaaccgaggtgtacgacttcgccagatgggagctgagaatcgtgtacagacgggataccgcctacggcgtgtgcaagctgtgcctgaggttccacagcaaagtgcggaagtacaggcggtacaactactccatctacggccccacactggaacggcggacaaagaagcagctcgaagaactcgtgatccggtgctactgctgccagaaacctcagtgccccgtggaaaagcagcgccacgttgaccagggccagagattccacaacattgccgagcagtggaccggcagatgcctgcaatgttggaggccaacagccgctgaaaccggctctatgatcggccctggacctacactgcaggatatcgtgcttgagctggaacccgagcctgtggacctgagaggatatgagcagctggactccagcgaggacgaggacgagattgaccaccaccaacagcaggacagacccgatgtgcaagaagatgacggcgagcggtttagaatcctgagcgactgtcacgtgtgccagaataccgtgtcaagagtggtgcacagcacccacgacgacctgcacattctcgaggacctgcttatgggcaccctcgagatcgtggcccctaattgtgccgtgggcagcggcgccaccaatttcagtctgcttaaacaggccggggacgtcgaagagaaccccggacctatgcatcggcgcagatctcggtcttgtagagaagaccaaaagcctgtcatggatgatcaaagagatttaatttctaataatgaacaattacccatgttgggacggcgccccggagcccccgaatctaagtgcagccggggagctttatatacaggattttctattttagtgaccttattattagctggccaagccacaacagcttatttcttataccaacaacaaggacggttagataaattaacagtcacatctcaaaatttacaattagagaatttaagaatgaaattacctaaaccacccaaacccgtcagtaaaatgagaatggctacccccttattaatgcaagccctccccatgggcgccttaccccaaggacccatgcaaaatgctacaaagtatggaaatatgacagaagatcatgtcatgcacttattacaaaacgctgaccccttaaaagtctatccccctttaaaaggatctttccctgaaaatttaagacatttaaaaaatacaatggagacaattgattggaaagtctttgaatcttggatgcatcattggttattatttgaaatgtctaggcattctttagagcaaaaacccaccgatgctccacccaaggaaagtttagagttagaggacccttctagcggattaggagtcaccaaacaggacttaggacccgtccccatgatggaagccctgagcgagagactgaacgcctaccaggacaagatcctgaccttctacgaagaggactccaaggacctgagggaccagatcgagcattggagatgtgtgcggggagagtgcgccgtgttctacaaggccagagagatgggccacagccacatcaaccaccagcaggttccacctctgcacgtgtccagaggcaaggcccacaatgccattgagctgcagatggccctggaaagcctgaaccagagcgacttcaacaccgaggaatggaccctgcaggacacaagcctggaaatgtggcggaccgagcctcagtgctgcttcaaaaagaaaggcgagacagtgaccgtgctgtatgactgcgacaaggacaacagcatggactacaccctgtggggccacgtgtacgtgtggggagatacaggctgggacaaagtgtgcggaaaggtggactacggcggcctgtactatgtgctgcacggcctgaaagtgtactacgttgagttccagcaagaggccgtgaagtacagcaagaccaacaagtgggaagtgcatatcggcagaacagtgatcccctacagcgagtccgtgtcctctacagccctgtgcgaaagagtgcctatcgccgagatcgccaatggcctccagcagaccagcattccctctcacacacacgccaccaccaaagagaacgcttgggtttcctctcagcctcctaccaagcggtccagaagatctgatccaggcggcgatcctgtcagagccctggatgccaatagcagaaccctgctgtctggaaccgcctgcgagaataccaccggcaactcttacagcgactgcacccctgtggtgcacctgaaaggcgaccccaattgtctgaaggccctgcggttcagattcgtgaaacacaagaatctgttcgtgaacgtgtcctccacctggcggtggaccaacaacaccgaagagaaggccatcgtgactgtgacctttaaggacgagcagcagagacagcagttcctcggcagcgtgaagatccccaactccatctgtgtgtgcaagggcgtgatgacagttggcagcgaacagaaactgatctccgaggaagatctctgaggaagaatgtgcacagtgctaaccagaaaattcaggacaagactagtgcggccgcttttat

SEQ ID NO: 89 - DNA, 3598 bp, Artificial Sequence
  MfPV3 Ii-E1E6E7 integrated into TK locus of the poxviral vector
ggccaaaaattgaaattttattttttttttttggaatataaataatccctatcagtgatagagatctccctatcagtgatagagatcgtcgacgagctcgtttagtgaaccgtcagatcgcctggagacgccatccacgctgttttgacctctagcaccggtgccaccatgcacagaaggcggagcagaagctgccgcgaggatcagaaacccgtgatggacgaccagcgggacctgatcagcaacaacgagcagctgcctatgctcggcagaaggcctggcgctcctgagagcaaatgttctagaggcgccctgtacaccggcttcagcatcctggttacactgctgctggccggacaggctaccaccgcctactttctgtatcagcagcagggcagactggacaagctgaccgtgaccagccagaacctgcagctggaaaacctgcggatgaagctgcccaagcctcctaagcctgtgtccaagatgcggatggccacacctctgctgatgcaggctttgcctatgggagcactgcctcagggccctatgcagaacgccaccaaatacggcaacatgaccgaggaccacgtgatgcatctgctgcagaatgccgatcctctgaaggtgtaccctccactgaagggcagctttcccgagaacctgcggcacctgaagaacaccatggaaaccatcgactggaaggtgttcgagagctggatgcaccactggctgctgttcgagatgagccggcacagcctggaacagaagcctacagacgcccctcctaaagagtccctggaactggaagatcccagctctggcctgggcgtgacaaagcaagatctgggccctgtgcctatgatggacccttctggaattcacggcgagggcaccagatgcaccggatggttcgatgtggaagccatcgtggaaagacggaccggcgacgtggtgtccgaggacgaagatgagaacctggaagataccggcgtggacctggtggacttcatcgacgatacctgcgagtttgagcaggccggcgacgaagctcctagagcactgctgcatgcccaagagacacaggcccatgtgaacgccgtgcactacctgaagcggaagttcacatgcagccctaccgtgtctcccctgggcaatgtgcagtgttctatcgagggcgagctgagccctagactgcacgccatccaactgaatgaaggcagcggcaaggccaagcggagactgtttctgcctgatagcggctacggcaataccgaggtggaaacccagctgtctcaggtggcaggatccgatggcgaatctcaagcccctggcggcaaagaaaatgtgcagcctgctgaaggcgctggcggagatgttcgacagctgctgagaagcagcaacctgaaggccacactgctgggcaagttcaaggacgtgtacggcatcggcttcaacgaactcgtgcggtgcttcaagagcgacaagaccgtgtgcaccgattgggttgtgggagctgctggcgtgcaccattctgtggccgaaggactgaagcacctgatcgagcctttctgcacatacgcccacatgcagtgcctgacctgcaactggggagtgtttctgctgctgctcatccggttcaagtgcggcaagaacagactgaccgtggccaagtgcatctctaccctgctgaacgtgcaagagccctacctgctgatcgaacctccaaagctgagatccacagccgccgctctgtactggtacagaaccggcatcagcaacgtgtccgaagtgatcggagagcctcctgagtggatcgtgcggcagaccatgtttcagcacagcctcgaggacagcatcttcgacctgtctcagatggtgcagtgggcctacgaccacgatctggtggacgatagcgccattgcctaccagtatgcccagctggccgacgtggactctaatgccgccgctttcctgaagtctaacgctcaggccaaatacgtgaaggactgcgccaccatgtgcagacactacaagagagccgagaagcaggccatgaccatgagccagtggatcagagccagatgcgataagaccgacgacggcggagattggaggcctatcgtgcagttcctgagataccagaacgtcgagttcatcacctttctgagcgcctttaaggccttcctgaagggaatccccaagagaagctgcatcgtgctgtacggccctccaaacaccggcaagagctacttcggaatgagcctgatgcagtttctgcagggcagcatcatcagctacgtgaacagcaacagccacttttggctggcccctctggccgaagctaaagtggccatgctggacgatgccacaccacagtgctggtcctacatcgacacctacatgcggagcgtgctggacggcaaccccatgagcattgaccggaagcacaagaacctgatccagatgaagtgtccgcctctgatcatcaccagcaacaccaacgtgggcgaagatgacagatggcgctacctgcactccagagtggtggtgttcaagttcgagcagacctttccattcgaccagaacggcaatcccgtgtacgagctgtccgacaagaattggaagtccttcttcagccggacctggtccagactcgagctgcaagaggatgaggacaccgagcaggatggctctacagtgcgggcctttaagtgtgtgcccggccagaacaccaatatcctgggctctatggtggaaggcagccaagagagagcccggacactgcacgaactgtgcgagcagagagaacagacccagcacgacatcgagctggactgcgtgtactgcctgaatcctctgaccagaaccgaggtgtacgacttcgccagatgggagctgagaatcgtgtacagacgggataccgcctacggcgtgtgcaagctgtgcctgaggttccacagcaaagtgcggaagtacaggcggtacaactactccatctacggccccacactggaacggcggacaaagaagcagctcgaagaactcgtgatccggtgctactgctgccagaaacctcagtgccccgtggaaaagcagcgccacgttgaccagggccagagattccacaacattgccgagcagtggaccggcagatgcctgcaatgttggaggccaacagccgctgaaaccggctctatgatcggccctggacctacactgcaggatatcgtgcttgagctggaacccgagcctgtggacctgagaggatatgagcagctggactccagcgaggacgaggacgagattgaccaccaccaacagcaggacagacccgatgtgcaagaagatgacggcgagcggtttagaatcctgagcgactgtcacgtgtgccagaataccgtgtcaagagtggtgcacagcacccacgacgacctgcacattctcgaggacctgcttatgggcaccctcgagatcgtggcccctaattgtgccgtgggcagcgaacagaaactgatctccgaggaagatctctgaggaagaatgtgcacagtgctaaccagaaaattcaggacaagactagtgcggccgcttttat

SEQ ID NO: 90 - DNA, 4744 bp, Artificial Sequence
  HPV16 Ii-E1E2E6E7 integrated into TK locus of the poxviral vector
ggccaaaaattgaaattttattttttttttttggaatataaataatccctatcagtgatagagatctccctatcagtgatagagatcgtcgacgagctcgtttagtgaaccgtcagatcgcctggagacgccatccacgctgttttgacctctagcaccggtgccaccatgcacagaaggcggagcagaagctgccgcgaggatcagaaacccgtgatggacgaccagcgggacctgatcagcaacaacgagcagctgcctatgctcggcagaaggcctggcgctcctgagagcaaatgttctagaggcgccctgtacaccggcttcagcatcctggttacactgctgctggccggacaggctaccaccgcctactttctgtatcagcagcagggcagactggacaagctgaccgtgaccagccagaacctgcagctggaaaacctgcggatgaagctgcccaagcctcctaagcctgtgtccaagatgcggatggccacacctctgctgatgcaggctttgcctatgggagcactgcctcagggccctatgcagaacgccaccaaatacggcaacatgaccgaggaccacgtgatgcatctgctgcagaatgccgatcctctgaaggtgtaccctccactgaagggcagctttcccgagaacctgcggcacctgaagaacaccatggaaaccatcgactggaaggtgttcgagagctggatgcaccactggctgctgttcgagatgagccggcacagcctggaacagaagcctacagacgcccctcctaaagagtccctggaactggaagatcccagctctggcctgggcgtgacaaagcaagatctgggccctgtgcctatgatggccgatcctgctggcacaaacggcgaagaaggcacaggctgcaacggctggttttacgtggaagccgtggtggaaaagaaaaccggcgacgccatcagcgacgacgagaacgagaatgacagcgacaccggcgaggacctggtggacttcatcgtgaacgacaacgactacctgacacaggccgagacagagacagcccacgctctgtttacagcccaagaggccaagcagcacagagatgccgttcaggtgctgaagagaaagtacctgggcagccctctgagcgacatcagcggctgtgtggacaacaacatcagccccagactgaaggccatctgcatcgagaagcagagcagagccgccaagcggagactgtttgagagcgaggatagcggctacggcaataccgaggtggaaacccagcaaatgctgcaggtcgagggcagacacgaaaccgagacaccttgcagccagtacagcggaggatctggcggaggctgtagccagtactcttctggaagtggcggagagggcgtgtccgagagacacaccatttgtcagacccctctgaccaacatcctgaacgtgctgaaaaccagcaacgccaaggccgccatgctggccaagttcaaagagctgtacggcgtcagcttcagcgaactcgtgcggcccttcaagagcaacaagtccacctgttgcgactggtgcattgccgcctttggcctgacaccttctatcgccgacagcatcaagaccctgctccagcagtactgtctgtacctgcacattcagagcctggcctgctcttggggaatggtggtgctgctgctcgtgcggtacaagtgcggcaagaacagagagacaattgagaagctgctgagcaaactgctgtgcgtgtcccctatgtgcatgatgatcgagcctccaaagctgcggtctacagccgccgctctgtactggtacaagaccggcatcagcaatatctccgaggtgtacggcgacacccctgagtggattcagagacagaccgtcctgcagcacagcttcaacgactgcaccttcgagctgtcccagatggtgcagtgggcctacgacaatgacatcgtggacgactccgagatcgcctataagtacgcccagctggccgacaccaacagcaatgccagcgccttcctgaagtccaacagccaggccaagatcgtgaaggactgcgccaccatgtgcagacactacaagcgggccgagaagaaacagatgagcatgagccagtggatcaagtacagatgcgacagagtggacgacggcggcgattggaagcagatcgtgatgttcctgagataccagggcgtcgagttcatgagctttctgacagccctgaagcggttcctgcagggcatccccaagaagaactgcatcctgctgtatggcgccgctaacaccggcaagagcctgttcggaatgagcctgatgaagtttctgcagggctccgtgatctgctttgtgaacagcaagagccacttctggctccagccactggccgatgccaagattggcatgctggacgatgccaccgtgccttgctggaactacatcgacgacaacctgagaaacgccctggacggcaacctggtttctatggacgtgaagcacagacccctggtgcagctgaagtgtcctccactgctgatcaccagcaacatcaacgccggcaccgattccagatggccctatctgcacaaccggctggtggtgtttacctttcctaacgagttccccttcgacgaaaacggcaaccccgtgtacgagctgaacgataagaattggaagtccttcttcagccggacctggtccagactgagcctgcacgaggatgaggacaaagagaacgacggcgacagcctgcctaccttcaaatgtgtcagcggccagaacaccaacacactgggcagcatggaaacactgtgccagcggctgaacgtgtgccaggacaagattctgacccactatgagaacgacagcaccgacctgagggaccacatcgactactggaagcacatgcggctggaatgcgccatctactacaaggctagagagatgggcttcaagcacatcaaccaccaggtggtgcctacactggccgtgtctaagaacaaggctctgcaggccatcgaactgcagctgaccctggaaacaatctacaactcccagtactccaacgagaagtggaccctccaggacgtgtcactggaagtgtacctgaccgctcctaccggctgcatcaagaaacacggctacaccgtggaagtgcagtttgacggcgatatctgcaataccatgcactacaccaactggacccacatctacatctgcgaagaggccagcgtgacagtggtggaaggccaggtcgactactacggcctgtactacgtgcacgagggcatcagaacctacttcgtgcagttcaaggatgacgccgagaagtacagcaagaacaaagtgtgggaagtgcacgctggcggccaagtgatcctgtgtcctacaagcgtgttcagcagcaacgaagtgtctagccccgagatcatcagacagcacctggccaatcatcctgccgccacacacacaaaagctgtggccctgggcaccgaggaaacacagaccacaattcagaggcccagaagcgagcccgataccggcaatccttgtcacaccaccaagctgctgcaccgggattccgtggattctgcccctatcctgaccgccttcaacagctcccacaaaggccggatcaactgcaacagcaacaccacacctatcgtgcacctgaaaggggacgccaacactctgaaggccctgcggtacagattcaagaagcactgtaccctgtataccgccgtgtccagcacatggcactggaccggacacaacgtgaaacacaagagcgccatcgtgaccctgacctacgatagcgagtggcagagggaccagttcctgagccaagtgaagatccctaagaccatcaccgtgtccaccggctttatgagcattggcagcatgcaccagaaacggacagccatgttccaggatcctcaagagcggccacggaagctgcctcagctgtgtacagaactgcagaccaccatccacgacatcatcctcgagtgcgtgtactgcaagcagcagctcctgcggagagaagtgtacgacttcgccttccgggatctgtgcatcgtgtacagagatggcaacccctacgccgtgtgcgacaagtgcctgaagttctactccaagatcagcgagtaccggcactactgctactccctgtacggcaccacacttgagcagcagtacaacaagcccctgtgcgatctgctgatccggtgcatcaactgccagaaacctcagtgccccgaggaaaagcagagacacctggacaagaagcagcggttccacaacattagaggcagatggacaggccggtgcatgagctgctgtagaagcagcagaacaagacggggctccatgcacggcgataccccaacactgcacgagtacatgctggatctgcagcccgagacaaccgatctgtacggctatgagcagctgaatgactccagcgaggaagaggacgagatcgacggacctgctggacaggctgaacctgatagagcccactacaatatcgtgaccttctgctgcaagtgcgatagcaccctgagaagatgcgtgcagagcacccacgtggacatcaggaccctcgaggatctgctcatgggcaccctgggaattgtggccccaatctgctctcagaagccttgaggaagaatgtgcacagtgctaaccagaaaattcaggacaagactagtgcggccgcttttat

SEQ ID NO: 91 - DNA, 5506 bp, Artificial Sequence
  HPV16 Ii-E1E2-p2a-Ii-E6E7 integrated into TK locus of the poxviral vector
ggccaaaaattgaaattttattttttttttttggaatataaataatccctatcagtgatagagatctccctatcagtgatagagatcgtcgacgagctcgtttagtgaaccgtcagatcgcctggagacgccatccacgctgttttgacctctagcaccggtgccaccatgcacagaaggcggagcagaagctgccgcgaggatcagaaacccgtgatggacgaccagcgggacctgatcagcaacaacgagcagctgcctatgctcggcagaaggcctggcgctcctgagagcaaatgttctagaggcgccctgtacaccggcttcagcatcctggttacactgctgctggccggacaggctaccaccgcctactttctgtatcagcagcagggcagactggacaagctgaccgtgaccagccagaacctgcagctggaaaacctgcggatgaagctgcccaagcctcctaagcctgtgtccaagatgcggatggccacacctctgctgatgcaggctttgcctatgggagcactgcctcagggccctatgcagaacgccaccaaatacggcaacatgaccgaggaccacgtgatgcatctgctgcagaatgccgatcctctgaaggtgtaccctccactgaagggcagctttcccgagaacctgcggcacctgaagaacaccatggaaaccatcgactggaaggtgttcgagagctggatgcaccactggctgctgttcgagatgagccggcacagcctggaacagaagcctacagacgcccctcctaaagagtccctggaactggaagatcccagctctggcctgggcgtgacaaagcaagatctgggccctgtgcctatgatggccgatcctgctggcacaaacggcgaagaaggcacaggctgcaacggctggttttacgtggaagccgtggtggaaaagaaaaccggcgacgccatcagcgacgacgagaacgagaatgacagcgacaccggcgaggacctggtggacttcatcgtgaacgacaacgactacctgacacaggccgagacagagacagcccacgctctgtttacagcccaagaggccaagcagcacagagatgccgttcaggtgctgaagagaaagtacctgggcagccctctgagcgacatcagcggctgtgtggacaacaacatcagccccagactgaaggccatctgcatcgagaagcagagcagagccgccaagcggagactgtttgagagcgaggatagcggctacggcaataccgaggtggaaacccagcaaatgctgcaggtcgagggcagacacgaaaccgagacaccttgcagccagtacagcggaggatctggcggaggctgtagccagtactcttctggaagtggcggagagggcgtgtccgagagacacaccatttgtcagacccctctgaccaacatcctgaacgtgctgaaaaccagcaacgccaaggccgccatgctggccaagttcaaagagctgtacggcgtcagcttcagcgaactcgtgcggcccttcaagagcaacaagtccacctgttgcgactggtgcattgccgcctttggcctgacaccttctatcgccgacagcatcaagaccctgctccagcagtactgtctgtacctgcacattcagagcctggcctgctcttggggaatggtggtgctgctgctcgtgcggtacaagtgcggcaagaacagagagacaattgagaagctgctgagcaaactgctgtgcgtgtcccctatgtgcatgatgatcgagcctccaaagctgcggtctacagccgccgctctgtactggtacaagaccggcatcagcaatatctccgaggtgtacggcgacacccctgagtggattcagagacagaccgtcctgcagcacagcttcaacgactgcaccttcgagctgtcccagatggtgcagtgggcctacgacaatgacatcgtggacgactccgagatcgcctataagtacgcccagctggccgacaccaacagcaatgccagcgccttcctgaagtccaacagccaggccaagatcgtgaaggactgcgccaccatgtgcagacactacaagcgggccgagaagaaacagatgagcatgagccagtggatcaagtacagatgcgacagagtggacgacggcggcgattggaagcagatcgtgatgttcctgagataccagggcgtcgagttcatgagctttctgacagccctgaagcggttcctgcagggcatccccaagaagaactgcatcctgctgtatggcgccgctaacaccggcaagagcctgttcggaatgagcctgatgaagtttctgcagggctccgtgatctgctttgtgaacagcaagagccacttctggctccagccactggccgatgccaagattggcatgctggacgatgccaccgtgccttgctggaactacatcgacgacaacctgagaaacgccctggacggcaacctggtttctatggacgtgaagcacagacccctggtgcagctgaagtgtcctccactgctgatcaccagcaacatcaacgccggcaccgattccagatggccctatctgcacaaccggctggtggtgtttacctttcctaacgagttccccttcgacgaaaacggcaaccccgtgtacgagctgaacgataagaattggaagtccttcttcagccggacctggtccagactgagcctgcacgaggatgaggacaaagagaacgacggcgacagcctgcctaccttcaaatgtgtcagcggccagaacaccaacacactgggcagcatggaaacactgtgccagcggctgaacgtgtgccaggacaagattctgacccactatgagaacgacagcaccgacctgagggaccacatcgactactggaagcacatgcggctggaatgcgccatctactacaaggctagagagatgggcttcaagcacatcaaccaccaggtggtgcctacactggccgtgtctaagaacaaggctctgcaggccatcgaactgcagctgaccctggaaacaatctacaactcccagtactccaacgagaagtggaccctccaggacgtgtcactggaagtgtacctgaccgctcctaccggctgcatcaagaaacacggctacaccgtggaagtgcagtttgacggcgatatctgcaataccatgcactacaccaactggacccacatctacatctgcgaagaggccagcgtgacagtggtggaaggccaggtcgactactacggcctgtactacgtgcacgagggcatcagaacctacttcgtgcagttcaaggatgacgccgagaagtacagcaagaacaaagtgtgggaagtgcacgctggcggccaagtgatcctgtgtcctacaagcgtgttcagcagcaacgaagtgtctagccccgagatcatcagacagcacctggccaatcatcctgccgccacacacacaaaagctgtggccctgggcaccgaggaaacacagaccacaattcagaggcccagaagcgagcccgataccggcaatccttgtcacaccaccaagctgctgcaccgggattccgtggattctgcccctatcctgaccgccttcaacagctcccacaaaggccggatcaactgcaacagcaacaccacacctatcgtgcacctgaaaggggacgccaacactctgaaggccctgcggtacagattcaagaagcactgtaccctgtataccgccgtgtccagcacatggcactggaccggacacaacgtgaaacacaagagcgccatcgtgaccctgacctacgatagcgagtggcagagggaccagttcctgagccaagtgaagatccctaagaccatcaccgtgtccaccggctttatgagcattggcagcggcagcggcgccaccaatttcagtctgcttaaacaggccggggacgtcgaagagaaccccggacctatgcatcggcgcagatctcggtcttgtagagaagaccaaaagcctgtcatggatgatcaaagagatttaatttctaataatgaacaattacccatgttgggacggcgccccggagcccccgaatctaagtgcagccggggagctttatatacaggattttctattttagtgaccttattattagctggccaagccacaacagcttatttcttataccaacaacaaggacggttagataaattaacagtcacatctcaaaatttacaattagagaatttaagaatgaaattacctaaaccacccaaacccgtcagtaaaatgagaatggctacccccttattaatgcaagccctccccatgggcgccttaccccaaggacccatgcaaaatgctacaaagtatggaaatatgacagaagatcatgtcatgcacttattacaaaacgctgaccccttaaaagtctatccccctttaaaaggatctttccctgaaaatttaagacatttaaaaaatacaatggagacaattgattggaaagtctttgaatcttggatgcatcattggttattatttgaaatgtctaggcattctttagagcaaaaacccaccgatgctccacccaaggaaagtttagagttagaggacccttctagcggattaggagtcaccaaacaggacttaggacccgtccccatgatgcaccagaaacggacagccatgttccaggatcctcaagagcggccacggaagctgcctcagctgtgtacagaactgcagaccaccatccacgacatcatcctcgagtgcgtgtactgcaagcagcagctcctgcggagagaagtgtacgacttcgccttccgggatctgtgcatcgtgtacagagatggcaacccctacgccgtgtgcgacaagtgcctgaagttctactccaagatcagcgagtaccggcactactgctactccctgtacggcaccacacttgagcagcagtacaacaagcccctgtgcgatctgctgatccggtgcatcaactgccagaaacctcagtgccccgaggaaaagcagagacacctggacaagaagcagcggttccacaacattagaggcagatggacaggccggtgcatgagctgctgtagaagcagcagaacaagacggggctccatgcacggcgataccccaacactgcacgagtacatgctggatctgcagcccgagacaaccgatctgtacggctatgagcagctgaatgactccagcgaggaagaggacgagatcgacggacctgctggacaggctgaacctgatagagcccactacaatatcgtgaccttctgctgcaagtgcgatagcaccctgagaagatgcgtgcagagcacccacgtggacatcaggaccctcgaggatctgctcatgggcaccctgggaattgtggccccaatctgctctcagaagccttgaggaagaatgtgcacagtgctaaccagaaaattcaggacaagactagtgcggccgcttttat

SEQ ID NO: 92 - DNA, 4048 bp, Artificial Sequence
  HPV16 E1E2E6E7 integrated into TK locus of the poxviral vector
ggccaaaaattgaaattttattttttttttttggaatataaataatccctatcagtgatagagatctccctatcagtgatagagatcgtcgacgagctcgtttagtgaaccgtcagatcgcctggagacgccatccacgctgttttgacctctagcaccggtgccaccatggccgatcctgctggcacaaacggcgaagaaggcacaggctgcaacggctggttttacgtggaagccgtggtggaaaagaaaaccggcgacgccatcagcgacgacgagaacgagaatgacagcgacaccggcgaggacctggtggacttcatcgtgaacgacaacgactacctgacacaggccgagacagagacagcccacgctctgtttacagcccaagaggccaagcagcacagagatgccgttcaggtgctgaagagaaagtacctgggcagccctctgagcgacatcagcggctgtgtggacaacaacatcagccccagactgaaggccatctgcatcgagaagcagagcagagccgccaagcggagactgtttgagagcgaggatagcggctacggcaataccgaggtggaaacccagcaaatgctgcaggtcgagggcagacacgaaaccgagacaccttgcagccagtacagcggaggatctggcggaggctgtagccagtactcttctggaagtggcggagagggcgtgtccgagagacacaccatttgtcagacccctctgaccaacatcctgaacgtgctgaaaaccagcaacgccaaggccgccatgctggccaagttcaaagagctgtacggcgtcagcttcagcgaactcgtgcggcccttcaagagcaacaagtccacctgttgcgactggtgcattgccgcctttggcctgacaccttctatcgccgacagcatcaagaccctgctccagcagtactgtctgtacctgcacattcagagcctggcctgctcttggggaatggtggtgctgctgctcgtgcggtacaagtgcggcaagaacagagagacaattgagaagctgctgagcaaactgctgtgcgtgtcccctatgtgcatgatgatcgagcctccaaagctgcggtctacagccgccgctctgtactggtacaagaccggcatcagcaatatctccgaggtgtacggcgacacccctgagtggattcagagacagaccgtcctgcagcacagcttcaacgactgcaccttcgagctgtcccagatggtgcagtgggcctacgacaatgacatcgtggacgactccgagatcgcctataagtacgcccagctggccgacaccaacagcaatgccagcgccttcctgaagtccaacagccaggccaagatcgtgaaggactgcgccaccatgtgcagacactacaagcgggccgagaagaaacagatgagcatgagccagtggatcaagtacagatgcgacagagtggacgacggcggcgattggaagcagatcgtgatgttcctgagataccagggcgtcgagttcatgagctttctgacagccctgaagcggttcctgcagggcatccccaagaagaactgcatcctgctgtatggcgccgctaacaccggcaagagcctgttcggaatgagcctgatgaagtttctgcagggctccgtgatctgctttgtgaacagcaagagccacttctggctccagccactggccgatgccaagattggcatgctggacgatgccaccgtgccttgctggaactacatcgacgacaacctgagaaacgccctggacggcaacctggtttctatggacgtgaagcacagacccctggtgcagctgaagtgtcctccactgctgatcaccagcaacatcaacgccggcaccgattccagatggccctatctgcacaaccggctggtggtgtttacctttcctaacgagttccccttcgacgaaaacggcaaccccgtgtacgagctgaacgataagaattggaagtccttcttcagccggacctggtccagactgagcctgcacgaggatgaggacaaagagaacgacggcgacagcctgcctaccttcaaatgtgtcagcggccagaacaccaacacactgggcagcatggaaacactgtgccagcggctgaacgtgtgccaggacaagattctgacccactatgagaacgacagcaccgacctgagggaccacatcgactactggaagcacatgcggctggaatgcgccatctactacaaggctagagagatgggcttcaagcacatcaaccaccaggtggtgcctacactggccgtgtctaagaacaaggctctgcaggccatcgaactgcagctgaccctggaaacaatctacaactcccagtactccaacgagaagtggaccctccaggacgtgtcactggaagtgtacctgaccgctcctaccggctgcatcaagaaacacggctacaccgtggaagtgcagtttgacggcgatatctgcaataccatgcactacaccaactggacccacatctacatctgcgaagaggccagcgtgacagtggtggaaggccaggtcgactactacggcctgtactacgtgcacgagggcatcagaacctacttcgtgcagttcaaggatgacgccgagaagtacagcaagaacaaagtgtgggaagtgcacgctggcggccaagtgatcctgtgtcctacaagcgtgttcagcagcaacgaagtgtctagccccgagatcatcagacagcacctggccaatcatcctgccgccacacacacaaaagctgtggccctgggcaccgaggaaacacagaccacaattcagaggcccagaagcgagcccgataccggcaatccttgtcacaccaccaagctgctgcaccgggattccgtggattctgcccctatcctgaccgccttcaacagctcccacaaaggccggatcaactgcaacagcaacaccacacctatcgtgcacctgaaaggggacgccaacactctgaaggccctgcggtacagattcaagaagcactgtaccctgtataccgccgtgtccagcacatggcactggaccggacacaacgtgaaacacaagagcgccatcgtgaccctgacctacgatagcgagtggcagagggaccagttcctgagccaagtgaagatccctaagaccatcaccgtgtccaccggctttatgagcattggcagcatgcaccagaaacggacagccatgttccaggatcctcaagagcggccacggaagctgcctcagctgtgtacagaactgcagaccaccatccacgacatcatcctcgagtgcgtgtactgcaagcagcagctcctgcggagagaagtgtacgacttcgccttccgggatctgtgcatcgtgtacagagatggcaacccctacgccgtgtgcgacaagtgcctgaagttctactccaagatcagcgagtaccggcactactgctactccctgtacggcaccacacttgagcagcagtacaacaagcccctgtgcgatctgctgatccggtgcatcaactgccagaaacctcagtgccccgaggaaaagcagagacacctggacaagaagcagcggttccacaacattagaggcagatggacaggccggtgcatgagctgctgtagaagcagcagaacaagacggggctccatgcacggcgataccccaacactgcacgagtacatgctggatctgcagcccgagacaaccgatctgtacggctatgagcagctgaatgactccagcgaggaagaggacgagatcgacggacctgctggacaggctgaacctgatagagcccactacaatatcgtgaccttctgctgcaagtgcgatagcaccctgagaagatgcgtgcagagcacccacgtggacatcaggaccctcgaggatctgctcatgggcaccctgggaattgtggccccaatctgctctcagaagccttgaggaagaatgtgcacagtgctaaccagaaaattcaggacaagactagtgcggccgcttttat

SEQ ID NO: 93 - DNA, 5500 bp, Artificial Sequence
  HPV16 Ii-E1E6E7-p2a-Ii-E2 integrated into TK locus of the poxviral vector
ggccaaaaattgaaattttattttttttttttggaatataaataatccctatcagtgatagagatctccctatcagtgatagagatcgtcgacgagctcgtttagtgaaccgtcagatcgcctggagacgccatccacgctgttttgacctctagcaccggtgccaccatgcacagaaggcggagcagaagctgccgcgaggatcagaaacccgtgatggacgaccagcgggacctgatcagcaacaacgagcagctgcctatgctcggcagaaggcctggcgctcctgagagcaaatgttctagaggcgccctgtacaccggcttcagcatcctggttacactgctgctggccggacaggctaccaccgcctactttctgtatcagcagcagggcagactggacaagctgaccgtgaccagccagaacctgcagctggaaaacctgcggatgaagctgcccaagcctcctaagcctgtgtccaagatgcggatggccacacctctgctgatgcaggctttgcctatgggagcactgcctcagggccctatgcagaacgccaccaaatacggcaacatgaccgaggaccacgtgatgcatctgctgcagaatgccgatcctctgaaggtgtaccctccactgaagggcagctttcccgagaacctgcggcacctgaagaacaccatggaaaccatcgactggaaggtgttcgagagctggatgcaccactggctgctgttcgagatgagccggcacagcctggaacagaagcctacagacgcccctcctaaagagtccctggaactggaagatcccagctctggcctgggcgtgacaaagcaagatctgggccctgtgcctatgatggccgatcctgctggcacaaacggcgaagaaggcacaggctgcaacggctggttttacgtggaagccgtggtggaaaagaaaaccggcgacgccatcagcgacgacgagaacgagaatgacagcgacaccggcgaggacctggtggacttcatcgtgaacgacaacgactacctgacacaggccgagacagagacagcccacgctctgtttacagcccaagaggccaagcagcacagagatgccgttcaggtgctgaagagaaagtacctgggcagccctctgagcgacatcagcggctgtgtggacaacaacatcagccccagactgaaggccatctgcatcgagaagcagagcagagccgccaagcggagactgtttgagagcgaggatagcggctacggcaataccgaggtggaaacccagcaaatgctgcaggtcgagggcagacacgaaaccgagacaccttgcagccagtacagcggaggatctggcggaggctgtagccagtactcttctggaagtggcggagagggcgtgtccgagagacacaccatttgtcagacccctctgaccaacatcctgaacgtgctgaaaaccagcaacgccaaggccgccatgctggccaagttcaaagagctgtacggcgtcagcttcagcgaactcgtgcggcccttcaagagcaacaagtccacctgttgcgactggtgcattgccgcctttggcctgacaccttctatcgccgacagcatcaagaccctgctccagcagtactgtctgtacctgcacattcagagcctggcctgctcttggggaatggtggtgctgctgctcgtgcggtacaagtgcggcaagaacagagagacaattgagaagctgctgagcaaactgctgtgcgtgtcccctatgtgcatgatgatcgagcctccaaagctgcggtctacagccgccgctctgtactggtacaagaccggcatcagcaatatctccgaggtgtacggcgacacccctgagtggattcagagacagaccgtcctgcagcacagcttcaacgactgcaccttcgagctgtcccagatggtgcagtgggcctacgacaatgacatcgtggacgactccgagatcgcctataagtacgcccagctggccgacaccaacagcaatgccagcgccttcctgaagtccaacagccaggccaagatcgtgaaggactgcgccaccatgtgcagacactacaagcgggccgagaagaaacagatgagcatgagccagtggatcaagtacagatgcgacagagtggacgacggcggcgattggaagcagatcgtgatgttcctgagataccagggcgtcgagttcatgagctttctgacagccctgaagcggttcctgcagggcatccccaagaagaactgcatcctgctgtatggcgccgctaacaccggcaagagcctgttcggaatgagcctgatgaagtttctgcagggctccgtgatctgctttgtgaacagcaagagccacttctggctccagccactggccgatgccaagattggcatgctggacgatgccaccgtgccttgctggaactacatcgacgacaacctgagaaacgccctggacggcaacctggtttctatggacgtgaagcacagacccctggtgcagctgaagtgtcctccactgctgatcaccagcaacatcaacgccggcaccgattccagatggccctatctgcacaaccggctggtggtgtttacctttcctaacgagttccccttcgacgaaaacggcaaccccgtgtacgagctgaacgataagaattggaagtccttcttcagccggacctggtccagactgagcctgcacgaggatgaggacaaagagaacgacggcgacagcctgcctaccttcaaatgtgtcagcggccagaacaccaacacactgggcagcatgcaccagaaacggacagccatgttccaggatcctcaagagcggccacggaagctgcctcagctgtgtacagaactgcagaccaccatccacgacatcatcctcgagtgcgtgtactgcaagcagcagctcctgcggagagaagtgtacgacttcgccttccgggatctgtgcatcgtgtacagagatggcaacccctacgccgtgtgcgacaagtgcctgaagttctactccaagatcagcgagtaccggcactactgctactccctgtacggcaccacacttgagcagcagtacaacaagcccctgtgcgatctgctgatccggtgcatcaactgccagaaacctcagtgccccgaggaaaagcagagacacctggacaagaagcagcggttccacaacattagaggcagatggacaggccggtgcatgagctgctgtagaagcagcagaacaagacggggctccatgcacggcgataccccaacactgcacgagtacatgctggatctgcagcccgagacaaccgatctgtacggctatgagcagctgaatgactccagcgaggaagaggacgagatcgacggacctgctggacaggctgaacctgatagagcccactacaatatcgtgaccttctgctgcaagtgcgatagcaccctgagaagatgcgtgcagagcacccacgtggacatcaggaccctcgaggatctgctcatgggcaccctgggaattgtggccccaatctgctctcagaagcctggcagcggcgccaccaatttcagtctgcttaaacaggccggggacgtcgaagagaaccccggacctatgcatcggcgcagatctcggtcttgtagagaagaccaaaagcctgtcatggatgatcaaagagatttaatttctaataatgaacaattacccatgttgggacggcgccccggagcccccgaatctaagtgcagccggggagctttatatacaggattttctattttagtgaccttattattagctggccaagccacaacagcttatttcttataccaacaacaaggacggttagataaattaacagtcacatctcaaaatttacaattagagaatttaagaatgaaattacctaaaccacccaaacccgtcagtaaaatgagaatggctacccccttattaatgcaagccctccccatgggcgccttaccccaaggacccatgcaaaatgctacaaagtatggaaatatgacagaagatcatgtcatgcacttattacaaaacgctgaccccttaaaagtctatccccctttaaaaggatctttccctgaaaatttaagacatttaaaaaatacaatggagacaattgattggaaagtctttgaatcttggatgcatcattggttattatttgaaatgtctaggcattctttagagcaaaaacccaccgatgctccacccaaggaaagtttagagttagaggacccttctagcggattaggagtcaccaaacaggacttaggacccgtccccatgatggaaacactgtgccagcggctgaacgtgtgccaggacaagattctgacccactatgagaacgacagcaccgacctgagggaccacatcgactactggaagcacatgcggctggaatgcgccatctactacaaggctagagagatgggcttcaagcacatcaaccaccaggtggtgcctacactggccgtgtctaagaacaaggctctgcaggccatcgaactgcagctgaccctggaaacaatctacaactcccagtactccaacgagaagtggaccctccaggacgtgtcactggaagtgtacctgaccgctcctaccggctgcatcaagaaacacggctacaccgtggaagtgcagtttgacggcgatatctgcaataccatgcactacaccaactggacccacatctacatctgcgaagaggccagcgtgacagtggtggaaggccaggtcgactactacggcctgtactacgtgcacgagggcatcagaacctacttcgtgcagttcaaggatgacgccgagaagtacagcaagaacaaagtgtgggaagtgcacgctggcggccaagtgatcctgtgtcctacaagcgtgttcagcagcaacgaagtgtctagccccgagatcatcagacagcacctggccaatcatcctgccgccacacacacaaaagctgtggccctgggcaccgaggaaacacagaccacaattcagaggcccagaagcgagcccgataccggcaatccttgtcacaccaccaagctgctgcaccgggattccgtggattctgcccctatcctgaccgccttcaacagctcccacaaaggccggatcaactgcaacagcaacaccacacctatcgtgcacctgaaaggggacgccaacactctgaaggccctgcggtacagattcaagaagcactgtaccctgtataccgccgtgtccagcacatggcactggaccggacacaacgtgaaacacaagagcgccatcgtgaccctgacctacgatagcgagtggcagagggaccagttcctgagccaagtgaagatccctaagaccatcaccgtgtccaccggctttatgagcatttgaggaagaatgtgcacagtgctaaccagaaaattcaggacaagactagtgcggccgcttttat

SEQ ID NO: 94 - DNA, 3643 bp, Artificial Sequence
  HPV16 Ii-E1E6E7 integrated into TK locus of the poxviral vector
ggccaaaaattgaaattttattttttttttttggaatataaataatccctatcagtgatagagatctccctatcagtgatagagatcgtcgacgagctcgtttagtgaaccgtcagatcgcctggagacgccatccacgctgttttgacctctagcaccggtgccaccatgcacagaaggcggagcagaagctgccgcgaggatcagaaacccgtgatggacgaccagcgggacctgatcagcaacaacgagcagctgcctatgctcggcagaaggcctggcgctcctgagagcaaatgttctagaggcgccctgtacaccggcttcagcatcctggttacactgctgctggccggacaggctaccaccgcctactttctgtatcagcagcagggcagactggacaagctgaccgtgaccagccagaacctgcagctggaaaacctgcggatgaagctgcccaagcctcctaagcctgtgtccaagatgcggatggccacacctctgctgatgcaggctttgcctatgggagcactgcctcagggccctatgcagaacgccaccaaatacggcaacatgaccgaggaccacgtgatgcatctgctgcagaatgccgatcctctgaaggtgtaccctccactgaagggcagctttcccgagaacctgcggcacctgaagaacaccatggaaaccatcgactggaaggtgttcgagagctggatgcaccactggctgctgttcgagatgagccggcacagcctggaacagaagcctacagacgcccctcctaaagagtccctggaactggaagatcccagctctggcctgggcgtgacaaagcaagatctgggccctgtgcctatgatggccgatcctgctggcacaaacggcgaagaaggcacaggctgcaacggctggttttacgtggaagccgtggtggaaaagaaaaccggcgacgccatcagcgacgacgagaacgagaatgacagcgacaccggcgaggacctggtggacttcatcgtgaacgacaacgactacctgacacaggccgagacagagacagcccacgctctgtttacagcccaagaggccaagcagcacagagatgccgttcaggtgctgaagagaaagtacctgggcagccctctgagcgacatcagcggctgtgtggacaacaacatcagccccagactgaaggccatctgcatcgagaagcagagcagagccgccaagcggagactgtttgagagcgaggatagcggctacggcaataccgaggtggaaacccagcaaatgctgcaggtcgagggcagacacgaaaccgagacaccttgcagccagtacagcggaggatctggcggaggctgtagccagtactcttctggaagtggcggagagggcgtgtccgagagacacaccatttgtcagacccctctgaccaacatcctgaacgtgctgaaaaccagcaacgccaaggccgccatgctggccaagttcaaagagctgtacggcgtcagcttcagcgaactcgtgcggcccttcaagagcaacaagtccacctgttgcgactggtgcattgccgcctttggcctgacaccttctatcgccgacagcatcaagaccctgctccagcagtactgtctgtacctgcacattcagagcctggcctgctcttggggaatggtggtgctgctgctcgtgcggtacaagtgcggcaagaacagagagacaattgagaagctgctgagcaaactgctgtgcgtgtcccctatgtgcatgatgatcgagcctccaaagctgcggtctacagccgccgctctgtactggtacaagaccggcatcagcaatatctccgaggtgtacggcgacacccctgagtggattcagagacagaccgtcctgcagcacagcttcaacgactgcaccttcgagctgtcccagatggtgcagtgggcctacgacaatgacatcgtggacgactccgagatcgcctataagtacgcccagctggccgacaccaacagcaatgccagcgccttcctgaagtccaacagccaggccaagatcgtgaaggactgcgccaccatgtgcagacactacaagcgggccgagaagaaacagatgagcatgagccagtggatcaagtacagatgcgacagagtggacgacggcggcgattggaagcagatcgtgatgttcctgagataccagggcgtcgagttcatgagctttctgacagccctgaagcggttcctgcagggcatccccaagaagaactgcatcctgctgtatggcgccgctaacaccggcaagagcctgttcggaatgagcctgatgaagtttctgcagggctccgtgatctgctttgtgaacagcaagagccacttctggctccagccactggccgatgccaagattggcatgctggacgatgccaccgtgccttgctggaactacatcgacgacaacctgagaaacgccctggacggcaacctggtttctatggacgtgaagcacagacccctggtgcagctgaagtgtcctccactgctgatcaccagcaacatcaacgccggcaccgattccagatggccctatctgcacaaccggctggtggtgtttacctttcctaacgagttccccttcgacgaaaacggcaaccccgtgtacgagctgaacgataagaattggaagtccttcttcagccggacctggtccagactgagcctgcacgaggatgaggacaaagagaacgacggcgacagcctgcctaccttcaaatgtgtcagcggccagaacaccaacacactgggcagcatgcaccagaaacggacagccatgttccaggatcctcaagagcggccacggaagctgcctcagctgtgtacagaactgcagaccaccatccacgacatcatcctcgagtgcgtgtactgcaagcagcagctcctgcggagagaagtgtacgacttcgccttccgggatctgtgcatcgtgtacagagatggcaacccctacgccgtgtgcgacaagtgcctgaagttctactccaagatcagcgagtaccggcactactgctactccctgtacggcaccacacttgagcagcagtacaacaagcccctgtgcgatctgctgatccggtgcatcaactgccagaaacctcagtgccccgaggaaaagcagagacacctggacaagaagcagcggttccacaacattagaggcagatggacaggccggtgcatgagctgctgtagaagcagcagaacaagacggggctccatgcacggcgataccccaacactgcacgagtacatgctggatctgcagcccgagacaaccgatctgtacggctatgagcagctgaatgactccagcgaggaagaggacgagatcgacggacctgctggacaggctgaacctgatagagcccactacaatatcgtgaccttctgctgcaagtgcgatagcaccctgagaagatgcgtgcagagcacccacgtggacatcaggaccctcgaggatctgctcatgggcaccctgggaattgtggccccaatctgctctcagaagccttgaggaagaatgtgcacagtgctaaccagaaaattcaggacaagactagtgcggccgcttttat

SEQ ID NO: 95 - DNA, 4789 bp, Artificial Sequence
  HPV18 Ii-E1E2E6E7 integrated into TK locus of the poxviral vector
ggccaaaaattgaaattttattttttttttttggaatataaataatccctatcagtgatagagatctccctatcagtgatagagatcgtcgacgagctcgtttagtgaaccgtcagatcgcctggagacgccatccacgctgttttgacctctagcaccggtgccaccatgcacagaaggcggagcagaagctgccgcgaggatcagaaacccgtgatggacgaccagcgggacctgatcagcaacaacgagcagctgcctatgctcggcagaaggcctggcgctcctgagagcaaatgttctagaggcgccctgtacaccggcttcagcatcctggttacactgctgctggccggacaggctaccaccgcctactttctgtatcagcagcagggcagactggacaagctgaccgtgaccagccagaacctgcagctggaaaacctgcggatgaagctgcccaagcctcctaagcctgtgtccaagatgcggatggccacacctctgctgatgcaggctttgcctatgggagcactgcctcagggccctatgcagaacgccaccaaatacggcaacatgaccgaggaccacgtgatgcatctgctgcagaatgccgatcctctgaaggtgtaccctccactgaagggcagctttcccgagaacctgcggcacctgaagaacaccatggaaaccatcgactggaaggtgttcgagagctggatgcaccactggctgctgttcgagatgagccggcacagcctggaacagaagcctacagacgcccctcctaaagagtccctggaactggaagatcccagctctggcctgggcgtgacaaagcaagatctgggccctgtgcctatgatggccgatcctgagggaacagatggcgaaggcacaggctgcaacggctggttttacgtgcaagccatcgtggacaagaagaccggcgacgtcatcagcgacgacgaggatgagaatgccaccgacaccggcagcgacatggtggactttatcgatacccagggcacgttctgcgagcaggccgaactggaaacagcccaggcactgtttcacgcccaagaggtgcacaacgatgcccaggtgctgcacgtgctgaagagaaagtttgccggcggaagcaccgagaacagcccactgggagaaagactggaagtggacaccgagctgagccccagactgcaagagatcagcctgaacagcggccagaagaaggccaagcggagactgttcaccatctccgacagcggctacggctgtagcgaagtggaagccacacagatccaagtgaccaccaatggcgagcacggcggcaatgtttgttctggcggatctaccgaggccatcgacaatggcggaaccgagggcaacaatagctccgtggatggcaccagcgacaacagcaacatcgagaacgtgaaccctcagtgcacaatcgcccagctgaaggacctgctgaaagtgaacaacaagcagggcgccatgctggccgtgtttaaggatacctacggcctgagcttcaccgacctcgtgcggaacttcaagagcgacaagaccacctgtaccgactgggtcaccgccatctttggcgtgaacccaacaatcgccgagggcttcaagaccctgatccagcctttcatcctgtacgcccacatccagtgtctggactgcaaatggggcgtgctgattctggccctgctgagatacaagtgcggcaagagcagactgaccgtggccaagggactgagcactctgctgcatgtgcccgagacatgcatgctgattcagcctccaaagctgcggtctagcgtggccgctctgtactggtacagaaccggcatcagcaatatcagcgaagtgatgggcgacacccctgagtggattcagcggctgacaatcatccagcacggcatcgacgactccaacttcgacctgagcgagatggtgcagtgggccttcgataacgagctgaccgacgagtccgacatggcctttgaatacgccctgctggcagacagcaactccaatgccgccgctttcctgaagtccaactgccaggccaagtacctgaaggactgcgccaccatgtgcaagcactaccgcagagcacagaaacggcagatgaacatgagccagtggatccggttccggtgcagcaagatcgatgaaggtggcgactggcggcctatcgtgcagttcctgagataccagcagatcgagttcatcacctttctgggcgccctgaagtcattcctgaagggaacccctaaaaagaactgcctggtgttctgcggccctgccaataccggcaagtcctacttcggcatgagctttatccacttcatccagggcgccgtgatcagcttcgtgaacagcaccagccacttttggctggaacccctgaccgataccaaggtggcaatgctggacgacgccaccaccacctgttggacctacttcgacacctacatgcggaacgccctggacggcaaccccatcagcatcgacagaaagcacaagcccctcatccagctgaaatgccctccaatcctgctgaccacaaacattcaccccgccaaggacaatcggtggccctacctggaaagccggatcaccgtgttcgagttccccaacgcctttccattcgacaagaacggcaatcccgtgtacgagatcaacgacaagaattggaagtgcttcttcgagcggacctggtccagactggatctgcacgaggaagaagaggacgccgacacagagggcaatcccttcggcacctttaagtgtgtggccgggcagaatcacagacccctgggatctatgcagaccccaaaagagacactgagcgagcggctgagcgccctccaggacaagatcatcgaccactacgagaacgacagcaaggacatcgacagccagattcagtactggcagctgatcagatgggagaacgccatcttcttcgccgctagagagcacggaattcagaccctgaaccaccaggtggtgcccgcctacaacatcagcaagagcaaggcccacaaggccattgaactccagatggccctgcaaggactggctcagagcgcctacaagaccgaggattggacactccaggatacctgcgaggaactgtggaacacagagcccacacactgcttcaagaaaggcggccagaccgtgcaggtctacttcgatggcaacaaggataactgcatgacctacgtggcctgggacagcgtgtactacatgacagatgccggcacctgggacaagaccgccacctgtgtttctcaccggggcctgtactacgtgaaagagggctacaacaccttctacatcgagtttaagagcgagtgcgagaagtatggcaacaccggcacatgggaagtgcatttcggcaacaacgtgatcgactgcaacgactccatgtgctccacctccgatgacaccgtgtctgccacacagctggtcaagcagctccagcacaccccatctccatacagctctacagtgtctgtgggcaccgccaagacctatggccaaacaagcgctgccacaagacctggccattgtggactggccgagaagcagcactgtggccctgttaatcctctgctgggagccgccacacctacaggcaacaacaagagaagaaagctgtgcagcggcaacaccacacctatcattcacctgaagggcgacagaaacagcctgaagtgcctgcggtacagactgaggaagcacagcgatcactaccgggacatcagctccacctggcactggacaggtgctggcaacgaaaagaccggcatcctgacagtgacctaccacagcgagactcagcggaccaagttcctgaacaccgtggctatccccgacagcgtgcagattctcgtgggctacatgaccatgggcagcatggccagattcgaggaccctaccagacggccctacaagctgcctgatctgtgcaccgaactgaacaccagccttcaggatatcgagatcacctgtgtgtactgcaagaccgtgctcgagctgacagaagtgtttgagttcgccttcaaggacctgttcgtggtgtacagagacagcatccctcacgccgcctgtcacaagtgcatcgacttctacagcagaatcagagagctgcggcactacagcgactccgtgtacggcgataccctggaaaaactgaccaacaccggactgtacaacctgctgatccggtgcctgagatgccagaaacctcagaaccccgccgagaaactgagacatctgaacgagaagcggcggttccacaatatcgccggccactacagaggccagtgccacagctgttgcaaccgggccagacaagaaagactccagcggagaagaggcagcatgcacggacctaaagccacacttcaggacatcgtgctgcacctcgagcctcagaatgagatccccgtggatctgctcggccatgagcagctgagcgatagcgaggaagagaacgacgagatcgacggcgtcaaccaccagcatctgcctgccagaagggccgaacctcagagacacaccatgctgtgcatgtgctgcaagtgcgaggcccggatcgagagagtggtggaatctagcgccgacgacctgagagctttccagcagctgttcctgaatactctgagcttcgtggccccttggtgcgctagtcagcagtgaggaagaatgtgcacagtgctaaccagaaaattcaggacaagactagtgcggccgcttttat

SEQ ID NO: 96 - DNA, 5545 bp, Artificial Sequence
  HPV18 Ii-E1E2-p2a-Ii-E6E7 integrated into TK locus of the poxviral vector
ggccaaaaattgaaattttattttttttttttggaatataaataatccctatcagtgatagagatctccctatcagtgatagagatcgtcgacgagctcgtttagtgaaccgtcagatcgcctggagacgccatccacgctgttttgacctctagcaccggtgccaccatgcacagaaggcggagcagaagctgccgcgaggatcagaaacccgtgatggacgaccagcgggacctgatcagcaacaacgagcagctgcctatgctcggcagaaggcctggcgctcctgagagcaaatgttctagaggcgccctgtacaccggcttcagcatcctggttacactgctgctggccggacaggctaccaccgcctactttctgtatcagcagcagggcagactggacaagctgaccgtgaccagccagaacctgcagctggaaaacctgcggatgaagctgcccaagcctcctaagcctgtgtccaagatgcggatggccacacctctgctgatgcaggctttgcctatgggagcactgcctcagggccctatgcagaacgccaccaaatacggcaacatgaccgaggaccacgtgatgcatctgctgcagaatgccgatcctctgaaggtgtaccctccactgaagggcagctttcccgagaacctgcggcacctgaagaacaccatggaaaccatcgactggaaggtgttcgagagctggatgcaccactggctgctgttcgagatgagccggcacagcctggaacagaagcctacagacgcccctcctaaagagtccctggaactggaagatcccagctctggcctgggcgtgacaaagcaagatctgggccctgtgcctatgatggccgatcctgagggaacagatggcgaaggcacaggctgcaacggctggttttacgtgcaagccatcgtggacaagaagaccggcgacgtcatcagcgacgacgaggatgagaatgccaccgacaccggcagcgacatggtggactttatcgatacccagggcacgttctgcgagcaggccgaactggaaacagcccaggcactgtttcacgcccaagaggtgcacaacgatgcccaggtgctgcacgtgctgaagagaaagtttgccggcggaagcaccgagaacagcccactgggagaaagactggaagtggacaccgagctgagccccagactgcaagagatcagcctgaacagcggccagaagaaggccaagcggagactgttcaccatctccgacagcggctacggctgtagcgaagtggaagccacacagatccaagtgaccaccaatggcgagcacggcggcaatgtttgttctggcggatctaccgaggccatcgacaatggcggaaccgagggcaacaatagctccgtggatggcaccagcgacaacagcaacatcgagaacgtgaaccctcagtgcacaatcgcccagctgaaggacctgctgaaagtgaacaacaagcagggcgccatgctggccgtgtttaaggatacctacggcctgagcttcaccgacctcgtgcggaacttcaagagcgacaagaccacctgtaccgactgggtcaccgccatctttggcgtgaacccaacaatcgccgagggcttcaagaccctgatccagcctttcatcctgtacgcccacatccagtgtctggactgcaaatggggcgtgctgattctggccctgctgagatacaagtgcggcaagagcagactgaccgtggccaagggactgagcactctgctgcatgtgcccgagacatgcatgctgattcagcctccaaagctgcggtctagcgtggccgctctgtactggtacagaaccggcatcagcaatatcagcgaagtgatgggcgacacccctgagtggattcagcggctgacaatcatccagcacggcatcgacgactccaacttcgacctgagcgagatggtgcagtgggccttcgataacgagctgaccgacgagtccgacatggcctttgaatacgccctgctggcagacagcaactccaatgccgccgctttcctgaagtccaactgccaggccaagtacctgaaggactgcgccaccatgtgcaagcactaccgcagagcacagaaacggcagatgaacatgagccagtggatccggttccggtgcagcaagatcgatgaaggtggcgactggcggcctatcgtgcagttcctgagataccagcagatcgagttcatcacctttctgggcgccctgaagtcattcctgaagggaacccctaaaaagaactgcctggtgttctgcggccctgccaataccggcaagtcctacttcggcatgagctttatccacttcatccagggcgccgtgatcagcttcgtgaacagcaccagccacttttggctggaacccctgaccgataccaaggtggcaatgctggacgacgccaccaccacctgttggacctacttcgacacctacatgcggaacgccctggacggcaaccccatcagcatcgacagaaagcacaagcccctcatccagctgaaatgccctccaatcctgctgaccacaaacattcaccccgccaaggacaatcggtggccctacctggaaagccggatcaccgtgttcgagttccccaacgcctttccattcgacaagaacggcaatcccgtgtacgagatcaacgacaagaattggaagtgcttcttcgagcggacctggtccagactggatctgcacgaggaagaagaggacgccgacacagagggcaatcccttcggcacctttaagtgtgtggccgggcagaatcacagacccctgggatctatgcagaccccaaaagagacactgagcgagcggctgagcgccctccaggacaagatcatcgaccactacgagaacgacagcaaggacatcgacagccagattcagtactggcagctgatcagatgggagaacgccatcttcttcgccgctagagagcacggaattcagaccctgaaccaccaggtggtgcccgcctacaacatcagcaagagcaaggcccacaaggccattgaactccagatggccctgcaaggactggctcagagcgcctacaagaccgaggattggacactccaggatacctgcgaggaactgtggaacacagagcccacacactgcttcaagaaaggcggccagaccgtgcaggtctacttcgatggcaacaaggataactgcatgacctacgtggcctgggacagcgtgtactacatgacagatgccggcacctgggacaagaccgccacctgtgtttctcaccggggcctgtactacgtgaaagagggctacaacaccttctacatcgagtttaagagcgagtgcgagaagtatggcaacaccggcacatgggaagtgcatttcggcaacaacgtgatcgactgcaacgactccatgtgctccacctccgatgacaccgtgtctgccacacagctggtcaagcagctccagcacaccccatctccatacagctctacagtgtctgtgggcaccgccaagacctatggccaaacaagcgctgccacaagacctggccattgtggactggccgagaagcagcactgtggccctgttaatcctctgctgggagccgccacacctacaggcaacaacaagagaagaaagctgtgcagcggcaacaccacacctatcattcacctgaagggcgacagaaacagcctgaagtgcctgcggtacagactgaggaagcacagcgatcactaccgggacatcagctccacctggcactggacaggtgctggcaacgaaaagaccggcatcctgacagtgacctaccacagcgagactcagcggaccaagttcctgaacaccgtggctatccccgacagcgtgcagattctcgtgggctacatgaccatgggcagcggcgccaccaatttcagtctgcttaaacaggccggggacgtcgaagagaaccccggacctatgcatcggcgcagatctcggtcttgtagagaagaccaaaagcctgtcatggatgatcaaagagatttaatttctaataatgaacaattacccatgttgggacggcgccccggagcccccgaatctaagtgcagccggggagctttatatacaggattttctattttagtgaccttattattagctggccaagccacaacagcttatttcttataccaacaacaaggacggttagataaattaacagtcacatctcaaaatttacaattagagaatttaagaatgaaattacctaaaccacccaaacccgtcagtaaaatgagaatggctacccccttattaatgcaagccctccccatgggcgccttaccccaaggacccatgcaaaatgctacaaagtatggaaatatgacagaagatcatgtcatgcacttattacaaaacgctgaccccttaaaagtctatccccctttaaaaggatctttccctgaaaatttaagacatttaaaaaatacaatggagacaattgattggaaagtctttgaatcttggatgcatcattggttattatttgaaatgtctaggcattctttagagcaaaaacccaccgatgctccacccaaggaaagtttagagttagaggacccttctagcggattaggagtcaccaaacaggacttaggacccgtccccatgatggccagattcgaggaccctaccagacggccctacaagctgcctgatctgtgcaccgaactgaacaccagccttcaggatatcgagatcacctgtgtgtactgcaagaccgtgctcgagctgacagaagtgtttgagttcgccttcaaggacctgttcgtggtgtacagagacagcatccctcacgccgcctgtcacaagtgcatcgacttctacagcagaatcagagagctgcggcactacagcgactccgtgtacggcgataccctggaaaaactgaccaacaccggactgtacaacctgctgatccggtgcctgagatgccagaaacctcagaaccccgccgagaaactgagacatctgaacgagaagcggcggttccacaatatcgccggccactacagaggccagtgccacagctgttgcaaccgggccagacaagaaagactccagcggagaagaggcagcatgcacggacctaaagccacacttcaggacatcgtgctgcacctcgagcctcagaatgagatccccgtggatctgctcggccatgagcagctgagcgatagcgaggaagagaacgacgagatcgacggcgtcaaccaccagcatctgcctgccagaagggccgaacctcagagacacaccatgctgtgcatgtgctgcaagtgcgaggcccggatcgagagagtggtggaatctagcgccgacgacctgagagctttccagcagctgttcctgaatactctgagcttcgtggccccttggtgcgctagtcagcagtgaggaagaatgtgcacagtgctaaccagaaaattcaggacaagactagtgcggccgcttttat

SEQ ID NO: 97 - DNA, 4093 bp, Artificial Sequence
  HPV18 E1E2E6E7 integrated into TK locus of the poxviral vector
ggccaaaaattgaaattttattttttttttttggaatataaataatccctatcagtgatagagatctccctatcagtgatagagatcgtcgacgagctcgtttagtgaaccgtcagatcgcctggagacgccatccacgctgttttgacctctagcaccggtgccaccatggccgatcctgagggaacagatggcgaaggcacaggctgcaacggctggttttacgtgcaagccatcgtggacaagaagaccggcgacgtcatcagcgacgacgaggatgagaatgccaccgacaccggcagcgacatggtggactttatcgatacccagggcacgttctgcgagcaggccgaactggaaacagcccaggcactgtttcacgcccaagaggtgcacaacgatgcccaggtgctgcacgtgctgaagagaaagtttgccggcggaagcaccgagaacagcccactgggagaaagactggaagtggacaccgagctgagccccagactgcaagagatcagcctgaacagcggccagaagaaggccaagcggagactgttcaccatctccgacagcggctacggctgtagcgaagtggaagccacacagatccaagtgaccaccaatggcgagcacggcggcaatgtttgttctggcggatctaccgaggccatcgacaatggcggaaccgagggcaacaatagctccgtggatggcaccagcgacaacagcaacatcgagaacgtgaaccctcagtgcacaatcgcccagctgaaggacctgctgaaagtgaacaacaagcagggcgccatgctggccgtgtttaaggatacctacggcctgagcttcaccgacctcgtgcggaacttcaagagcgacaagaccacctgtaccgactgggtcaccgccatctttggcgtgaacccaacaatcgccgagggcttcaagaccctgatccagcctttcatcctgtacgcccacatccagtgtctggactgcaaatggggcgtgctgattctggccctgctgagatacaagtgcggcaagagcagactgaccgtggccaagggactgagcactctgctgcatgtgcccgagacatgcatgctgattcagcctccaaagctgcggtctagcgtggccgctctgtactggtacagaaccggcatcagcaatatcagcgaagtgatgggcgacacccctgagtggattcagcggctgacaatcatccagcacggcatcgacgactccaacttcgacctgagcgagatggtgcagtgggccttcgataacgagctgaccgacgagtccgacatggcctttgaatacgccctgctggcagacagcaactccaatgccgccgctttcctgaagtccaactgccaggccaagtacctgaaggactgcgccaccatgtgcaagcactaccgcagagcacagaaacggcagatgaacatgagccagtggatccggttccggtgcagcaagatcgatgaaggtggcgactggcggcctatcgtgcagttcctgagataccagcagatcgagttcatcacctttctgggcgccctgaagtcattcctgaagggaacccctaaaaagaactgcctggtgttctgcggccctgccaataccggcaagtcctacttcggcatgagctttatccacttcatccagggcgccgtgatcagcttcgtgaacagcaccagccacttttggctggaacccctgaccgataccaaggtggcaatgctggacgacgccaccaccacctgttggacctacttcgacacctacatgcggaacgccctggacggcaaccccatcagcatcgacagaaagcacaagcccctcatccagctgaaatgccctccaatcctgctgaccacaaacattcaccccgccaaggacaatcggtggccctacctggaaagccggatcaccgtgttcgagttccccaacgcctttccattcgacaagaacggcaatcccgtgtacgagatcaacgacaagaattggaagtgcttcttcgagcggacctggtccagactggatctgcacgaggaagaagaggacgccgacacagagggcaatcccttcggcacctttaagtgtgtggccgggcagaatcacagacccctgggatctatgcagaccccaaaagagacactgagcgagcggctgagcgccctccaggacaagatcatcgaccactacgagaacgacagcaaggacatcgacagccagattcagtactggcagctgatcagatgggagaacgccatcttcttcgccgctagagagcacggaattcagaccctgaaccaccaggtggtgcccgcctacaacatcagcaagagcaaggcccacaaggccattgaactccagatggccctgcaaggactggctcagagcgcctacaagaccgaggattggacactccaggatacctgcgaggaactgtggaacacagagcccacacactgcttcaagaaaggcggccagaccgtgcaggtctacttcgatggcaacaaggataactgcatgacctacgtggcctgggacagcgtgtactacatgacagatgccggcacctgggacaagaccgccacctgtgtttctcaccggggcctgtactacgtgaaagagggctacaacaccttctacatcgagtttaagagcgagtgcgagaagtatggcaacaccggcacatgggaagtgcatttcggcaacaacgtgatcgactgcaacgactccatgtgctccacctccgatgacaccgtgtctgccacacagctggtcaagcagctccagcacaccccatctccatacagctctacagtgtctgtgggcaccgccaagacctatggccaaacaagcgctgccacaagacctggccattgtggactggccgagaagcagcactgtggccctgttaatcctctgctgggagccgccacacctacaggcaacaacaagagaagaaagctgtgcagcggcaacaccacacctatcattcacctgaagggcgacagaaacagcctgaagtgcctgcggtacagactgaggaagcacagcgatcactaccgggacatcagctccacctggcactggacaggtgctggcaacgaaaagaccggcatcctgacagtgacctaccacagcgagactcagcggaccaagttcctgaacaccgtggctatccccgacagcgtgcagattctcgtgggctacatgaccatgggcagcatggccagattcgaggaccctaccagacggccctacaagctgcctgatctgtgcaccgaactgaacaccagccttcaggatatcgagatcacctgtgtgtactgcaagaccgtgctcgagctgacagaagtgtttgagttcgccttcaaggacctgttcgtggtgtacagagacagcatccctcacgccgcctgtcacaagtgcatcgacttctacagcagaatcagagagctgcggcactacagcgactccgtgtacggcgataccctggaaaaactgaccaacaccggactgtacaacctgctgatccggtgcctgagatgccagaaacctcagaaccccgccgagaaactgagacatctgaacgagaagcggcggttccacaatatcgccggccactacagaggccagtgccacagctgttgcaaccgggccagacaagaaagactccagcggagaagaggcagcatgcacggacctaaagccacacttcaggacatcgtgctgcacctcgagcctcagaatgagatccccgtggatctgctcggccatgagcagctgagcgatagcgaggaagagaacgacgagatcgacggcgtcaaccaccagcatctgcctgccagaagggccgaacctcagagacacaccatgctgtgcatgtgctgcaagtgcgaggcccggatcgagagagtggtggaatctagcgccgacgacctgagagctttccagcagctgttcctgaatactctgagcttcgtggccccttggtgcgctagtcagcagtgaggaagaatgtgcacagtgctaaccagaaaattcaggacaagactagtgcggccgcttttat

SEQ ID NO: 98 - DNA, 5545 bp, Artificial Sequence
  HPV18 Ii-E1E6E7-p2a-Ii-E2 integrated into TK locus of the poxviral vector
ggccaaaaattgaaattttattttttttttttggaatataaataatccctatcagtgatagagatctccctatcagtgatagagatcgtcgacgagctcgtttagtgaaccgtcagatcgcctggagacgccatccacgctgttttgacctctagcaccggtgccaccatgcacagaaggcggagcagaagctgccgcgaggatcagaaacccgtgatggacgaccagcgggacctgatcagcaacaacgagcagctgcctatgctcggcagaaggcctggcgctcctgagagcaaatgttctagaggcgccctgtacaccggcttcagcatcctggttacactgctgctggccggacaggctaccaccgcctactttctgtatcagcagcagggcagactggacaagctgaccgtgaccagccagaacctgcagctggaaaacctgcggatgaagctgcccaagcctcctaagcctgtgtccaagatgcggatggccacacctctgctgatgcaggctttgcctatgggagcactgcctcagggccctatgcagaacgccaccaaatacggcaacatgaccgaggaccacgtgatgcatctgctgcagaatgccgatcctctgaaggtgtaccctccactgaagggcagctttcccgagaacctgcggcacctgaagaacaccatggaaaccatcgactggaaggtgttcgagagctggatgcaccactggctgctgttcgagatgagccggcacagcctggaacagaagcctacagacgcccctcctaaagagtccctggaactggaagatcccagctctggcctgggcgtgacaaagcaagatctgggccctgtgcctatgatggccgatcctgagggaacagatggcgaaggcacaggctgcaacggctggttttacgtgcaagccatcgtggacaagaagaccggcgacgtcatcagcgacgacgaggatgagaatgccaccgacaccggcagcgacatggtggactttatcgatacccagggcacgttctgcgagcaggccgaactggaaacagcccaggcactgtttcacgcccaagaggtgcacaacgatgcccaggtgctgcacgtgctgaagagaaagtttgccggcggaagcaccgagaacagcccactgggagaaagactggaagtggacaccgagctgagccccagactgcaagagatcagcctgaacagcggccagaagaaggccaagcggagactgttcaccatctccgacagcggctacggctgtagcgaagtggaagccacacagatccaagtgaccaccaatggcgagcacggcggcaatgtttgttctggcggatctaccgaggccatcgacaatggcggaaccgagggcaacaatagctccgtggatggcaccagcgacaacagcaacatcgagaacgtgaaccctcagtgcacaatcgcccagctgaaggacctgctgaaagtgaacaacaagcagggcgccatgctggccgtgtttaaggatacctacggcctgagcttcaccgacctcgtgcggaacttcaagagcgacaagaccacctgtaccgactgggtcaccgccatctttggcgtgaacccaacaatcgccgagggcttcaagaccctgatccagcctttcatcctgtacgcccacatccagtgtctggactgcaaatggggcgtgctgattctggccctgctgagatacaagtgcggcaagagcagactgaccgtggccaagggactgagcactctgctgcatgtgcccgagacatgcatgctgattcagcctccaaagctgcggtctagcgtggccgctctgtactggtacagaaccggcatcagcaatatcagcgaagtgatgggcgacacccctgagtggattcagcggctgacaatcatccagcacggcatcgacgactccaacttcgacctgagcgagatggtgcagtgggccttcgataacgagctgaccgacgagtccgacatggcctttgaatacgccctgctggcagacagcaactccaatgccgccgctttcctgaagtccaactgccaggccaagtacctgaaggactgcgccaccatgtgcaagcactaccgcagagcacagaaacggcagatgaacatgagccagtggatccggttccggtgcagcaagatcgatgaaggtggcgactggcggcctatcgtgcagttcctgagataccagcagatcgagttcatcacctttctgggcgccctgaagtcattcctgaagggaacccctaaaaagaactgcctggtgttctgcggccctgccaataccggcaagtcctacttcggcatgagctttatccacttcatccagggcgccgtgatcagcttcgtgaacagcaccagccacttttggctggaacccctgaccgataccaaggtggcaatgctggacgacgccaccaccacctgttggacctacttcgacacctacatgcggaacgccctggacggcaaccccatcagcatcgacagaaagcacaagcccctcatccagctgaaatgccctccaatcctgctgaccacaaacattcaccccgccaaggacaatcggtggccctacctggaaagccggatcaccgtgttcgagttccccaacgcctttccattcgacaagaacggcaatcccgtgtacgagatcaacgacaagaattggaagtgcttcttcgagcggacctggtccagactggatctgcacgaggaagaagaggacgccgacacagagggcaatcccttcggcacctttaagtgtgtggccgggcagaatcacagacccctgggcagcatggccagattcgaggaccctaccagacggccctacaagctgcctgatctgtgcaccgaactgaacaccagccttcaggatatcgagatcacctgtgtgtactgcaagaccgtgctcgagctgacagaagtgtttgagttcgccttcaaggacctgttcgtggtgtacagagacagcatccctcacgccgcctgtcacaagtgcatcgacttctacagcagaatcagagagctgcggcactacagcgactccgtgtacggcgataccctggaaaaactgaccaacaccggactgtacaacctgctgatccggtgcctgagatgccagaaacctcagaaccccgccgagaaactgagacatctgaacgagaagcggcggttccacaatatcgccggccactacagaggccagtgccacagctgttgcaaccgggccagacaagaaagactccagcggagaagaggcagcatgcacggacctaaagccacacttcaggacatcgtgctgcacctcgagcctcagaatgagatccccgtggatctgctcggccatgagcagctgagcgatagcgaggaagagaacgacgagatcgacggcgtcaaccaccagcatctgcctgccagaagggccgaacctcagagacacaccatgctgtgcatgtgctgcaagtgcgaggcccggatcgagagagtggtggaatctagcgccgacgacctgagagctttccagcagctgttcctgaatactctgagcttcgtggccccttggtgcgctagtcagcagggcagcggcgccaccaatttcagtctgcttaaacaggccggggacgtcgaagagaaccccggacctatgcatcggcgcagatctcggtcttgtagagaagaccaaaagcctgtcatggatgatcaaagagatttaatttctaataatgaacaattacccatgttgggacggcgccccggagcccccgaatctaagtgcagccggggagctttatatacaggattttctattttagtgaccttattattagctggccaagccacaacagcttatttcttataccaacaacaaggacggttagataaattaacagtcacatctcaaaatttacaattagagaatttaagaatgaaattacctaaaccacccaaacccgtcagtaaaatgagaatggctacccccttattaatgcaagccctccccatgggcgccttaccccaaggacccatgcaaaatgctacaaagtatggaaatatgacagaagatcatgtcatgcacttattacaaaacgctgaccccttaaaagtctatccccctttaaaaggatctttccctgaaaatttaagacatttaaaaaatacaatggagacaattgattggaaagtctttgaatcttggatgcatcattggttattatttgaaatgtctaggcattctttagagcaaaaacccaccgatgctccacccaaggaaagtttagagttagaggacccttctagcggattaggagtcaccaaacaggacttaggacccgtccccatgatgcagaccccaaaagagacactgagcgagcggctgagcgccctccaggacaagatcatcgaccactacgagaacgacagcaaggacatcgacagccagattcagtactggcagctgatcagatgggagaacgccatcttcttcgccgctagagagcacggaattcagaccctgaaccaccaggtggtgcccgcctacaacatcagcaagagcaaggcccacaaggccattgaactccagatggccctgcaaggactggctcagagcgcctacaagaccgaggattggacactccaggatacctgcgaggaactgtggaacacagagcccacacactgcttcaagaaaggcggccagaccgtgcaggtctacttcgatggcaacaaggataactgcatgacctacgtggcctgggacagcgtgtactacatgacagatgccggcacctgggacaagaccgccacctgtgtttctcaccggggcctgtactacgtgaaagagggctacaacaccttctacatcgagtttaagagcgagtgcgagaagtatggcaacaccggcacatgggaagtgcatttcggcaacaacgtgatcgactgcaacgactccatgtgctccacctccgatgacaccgtgtctgccacacagctggtcaagcagctccagcacaccccatctccatacagctctacagtgtctgtgggcaccgccaagacctatggccaaacaagcgctgccacaagacctggccattgtggactggccgagaagcagcactgtggccctgttaatcctctgctgggagccgccacacctacaggcaacaacaagagaagaaagctgtgcagcggcaacaccacacctatcattcacctgaagggcgacagaaacagcctgaagtgcctgcggtacagactgaggaagcacagcgatcactaccgggacatcagctccacctggcactggacaggtgctggcaacgaaaagaccggcatcctgacagtgacctaccacagcgagactcagcggaccaagttcctgaacaccgtggctatccccgacagcgtgcagattctcgtgggctacatgaccatgtgaggaagaatgtgcacagtgctaaccagaaaattcaggacaagactagtgcggccgcttttat

SEQ ID NO: 99 - DNA, 3688 bp, Artificial Sequence
  HPV18 Ii-E1E6E7 integrated into TK locus of the poxviral vector
ggccaaaaattgaaattttattttttttttttggaatataaataatccctatcagtgatagagatctccctatcagtgatagagatcgtcgacgagctcgtttagtgaaccgtcagatcgcctggagacgccatccacgctgttttgacctctagcaccggtgccaccatgcacagaaggcggagcagaagctgccgcgaggatcagaaacccgtgatggacgaccagcgggacctgatcagcaacaacgagcagctgcctatgctcggcagaaggcctggcgctcctgagagcaaatgttctagaggcgccctgtacaccggcttcagcatcctggttacactgctgctggccggacaggctaccaccgcctactttctgtatcagcagcagggcagactggacaagctgaccgtgaccagccagaacctgcagctggaaaacctgcggatgaagctgcccaagcctcctaagcctgtgtccaagatgcggatggccacacctctgctgatgcaggctttgcctatgggagcactgcctcagggccctatgcagaacgccaccaaatacggcaacatgaccgaggaccacgtgatgcatctgctgcagaatgccgatcctctgaaggtgtaccctccactgaagggcagctttcccgagaacctgcggcacctgaagaacaccatggaaaccatcgactggaaggtgttcgagagctggatgcaccactggctgctgttcgagatgagccggcacagcctggaacagaagcctacagacgcccctcctaaagagtccctggaactggaagatcccagctctggcctgggcgtgacaaagcaagatctgggccctgtgcctatgatggccgatcctgagggaacagatggcgaaggcacaggctgcaacggctggttttacgtgcaagccatcgtggacaagaagaccggcgacgtcatcagcgacgacgaggatgagaatgccaccgacaccggcagcgacatggtggactttatcgatacccagggcacgttctgcgagcaggccgaactggaaacagcccaggcactgtttcacgcccaagaggtgcacaacgatgcccaggtgctgcacgtgctgaagagaaagtttgccggcggaagcaccgagaacagcccactgggagaaagactggaagtggacaccgagctgagccccagactgcaagagatcagcctgaacagcggccagaagaaggccaagcggagactgttcaccatctccgacagcggctacggctgtagcgaagtggaagccacacagatccaagtgaccaccaatggcgagcacggcggcaatgtttgttctggcggatctaccgaggccatcgacaatggcggaaccgagggcaacaatagctccgtggatggcaccagcgacaacagcaacatcgagaacgtgaaccctcagtgcacaatcgcccagctgaaggacctgctgaaagtgaacaacaagcagggcgccatgctggccgtgtttaaggatacctacggcctgagcttcaccgacctcgtgcggaacttcaagagcgacaagaccacctgtaccgactgggtcaccgccatctttggcgtgaacccaacaatcgccgagggcttcaagaccctgatccagcctttcatcctgtacgcccacatccagtgtctggactgcaaatggggcgtgctgattctggccctgctgagatacaagtgcggcaagagcagactgaccgtggccaagggactgagcactctgctgcatgtgcccgagacatgcatgctgattcagcctccaaagctgcggtctagcgtggccgctctgtactggtacagaaccggcatcagcaatatcagcgaagtgatgggcgacacccctgagtggattcagcggctgacaatcatccagcacggcatcgacgactccaacttcgacctgagcgagatggtgcagtgggccttcgataacgagctgaccgacgagtccgacatggcctttgaatacgccctgctggcagacagcaactccaatgccgccgctttcctgaagtccaactgccaggccaagtacctgaaggactgcgccaccatgtgcaagcactaccgcagagcacagaaacggcagatgaacatgagccagtggatccggttccggtgcagcaagatcgatgaaggtggcgactggcggcctatcgtgcagttcctgagataccagcagatcgagttcatcacctttctgggcgccctgaagtcattcctgaagggaacccctaaaaagaactgcctggtgttctgcggccctgccaataccggcaagtcctacttcggcatgagctttatccacttcatccagggcgccgtgatcagcttcgtgaacagcaccagccacttttggctggaacccctgaccgataccaaggtggcaatgctggacgacgccaccaccacctgttggacctacttcgacacctacatgcggaacgccctggacggcaaccccatcagcatcgacagaaagcacaagcccctcatccagctgaaatgccctccaatcctgctgaccacaaacattcaccccgccaaggacaatcggtggccctacctggaaagccggatcaccgtgttcgagttccccaacgcctttccattcgacaagaacggcaatcccgtgtacgagatcaacgacaagaattggaagtgcttcttcgagcggacctggtccagactggatctgcacgaggaagaagaggacgccgacacagagggcaatcccttcggcacctttaagtgtgtggccgggcagaatcacagacccctgggcagcatggccagattcgaggaccctaccagacggccctacaagctgcctgatctgtgcaccgaactgaacaccagccttcaggatatcgagatcacctgtgtgtactgcaagaccgtgctcgagctgacagaagtgtttgagttcgccttcaaggacctgttcgtggtgtacagagacagcatccctcacgccgcctgtcacaagtgcatcgacttctacagcagaatcagagagctgcggcactacagcgactccgtgtacggcgataccctggaaaaactgaccaacaccggactgtacaacctgctgatccggtgcctgagatgccagaaacctcagaaccccgccgagaaactgagacatctgaacgagaagcggcggttccacaatatcgccggccactacagaggccagtgccacagctgttgcaaccgggccagacaagaaagactccagcggagaagaggcagcatgcacggacctaaagccacacttcaggacatcgtgctgcacctcgagcctcagaatgagatccccgtggatctgctcggccatgagcagctgagcgatagcgaggaagagaacgacgagatcgacggcgtcaaccaccagcatctgcctgccagaagggccgaacctcagagacacaccatgctgtgcatgtgctgcaagtgcgaggcccggatcgagagagtggtggaatctagcgccgacgacctgagagctttccagcagctgttcctgaatactctgagcttcgtggccccttggtgcgctagtcagcagtgaggaagaatgtgcacagtgctaaccagaaaattcaggacaagactagtgcggccgcttttat

SEQ ID NO: 100 - DNA, 3462 bp, Human papillomavirus type 18
  HPV18 Ii-E1E6E7 different linker
atgcacagaaggcggagcagaagctgccgcgaggatcagaaacccgtgatggacgaccagcgggacctgatcagcaacaacgagcagctgcctatgctcggcagaaggcctggcgctcctgagagcaaatgttctagaggcgccctgtacaccggcttcagcatcctggttacactgctgctggccggacaggctaccaccgcctactttctgtatcagcagcagggcagactggacaagctgaccgtgaccagccagaacctgcagctggaaaacctgcggatgaagctgcccaagcctcctaagcctgtgtccaagatgcggatggccacacctctgctgatgcaggctttgcctatgggagcactgcctcagggccctatgcagaacgccaccaaatacggcaacatgaccgaggaccacgtgatgcatctgctgcagaatgccgatcctctgaaggtgtaccctccactgaagggcagctttcccgagaacctgcggcacctgaagaacaccatggaaaccatcgactggaaggtgttcgagagctggatgcaccactggctgctgttcgagatgagccggcacagcctggaacagaagcctacagacgcccctcctaaagagtccctggaactggaagatcccagctctggcctgggcgtgacaaagcaagatctgggccctgtgcctatgatggccgatcctgagggaacagatggcgaaggcacaggctgcaacggctggttttacgtgcaagccatcgtggacaagaagaccggcgacgtcatcagcgacgacgaggatgagaatgccaccgacaccggcagcgacatggtggactttatcgatacccagggcacgttctgcgagcaggccgaactggaaacagcccaggcactgtttcacgcccaagaggtgcacaacgatgcccaggtgctgcacgtgctgaagagaaagtttgccggcggaagcaccgagaacagcccactgggagaaagactggaagtggacaccgagctgagccccagactgcaagagatcagcctgaacagcggccagaagaaggccaagcggagactgttcaccatctccgacagcggctacggctgtagcgaagtggaagccacacagatccaagtgaccaccaatggcgagcacggcggcaatgtttgttctggcggatctaccgaggccatcgacaatggcggaaccgagggcaacaatagctccgtggatggcaccagcgacaacagcaacatcgagaacgtgaaccctcagtgcacaatcgcccagctgaaggacctgctgaaagtgaacaacaagcagggcgccatgctggccgtgtttaaggatacctacggcctgagcttcaccgacctcgtgcggaacttcaagagcgacaagaccacctgtaccgactgggtcaccgccatctttggcgtgaacccaacaatcgccgagggcttcaagaccctgatccagcctttcatcctgtacgcccacatccagtgtctggactgcaaatggggcgtgctgattctggccctgctgagatacaagtgcggcaagagcagactgaccgtggccaagggactgagcactctgctgcatgtgcccgagacatgcatgctgattcagcctccaaagctgcggtctagcgtggccgctctgtactggtacagaaccggcatcagcaatatcagcgaagtgatgggcgacacccctgagtggattcagcggctgacaatcatccagcacggcatcgacgactccaacttcgacctgagcgagatggtgcagtgggccttcgataacgagctgaccgacgagtccgacatggcctttgaatacgccctgctggcagacagcaactccaatgccgccgctttcctgaagtccaactgccaggccaagtacctgaaggactgcgccaccatgtgcaagcactaccgcagagcacagaaacggcagatgaacatgagccagtggatccggttccggtgcagcaagatcgatgaaggtggcgactggcggcctatcgtgcagttcctgagataccagcagatcgagttcatcacctttctgggcgccctgaagtcattcctgaagggaacccctaaaaagaactgcctggtgttctgcggccctgccaataccggcaagtcctacttcggcatgagctttatccacttcatccagggcgccgtgatcagcttcgtgaacagcaccagccacttttggctggaacccctgaccgataccaaggtggcaatgctggacgacgccaccaccacctgttggacctacttcgacacctacatgcggaacgccctggacggcaaccccatcagcatcgacagaaagcacaagcccctcatccagctgaaatgccctccaatcctgctgaccacaaacattcaccccgccaaggacaatcggtggccctacctggaaagccggatcaccgtgttcgagttccccaacgcctttccattcgacaagaacggcaatcccgtgtacgagatcaacgacaagaattggaagtgcttcttcgagcggacctggtccagactggatctgcacgaggaagaagaggacgccgacacagagggcaatcccttcggcacctttaagtgtgtggccgggcagaatcacagacccctgggctgcagcatggccagattcgaggaccctaccagacggccctacaagctgcctgatctgtgcaccgaactgaacaccagccttcaggatatcgagatcacctgtgtgtactgcaagaccgtgctcgagctgacagaagtgtttgagttcgccttcaaggacctgttcgtggtgtacagagacagcatccctcacgccgcctgtcacaagtgcatcgacttctacagcagaatcagagagctgcggcactacagcgactccgtgtacggcgataccctggaaaaactgaccaacaccggactgtacaacctgctgatccggtgcctgagatgccagaaacctcagaaccccgccgagaaactgagacatctgaacgagaagcggcggttccacaatatcgccggccactacagaggccagtgccacagctgttgcaaccgggccagacaagaaagactccagcggagaagaggcagcatgcacggacctaaagccacacttcaggacatcgtgctgcacctcgagcctcagaatgagatccccgtggatctgctcggccatgagcagctgagcgatagcgaggaagagaacgacgagatcgacggcgtcaaccaccagcatctgcctgccagaagggccgaacctcagagacacaccatgctgtgcatgtgctgcaagtgcgaggcccggatcgagagagtggtggaatctagcgccgacgacctgagagctttccagcagctgttcctgaatactctgagcttcgtggccccttggtgcgctagtcagcagtga

SEQ ID NO: 101 - protein, 1153 aa, Human papillomavirus type 18
  HPV18 Ii-E1E6E7 translated different linker
MHRRRSRSCREDQKPVMDDQRDLISNNEQLPMLGRRPGAPESKCSRGALYTGFSILVTLLLAGQATTAYFLYQQQGRLDKLTVTSQNLQLENLRMKLPKPPKPVSKMRMATPLLMQALPMGALPQGPMQNATKYGNMTEDHVMHLLQNADPLKVYPPLKGSFPENLRHLKNTMETIDWKVFESWMHHWLLFEMSRHSLEQKPTDAPPKESLELEDPSSGLGVTKQDLGPVPMMADPEGTDGEGTGCNGWFYVQAIVDKKTGDVISDDEDENATDTGSDMVDFIDTQGTFCEQAELETAQALFHAQEVHNDAQVLHVLKRKFAGGSTENSPLGERLEVDTELSPRLQEISLNSGQKKAKRRLFTISDSGYGCSEVEATQIQVTTNGEHGGNVCSGGSTEAIDNGGTEGNNSSVDGTSDNSNIENVNPQCTIAQLKDLLKVNNKQGAMLAVFKDTYGLSFTDLVRNFKSDKTTCTDWVTAIFGVNPTIAEGFKTLIQPFILYAHIQCLDCKWGVLILALLRYKCGKSRLTVAKGLSTLLHVPETCMLIQPPKLRSSVAALYWYRTGISNISEVMGDTPEWIQRLTIIQHGIDDSNFDLSEMVQWAFDNELTDESDMAFEYALLADSNSNAAAFLKSNCQAKYLKDCATMCKHYRRAQKRQMNMSQWIRFRCSKIDEGGDWRPIVQFLRYQQIEFITFLGALKSFLKGTPKKNCLVFCGPANTGKSYFGMSFIHFIQGAVISFVNSTSHFWLEPLTDTKVAMLDDATTTCWTYFDTYMRNALDGNPISIDRKHKPLIQLKCPPILLTTNIHPAKDNRWPYLESRITVFEFPNAFPFDKNGNPVYEINDKNWKCFFERTWSRLDLHEEEEDADTEGNPFGTFKCVAGQNHRPLGCSMARFEDPTRRPYKLPDLCTELNTSLQDIEITCVYCKTVLELTEVFEFAFKDLFVVYRDSIPHAACHKCIDFYSRIRELRHYSDSVYGDTLEKLTNTGLYNLLIRCLRCQKPQNPAEKLRHLNEKRRFHNIAGHYRGQCHSCCNRARQERLQRRRGSMHGPKATLQDIVLHLEPQNEIPVDLLGHEQLSDSEEENDEIDGVNHQHLPARRAEPQRHTMLCMCCKCEARIERVVESSADDLRAFQQLFLNTLSFVAPWCASQQ

SEQ ID NO: 102 - DNA, 4040 bp, Artificial Sequence
  HPV18 Ii-E1E6E7 different linker as carried by Adenoviral vector
gtgatgcggttttggcagtacatcaatgggcgtggatagcggtttgactcacggggatttccaagtctccaccccattgacgtcaatgggagtttgttttggaaccaaaatcaacgggactttccaaaatgtcgtaacaactccgccccattgacgcaaatgggcggtaggcgtgtacggtgggaggtctatataagcagagctctccctatcagtgatagagatctccctatcagtgatagagatcgtcgacgagctcgtttagtgaaccgtcagatcgcctggagacgccatccacgctgttttgacctctagcaccggtgccaccatgcacagaaggcggagcagaagctgccgcgaggatcagaaacccgtgatggacgaccagcgggacctgatcagcaacaacgagcagctgcctatgctcggcagaaggcctggcgctcctgagagcaaatgttctagaggcgccctgtacaccggcttcagcatcctggttacactgctgctggccggacaggctaccaccgcctactttctgtatcagcagcagggcagactggacaagctgaccgtgaccagccagaacctgcagctggaaaacctgcggatgaagctgcccaagcctcctaagcctgtgtccaagatgcggatggccacacctctgctgatgcaggctttgcctatgggagcactgcctcagggccctatgcagaacgccaccaaatacggcaacatgaccgaggaccacgtgatgcatctgctgcagaatgccgatcctctgaaggtgtaccctccactgaagggcagctttcccgagaacctgcggcacctgaagaacaccatggaaaccatcgactggaaggtgttcgagagctggatgcaccactggctgctgttcgagatgagccggcacagcctggaacagaagcctacagacgcccctcctaaagagtccctggaactggaagatcccagctctggcctgggcgtgacaaagcaagatctgggccctgtgcctatgatggccgatcctgagggaacagatggcgaaggcacaggctgcaacggctggttttacgtgcaagccatcgtggacaagaagaccggcgacgtcatcagcgacgacgaggatgagaatgccaccgacaccggcagcgacatggtggactttatcgatacccagggcacgttctgcgagcaggccgaactggaaacagcccaggcactgtttcacgcccaagaggtgcacaacgatgcccaggtgctgcacgtgctgaagagaaagtttgccggcggaagcaccgagaacagcccactgggagaaagactggaagtggacaccgagctgagccccagactgcaagagatcagcctgaacagcggccagaagaaggccaagcggagactgttcaccatctccgacagcggctacggctgtagcgaagtggaagccacacagatccaagtgaccaccaatggcgagcacggcggcaatgtttgttctggcggatctaccgaggccatcgacaatggcggaaccgagggcaacaatagctccgtggatggcaccagcgacaacagcaacatcgagaacgtgaaccctcagtgcacaatcgcccagctgaaggacctgctgaaagtgaacaacaagcagggcgccatgctggccgtgtttaaggatacctacggcctgagcttcaccgacctcgtgcggaacttcaagagcgacaagaccacctgtaccgactgggtcaccgccatctttggcgtgaacccaacaatcgccgagggcttcaagaccctgatccagcctttcatcctgtacgcccacatccagtgtctggactgcaaatggggcgtgctgattctggccctgctgagatacaagtgcggcaagagcagactgaccgtggccaagggactgagcactctgctgcatgtgcccgagacatgcatgctgattcagcctccaaagctgcggtctagcgtggccgctctgtactggtacagaaccggcatcagcaatatcagcgaagtgatgggcgacacccctgagtggattcagcggctgacaatcatccagcacggcatcgacgactccaacttcgacctgagcgagatggtgcagtgggccttcgataacgagctgaccgacgagtccgacatggcctttgaatacgccctgctggcagacagcaactccaatgccgccgctttcctgaagtccaactgccaggccaagtacctgaaggactgcgccaccatgtgcaagcactaccgcagagcacagaaacggcagatgaacatgagccagtggatccggttccggtgcagcaagatcgatgaaggtggcgactggcggcctatcgtgcagttcctgagataccagcagatcgagttcatcacctttctgggcgccctgaagtcattcctgaagggaacccctaaaaagaactgcctggtgttctgcggccctgccaataccggcaagtcctacttcggcatgagctttatccacttcatccagggcgccgtgatcagcttcgtgaacagcaccagccacttttggctggaacccctgaccgataccaaggtggcaatgctggacgacgccaccaccacctgttggacctacttcgacacctacatgcggaacgccctggacggcaaccccatcagcatcgacagaaagcacaagcccctcatccagctgaaatgccctccaatcctgctgaccacaaacattcaccccgccaaggacaatcggtggccctacctggaaagccggatcaccgtgttcgagttccccaacgcctttccattcgacaagaacggcaatcccgtgtacgagatcaacgacaagaattggaagtgcttcttcgagcggacctggtccagactggatctgcacgaggaagaagaggacgccgacacagagggcaatcccttcggcacctttaagtgtgtggccgggcagaatcacagacccctgggctgcagcatggccagattcgaggaccctaccagacggccctacaagctgcctgatctgtgcaccgaactgaacaccagccttcaggatatcgagatcacctgtgtgtactgcaagaccgtgctcgagctgacagaagtgtttgagttcgccttcaaggacctgttcgtggtgtacagagacagcatccctcacgccgcctgtcacaagtgcatcgacttctacagcagaatcagagagctgcggcactacagcgactccgtgtacggcgataccctggaaaaactgaccaacaccggactgtacaacctgctgatccggtgcctgagatgccagaaacctcagaaccccgccgagaaactgagacatctgaacgagaagcggcggttccacaatatcgccggccactacagaggccagtgccacagctgttgcaaccgggccagacaagaaagactccagcggagaagaggcagcatgcacggacctaaagccacacttcaggacatcgtgctgcacctcgagcctcagaatgagatccccgtggatctgctcggccatgagcagctgagcgatagcgaggaagagaacgacgagatcgacggcgtcaaccaccagcatctgcctgccagaagggccgaacctcagagacacaccatgctgtgcatgtgctgcaagtgcgaggcccggatcgagagagtggtggaatctagcgccgacgacctgagagctttccagcagctgttcctgaatactctgagcttcgtggccccttggtgcgctagtcagcagtgagcggccgcggaagaatgtgcacagtgctaaccagaaaattcaggacaagactagtgactctagatcataatcagccataccacatttgtagaggttttacttgctttaaaaaacctcccacacctccccctgaacctgaaacataaaatgaatgcaattgttgttgttaacttgtttattgcagcttataatggttacaaataaagcaatagcatcacaaatttcacaaataaagcatttttttcactgc

SEQ ID NO: 103 - DNA, 3755 bp, Artificial Sequence
  HPV18 Ii-E1E6E7 different linker integrated into DelIII locus of the poxviral vector
aaaaattaaaattttattttttttttttggaatataaataagatctatccctatcagtgatagagatctccctatcagtgatagagatcgtcgacgagctcgtttagtgaaccgtcagatcgcctggagacgccatccacgctgttttgacctctagcaccggtgccaccatgcacagaaggcggagcagaagctgccgcgaggatcagaaacccgtgatggacgaccagcgggacctgatcagcaacaacgagcagctgcctatgctcggcagaaggcctggcgctcctgagagcaaatgttctagaggcgccctgtacaccggcttcagcatcctggttacactgctgctggccggacaggctaccaccgcctactttctgtatcagcagcagggcagactggacaagctgaccgtgaccagccagaacctgcagctggaaaacctgcggatgaagctgcccaagcctcctaagcctgtgtccaagatgcggatggccacacctctgctgatgcaggctttgcctatgggagcactgcctcagggccctatgcagaacgccaccaaatacggcaacatgaccgaggaccacgtgatgcatctgctgcagaatgccgatcctctgaaggtgtaccctccactgaagggcagctttcccgagaacctgcggcacctgaagaacaccatggaaaccatcgactggaaggtgttcgagagctggatgcaccactggctgctgttcgagatgagccggcacagcctggaacagaagcctacagacgcccctcctaaagagtccctggaactggaagatcccagctctggcctgggcgtgacaaagcaagatctgggccctgtgcctatgatggccgatcctgagggaacagatggcgaaggcacaggctgcaacggctggttttacgtgcaagccatcgtggacaagaagaccggcgacgtcatcagcgacgacgaggatgagaatgccaccgacaccggcagcgacatggtggactttatcgatacccagggcacgttctgcgagcaggccgaactggaaacagcccaggcactgtttcacgcccaagaggtgcacaacgatgcccaggtgctgcacgtgctgaagagaaagtttgccggcggaagcaccgagaacagcccactgggagaaagactggaagtggacaccgagctgagccccagactgcaagagatcagcctgaacagcggccagaagaaggccaagcggagactgttcaccatctccgacagcggctacggctgtagcgaagtggaagccacacagatccaagtgaccaccaatggcgagcacggcggcaatgtttgttctggcggatctaccgaggccatcgacaatggcggaaccgagggcaacaatagctccgtggatggcaccagcgacaacagcaacatcgagaacgtgaaccctcagtgcacaatcgcccagctgaaggacctgctgaaagtgaacaacaagcagggcgccatgctggccgtgtttaaggatacctacggcctgagcttcaccgacctcgtgcggaacttcaagagcgacaagaccacctgtaccgactgggtcaccgccatctttggcgtgaacccaacaatcgccgagggcttcaagaccctgatccagcctttcatcctgtacgcccacatccagtgtctggactgcaaatggggcgtgctgattctggccctgctgagatacaagtgcggcaagagcagactgaccgtggccaagggactgagcactctgctgcatgtgcccgagacatgcatgctgattcagcctccaaagctgcggtctagcgtggccgctctgtactggtacagaaccggcatcagcaatatcagcgaagtgatgggcgacacccctgagtggattcagcggctgacaatcatccagcacggcatcgacgactccaacttcgacctgagcgagatggtgcagtgggccttcgataacgagctgaccgacgagtccgacatggcctttgaatacgccctgctggcagacagcaactccaatgccgccgctttcctgaagtccaactgccaggccaagtacctgaaggactgcgccaccatgtgcaagcactaccgcagagcacagaaacggcagatgaacatgagccagtggatccggttccggtgcagcaagatcgatgaaggtggcgactggcggcctatcgtgcagttcctgagataccagcagatcgagttcatcacctttctgggcgccctgaagtcattcctgaagggaacccctaaaaagaactgcctggtgttctgcggccctgccaataccggcaagtcctacttcggcatgagctttatccacttcatccagggcgccgtgatcagcttcgtgaacagcaccagccacttttggctggaacccctgaccgataccaaggtggcaatgctggacgacgccaccaccacctgttggacctacttcgacacctacatgcggaacgccctggacggcaaccccatcagcatcgacagaaagcacaagcccctcatccagctgaaatgccctccaatcctgctgaccacaaacattcaccccgccaaggacaatcggtggccctacctggaaagccggatcaccgtgttcgagttccccaacgcctttccattcgacaagaacggcaatcccgtgtacgagatcaacgacaagaattggaagtgcttcttcgagcggacctggtccagactggatctgcacgaggaagaagaggacgccgacacagagggcaatcccttcggcacctttaagtgtgtggccgggcagaatcacagacccctgggctgcagcatggccagattcgaggaccctaccagacggccctacaagctgcctgatctgtgcaccgaactgaacaccagccttcaggatatcgagatcacctgtgtgtactgcaagaccgtgctcgagctgacagaagtgtttgagttcgccttcaaggacctgttcgtggtgtacagagacagcatccctcacgccgcctgtcacaagtgcatcgacttctacagcagaatcagagagctgcggcactacagcgactccgtgtacggcgataccctggaaaaactgaccaacaccggactgtacaacctgctgatccggtgcctgagatgccagaaacctcagaaccccgccgagaaactgagacatctgaacgagaagcggcggttccacaatatcgccggccactacagaggccagtgccacagctgttgcaaccgggccagacaagaaagactccagcggagaagaggcagcatgcacggacctaaagccacacttcaggacatcgtgctgcacctcgagcctcagaatgagatccccgtggatctgctcggccatgagcagctgagcgatagcgaggaagagaacgacgagatcgacggcgtcaaccaccagcatctgcctgccagaagggccgaacctcagagacacaccatgctgtgcatgtgctgcaagtgcgaggcccggatcgagagagtggtggaatctagcgccgacgacctgagagctttccagcagctgttcctgaatactctgagcttcgtggccccttggtgcgctagtcagcagtgaggaagaatgtgcacagtgctaaccagaaaattcaggacaagactagtgcggccgctttggaaagttttataggtagttgatagaacaaaatacataattttgtaaaaataaatcactttttat

SEQ ID NO: 104 - DNA, 3691 bp, Artificial Sequence
  HPV18 Ii-E1E6E7 different linker integrated into TK locus of the poxviral vector
ggccaaaaattgaaattttattttttttttttggaatataaataatccctatcagtgatagagatctccctatcagtgatagagatcgtcgacgagctcgtttagtgaaccgtcagatcgcctggagacgccatccacgctgttttgacctctagcaccggtgccaccatgcacagaaggcggagcagaagctgccgcgaggatcagaaacccgtgatggacgaccagcgggacctgatcagcaacaacgagcagctgcctatgctcggcagaaggcctggcgctcctgagagcaaatgttctagaggcgccctgtacaccggcttcagcatcctggttacactgctgctggccggacaggctaccaccgcctactttctgtatcagcagcagggcagactggacaagctgaccgtgaccagccagaacctgcagctggaaaacctgcggatgaagctgcccaagcctcctaagcctgtgtccaagatgcggatggccacacctctgctgatgcaggctttgcctatgggagcactgcctcagggccctatgcagaacgccaccaaatacggcaacatgaccgaggaccacgtgatgcatctgctgcagaatgccgatcctctgaaggtgtaccctccactgaagggcagctttcccgagaacctgcggcacctgaagaacaccatggaaaccatcgactggaaggtgttcgagagctggatgcaccactggctgctgttcgagatgagccggcacagcctggaacagaagcctacagacgcccctcctaaagagtccctggaactggaagatcccagctctggcctgggcgtgacaaagcaagatctgggccctgtgcctatgatggccgatcctgagggaacagatggcgaaggcacaggctgcaacggctggttttacgtgcaagccatcgtggacaagaagaccggcgacgtcatcagcgacgacgaggatgagaatgccaccgacaccggcagcgacatggtggactttatcgatacccagggcacgttctgcgagcaggccgaactggaaacagcccaggcactgtttcacgcccaagaggtgcacaacgatgcccaggtgctgcacgtgctgaagagaaagtttgccggcggaagcaccgagaacagcccactgggagaaagactggaagtggacaccgagctgagccccagactgcaagagatcagcctgaacagcggccagaagaaggccaagcggagactgttcaccatctccgacagcggctacggctgtagcgaagtggaagccacacagatccaagtgaccaccaatggcgagcacggcggcaatgtttgttctggcggatctaccgaggccatcgacaatggcggaaccgagggcaacaatagctccgtggatggcaccagcgacaacagcaacatcgagaacgtgaaccctcagtgcacaatcgcccagctgaaggacctgctgaaagtgaacaacaagcagggcgccatgctggccgtgtttaaggatacctacggcctgagcttcaccgacctcgtgcggaacttcaagagcgacaagaccacctgtaccgactgggtcaccgccatctttggcgtgaacccaacaatcgccgagggcttcaagaccctgatccagcctttcatcctgtacgcccacatccagtgtctggactgcaaatggggcgtgctgattctggccctgctgagatacaagtgcggcaagagcagactgaccgtggccaagggactgagcactctgctgcatgtgcccgagacatgcatgctgattcagcctccaaagctgcggtctagcgtggccgctctgtactggtacagaaccggcatcagcaatatcagcgaagtgatgggcgacacccctgagtggattcagcggctgacaatcatccagcacggcatcgacgactccaacttcgacctgagcgagatggtgcagtgggccttcgataacgagctgaccgacgagtccgacatggcctttgaatacgccctgctggcagacagcaactccaatgccgccgctttcctgaagtccaactgccaggccaagtacctgaaggactgcgccaccatgtgcaagcactaccgcagagcacagaaacggcagatgaacatgagccagtggatccggttccggtgcagcaagatcgatgaaggtggcgactggcggcctatcgtgcagttcctgagataccagcagatcgagttcatcacctttctgggcgccctgaagtcattcctgaagggaacccctaaaaagaactgcctggtgttctgcggccctgccaataccggcaagtcctacttcggcatgagctttatccacttcatccagggcgccgtgatcagcttcgtgaacagcaccagccacttttggctggaacccctgaccgataccaaggtggcaatgctggacgacgccaccaccacctgttggacctacttcgacacctacatgcggaacgccctggacggcaaccccatcagcatcgacagaaagcacaagcccctcatccagctgaaatgccctccaatcctgctgaccacaaacattcaccccgccaaggacaatcggtggccctacctggaaagccggatcaccgtgttcgagttccccaacgcctttccattcgacaagaacggcaatcccgtgtacgagatcaacgacaagaattggaagtgcttcttcgagcggacctggtccagactggatctgcacgaggaagaagaggacgccgacacagagggcaatcccttcggcacctttaagtgtgtggccgggcagaatcacagacccctgggctgcagcatggccagattcgaggaccctaccagacggccctacaagctgcctgatctgtgcaccgaactgaacaccagccttcaggatatcgagatcacctgtgtgtactgcaagaccgtgctcgagctgacagaagtgtttgagttcgccttcaaggacctgttcgtggtgtacagagacagcatccctcacgccgcctgtcacaagtgcatcgacttctacagcagaatcagagagctgcggcactacagcgactccgtgtacggcgataccctggaaaaactgaccaacaccggactgtacaacctgctgatccggtgcctgagatgccagaaacctcagaaccccgccgagaaactgagacatctgaacgagaagcggcggttccacaatatcgccggccactacagaggccagtgccacagctgttgcaaccgggccagacaagaaagactccagcggagaagaggcagcatgcacggacctaaagccacacttcaggacatcgtgctgcacctcgagcctcagaatgagatccccgtggatctgctcggccatgagcagctgagcgatagcgaggaagagaacgacgagatcgacggcgtcaaccaccagcatctgcctgccagaagggccgaacctcagagacacaccatgctgtgcatgtgctgcaagtgcgaggcccggatcgagagagtggtggaatctagcgccgacgacctgagagctttccagcagctgttcctgaatactctgagcttcgtggccccttggtgcgctagtcagcagtgaggaagaatgtgcacagtgctaaccagaaaattcaggacaagactagtgcggccgcttttat

SEQ ID NO: 105 - DNA, 18 bp, Artificial Sequence
  Tet operator site
ccctatcagtgatagaga